European Patent Specification EP 3 434 771 B1, published September 13, 2023. Title: PLANT REGULATORY ELEMENTS AND USES THEREOF. Applicant: Monsanto Technology LLC. Application Unknown. The sequence listing filed with the application follows.

SEQUENCE LISTING (171 sequences)

SEQ ID NO: 1 - DNA, 3143 bp, Agrostis nebulosa
ggcctctttacgtttggcacaatttaattgaatcccggcatggcatgttagaccggagtgagccggcccttttactggtatgacactccctctgtcttgagtgtcgctgtgccagcttgtacctctgtctatgttcacagcccgtgctgtgtacctagaccctccgtttgtccacattcattttaatctctattgtatcttgtcaaaacctaaaagcctaaaacgactctgataaagggacagaaagattatacaagagcaagtgtataatgaaataatgtaagcgagctatatgaattgtcacgtgtcatatttatgttgagacgaagaagagaaaataaacaccatgcaaatttatggcgagtgatagatggccagatgggcacaaggcctcctatttcttaaatcggattttgtaagaacgaaaaaagggacttataagagaataggatagaccatatatcaatgatgtagtatgcatcaagatctaactattatatgagtgaattgataaatttattctaggtgacatggccttaacgatgaacagtacatggttaaatcaatagaacaatagccaactctagcagctctaaaaaaagatatatattcgtcgaggcactattatgcaaccacatagtcaacttcaacaccgcttgagtgcgttctcatgttttttttttcttgcaaattacgcttttctaaaataaaataatttggatcgtgcaattatttcactttaggtgtgcgtgactacgtgagtaacatttttgaatctcagaaaggaaataaaagtataatactgctgcctactttgaggattcggcttgttatttaaaaccgtctttaaggtcaaatgctcaagattcattcaacaattgaaacgtctcacatgattaaatcatgtataaggatgctaaggtcttgcttgacaatgtttttctaggaatttcatctaactttttgagtgaaactatcaaataataattttaaaacaattttataagagaagctccggagataaaaggccatctaatctatgttagaagagtgaagtttactccctctgtcccaaaaatagaattctaagtatgaaatgatttttttgttatacaaaaggagtatatatcacaagattgatgtcagttatgcttagggcacgtacacgacgctggtgctttaggtagacgttaatcgttgtttctgcattttattttattttgttgccacggtgtacatttgggtagacgtttgtcacaggcattgccactcaaacaagcagccggcgcttggagcttttatagtttgaaaagtgacggttttaaggatgggtaagctgattagtatatgtaagtttagctttttccattgtaggttaagccttaaggctcttacacaattgtttcattattctcattctttaagagcccatataagcgttcatgaattgtacatatccttagatttttttttttgggtaaagctcgagcttctgtatctaaaagtagagaaatcagaaaaagattcatgttttggtagttttgatttcttgcctccataataattttggtttaccattttttgtttgattttagttttagaagcgtttatagcaggatttaaaatccaaaactaccattatcttcaagtgaccgtcagtgagccgtttaacggcgtcgacaagtccaacggacaccaaccagtgaaccaccagcgtcgagccaagcgatgcaaacggaacggccgagacgttgacacctttggcgcggcacggcatgtcggatctccctctctggccccctctcgagagttccagctccacctccaccggtggcggtttccaagtccgttccgttccgttccgcctcctgcctgctcctctcagacggcacgaaaccgtgacggcaccggcagcacggggggattccttttccactgctccttccttttcccttcctcgcccgccgctataaatagccagccccgtccccagattctttcccaacctcatctttgttcggagcacccacacaacccgatccccaattccctcgtctctcctcgcgagcctcgtcgacccccccttcaaggtacggcgatcgtcctccctccctctctctctctaccttctcttctctagactagatcggcgacccggtccatggttagggcctgctagttctgttcctgttttttccatggctgcgaggtaaaatagatctgatggcgttatgatggttaactcgtcatactcttgcgatctatggtccctttaggacatcgatttaatttcggatggttcgagatcggtgatccatggttagtaccctaggcagtggggttagatccgtgctgttagggttcgtagatggattctgattgctcagtaactgggaaacctgggatggttctagctgggaatcctgggatggttctagctggttcgcagatgagatcgatttcatggtctgctatatcttgtttcgttgcctaggttccgtttaatctgtccgtggtatgatgttagcctttgataaggttcgatcgtgctagctacgtcctgcgcagcatttaattgtcaggtcataatttttagcattcctgtttttgtttggtttggttttgtctggttgggctgtagatagtttcaatctacctgtcggtttattttattaaatttggattggatctgtatgtgtcacatatatcttcatgattaatatggttggaattatctcttcatcttttagatatatatggataggtatatatgttgctgtgggttttactggtactttattagatatattcatgcttagatacatgaagcaacgtgctgttacagtttaataattcttgtttatctaataaacaaataaggataggtatatatgttgctgatggttttactgatactttattagatagtacttctttgacatgaaggaacatcctgcgacagcttaataattattcttcatctaataaaaagcttgctttttaattattttgatatacttggatgatgtcatgcagcagctatgtgtgaattttcggccctgtcttcatatgatgtttatttgcttgggactgtttctttggctgataactcaccctgttgtttggtgatccttctgcaggtg

SEQ ID NO: 2 - DNA, 2005 bp, Agrostis nebulosa
ggcctctttacgtttggcacaatttaattgaatcccggcatggcatgttagaccggagtgagccggcccttttactggtatgacactccctctgtcttgagtgtcgctgtgccagcttgtacctctgtctatgttcacagcccgtgctgtgtacctagaccctccgtttgtccacattcattttaatctctattgtatcttgtcaaaacctaaaagcctaaaacgactctgataaagggacagaaagattatacaagagcaagtgtataatgaaataatgtaagcgagctatatgaattgtcacgtgtcatatttatgttgagacgaagaagagaaaataaacaccatgcaaatttatggcgagtgatagatggccagatgggcacaaggcctcctatttcttaaatcggattttgtaagaacgaaaaaagggacttataagagaataggatagaccatatatcaatgatgtagtatgcatcaagatctaactattatatgagtgaattgataaatttattctaggtgacatggccttaacgatgaacagtacatggttaaatcaatagaacaatagccaactctagcagctctaaaaaaagatatatattcgtcgaggcactattatgcaaccacatagtcaacttcaacaccgcttgagtgcgttctcatgttttttttttcttgcaaattacgcttttctaaaataaaataatttggatcgtgcaattatttcactttaggtgtgcgtgactacgtgagtaacatttttgaatctcagaaaggaaataaaagtataatactgctgcctactttgaggattcggcttgttatttaaaaccgtctttaaggtcaaatgctcaagattcattcaacaattgaaacgtctcacatgattaaatcatgtataaggatgctaaggtcttgcttgacaatgtttttctaggaatttcatctaactttttgagtgaaactatcaaataataattttaaaacaattttataagagaagctccggagataaaaggccatctaatctatgttagaagagtgaagtttactccctctgtcccaaaaatagaattctaagtatgaaatgatttttttgttatacaaaaggagtatatatcacaagattgatgtcagttatgcttagggcacgtacacgacgctggtgctttaggtagacgttaatcgttgtttctgcattttattttattttgttgccacggtgtacatttgggtagacgtttgtcacaggcattgccactcaaacaagcagccggcgcttggagcttttatagtttgaaaagtgacggttttaaggatgggtaagctgattagtatatgtaagtttagctttttccattgtaggttaagccttaaggctcttacacaattgtttcattattctcattctttaagagcccatataagcgttcatgaattgtacatatccttagatttttttttttgggtaaagctcgagcttctgtatctaaaagtagagaaatcagaaaaagattcatgttttggtagttttgatttcttgcctccataataattttggtttaccattttttgtttgattttagttttagaagcgtttatagcaggatttaaaatccaaaactaccattatcttcaagtgaccgtcagtgagccgtttaacggcgtcgacaagtccaacggacaccaaccagtgaaccaccagcgtcgagccaagcgatgcaaacggaacggccgagacgttgacacctttggcgcggcacggcatgtcggatctccctctctggccccctctcgagagttccagctccacctccaccggtggcggtttccaagtccgttccgttccgttccgcctcctgcctgctcctctcagacggcacgaaaccgtgacggcaccggcagcacggggggattccttttccactgctccttccttttcccttcctcgcccgccgctataaatagccagccccgtccccagattctttcccaa

SEQ ID NO: 3 - DNA, 85 bp, Agrostis nebulosa
cctcatctttgttcggagcacccacacaacccgatccccaattccctcgtctctcctcgcgagcctcgtcgacccccccttcaag

SEQ ID NO: 4 - DNA, 1053 bp, Agrostis nebulosa
gtacggcgatcgtcctccctccctctctctctctaccttctcttctctagactagatcggcgacccggtccatggttagggcctgctagttctgttcctgttttttccatggctgcgaggtaaaatagatctgatggcgttatgatggttaactcgtcatactcttgcgatctatggtccctttaggacatcgatttaatttcggatggttcgagatcggtgatccatggttagtaccctaggcagtggggttagatccgtgctgttagggttcgtagatggattctgattgctcagtaactgggaaacctgggatggttctagctgggaatcctgggatggttctagctggttcgcagatgagatcgatttcatggtctgctatatcttgtttcgttgcctaggttccgtttaatctgtccgtggtatgatgttagcctttgataaggttcgatcgtgctagctacgtcctgcgcagcatttaattgtcaggtcataatttttagcattcctgtttttgtttggtttggttttgtctggttgggctgtagatagtttcaatctacctgtcggtttattttattaaatttggattggatctgtatgtgtcacatatatcttcatgattaatatggttggaattatctcttcatcttttagatatatatggataggtatatatgttgctgtgggttttactggtactttattagatatattcatgcttagatacatgaagcaacgtgctgttacagtttaataattcttgtttatctaataaacaaataaggataggtatatatgttgctgatggttttactgatactttattagatagtacttctttgacatgaaggaacatcctgcgacagcttaataattattcttcatctaataaaaagcttgctttttaattattttgatatacttggatgatgtcatgcagcagctatgtgtgaattttcggccctgtcttcatatgatgtttatttgcttgggactgtttctttggctgataactcaccctgttgtttggtgatccttctgcaggtg

SEQ ID NO: 5 - DNA, 2137 bp, Agrostis nebulosa
gagaagctccggagataaaaggccatctaatctatgttagaagagtgaagtttactccctctgtcccaaaaatagaattctaagtatgaaatgatttttttgttatacaaaaggagtatatatcacaagattgatgtcagttatgcttagggcacgtacacgacgctggtgctttaggtagacgttaatcgttgtttctgcattttattttattttgttgccacggtgtacatttgggtagacgtttgtcacaggcattgccactcaaacaagcagccggcgcttggagcttttatagtttgaaaagtgacggttttaaggatgggtaagctgattagtatatgtaagtttagctttttccattgtaggttaagccttaaggctcttacacaattgtttcattattctcattctttaagagcccatataagcgttcatgaattgtacatatccttagatttttttttttgggtaaagctcgagcttctgtatctaaaagtagagaaatcagaaaaagattcatgttttggtagttttgatttcttgcctccataataattttggtttaccattttttgtttgattttagttttagaagcgtttatagcaggatttaaaatccaaaactaccattatcttcaagtgaccgtcagtgagccgtttaacggcgtcgacaagtccaacggacaccaaccagtgaaccaccagcgtcgagccaagcgatgcaaacggaacggccgagacgttgacacctttggcgcggcacggcatgtcggatctccctctctggccccctctcgagagttccagctccacctccaccggtggcggtttccaagtccgttccgttccgttccgcctcctgcctgctcctctcagacggcacgaaaccgtgacggcaccggcagcacggggggattccttttccactgctccttccttttcccttcctcgcccgccgctataaatagccagccccgtccccagattctttcccaacctcatctttgttcggagcacccacacaacccgatccccaattccctcgtctctcctcgcgagcctcgtcgacccccccttcaaggtacggcgatcgtcctccctccctctctctctctaccttctcttctctagactagatcggcgacccggtccatggttagggcctgctagttctgttcctgttttttccatggctgcgaggtaaaatagatctgatggcgttatgatggttaactcgtcatactcttgcgatctatggtccctttaggacatcgatttaatttcggatggttcgagatcggtgatccatggttagtaccctaggcagtggggttagatccgtgctgttagggttcgtagatggattctgattgctcagtaactgggaaacctgggatggttctagctgggaatcctgggatggttctagctggttcgcagatgagatcgatttcatggtctgctatatcttgtttcgttgcctaggttccgtttaatctgtccgtggtatgatgttagcctttgataaggttcgatcgtgctagctacgtcctgcgcagcatttaattgtcaggtcataatttttagcattcctgtttttgtttggtttggttttgtctggttgggctgtagatagtttcaatctacctgtcggtttattttattaaatttggattggatctgtatgtgtcacatatatcttcatgattaatatggttggaattatctcttcatcttttagatatatatggataggtatatatgttgctgtgggttttactggtactttattagatatattcatgcttagatacatgaagcaacgtgctgttacagtttaataattcttgtttatctaataaacaaataaggataggtatatatgttgctgatggttttactgatactttattagatagtacttctttgacatgaaggaacatcctgcgacagcttaataattattcttcatctaataaaaagcttgctttttaattattttgatatacttggatgatgtcatgcagcagctatgtgtgaattttcggccctgtcttcatatgatgtttatttgcttgggactgtttctttggctgataactcaccctgttgtttggtgatccttctgcaggtg

SEQ ID NO: 6 - DNA, 999 bp, Agrostis nebulosa
gagaagctccggagataaaaggccatctaatctatgttagaagagtgaagtttactccctctgtcccaaaaatagaattctaagtatgaaatgatttttttgttatacaaaaggagtatatatcacaagattgatgtcagttatgcttagggcacgtacacgacgctggtgctttaggtagacgttaatcgttgtttctgcattttattttattttgttgccacggtgtacatttgggtagacgtttgtcacaggcattgccactcaaacaagcagccggcgcttggagcttttatagtttgaaaagtgacggttttaaggatgggtaagctgattagtatatgtaagtttagctttttccattgtaggttaagccttaaggctcttacacaattgtttcattattctcattctttaagagcccatataagcgttcatgaattgtacatatccttagatttttttttttgggtaaagctcgagcttctgtatctaaaagtagagaaatcagaaaaagattcatgttttggtagttttgatttcttgcctccataataattttggtttaccattttttgtttgattttagttttagaagcgtttatagcaggatttaaaatccaaaactaccattatcttcaagtgaccgtcagtgagccgtttaacggcgtcgacaagtccaacggacaccaaccagtgaaccaccagcgtcgagccaagcgatgcaaacggaacggccgagacgttgacacctttggcgcggcacggcatgtcggatctccctctctggccccctctcgagagttccagctccacctccaccggtggcggtttccaagtccgttccgttccgttccgcctcctgcctgctcctctcagacggcacgaaaccgtgacggcaccggcagcacggggggattccttttccactgctccttccttttcccttcctcgcccgccgctataaatagccagccccgtccccagattctttcccaa

SEQ ID NO: 7 - DNA, 1900 bp, Agrostis nebulosa
gtagacgtttgtcacaggcattgccactcaaacaagcagccggcgcttggagcttttatagtttgaaaagtgacggttttaaggatgggtaagctgattagtatatgtaagtttagctttttccattgtaggttaagccttaaggctcttacacaattgtttcattattctcattctttaagagcccatataagcgttcatgaattgtacatatccttagatttttttttttgggtaaagctcgagcttctgtatctaaaagtagagaaatcagaaaaagattcatgttttggtagttttgatttcttgcctccataataattttggtttaccattttttgtttgattttagttttagaagcgtttatagcaggatttaaaatccaaaactaccattatcttcaagtgaccgtcagtgagccgtttaacggcgtcgacaagtccaacggacaccaaccagtgaaccaccagcgtcgagccaagcgatgcaaacggaacggccgagacgttgacacctttggcgcggcacggcatgtcggatctccctctctggccccctctcgagagttccagctccacctccaccggtggcggtttccaagtccgttccgttccgttccgcctcctgcctgctcctctcagacggcacgaaaccgtgacggcaccggcagcacggggggattccttttccactgctccttccttttcccttcctcgcccgccgctataaatagccagccccgtccccagattctttcccaacctcatctttgttcggagcacccacacaacccgatccccaattccctcgtctctcctcgcgagcctcgtcgacccccccttcaaggtacggcgatcgtcctccctccctctctctctctaccttctcttctctagactagatcggcgacccggtccatggttagggcctgctagttctgttcctgttttttccatggctgcgaggtaaaatagatctgatggcgttatgatggttaactcgtcatactcttgcgatctatggtccctttaggacatcgatttaatttcggatggttcgagatcggtgatccatggttagtaccctaggcagtggggttagatccgtgctgttagggttcgtagatggattctgattgctcagtaactgggaaacctgggatggttctagctgggaatcctgggatggttctagctggttcgcagatgagatcgatttcatggtctgctatatcttgtttcgttgcctaggttccgtttaatctgtccgtggtatgatgttagcctttgataaggttcgatcgtgctagctacgtcctgcgcagcatttaattgtcaggtcataatttttagcattcctgtttttgtttggtttggttttgtctggttgggctgtagatagtttcaatctacctgtcggtttattttattaaatttggattggatctgtatgtgtcacatatatcttcatgattaatatggttggaattatctcttcatcttttagatatatatggataggtatatatgttgctgtgggttttactggtactttattagatatattcatgcttagatacatgaagcaacgtgctgttacagtttaataattcttgtttatctaataaacaaataaggataggtatatatgttgctgatggttttactgatactttattagatagtacttctttgacatgaaggaacatcctgcgacagcttaataattattcttcatctaataaaaagcttgctttttaattattttgatatacttggatgatgtcatgcagcagctatgtgtgaattttcggccctgtcttcatatgatgtttatttgcttgggactgtttctttggctgataactcaccctgttgtttggtgatccttctgcaggtg

SEQ ID NO: 8 - DNA, 762 bp, Agrostis nebulosa
gtagacgtttgtcacaggcattgccactcaaacaagcagccggcgcttggagcttttatagtttgaaaagtgacggttttaaggatgggtaagctgattagtatatgtaagtttagctttttccattgtaggttaagccttaaggctcttacacaattgtttcattattctcattctttaagagcccatataagcgttcatgaattgtacatatccttagatttttttttttgggtaaagctcgagcttctgtatctaaaagtagagaaatcagaaaaagattcatgttttggtagttttgatttcttgcctccataataattttggtttaccattttttgtttgattttagttttagaagcgtttatagcaggatttaaaatccaaaactaccattatcttcaagtgaccgtcagtgagccgtttaacggcgtcgacaagtccaacggacaccaaccagtgaaccaccagcgtcgagccaagcgatgcaaacggaacggccgagacgttgacacctttggcgcggcacggcatgtcggatctccctctctggccccctctcgagagttccagctccacctccaccggtggcggtttccaagtccgttccgttccgttccgcctcctgcctgctcctctcagacggcacgaaaccgtgacggcaccggcagcacggggggattccttttccactgctccttccttttcccttcctcgcccgccgctataaatagccagccccgtccccagattctttcccaa

SEQ ID NO: 9 - DNA, 5068 bp, Arundo donax
ggcctctttacgtttggcacaatttgatcgaatccaacacggcaagttaacatttgaagattgaaccgggcactaatgcaagtctacaactaagaactacaagaaagcatgttccttgaggtacttggatgcaacctcacaattatcaaattaattaacaactacagttagaattttagatcacaagaatatcacgaactgtggatactacttcaagggctattcttttctgaatgttgcagttggttgttttaaacatattacaaactaggtgtttaaatgccaaaaagttcatggaaaaagattaagctaatattccatccgtccacaaaatttaaatgctaggaatcattatatttgtggatagaaggagtagttagtaagacctacacttaattacacattggtcattcctggaggaataatcccccatagcaagttgttttgagtttgactacccaaacttgcataaattttttcttaaaaaaagggggagcttcaccattccatcaagatggcgaggctaaatgaaacgcacgatgggcaaaacggactaacgtacaaacaacaaggcaatgaaagatagggttttgataaatatcaaatatacaaagtcaaccaaagaaaaaagagatcccaatggctaacctttggatccgtgtcgcaatttgtgctttaggacatacaaggtggatttcttctttggcaaactctataataattgggtgacggtggcctcacggcagcctcaaagagtcggtagcaacttttagatcttttgagctgaaactcaattatgtagtagaatgatatttagatagatagatcgaaatttgggggtgtgaaaacaaagaggttctcaatattgatagcaactccaacgaatggatatggaaaatacatgattttttattcgagtagaaaaaggaggggaacggaacaaatctagcaatagtagccaccaaagatgaggaccctggatttcggatccaatagtggtaaggaagaaagggccggactatccagaataaggtgaattggtcaaggaagcggaagtctccataaagaaattgtgggctcacttgatgtgagaaagaagaccgaccaagaagcgggttttgggggacagaggagattggtgccaggttgcagtggcatgtatgtgggggaagaggcaatgacaacggccgagagaggagaagggaatgaggtaagtatttgaagtgaagaggtgcccatataggttaaaaaatgagctgtggatttaaatcaaaggtgtcagcgacacaggcacggaagtaccctaagttacctatgtgggtcgcatatcacgctaagttccttcaccgtacaaggtgaaagtaacactggcaatgtgccccagctgcaaggcttgtctatcaatgtggccctacaaggctcctggctaccccaggagctcaaaacacgtggcacatggtggtacttcgcccgacctctatgctcaccgtgcacccggccccgaggtcaatggctcctgagcacccgactgcatgactggacccctgagtacccgacccccgggacaagctcccgtggaccttccccggggatcaggctcacgagtactcgacctcacgtcaatggctctcccgagtacccaaccttgtgtcgatagctcactaaggatcatgtgctaatccttagcatctcggattttgagtactaggccattatttgcatgccatcctcttggatctatgcggattttcaaggaccttacctaagcatcaacatgcacaaacacaaacccttcgtgaagccatccccaactactcgggtggcaggaccctcgacacgtgcgatgcgagctcggacagagctgacaagaacctcccgacggcgcattaaatgccctggcaagggcgccccgcctcgtcgagctctggacttcatcaagtcacatcaacagcaggcaggcgctccttccgcagacttcatcatgagggaatccgttaccctctatttacatagtgcagcggggaatgtggagatcaaatctctccaatgatgtcactgtgtagcatgtattagcacgccaacaccctgtcgcttaccacgaggatcagccatgcaagcaagagatgttggtcgggcctcggtggcaactgaggctatagtgacctatgacgagcaggccatagataggcccactggcaagcccaagaatcgctagacgggctagatctggacacttgtccgcaccaagcactaccgttgcaactgcaacctctatatgtaactatagattcacatgttgcgacatctttgcccaatacgtattgtaccctagacagctcaccctatctttttcttttttttcctctttcttcttcctcctccttgcatggagacgtagaaggactcctcccttgtgactattaaaggaaggacttagggctgtgctaggggagagaacttttggacttgggagagctctgcactgaacatcttcctctccacgcttgtaatattttccacaacaaagaattccataaagccggatgtagggctattatccctctcgggaggcctgaaccagggtaaaacaccactcttctcaccagcgttcgccgcattagtctagactagcatcttttgaccctatatcgaaccatctagggactttacgtcccctgcctgcagtttcccggtgacagaatgactatgatttttcgtcgattttataaaagtgaaaacaaccggttgatatctatgcgcactattttcctacatatatttctaacttcttgcttagccatgtcggttaagagcaagtggagagcactctcatttcgtagaacaagtgatgaatgccgacctgcatcatcttacttagacttgatcatcaagtggaatccccattcatcttaataatctcatattgagtgccaatgcaacattgttataatcctcttcatatgctaattcttcaaagctaacgtagttaaatgaaggcaaaatatgcaacttcgtcctctaagtttgctcaaaggctcatttttaccctttaactatcaaaccgattactttcgtccctgaactttcatgtttggtccaatttaatccctgggctgatgtatccgtccacggtggtgtgtccaatcagtgaataatctagttagtgaagccagaagtccatagtgccccttgctctgtcaccatatatccagttcaaccgcaccaatttgccatctcgaactggttcatgttttattcaggttggtaaatgaattttgccaattcaatgtagttagatatttccatgtcattttagtacatttaccaattttttatattctggctagaaaaggagaatggtgacgtctttcggaagatcaagatcaattatcaagtatcagcaacagcacctgaaggttggagtgcattagttgtcattgagaataatgctagctattcattgcactggcattagagacagagagggcgagccagtttgacatggcaaattagcacagtcaaactggatacgtggtgacggagggaggggcactatgaatttttggtgacggagggaggggcactatgaatttttggctttgctgacgggacacgccactatggatgaaattggacaaaatacgaatattcaaggatgaaagtggtcggtttgatagttcagggatgaaatgtgtctttgggcaaactttgaggacgaagttgcctattttgcattaaacgaatatatttatataccccaaaaaaaagaatacacatctccactccgagccggcatgtggggtccccactagtcagccactgtatggcgccgactagctcaacggccacgaaccagccaaccaccagcgcaacctaaacggcgtaaacgttgacggcatctctctctcgccccgtctcgaagcttccgcaccgctcgctggtcgctgcccggcgccgctcgtgctggactctttccgtggcggcttccgcgaaattgcgtggtggagaggagagacggaaccgtcacggcactggattccttccccacccggcttggccggcccctcctcgcctccataaataggcaccccgtcctcgcctcctctccccacctcatctcctcctttcccgtgaaccgtgaacacaacccgacccagatcccctcttgcgagcttcgtcgatccctcctccgcgtcaaggtacggagcttctcctcccccttcttctctagatcggcgtgttatgttgtttccgtggttgcttggttggatgaatcgaatgattcttagggcctaggaggctggttagatctgttgcgttctgtttcgtagatggattttggtgtaagatcaggtcggttccgctgtttaacttgtgatgctagtgtgatttttgggaggatttgagttgttaatctgggagttgttgggaggttctcgtaggcggattgtagatgaagtcgcccgcacgatttgcgtggcttgttgggtagctagggttagatctgctcggatttttcattgttacttattgagagataatgtagctaacctttacttgttcatctatgtatctcgtattcgtattcatctggttcgatggtgctagatagatgcgcctgatttgtccgatcgaattgggtagcatccgcggcttgtttggtagtgttctgattgatttgtcgctctagatctgagtggaataatattacatctcaacatgttactagaaacttggtttatagctccggatttacatgtttattcttatgtaaggttttaaatgaaagatttatgctactgctgctcgttgatcctttagcatccacctgaggaacatgcatgcatctgttacttcttttgatatatgcttagatagttgttagtatatactgctgttgttcgatgatccttcaggatgaacatgcatgatcatgttacttgtttttatatgcttctgctgttcgttgattctttagtactacctacctgatcatcttgcatgtttcctgcttgttagagattaattgattaggcttaccttgttgcctggtgattcttccttgcag

SEQ ID NO: 10 - DNA, 4114 bp, Arundo donax
ggcctctttacgtttggcacaatttgatcgaatccaacacggcaagttaacatttgaagattgaaccgggcactaatgcaagtctacaactaagaactacaagaaagcatgttccttgaggtacttggatgcaacctcacaattatcaaattaattaacaactacagttagaattttagatcacaagaatatcacgaactgtggatactacttcaagggctattcttttctgaatgttgcagttggttgttttaaacatattacaaactaggtgtttaaatgccaaaaagttcatggaaaaagattaagctaatattccatccgtccacaaaatttaaatgctaggaatcattatatttgtggatagaaggagtagttagtaagacctacacttaattacacattggtcattcctggaggaataatcccccatagcaagttgttttgagtttgactacccaaacttgcataaattttttcttaaaaaaagggggagcttcaccattccatcaagatggcgaggctaaatgaaacgcacgatgggcaaaacggactaacgtacaaacaacaaggcaatgaaagatagggttttgataaatatcaaatatacaaagtcaaccaaagaaaaaagagatcccaatggctaacctttggatccgtgtcgcaatttgtgctttaggacatacaaggtggatttcttctttggcaaactctataataattgggtgacggtggcctcacggcagcctcaaagagtcggtagcaacttttagatcttttgagctgaaactcaattatgtagtagaatgatatttagatagatagatcgaaatttgggggtgtgaaaacaaagaggttctcaatattgatagcaactccaacgaatggatatggaaaatacatgattttttattcgagtagaaaaaggaggggaacggaacaaatctagcaatagtagccaccaaagatgaggaccctggatttcggatccaatagtggtaaggaagaaagggccggactatccagaataaggtgaattggtcaaggaagcggaagtctccataaagaaattgtgggctcacttgatgtgagaaagaagaccgaccaagaagcgggttttgggggacagaggagattggtgccaggttgcagtggcatgtatgtgggggaagaggcaatgacaacggccgagagaggagaagggaatgaggtaagtatttgaagtgaagaggtgcccatataggttaaaaaatgagctgtggatttaaatcaaaggtgtcagcgacacaggcacggaagtaccctaagttacctatgtgggtcgcatatcacgctaagttccttcaccgtacaaggtgaaagtaacactggcaatgtgccccagctgcaaggcttgtctatcaatgtggccctacaaggctcctggctaccccaggagctcaaaacacgtggcacatggtggtacttcgcccgacctctatgctcaccgtgcacccggccccgaggtcaatggctcctgagcacccgactgcatgactggacccctgagtacccgacccccgggacaagctcccgtggaccttccccggggatcaggctcacgagtactcgacctcacgtcaatggctctcccgagtacccaaccttgtgtcgatagctcactaaggatcatgtgctaatccttagcatctcggattttgagtactaggccattatttgcatgccatcctcttggatctatgcggattttcaaggaccttacctaagcatcaacatgcacaaacacaaacccttcgtgaagccatccccaactactcgggtggcaggaccctcgacacgtgcgatgcgagctcggacagagctgacaagaacctcccgacggcgcattaaatgccctggcaagggcgccccgcctcgtcgagctctggacttcatcaagtcacatcaacagcaggcaggcgctccttccgcagacttcatcatgagggaatccgttaccctctatttacatagtgcagcggggaatgtggagatcaaatctctccaatgatgtcactgtgtagcatgtattagcacgccaacaccctgtcgcttaccacgaggatcagccatgcaagcaagagatgttggtcgggcctcggtggcaactgaggctatagtgacctatgacgagcaggccatagataggcccactggcaagcccaagaatcgctagacgggctagatctggacacttgtccgcaccaagcactaccgttgcaactgcaacctctatatgtaactatagattcacatgttgcgacatctttgcccaatacgtattgtaccctagacagctcaccctatctttttcttttttttcctctttcttcttcctcctccttgcatggagacgtagaaggactcctcccttgtgactattaaaggaaggacttagggctgtgctaggggagagaacttttggacttgggagagctctgcactgaacatcttcctctccacgcttgtaatattttccacaacaaagaattccataaagccggatgtagggctattatccctctcgggaggcctgaaccagggtaaaacaccactcttctcaccagcgttcgccgcattagtctagactagcatcttttgaccctatatcgaaccatctagggactttacgtcccctgcctgcagtttcccggtgacagaatgactatgatttttcgtcgattttataaaagtgaaaacaaccggttgatatctatgcgcactattttcctacatatatttctaacttcttgcttagccatgtcggttaagagcaagtggagagcactctcatttcgtagaacaagtgatgaatgccgacctgcatcatcttacttagacttgatcatcaagtggaatccccattcatcttaataatctcatattgagtgccaatgcaacattgttataatcctcttcatatgctaattcttcaaagctaacgtagttaaatgaaggcaaaatatgcaacttcgtcctctaagtttgctcaaaggctcatttttaccctttaactatcaaaccgattactttcgtccctgaactttcatgtttggtccaatttaatccctgggctgatgtatccgtccacggtggtgtgtccaatcagtgaataatctagttagtgaagccagaagtccatagtgccccttgctctgtcaccatatatccagttcaaccgcaccaatttgccatctcgaactggttcatgttttattcaggttggtaaatgaattttgccaattcaatgtagttagatatttccatgtcattttagtacatttaccaattttttatattctggctagaaaaggagaatggtgacgtctttcggaagatcaagatcaattatcaagtatcagcaacagcacctgaaggttggagtgcattagttgtcattgagaataatgctagctattcattgcactggcattagagacagagagggcgagccagtttgacatggcaaattagcacagtcaaactggatacgtggtgacggagggaggggcactatgaatttttggtgacggagggaggggcactatgaatttttggctttgctgacgggacacgccactatggatgaaattggacaaaatacgaatattcaaggatgaaagtggtcggtttgatagttcagggatgaaatgtgtctttgggcaaactttgaggacgaagttgcctattttgcattaaacgaatatatttatataccccaaaaaaaagaatacacatctccactccgagccggcatgtggggtccccactagtcagccactgtatggcgccgactagctcaacggccacgaaccagccaaccaccagcgcaacctaaacggcgtaaacgttgacggcatctctctctcgccccgtctcgaagcttccgcaccgctcgctggtcgctgcccggcgccgctcgtgctggactctttccgtggcggcttccgcgaaattgcgtggtggagaggagagacggaaccgtcacggcactggattccttccccacccggcttggccggcccctcctcgcctccataaataggcaccccgtcctcgcctcctctccccacct

SEQ ID NO: 11 - DNA, 85 bp, Arundo donax
catctcctcctttcccgtgaaccgtgaacacaacccgacccagatcccctcttgcgagcttcgtcgatccctcctccgcgtcaag

SEQ ID NO: 12 - DNA, 869 bp, Arundo donax
gtacggagcttctcctcccccttcttctctagatcggcgtgttatgttgtttccgtggttgcttggttggatgaatcgaatgattcttagggcctaggaggctggttagatctgttgcgttctgtttcgtagatggattttggtgtaagatcaggtcggttccgctgtttaacttgtgatgctagtgtgatttttgggaggatttgagttgttaatctgggagttgttgggaggttctcgtaggcggattgtagatgaagtcgcccgcacgatttgcgtggcttgttgggtagctagggttagatctgctcggatttttcattgttacttattgagagataatgtagctaacctttacttgttcatctatgtatctcgtattcgtattcatctggttcgatggtgctagatagatgcgcctgatttgtccgatcgaattgggtagcatccgcggcttgtttggtagtgttctgattgatttgtcgctctagatctgagtggaataatattacatctcaacatgttactagaaacttggtttatagctccggatttacatgtttattcttatgtaaggttttaaatgaaagatttatgctactgctgctcgttgatcctttagcatccacctgaggaacatgcatgcatctgttacttcttttgatatatgcttagatagttgttagtatatactgctgttgttcgatgatccttcaggatgaacatgcatgatcatgttacttgtttttatatgcttctgctgttcgttgattctttagtactacctacctgatcatcttgcatgtttcctgcttgttagagattaattgattaggcttaccttgttgcctggtgattcttccttgcag

SEQ ID NO: 13 - DNA, 2969 bp, Arundo donax
gatcagccatgcaagcaagagatgttggtcgggcctcggtggcaactgaggctatagtgacctatgacgagcaggccatagataggcccactggcaagcccaagaatcgctagacgggctagatctggacacttgtccgcaccaagcactaccgttgcaactgcaacctctatatgtaactatagattcacatgttgcgacatctttgcccaatacgtattgtaccctagacagctcaccctatctttttcttttttttcctctttcttcttcctcctccttgcatggagacgtagaaggactcctcccttgtgactattaaaggaaggacttagggctgtgctaggggagagaacttttggacttgggagagctctgcactgaacatcttcctctccacgcttgtaatattttccacaacaaagaattccataaagccggatgtagggctattatccctctcgggaggcctgaaccagggtaaaacaccactcttctcaccagcgttcgccgcattagtctagactagcatcttttgaccctatatcgaaccatctagggactttacgtcccctgcctgcagtttcccggtgacagaatgactatgatttttcgtcgattttataaaagtgaaaacaaccggttgatatctatgcgcactattttcctacatatatttctaacttcttgcttagccatgtcggttaagagcaagtggagagcactctcatttcgtagaacaagtgatgaatgccgacctgcatcatcttacttagacttgatcatcaagtggaatccccattcatcttaataatctcatattgagtgccaatgcaacattgttataatcctcttcatatgctaattcttcaaagctaacgtagttaaatgaaggcaaaatatgcaacttcgtcctctaagtttgctcaaaggctcatttttaccctttaactatcaaaccgattactttcgtccctgaactttcatgtttggtccaatttaatccctgggctgatgtatccgtccacggtggtgtgtccaatcagtgaataatctagttagtgaagccagaagtccatagtgccccttgctctgtcaccatatatccagttcaaccgcaccaatttgccatctcgaactggttcatgttttattcaggttggtaaatgaattttgccaattcaatgtagttagatatttccatgtcattttagtacatttaccaattttttatattctggctagaaaaggagaatggtgacgtctttcggaagatcaagatcaattatcaagtatcagcaacagcacctgaaggttggagtgcattagttgtcattgagaataatgctagctattcattgcactggcattagagacagagagggcgagccagtttgacatggcaaattagcacagtcaaactggatacgtggtgacggagggaggggcactatgaatttttggtgacggagggaggggcactatgaatttttggctttgctgacgggacacgccactatggatgaaattggacaaaatacgaatattcaaggatgaaagtggtcggtttgatagttcagggatgaaatgtgtctttgggcaaactttgaggacgaagttgcctattttgcattaaacgaatatatttatataccccaaaaaaaagaatacacatctccactccgagccggcatgtggggtccccactagtcagccactgtatggcgccgactagctcaacggccacgaaccagccaaccaccagcgcaacctaaacggcgtaaacgttgacggcatctctctctcgccccgtctcgaagcttccgcaccgctcgctggtcgctgcccggcgccgctcgtgctggactctttccgtggcggcttccgcgaaattgcgtggtggagaggagagacggaaccgtcacggcactggattccttccccacccggcttggccggcccctcctcgcctccataaataggcaccccgtcctcgcctcctctccccacctcatctcctcctttcccgtgaaccgtgaacacaacccgacccagatcccctcttgcgagcttcgtcgatccctcctccgcgtcaaggtacggagcttctcctcccccttcttctctagatcggcgtgttatgttgtttccgtggttgcttggttggatgaatcgaatgattcttagggcctaggaggctggttagatctgttgcgttctgtttcgtagatggattttggtgtaagatcaggtcggttccgctgtttaacttgtgatgctagtgtgatttttgggaggatttgagttgttaatctgggagttgttgggaggttctcgtaggcggattgtagatgaagtcgcccgcacgatttgcgtggcttgttgggtagctagggttagatctgctcggatttttcattgttacttattgagagataatgtagctaacctttacttgttcatctatgtatctcgtattcgtattcatctggttcgatggtgctagatagatgcgcctgatttgtccgatcgaattgggtagcatccgcggcttgtttggtagtgttctgattgatttgtcgctctagatctgagtggaataatattacatctcaacatgttactagaaacttggtttatagctccggatttacatgtttattcttatgtaaggttttaaatgaaagatttatgctactgctgctcgttgatcctttagcatccacctgaggaacatgcatgcatctgttacttcttttgatatatgcttagatagttgttagtatatactgctgttgttcgatgatccttcaggatgaacatgcatgatcatgttacttgtttttatatgcttctgctgttcgttgattctttagtactacctacctgatcatcttgcatgtttcctgcttgttagagattaattgattaggcttaccttgttgcctggtgattcttccttgcaggtg

SEQ ID NO: 14 - DNA, 2012 bp, Arundo donax
gatcagccatgcaagcaagagatgttggtcgggcctcggtggcaactgaggctatagtgacctatgacgagcaggccatagataggcccactggcaagcccaagaatcgctagacgggctagatctggacacttgtccgcaccaagcactaccgttgcaactgcaacctctatatgtaactatagattcacatgttgcgacatctttgcccaatacgtattgtaccctagacagctcaccctatctttttcttttttttcctctttcttcttcctcctccttgcatggagacgtagaaggactcctcccttgtgactattaaaggaaggacttagggctgtgctaggggagagaacttttggacttgggagagctctgcactgaacatcttcctctccacgcttgtaatattttccacaacaaagaattccataaagccggatgtagggctattatccctctcgggaggcctgaaccagggtaaaacaccactcttctcaccagcgttcgccgcattagtctagactagcatcttttgaccctatatcgaaccatctagggactttacgtcccctgcctgcagtttcccggtgacagaatgactatgatttttcgtcgattttataaaagtgaaaacaaccggttgatatctatgcgcactattttcctacatatatttctaacttcttgcttagccatgtcggttaagagcaagtggagagcactctcatttcgtagaacaagtgatgaatgccgacctgcatcatcttacttagacttgatcatcaagtggaatccccattcatcttaataatctcatattgagtgccaatgcaacattgttataatcctcttcatatgctaattcttcaaagctaacgtagttaaatgaaggcaaaatatgcaacttcgtcctctaagtttgctcaaaggctcatttttaccctttaactatcaaaccgattactttcgtccctgaactttcatgtttggtccaatttaatccctgggctgatgtatccgtccacggtggtgtgtccaatcagtgaataatctagttagtgaagccagaagtccatagtgccccttgctctgtcaccatatatccagttcaaccgcaccaatttgccatctcgaactggttcatgttttattcaggttggtaaatgaattttgccaattcaatgtagttagatatttccatgtcattttagtacatttaccaattttttatattctggctagaaaaggagaatggtgacgtctttcggaagatcaagatcaattatcaagtatcagcaacagcacctgaaggttggagtgcattagttgtcattgagaataatgctagctattcattgcactggcattagagacagagagggcgagccagtttgacatggcaaattagcacagtcaaactggatacgtggtgacggagggaggggcactatgaatttttggtgacggagggaggggcactatgaatttttggctttgctgacgggacacgccactatggatgaaattggacaaaatacgaatattcaaggatgaaagtggtcggtttgatagttcagggatgaaatgtgtctttgggcaaactttgaggacgaagttgcctattttgcattaaacgaatatatttatataccccaaaaaaaagaatacacatctccactccgagccggcatgtggggtccccactagtcagccactgtatggcgccgactagctcaacggccacgaaccagccaaccaccagcgcaacctaaacggcgtaaacgttgacggcatctctctctcgccccgtctcgaagcttccgcaccgctcgctggtcgctgcccggcgccgctcgtgctggactctttccgtggcggcttccgcgaaattgcgtggtggagaggagagacggaaccgtcacggcactggattccttccccacccggcttggccggcccctcctcgcctccataaataggcaccccgtcctcgcctcctctccccacct

SEQ ID NO: 15 - DNA, 872 bp, Arundo donax
gtacggagcttctcctcccccttcttctctagatcggcgtgttatgttgtttccgtggttgcttggttggatgaatcgaatgattcttagggcctaggaggctggttagatctgttgcgttctgtttcgtagatggattttggtgtaagatcaggtcggttccgctgtttaacttgtgatgctagtgtgatttttgggaggatttgagttgttaatctgggagttgttgggaggttctcgtaggcggattgtagatgaagtcgcccgcacgatttgcgtggcttgttgggtagctagggttagatctgctcggatttttcattgttacttattgagagataatgtagctaacctttacttgttcatctatgtatctcgtattcgtattcatctggttcgatggtgctagatagatgcgcctgatttgtccgatcgaattgggtagcatccgcggcttgtttggtagtgttctgattgatttgtcgctctagatctgagtggaataatattacatctcaacatgttactagaaacttggtttatagctccggatttacatgtttattcttatgtaaggttttaaatgaaagatttatgctactgctgctcgttgatcctttagcatccacctgaggaacatgcatgcatctgttacttcttttgatatatgcttagatagttgttagtatatactgctgttgttcgatgatccttcaggatgaacatgcatgatcatgttacttgtttttatatgcttctgctgttcgttgattctttagtactacctacctgatcatcttgcatgtttcctgcttgttagagattaattgattaggcttaccttgttgcctggtgattcttccttgcaggtg

SEQ ID NO: 16 - DNA, 1954 bp, Arundo donax
tgatgtatccgtccacggtggtgtgtccaatcagtgaataatctagttagtgaagccagaagtccatagtgccccttgctctgtcaccatatatccagttcaaccgcaccaatttgccatctcgaactggttcatgttttattcaggttggtaaatgaattttgccaattcaatgtagttagatatttccatgtcattttagtacatttaccaattttttatattctggctagaaaaggagaatggtgacgtctttcggaagatcaagatcaattatcaagtatcagcaacagcacctgaaggttggagtgcattagttgtcattgagaataatgctagctattcattgcactggcattagagacagagagggcgagccagtttgacatggcaaattagcacagtcaaactggatacgtggtgacggagggaggggcactatgaatttttggtgacggagggaggggcactatgaatttttggctttgctgacgggacacgccactatggatgaaattggacaaaatacgaatattcaaggatgaaagtggtcggtttgatagttcagggatgaaatgtgtctttgggcaaactttgaggacgaagttgcctattttgcattaaacgaatatatttatataccccaaaaaaaagaatacacatctccactccgagccggcatgtggggtccccactagtcagccactgtatggcgccgactagctcaacggccacgaaccagccaaccaccagcgcaacctaaacggcgtaaacgttgacggcatctctctctcgccccgtctcgaagcttccgcaccgctcgctggtcgctgcccggcgccgctcgtgctggactctttccgtggcggcttccgcgaaattgcgtggtggagaggagagacggaaccgtcacggcactggattccttccccacccggcttggccggcccctcctcgcctccataaataggcaccccgtcctcgcctcctctccccacctcatctcctcctttcccgtgaaccgtgaacacaacccgacccagatcccctcttgcgagcttcgtcgatccctcctccgcgtcaaggtacggagcttctcctcccccttcttctctagatcggcgtgttatgttgtttccgtggttgcttggttggatgaatcgaatgattcttagggcctaggaggctggttagatctgttgcgttctgtttcgtagatggattttggtgtaagatcaggtcggttccgctgtttaacttgtgatgctagtgtgatttttgggaggatttgagttgttaatctgggagttgttgggaggttctcgtaggcggattgtagatgaagtcgcccgcacgatttgcgtggcttgttgggtagctagggttagatctgctcggatttttcattgttacttattgagagataatgtagctaacctttacttgttcatctatgtatctcgtattcgtattcatctggttcgatggtgctagatagatgcgcctgatttgtccgatcgaattgggtagcatccgcggcttgtttggtagtgttctgattgatttgtcgctctagatctgagtggaataatattacatctcaacatgttactagaaacttggtttatagctccggatttacatgtttattcttatgtaaggttttaaatgaaagatttatgctactgctgctcgttgatcctttagcatccacctgaggaacatgcatgcatctgttacttcttttgatatatgcttagatagttgttagtatatactgctgttgttcgatgatccttcaggatgaacatgcatgatcatgttacttgtttttatatgcttctgctgttcgttgattctttagtactacctacctgatcatcttgcatgtttcctgcttgttagagattaattgattaggcttaccttgttgcctggtgattcttccttgcag

SEQ ID NO: 17 - DNA, 1000 bp, Arundo donax
tgatgtatccgtccacggtggtgtgtccaatcagtgaataatctagttagtgaagccagaagtccatagtgccccttgctctgtcaccatatatccagttcaaccgcaccaatttgccatctcgaactggttcatgttttattcaggttggtaaatgaattttgccaattcaatgtagttagatatttccatgtcattttagtacatttaccaattttttatattctggctagaaaaggagaatggtgacgtctttcggaagatcaagatcaattatcaagtatcagcaacagcacctgaaggttggagtgcattagttgtcattgagaataatgctagctattcattgcactggcattagagacagagagggcgagccagtttgacatggcaaattagcacagtcaaactggatacgtggtgacggagggaggggcactatgaatttttggtgacggagggaggggcactatgaatttttggctttgctgacgggacacgccactatggatgaaattggacaaaatacgaatattcaaggatgaaagtggtcggtttgatagttcagggatgaaatgtgtctttgggcaaactttgaggacgaagttgcctattttgcattaaacgaatatatttatataccccaaaaaaaagaatacacatctccactccgagccggcatgtggggtccccactagtcagccactgtatggcgccgactagctcaacggccacgaaccagccaaccaccagcgcaacctaaacggcgtaaacgttgacggcatctctctctcgccccgtctcgaagcttccgcaccgctcgctggtcgctgcccggcgccgctcgtgctggactctttccgtggcggcttccgcgaaattgcgtggtggagaggagagacggaaccgtcacggcactggattccttccccacccggcttggccggcccctcctcgcctccataaataggcaccccgtcctcgcctcctctccccacct

SEQ ID NO: 18 - DNA, 1957 bp, Arundo donax
tgatgtatccgtccacggtggtgtgtccaatcagtgaataatctagttagtgaagccagaagtccatagtgccccttgctctgtcaccatatatccagttcaaccgcaccaatttgccatctcgaactggttcatgttttattcaggttggtaaatgaattttgccaattcaatgtagttagatatttccatgtcattttagtacatttaccaattttttatattctggctagaaaaggagaatggtgacgtctttcggaagatcaagatcaattatcaagtatcagcaacagcacctgaaggttggagtgcattagttgtcattgagaataatgctagctattcattgcactggcattagagacagagagggcgagccagtttgacatggcaaattagcacagtcaaactggatacgtggtgacggagggaggggcactatgaatttttggtgacggagggaggggcactatgaatttttggctttgctgacgggacacgccactatggatgaaattggacaaaatacgaatattcaaggatgaaagtggtcggtttgatagttcagggatgaaatgtgtctttgggcaaactttgaggacgaagttgcctattttgcattaaacgaatatatttatataccccaaaaaaaagaatacacatctccactccgagccggcatgtggggtccccactagtcagccactgtatggcgccgactagctcaacggccacgaaccagccaaccaccagcgcaacctaaacggcgtaaacgttgacggcatctctctctcgccccgtctcgaagcttccgcaccgctcgctggtcgctgcccggcgccgctcgtgctggactctttccgtggcggcttccgcgaaattgcgtggtggagaggagagacggaaccgtcacggcactggattccttccccacccggcttggccggcccctcctcgcctccataaataggcaccccgtcctcgcctcctctccccacctcatctcctcctttcccgtgaaccgtgaacacaacccgacccagatcccctcttgcgagcttcgtcgatccctcctccgcgtcaaggtacggagcttctcctcccccttcttctctagatcggcgtgttatgttgtttccgtggttgcttggttggatgaatcgaatgattcttagggcctaggaggctggttagatctgttgcgttctgtttcgtagatggattttggtgtaagatcaggtcggttccgctgtttaacttgtgatgctagtgtgatttttgggaggatttgagttgttaatctgggagttgttgggaggttctcgtaggcggattgtagatgaagtcgcccgcacgatttgcgtggcttgttgggtagctagggttagatctgctcggatttttcattgttacttattgagagataatgtagctaacctttacttgttcatctatgtatctcgtattcgtattcatctggttcgatggtgctagatagatgcgcctgatttgtccgatcgaattgggtagcatccgcggcttgtttggtagtgttctgattgatttgtcgctctagatctgagtggaataatattacatctcaacatgttactagaaacttggtttatagctccggatttacatgtttattcttatgtaaggttttaaatgaaagatttatgctactgctgctcgttgatcctttagcatccacctgaggaacatgcatgcatctgttacttcttttgatatatgcttagatagttgttagtatatactgctgttgttcgatgatccttcaggatgaacatgcatgatcatgttacttgtttttatatgcttctgctgttcgttgattctttagtactacctacctgatcatcttgcatgtttcctgcttgttagagattaattgattaggcttaccttgttgcctggtgattcttccttgcaggtg

SEQ ID NO: 19 - DNA, 1957 bp, Arundo donax
tgatgtatccgtccacggtggtgtgtccaatcagtgaataatctagttagtgaagccagaagtccatagtgccccttgctctgtcaccatatatccagttcaaccgcaccaatttgccatctcgaactggttcatgttttattcaggttggtaaatgaattttgccaattcaatgtagttagatatttccatgtcattttagtacatttaccaattttttatattctggctagaaaaggagaatggtgacgtctttcggaagatcaagatcaattatcaagtatcagcaacagcacctgaaggttggagtgcattagttgtcattgagaataatgctagctattcattgcactggcattagagacagagagggcgagccagtttgacatggcaaattagcacagtcaaactggatacgtggtgacggagggaggggcactatgaatttttggtgacggagggaggggcactatgaatttttggctttgctgacgggacacgccactatggatgaaattggacaaaatacgaatattcaaggatgaaagtggtcggtttgatagttcagggatgaaatgtgtctttgggcaaactttgaggacgaagttgcctattttgcattaaacgaatatatttatataccccaaaaaaaagaatacacatctccactccgagccggcatgtggggtccccactagtcagccactgtatggcgccgactagctcaacggccacgaaccagccaaccaccagcgcaacctaaacggcgtaaacgttgacggcatctctctctcgccccgtctcgaagcttccgcaccgctcgctggtcgctgcccggcgccgctcgtgctggactctttccgtggcggcttccgcgaaattgcgtggtggagaggagagacggaaccgtcacggcactggattccttccccacccggcttggccggcccctcctcgcctccataaataggcaccccgtcctcgcctcctctccccacctcatctcctcctttcccgtgaaccgtgaacacaacccgacccagatcccctcttgcgagcttcgtcgatccctcctccgcgtcaaggtacggagcttctcctcccccttcttctctagatcggcgtgttatgttgtttccgtggttgcttggttggatgaatcgaatgattcttagggcctaggaggctggttagatctgttgcgttctgtttcgtagatggattttggtgtaagatcaggtcggttccgctgtttaacttgtgatgctagtgtgatttttgggaggatttgagttgttaatctgggagttgttgggaggttctcgtaggcggattgtagatgaagtcgcccgcacgatttgcgtggcttgttgggtagctagggttagatctgctcggatttttcattgttacttattgagagataatgtagctaacctttacttgttcatctatgtatatcgtattcgtattcatctggttcgatggtgctagatagatgcgcctgatttgtccgatcgaattgggtagcatccgcggcttgtttggtagtgttctgattgatttgtcgctctagatctgagtggaataatattacatctcaacatgttactagaaacttggtttatagctccggatttacatgtttattcttatgtaaggttttaaatgaaagatttatgctactgctgctcgttgatcctttagcatccacctgaggaacatgcatgcatctgttacttcttttgatatatgcttagatagttgttagtatatactgctgttgttcgatgatccttcaggatgaacatgcatgatcatgttacttgtttttatatgcttctgctgttcgttgattctttagtactacctacctgatcatcttgcatgtttcctgcttgttagagattaattgattaggcttaccttgttgcctggtgattcttccttgcaggtg

SEQ ID NO: 20 - DNA, 872 bp, Arundo donax
gtacggagcttctcctcccccttcttctctagatcggcgtgttatgttgtttccgtggttgcttggttggatgaatcgaatgattcttagggcctaggaggctggttagatctgttgcgttctgtttcgtagatggattttggtgtaagatcaggtcggttccgctgtttaacttgtgatgctagtgtgatttttgggaggatttgagttgttaatctgggagttgttgggaggttctcgtaggcggattgtagatgaagtcgcccgcacgatttgcgtggcttgttgggtagctagggttagatctgctcggatttttcattgttacttattgagagataatgtagctaacctttacttgttcatctatgtatatcgtattcgtattcatctggttcgatggtgctagatagatgcgcctgatttgtccgatcgaattgggtagcatccgcggcttgtttggtagtgttctgattgatttgtcgctctagatctgagtggaataatattacatctcaacatgttactagaaacttggtttatagctccggatttacatgtttattcttatgtaaggttttaaatgaaagatttatgctactgctgctcgttgatcctttagcatccacctgaggaacatgcatgcatctgttacttcttttgatatatgcttagatagttgttagtatatactgctgttgttcgatgatccttcaggatgaacatgcatgatcatgttacttgtttttatatgcttctgctgttcgttgattctttagtactacctacctgatcatcttgcatgtttcctgcttgttagagattaattgattaggcttaccttgttgcctggtgattcttccttgcaggtg

SEQ ID NO: 21 - DNA, 1712 bp, Arundo donax
gtgacgtctttcggaagatcaagatcaattatcaagtatcagcaacagcacctgaaggttggagtgcattagttgtcattgagaataatgctagctattcattgcactggcattagagacagagagggcgagccagtttgacatggcaaattagcacagtcaaactggatacgtggtgacggagggaggggcactatgaatttttggtgacggagggaggggcactatgaatttttggctttgctgacgggacacgccactatggatgaaattggacaaaatacgaatattcaaggatgaaagtggtcggtttgatagttcagggatgaaatgtgtctttgggcaaactttgaggacgaagttgcctattttgcattaaacgaatatatttatataccccaaaaaaaagaatacacatctccactccgagccggcatgtggggtccccactagtcagccactgtatggcgccgactagctcaacggccacgaaccagccaaccaccagcgcaacctaaacggcgtaaacgttgacggcatctctctctcgccccgtctcgaagcttccgcaccgctcgctggtcgctgcccggcgccgctcgtgctggactctttccgtggcggcttccgcgaaattgcgtggtggagaggagagacggaaccgtcacggcactggattccttccccacccggcttggccggcccctcctcgcctccataaataggcaccccgtcctcgcctcctctccccacctcatctcctcctttcccgtgaaccgtgaacacaacccgacccagatcccctcttgcgagcttcgtcgatccctcctccgcgtcaaggtacggagcttctcctcccccttcttctctagatcggcgtgttatgttgtttccgtggttgcttggttggatgaatcgaatgattcttagggcctaggaggctggttagatctgttgcgttctgtttcgtagatggattttggtgtaagatcaggtcggttccgctgtttaacttgtgatgctagtgtgatttttgggaggatttgagttgttaatctgggagttgttgggaggttctcgtaggcggattgtagatgaagtcgcccgcacgatttgcgtggcttgttgggtagctagggttagatctgctcggatttttcattgttacttattgagagataatgtagctaacctttacttgttcatctatgtatctcgtattcgtattcatctggttcgatggtgctagatagatgcgcctgatttgtccgatcgaattgggtagcatccgcggcttgtttggtagtgttctgattgatttgtcgctctagatctgagtggaataatattacatctcaacatgttactagaaacttggtttatagctccggatttacatgtttattcttatgtaaggttttaaatgaaagatttatgctactgctgctcgttgatcctttagcatccacctgaggaacatgcatgcatctgttacttcttttgatatatgcttagatagttgttagtatatactgctgttgttcgatgatccttcaggatgaacatgcatgatcatgttacttgtttttatatgcttctgctgttcgttgattctttagtactacctacctgatcatcttgcatgtttcctgcttgttagagattaattgattaggcttaccttgttgcctggtgattcttccttgcaggtg

SEQ ID NO: 22 - DNA, 755 bp, Arundo donax
gtgacgtctttcggaagatcaagatcaattatcaagtatcagcaacagcacctgaaggttggagtgcattagttgtcattgagaataatgctagctattcattgcactggcattagagacagagagggcgagccagtttgacatggcaaattagcacagtcaaactggatacgtggtgacggagggaggggcactatgaatttttggtgacggagggaggggcactatgaatttttggctttgctgacgggacacgccactatggatgaaattggacaaaatacgaatattcaaggatgaaagtggtcggtttgatagttcagggatgaaatgtgtctttgggcaaactttgaggacgaagttgcctattttgcattaaacgaatatatttatataccccaaaaaaaagaatacacatctccactccgagccggcatgtggggtccccactagtcagccactgtatggcgccgactagctcaacggccacgaaccagccaaccaccagcgcaacctaaacggcgtaaacgttgacggcatctctctctcgccccgtctcgaagcttccgcaccgctcgctggtcgctgcccggcgccgctcgtgctggactctttccgtggcggcttccgcgaaattgcgtggtggagaggagagacggaaccgtcacggcactggattccttccccacccggcttggccggcccctcctcgcctccataaataggcaccccgtcctcgcctcctctccccacct

SEQ ID NO: 23 - DNA, 3276 bp, Arundo donax
ggcctctttacgtttggcacaatttgatcgaatccaacacggcaagttagcctttgaagcttgaaccgggcactaatgcaagtatataataactgagaactacaagaaagcatattccttgaggtacttatgcaaccttacaattatcaaattaattaacaactagcagttagaattttatatcacaagaatatcatgaaccgtggatactacttcttaaagggctattctttttctgaatgtcgcagttggttattttaaccatattacaaactaggggtttaaatcccaaaaagttcacggaaagggattaagcaagtagttagcaagactcacacttatgaccgttagccaaattacacattggtcattccaggaggagtaatcccccatagctagttgttttgagtttgactacccaaacttgcataatcgttttcctagagggggggggggggttcaccattccatcaagatgaggcaaagctaaatgaaacacacgagaggcaaaacggactgacgtgatagagtttttaataaatatcaaatatgtagagtcaaccaaagaaaaaagatatcccaatggctaaactttggatctatgtcgtaattcgtgttttaggacatacaaggcgaattccttctacggcaaactctagaatagctgggcgacaatggcctcacgatagcctcaaagagttggtagcaactttgagatcttttgatccgaaactcaattatgtagtacaatgatatttagatagattgattgaaagttgggggtgggggcgaaagcgaaggggatctcaatattaatacatctatagtgaatggatatagaaaacacaggatttccaattcaagtagaaataggaggaacggaacagatctagcaatagtagccaccaaagacgaggaggattctagattgcaaatccaaggtgaaaggaagaaatgttgaactatccagaataaggcggattggccaaggaggcggaagtctctagaaagaagtcatttggctctgagggctcacttgatgcgagaaggaagactgactgaggaatggattttggtggaccgaggaaattggtgctgggttgcagaggcatgtatgtgggaaaagaggcagtggcaacgatcgagagaggagaagggaatgaggtaagtatttgaagtgaagaggagcccatataggtgaaaaataaaaataatccatcgtggattcaaataatcaaagggctatgacctttcatcaattttagaaaagtgaaaacaaccggtttaacacctatatgcaccattttcctacatagatttttaacttcttacttaaccatgttgactaagagcaagtggagagcactctcatttcatagaacaagtgatgaatgccaacctgcattattatcttaattagactttgatcatcaagtggaatcccatttatcttaataatcttggcaacattgttataatgctacttcatatgctaattcttcaaagctaacatcgttaaacgaatacatatctcctgtattctaagaccctatttagaatacagaaattttacagaaatcagttcaattctcgtagaattgggaaagaaatcctccgttccaaacgtgacctaagccggcatggcacgaccccactcgtcaggcactgtatgtaaacgtcagcaactccgtggcaagtaacgtcgagaggaggagcgggcctaacggcgccgactagctcaacggccaccaaccagccaaccaccagcgcaaccgaaacggcgcaaacgttgacgtcatctctctctctctcgcgccccgcgtcccgaagcttccgcaccactcgctggtcgctgctagctgggccccaccggccggccccgttcgtgctggactcttcttcctcgaaattgcgtggtggagagggagagggggcacctcgagacggaaccgtcacggcacgggattccttccccacccggcccctcctcgtctccataaataggcgccccctcctcgcgtcctctcccccgtctcatctcctcctgttccgtgaaccgtgaacgcaacccgacccccagatctctctcgcgagcatcgtcgatccctcctccgcgtcaaggtacggatcttctccttcctcccccttcccctctgggtcggcgtgtcgtgttgtttctctagttgcttggctggatggatcgagtggttcttagggcttagatggctggttagatctgttgcgttctgtttcgtagatggatttttggtgtagatctggtaggttatgctggttaactggtgatgctcctgcgatttttgggggatctgagttgttaatctggtagttgtatggggttctcgtagccggattgtagatgaaatcgtccgcgcggtttgcgtggctcgttggttagctagggttagatctgctcggatttttcattgttcctgattcagagatgtagttaacctttacttgttcatctttgtatctcgtattcgtacctgcatgtatgatctgtttcgatggtgctagataggtgcgcctgatttgtccgatcgaatctggtagcatgcgctgtttgtttggtagtgttctgattgatttgtcgctctagatctgagtagaataggattatttctcaacatgatattagaagcttggtttatagctccggattagcatgtatgttacatgtttattcttatgtaaggttttaaacggaagatatatgctactgctgctcattgattctttatcatccacctgagtccatgcatgcttctgttacttcttttgatatgtgcttagatagctgttgatatgtactgctgctgttagatgatccttcaggatgaacatgcatgattctgttacttgttttggtatgcttagataaatcaagatacgcttctgctgttcgttgattctttagtactacctacctgatcagcttagatagatcaagatatgcttctgctgttcgttgattctttagtaatacctacctgatcagcttagatagatcaagatacgcttctgctgttcgttgattctctagtactacctacctgataaacatgcatgttttctgcttgttaaaggttgattgcttaggctcatctttttcttttcgttgattctctagtactacctacctgataaacatgcatgttttctgcttgttaaagattgattgcttagtctcatctttttctttctcttttgtctaccgccaggcctaaccttgttgctggtgactctttcttgcag

SEQ ID NO: 24 - DNA, 2033 bp, Arundo donax
ggcctctttacgtttggcacaatttgatcgaatccaacacggcaagttagcctttgaagcttgaaccgggcactaatgcaagtatataataactgagaactacaagaaagcatattccttgaggtacttatgcaaccttacaattatcaaattaattaacaactagcagttagaattttatatcacaagaatatcatgaaccgtggatactacttcttaaagggctattctttttctgaatgtcgcagttggttattttaaccatattacaaactaggggtttaaatcccaaaaagttcacggaaagggattaagcaagtagttagcaagactcacacttatgaccgttagccaaattacacattggtcattccaggaggagtaatcccccatagctagttgttttgagtttgactacccaaacttgcataatcgttttcctagagggggggggggggttcaccattccatcaagatgaggcaaagctaaatgaaacacacgagaggcaaaacggactgacgtgatagagtttttaataaatatcaaatatgtagagtcaaccaaagaaaaaagatatcccaatggctaaactttggatctatgtcgtaattcgtgttttaggacatacaaggcgaattccttctacggcaaactctagaatagctgggcgacaatggcctcacgatagcctcaaagagttggtagcaactttgagatcttttgatccgaaactcaattatgtagtacaatgatatttagatagattgattgaaagttgggggtgggggcgaaagcgaaggggatctcaatattaatacatctatagtgaatggatatagaaaacacaggatttccaattcaagtagaaataggaggaacggaacagatctagcaatagtagccaccaaagacgaggaggattctagattgcaaatccaaggtgaaaggaagaaatgttgaactatccagaataaggcggattggccaaggaggcggaagtctctagaaagaagtcatttggctctgagggctcacttgatgcgagaaggaagactgactgaggaatggattttggtggaccgaggaaattggtgctgggttgcagaggcatgtatgtgggaaaagaggcagtggcaacgatcgagagaggagaagggaatgaggtaagtatttgaagtgaagaggagcccatataggtgaaaaataaaaataatccatcgtggattcaaataatcaaagggctatgacctttcatcaattttagaaaagtgaaaacaaccggtttaacacctatatgcaccattttcctacatagatttttaacttcttacttaaccatgttgactaagagcaagtggagagcactctcatttcatagaacaagtgatgaatgccaacctgcattattatcttaattagactttgatcatcaagtggaatcccatttatcttaataatcttggcaacattgttataatgctacttcatatgctaattcttcaaagctaacatcgttaaacgaatacatatctcctgtattctaagaccctatttagaatacagaaattttacagaaatcagttcaattctcgtagaattgggaaagaaatcctccgttccaaacgtgacctaagccggcatggcacgaccccactcgtcaggcactgtatgtaaacgtcagcaactccgtggcaagtaacgtcgagaggaggagcgggcctaacggcgccgactagctcaacggccaccaaccagccaaccaccagcgcaaccgaaacggcgcaaacgttgacgtcatctctctctctctcgcgccccgcgtcccgaagcttccgcaccactcgctggtcgctgctagctgggccccaccggccggccccgttcgtgctggactcttcttcctcgaaattgcgtggtggagagggagagggggcacctcgagacggaaccgtcacggcacgggattccttccccacccggcccctcctcgtctccataaataggcgccccctcctcgcgtcctctcccccgt

SEQ ID NO: 25 - DNA, 88 bp, Arundo donax
ctcatctcctcctgttccgtgaaccgtgaacgcaacccgacccccagatctctctcgcgagcatcgtcgatccctcctccgcgtcaag

SEQ ID NO: 26 - DNA, 1155 bp, Arundo donax
gtacggatcttctccttcctcccccttcccctctgggtcggcgtgtcgtgttgtttctctagttgcttggctggatggatcgagtggttcttagggcttagatggctggttagatctgttgcgttctgtttcgtagatggatttttggtgtagatctggtaggttatgctggttaactggtgatgctcctgcgatttttgggggatctgagttgttaatctggtagttgtatggggttctcgtagccggattgtagatgaaatcgtccgcgcggtttgcgtggctcgttggttagctagggttagatctgctcggatttttcattgttcctgattcagagatgtagttaacctttacttgttcatctttgtatctcgtattcgtacctgcatgtatgatctgtttcgatggtgctagataggtgcgcctgatttgtccgatcgaatctggtagcatgcgctgtttgtttggtagtgttctgattgatttgtcgctctagatctgagtagaataggattatttctcaacatgatattagaagcttggtttatagctccggattagcatgtatgttacatgtttattcttatgtaaggttttaaacggaagatatatgctactgctgctcattgattctttatcatccacctgagtccatgcatgcttctgttacttcttttgatatgtgcttagatagctgttgatatgtactgctgctgttagatgatccttcaggatgaacatgcatgattctgttacttgttttggtatgcttagataaatcaagatacgcttctgctgttcgttgattctttagtactacctacctgatcagcttagatagatcaagatatgcttctgctgttcgttgattctttagtaatacctacctgatcagcttagatagatcaagatacgcttctgctgttcgttgattctctagtactacctacctgataaacatgcatgttttctgcttgttaaaggttgattgcttaggctcatctttttcttttcgttgattctctagtactacctacctgataaacatgcatgttttctgcttgttaaagattgattgcttagtctcatctttttctttctcttttgtctaccgccaggcctaaccttgttgctggtgactctttcttgcag

SEQ ID NO: 27 - DNA, 3250 bp, Arundo donax
gaatccaacacggcaagttagcctttgaagcttgaaccgggcactaatgcaagtatataataactgagaactacaagaaagcatattccttgaggtacttatgcaaccttacaattatcaaattaattaacaactagcagttagaattttatatcacaagaatatcatgaaccgtggatactacttcttaaagggctattctttttctgaatgtcgcagttggttattttaaccatattacaaactaggggtttaaatcccaaaaagttcacggaaagggattaagcaagtagttagcaagactcacacttatgaccgttagccaaattacacattggtcattccaggaggagtaatcccccatagctagttgttttgagtttgactacccaaacttgcataatcgttttcctagagggggggggggggttcaccattccatcaagatgaggcaaagctaaatgaaacacacgagaggcaaaacggactgacgtgatagagtttttaataaatatcaaatatgtagagtcaaccaaagaaaaaagatatcccaatggctaaactttggatctatgtcgtaattcgtgttttaggacatacaaggcgaattccttctacggcaaactctagaatagctgggcgacaatggcctcacgatagcctcaaagagttggtagcaactttgagatcttttgatccgaaactcaattatgtagtacaatgatatttagatagattgattgaaagttgggggtgggggcgaaagcgaaggggatctcaatattaatacatctatagtgaatggatatagaaaacacaggatttccaattcaagtagaaataggaggaacggaacagatctagcaatagtagccaccaaagacgaggaggattctagattgcaaatccaaggtgaaaggaagaaatgttgaactatccagaataaggcggattggccaaggaggcggaagtctctagaaagaagtcatttggctctgagggctcacttgatgcgagaaggaagactgactgaggaatggattttggtggaccgaggaaattggtgctgggttgcagaggcatgtatgtgggaaaagaggcagtggcaacgatcgagagaggagaagggaatgaggtaagtatttgaagtgaagaggagcccatataggtgaaaaataaaaataatccatcgtggattcaaataatcaaagggctatgacctttcatcaattttagaaaagtgaaaacaaccggtttaacacctatatgcaccattttcctacatagatttttaacttcttacttaaccatgttgactaagagcaagtggagagcactctcatttcatagaacaagtgatgaatgccaacctgcattattatcttaattagactttgatcatcaagtggaatcccatttatcttaataatcttggcaacattgttataatgctacttcatatgctaattcttcaaagctaacatcgttaaacgaatacatatctcctgtattctaagaccctatttagaatacagaaattttacagaaatcagttcaattctcgtagaattgggaaagaaatcctccgttccaaacgtgacctaagccggcatggcacgaccccactcgtcaggcactgtatgtaaacgtcagcaactccgtggcaagtaacgtcgagaggaggagcgggcctaacggcgccgactagctcaacggccaccaaccagccaaccaccagcgcaaccgaaacggcgcaaacgttgacgtcatctctctctctctcgcgccccgcgtcccgaagcttccgcaccactcgctggtcgctgctagctgggccccaccggccggccccgttcgtgctggactcttcttcctcgaaattgcgtggtggagagggagagggggcacctcgagacggaaccgtcacggcacgggattccttccccacccggcccctcctcgtctccataaataggcgccccctcctcgcgtcctctcccccgtctcatctcctcctgttccgtgaaccgtgaacgcaacccgacccccagatctctctcgcgagcatcgtcgatccctcctccgcgtcaaggtacggatcttctccttcctcccccttcccctctgggtcggcgtgtcgtgttgtttctctagttgcttggctggatggatcgagtggttcttagggcttagatggctggttagatctgttgcgttctgtttcgtagatggatttttggtgtagatctggtaggttatgctggttaactggtgatgctcctgcgatttttgggggatctgagttgttaatctggtagttgtatggggttctcgtagccggattgtagatgaaatcgtccgcgcggtttgcgtggctcgttggttagctagggttagatctgctcggatttttcattgttcctgattcagagatgtagttaacctttacttgttcatctttgtatctcgtattcgtacctgcatgtatgatctgtttcgatggtgctagataggtgcgcctgatttgtccgatcgaatctggtagcatgcgctgtttgtttggtagtgttctgattgatttgtcgctctagatctgagtagaataggattatttctcaacatgatattagaagcttggtttatagctccggattagcatgtatgttacatgtttattcttatgtaaggttttaaacggaagatatatgctactgctgctcattgattctttatcatccacctgagtccatgcatgcttctgttacttcttttgatatgtgcttagatagctgttgatatgtactgctgctgttagatgatccttcaggatgaacatgcatgattctgttacttgttttggtatgcttagataaatcaagatacgcttctgctgttcgttgattctttagtactacctacctgatcagcttagatagatcaagatatgcttctgctgttcgttgattctttagtaatacctacctgatcagcttagatagatcaagatacgcttctgctgttcgttgattctctagtactacctacctgataaacatgcatgttttctgcttgttaaaggttgattgcttaggctcatctttttcttttcgttgattctctagtactacctacctgataaacatgcatgttttctgcttgttaaagattgattgcttagtctcatctttttctttctcttttgtctaccgccaggcctaaccttgttgctggtgactctttcttgcaggtg

SEQ ID NO: 28 - DNA, 2004 bp, Arundo donax
gaatccaacacggcaagttagcctttgaagcttgaaccgggcactaatgcaagtatataataactgagaactacaagaaagcatattccttgaggtacttatgcaaccttacaattatcaaattaattaacaactagcagttagaattttatatcacaagaatatcatgaaccgtggatactacttcttaaagggctattctttttctgaatgtcgcagttggttattttaaccatattacaaactaggggtttaaatcccaaaaagttcacggaaagggattaagcaagtagttagcaagactcacacttatgaccgttagccaaattacacattggtcattccaggaggagtaatcccccatagctagttgttttgagtttgactacccaaacttgcataatcgttttcctagagggggggggggggttcaccattccatcaagatgaggcaaagctaaatgaaacacacgagaggcaaaacggactgacgtgatagagtttttaataaatatcaaatatgtagagtcaaccaaagaaaaaagatatcccaatggctaaactttggatctatgtcgtaattcgtgttttaggacatacaaggcgaattccttctacggcaaactctagaatagctgggcgacaatggcctcacgatagcctcaaagagttggtagcaactttgagatcttttgatccgaaactcaattatgtagtacaatgatatttagatagattgattgaaagttgggggtgggggcgaaagcgaaggggatctcaatattaatacatctatagtgaatggatatagaaaacacaggatttccaattcaagtagaaataggaggaacggaacagatctagcaatagtagccaccaaagacgaggaggattctagattgcaaatccaaggtgaaaggaagaaatgttgaactatccagaataaggcggattggccaaggaggcggaagtctctagaaagaagtcatttggctctgagggctcacttgatgcgagaaggaagactgactgaggaatggattttggtggaccgaggaaattggtgctgggttgcagaggcatgtatgtgggaaaagaggcagtggcaacgatcgagagaggagaagggaatgaggtaagtatttgaagtgaagaggagcccatataggtgaaaaataaaaataatccatcgtggattcaaataatcaaagggctatgacctttcatcaattttagaaaagtgaaaacaaccggtttaacacctatatgcaccattttcctacatagatttttaacttcttacttaaccatgttgactaagagcaagtggagagcactctcatttcatagaacaagtgatgaatgccaacctgcattattatcttaattagactttgatcatcaagtggaatcccatttatcttaataatcttggcaacattgttataatgctacttcatatgctaattcttcaaagctaacatcgttaaacgaatacatatctcctgtattctaagaccctatttagaatacagaaattttacagaaatcagttcaattctcgtagaattgggaaagaaatcctccgttccaaacgtgacctaagccggcatggcacgaccccactcgtcaggcactgtatgtaaacgtcagcaactccgtggcaagtaacgtcgagaggaggagcgggcctaacggcgccgactagctcaacggccaccaaccagccaaccaccagcgcaaccgaaacggcgcaaacgttgacgtcatctctctctctctcgcgccccgcgtcccgaagcttccgcaccactcgctggtcgctgctagctgggccccaccggccggccccgttcgtgctggactcttcttcctcgaaattgcgtggtggagagggagagggggcacctcgagacggaaccgtcacggcacgggattccttccccacccggcccctcctcgtctccataaataggcgccccctcctcgcgtcctctcccccgt

SEQ ID NO: 29 - DNA, 1158 bp, Arundo donax
gtacggatcttctccttcctcccccttcccctctgggtcggcgtgtcgtgttgtttctctagttgcttggctggatggatcgagtggttcttagggcttagatggctggttagatctgttgcgttctgtttcgtagatggatttttggtgtagatctggtaggttatgctggttaactggtgatgctcctgcgatttttgggggatctgagttgttaatctggtagttgtatggggttctcgtagccggattgtagatgaaatcgtccgcgcggtttgcgtggctcgttggttagctagggttagatctgctcggatttttcattgttcctgattcagagatgtagttaacctttacttgttcatctttgtatctcgtattcgtacctgcatgtatgatctgtttcgatggtgctagataggtgcgcctgatttgtccgatcgaatctggtagcatgcgctgtttgtttggtagtgttctgattgatttgtcgctctagatctgagtagaataggattatttctcaacatgatattagaagcttggtttatagctccggattagcatgtatgttacatgtttattcttatgtaaggttttaaacggaagatatatgctactgctgctcattgattctttatcatccacctgagtccatgcatgcttctgttacttcttttgatatgtgcttagatagctgttgatatgtactgctgctgttagatgatccttcaggatgaacatgcatgattctgttacttgttttggtatgcttagataaatcaagatacgcttctgctgttcgttgattctttagtactacctacctgatcagcttagatagatcaagatatgcttctgctgttcgttgattctttagtaatacctacctgatcagcttagatagatcaagatacgcttctgctgttcgttgattctctagtactacctacctgataaacatgcatgttttctgcttgttaaaggttgattgcttaggctcatctttttcttttcgttgattctctagtactacctacctgataaacatgcatgttttctgcttgttaaagattgattgcttagtctcatctttttctttctcttttgtctaccgccaggcctaaccttgttgctggtgactctttcttgcaggtg

SEQ ID NO: 30 - DNA, 2247 bp, Arundo donax
tcacttgatgcgagaaggaagactgactgaggaatggattttggtggaccgaggaaattggtgctgggttgcagaggcatgtatgtgggaaaagaggcagtggcaacgatcgagagaggagaagggaatgaggtaagtatttgaagtgaagaggagcccatataggtgaaaaataaaaataatccatcgtggattcaaataatcaaagggctatgacctttcatcaattttagaaaagtgaaaacaaccggtttaacacctatatgcaccattttcctacatagatttttaacttcttacttaaccatgttgactaagagcaagtggagagcactctcatttcatagaacaagtgatgaatgccaacctgcattattatcttaattagactttgatcatcaagtggaatcccatttatcttaataatcttggcaacattgttataatgctacttcatatgctaattcttcaaagctaacatcgttaaacgaatacatatctcctgtattctaagaccctatttagaatacagaaattttacagaaatcagttcaattctcgtagaattgggaaagaaatcctccgttccaaacgtgacctaagccggcatggcacgaccccactcgtcaggcactgtatgtaaacgtcagcaactccgtggcaagtaacgtcgagaggaggagcgggcctaacggcgccgactagctcaacggccaccaaccagccaaccaccagcgcaaccgaaacggcgcaaacgttgacgtcatctctctctctctcgcgccccgcgtcccgaagcttccgcaccactcgctggtcgctgctagctgggccccaccggccggccccgttcgtgctggactcttcttcctcgaaattgcgtggtggagagggagagggggcacctcgagacggaaccgtcacggcacgggattccttccccacccggcccctcctcgtctccataaataggcgccccctcctcgcgtcctctcccccgtctcatctcctcctgttccgtgaaccgtgaacgcaacccgacccccagatctctctcgcgagcatcgtcgatccctcctccgcgtcaaggtacggatcttctccttcctcccccttcccctctgggtcggcgtgtcgtgttgtttctctagttgcttggctggatggatcgagtggttcttagggcttagatggctggttagatctgttgcgttctgtttcgtagatggatttttggtgtagatctggtaggttatgctggttaactggtgatgctcctgcgatttttgggggatctgagttgttaatctggtagttgtatggggttctcgtagccggattgtagatgaaatcgtccgcgcggtttgcgtggctcgttggttagctagggttagatctgctcggatttttcattgttcctgattcagagatgtagttaacctttacttgttcatctttgtatctcgtattcgtacctgcatgtatgatctgtttcgatggtgctagataggtgcgcctgatttgtccgatcgaatctggtagcatgcgctgtttgtttggtagtgttctgattgatttgtcgctctagatctgagtagaataggattatttctcaacatgatattagaagcttggtttatagctccggattagcatgtatgttacatgtttattcttatgtaaggttttaaacggaagatatatgctactgctgctcattgattctttatcatccacctgagtccatgcatgcttctgttacttcttttgatatgtgcttagatagctgttgatatgtactgctgctgttagatgatccttcaggatgaacatgcatgattctgttacttgttttggtatgcttagataaatcaagatacgcttctgctgttcgttgattctttagtactacctacctgatcagcttagatagatcaagatatgcttctgctgttcgttgattctttagtaatacctacctgatcagcttagatagatcaagatacgcttctgctgttcgttgattctctagtactacctacctgataaacatgcatgttttctgcttgttaaaggttgattgcttaggctcatctttttcttttcgttgattctctagtactacctacctgataaacatgcatgttttctgcttgttaaagattgattgcttagtctcatctttttctttctcttttgtctaccgccaggcctaaccttgttgctggtgactctttcttgcaggtg

SEQ ID NO: 31 - DNA, 1001 bp, Arundo donax
tcacttgatgcgagaaggaagactgactgaggaatggattttggtggaccgaggaaattggtgctgggttgcagaggcatgtatgtgggaaaagaggcagtggcaacgatcgagagaggagaagggaatgaggtaagtatttgaagtgaagaggagcccatataggtgaaaaataaaaataatccatcgtggattcaaataatcaaagggctatgacctttcatcaattttagaaaagtgaaaacaaccggtttaacacctatatgcaccattttcctacatagatttttaacttcttacttaaccatgttgactaagagcaagtggagagcactctcatttcatagaacaagtgatgaatgccaacctgcattattatcttaattagactttgatcatcaagtggaatcccatttatcttaataatcttggcaacattgttataatgctacttcatatgctaattcttcaaagctaacatcgttaaacgaatacatatctcctgtattctaagaccctatttagaatacagaaattttacagaaatcagttcaattctcgtagaattgggaaagaaatcctccgttccaaacgtgacctaagccggcatggcacgaccccactcgtcaggcactgtatgtaaacgtcagcaactccgtggcaagtaacgtcgagaggaggagcgggcctaacggcgccgactagctcaacggccaccaaccagccaaccaccagcgcaaccgaaacggcgcaaacgttgacgtcatctctctctctctcgcgccccgcgtcccgaagcttccgcaccactcgctggtcgctgctagctgggccccaccggccggccccgttcgtgctggactcttcttcctcgaaattgcgtggtggagagggagagggggcacctcgagacggaaccgtcacggcacgggattccttccccacccggcccctcctcgtctccataaataggcgccccctcctcgcgtcctctcccccgt

SEQ ID NO: 32 - DNA, 1942 bp, Arundo donax
catgttgactaagagcaagtggagagcactctcatttcatagaacaagtgatgaatgccaacctgcattattatcttaattagactttgatcatcaagtggaatcccatttatcttaataatcttggcaacattgttataatgctacttcatatgctaattcttcaaagctaacatcgttaaacgaatacatatctcctgtattctaagaccctatttagaatacagaaattttacagaaatcagttcaattctcgtagaattgggaaagaaatcctccgttccaaacgtgacctaagccggcatggcacgaccccactcgtcaggcactgtatgtaaacgtcagcaactccgtggcaagtaacgtcgagaggaggagcgggcctaacggcgccgactagctcaacggccaccaaccagccaaccaccagcgcaaccgaaacggcgcaaacgttgacgtcatctctctctctctcgcgccccgcgtcccgaagcttccgcaccactcgctggtcgctgctagctgggccccaccggccggccccgttcgtgctggactcttcttcctcgaaattgcgtggtggagagggagagggggcacctcgagacggaaccgtcacggcacgggattccttccccacccggcccctcctcgtctccataaataggcgccccctcctcgcgtcctctcccccgtctcatctcctcctgttccgtgaaccgtgaacgcaacccgacccccagatctctctcgcgagcatcgtcgatccctcctccgcgtcaaggtacggatcttctccttcctcccccttcccctctgggtcggcgtgtcgtgttgtttctctagttgcttggctggatggatcgagtggttcttagggcttagatggctggttagatctgttgcgttctgtttcgtagatggatttttggtgtagatctggtaggttatgctggttaactggtgatgctcctgcgatttttgggggatctgagttgttaatctggtagttgtatggggttctcgtagccggattgtagatgaaatcgtccgcgcggtttgcgtggctcgttggttagctagggttagatctgctcggatttttcattgttcctgattcagagatgtagttaacctttacttgttcatctttgtatctcgtattcgtacctgcatgtatgatctgtttcgatggtgctagataggtgcgcctgatttgtccgatcgaatctggtagcatgcgctgtttgtttggtagtgttctgattgatttgtcgctctagatctgagtagaataggattatttctcaacatgatattagaagcttggtttatagctccggattagcatgtatgttacatgtttattcttatgtaaggttttaaacggaagatatatgctactgctgctcattgattctttatcatccacctgagtccatgcatgcttctgttacttcttttgatatgtgcttagatagctgttgatatgtactgctgctgttagatgatccttcaggatgaacatgcatgattctgttacttgttttggtatgcttagataaatcaagatacgcttctgctgttcgttgattctttagtactacctacctgatcagcttagatagatcaagatatgcttctgctgttcgttgattctttagtaatacctacctgatcagcttagatagatcaagatacgcttctgctgttcgttgattctctagtactacctacctgataaacatgcatgttttctgcttgttaaaggttgattgcttaggctcatctttttcttttcgttgattctctagtactacctacctgataaacatgcatgttttctgcttgttaaagattgattgcttagtctcatctttttctttctcttttgtctaccgccaggcctaaccttgttgctggtgactctttcttgcaggtg

SEQ ID NO: 33 - DNA, 696 bp, Arundo donax
catgttgactaagagcaagtggagagcactctcatttcatagaacaagtgatgaatgccaacctgcattattatcttaattagactttgatcatcaagtggaatcccatttatcttaataatcttggcaacattgttataatgctacttcatatgctaattcttcaaagctaacatcgttaaacgaatacatatctcctgtattctaagaccctatttagaatacagaaattttacagaaatcagttcaattctcgtagaattgggaaagaaatcctccgttccaaacgtgacctaagccggcatggcacgaccccactcgtcaggcactgtatgtaaacgtcagcaactccgtggcaagtaacgtcgagaggaggagcgggcctaacggcgccgactagctcaacggccaccaaccagccaaccaccagcgcaaccgaaacggcgcaaacgttgacgtcatctctctctctctcgcgccccgcgtcccgaagcttccgcaccactcgctggtcgctgctagctgggccccaccggccggccccgttcgtgctggactcttcttcctcgaaattgcgtggtggagagggagagggggcacctcgagacggaaccgtcacggcacgggattccttccccacccggcccctcctcgtctccataaataggcgccccctcctcgcgtcctctcccccgt

SEQ ID NO: 34 - DNA, 3511 bp, Bouteloua gracilis
gtggccagcttttgttctagttcaacggtcccggccttccgtgcacctaatactacactgattaatctattgcagctaacctcaaaagaaatacacttgcagttgtctgtcccaatcaagccactagcagactctcatgtcattgatggaggaaattaaattcagtctttgacgtggatgcaacaactgcacagtataccatgcatcttaattagccgttgtgtcaaagtttgttttgctgacgttttgagaaaaccaactttgaccaacaggagatgagcgtcttgcgtttggcacagtgtaatggaatccggcacggcaagttagactctgtagtgttagcggtctctttacgtttggcacaatttaattgaatcccggcatggcatgttagaccggagtgagccggcccttttactggtatgacactccctctgtcttgagtgtcgctgtgccagcttgtacctctgtctatgttcacagcccgtgctgtgtacctagaccctccgtttgtccacattcattttaatctctattgtatcttgtcaaaacctaaaagcctaaaacgactctgataaagggacagaaagattatacaagagcaagtgtataatgaaataatgtaagcgagctatatgaattgtcacgtgtcatatttatgttgagacgaagaagagaaaataaacaccatgcaaatttatggcgagtgatagatggccagatgggcacaaggcctcctatttcttaaatcggattttgtaagaacgaaaaaagggacttataagagaataggatagaccatatatcaatgatgtagtatgcatcaagatctaactattatatgagtgaattgataaatttattctaggtgacatggccttaacgatgaacagtacgtggttaaatcaatagaacaatagccaactctagcggctctaaaaaaagatatatattcgtcgaggcactattatgcaaccacatagtcaacttcaacgccgcttgagtgcgttctcatgttttttttttcttgcaaattacgcttttctaaaataaaataatttggatcgtgcaattatttcactttaggtgtgcgtgactacgtgagtaacaattttgaatctcagaaaggaaataaaagtataatactgctacctactttgaggattcagcttgttacttaaaaccgtctttaaggtcaaatgctcaagattcattcaacaattgaaacgtctcacatgattaaaccatgtataaggatgctaaggtcttgcttgacaatgtttttctaggaatttcatctaactttttgagtgaaactatcaaataataattttaaaacaattttataagagaagctccggagataaaagggcatctaatctatgttagaagagtgaagtttactccctctgtcccaaaaatagaattctaagtatgaaatgatttttttgttatacgaaaggagtatatatcacaagattgatgtcagttatgcttagggcacgtacacgacgctggtgctttaggtagacgttaatcgttgtttctgcattttattttattttgttgccacggtgtacatttgggtagacgtttgtcacaggcattgccactcaaacaagcagccggcgcttggagcttttatagtttgaaaagtgacggttttaatgatgggtaagctgattagtatatgtaagtttagctttttccattgtaggttaagccttaaggctcttacacaattgtttcattattctcattctttaagagcccatataagcgttcatgaattgtacatatccttagatgtttttttttttgggtaaagctcgagcttctctatctaaaagtagagaaatcagaaaaagattcatgttttggtagttttgatttcttgcctccataataattttggtttaccattttttgtttgattttagttttagaagcgtttatagcaggatttaaaatccaaaactaccattatcttcaagtgaccgtcagtgagccgtttaacggcgtcgacaagtccaacggacaccaaccagtgaaccaccagcgtcgagccaagcgatgcaaacggaacggccgagacgttgacacctttggcgcggcacggcatgtcggatctccctctctggccagagagttccagctccacctccacctccacctccaccggtggcggtttccaagtccgttccgttccgttccgttccgttccgttccgcctcctgcctgctcctctcagacggcacgaaaccgtgacggcaccggcagcacggggggattccttttccactgctccttcctcttcccttcctcgcccgccgctataaatagccagccccgtccccagattctttcccaacctcatctttgttcggagcacgcacacaacccgatccccaattccctcgtctctcctcgcgagcctcgtcgaccccccccttcaaggtacggcgatcatcctccctccctccctctctctaccttctcttctctagactagatcggcgacccggtccatggttagggcctgctagttctgttcctgttttttccatggctgcgaggtaaaatagatctgatggcgttatgatggttaactcgtcatactcttgcgatctatggtccctttaggacatcgatttaatttcggatggttcgagatcggtgatccatggttagtaccctaggcagtggggttagatccgtgctgttagggttcgtagatggattctgattgctcagtaactgggaaacctgggatggttctagctgggaatcctgggatggttctagctggttcgcagatgagatcgatttcatggtctgctatatcttgtttcgttgcctaggttccgtttaatctgtccgtggtatgatgttagcctttgataaggttcgatcgtgctagctacgtcctgcgcagcatttaattgtcaggtcataatttttagcattcctgtttttgtttggtttggttttgtctggttgggctgtagatagtttcaatctacctgtcggtttattttattaaatttggattggatctgtatgtgtcacatatatcttcatgattaagatggttggaattatctcttcatcttttagatatatatggataggtatatatgttgctgtgggttttactggtactttattagatatattcatgcttagatacatgaagcaacgtgctgttacagtttaataattcttgtttatctaataaacaaataaggataggtatatgttgctgatggttttactgatactttattagatagtactttgacatgaaggaacatcctgcgacagcttaataattattcttcatctaataaaaagcttgctttttaattattttaattattttgatatacttggatgatgtcatgcagcagctatgtgtgaattttcggccctgtcttcatatgatgtttatttgcttgggactgtttctttggctgataacttaccctgttgtttggtgatccttctgcag

SEQ ID NO: 35 - DNA, 2371 bp, Bouteloua gracilis
gtggccagcttttgttctagttcaacggtcccggccttccgtgcacctaatactacactgattaatctattgcagctaacctcaaaagaaatacacttgcagttgtctgtcccaatcaagccactagcagactctcatgtcattgatggaggaaattaaattcagtctttgacgtggatgcaacaactgcacagtataccatgcatcttaattagccgttgtgtcaaagtttgttttgctgacgttttgagaaaaccaactttgaccaacaggagatgagcgtcttgcgtttggcacagtgtaatggaatccggcacggcaagttagactctgtagtgttagcggtctctttacgtttggcacaatttaattgaatcccggcatggcatgttagaccggagtgagccggcccttttactggtatgacactccctctgtcttgagtgtcgctgtgccagcttgtacctctgtctatgttcacagcccgtgctgtgtacctagaccctccgtttgtccacattcattttaatctctattgtatcttgtcaaaacctaaaagcctaaaacgactctgataaagggacagaaagattatacaagagcaagtgtataatgaaataatgtaagcgagctatatgaattgtcacgtgtcatatttatgttgagacgaagaagagaaaataaacaccatgcaaatttatggcgagtgatagatggccagatgggcacaaggcctcctatttcttaaatcggattttgtaagaacgaaaaaagggacttataagagaataggatagaccatatatcaatgatgtagtatgcatcaagatctaactattatatgagtgaattgataaatttattctaggtgacatggccttaacgatgaacagtacgtggttaaatcaatagaacaatagccaactctagcggctctaaaaaaagatatatattcgtcgaggcactattatgcaaccacatagtcaacttcaacgccgcttgagtgcgttctcatgttttttttttcttgcaaattacgcttttctaaaataaaataatttggatcgtgcaattatttcactttaggtgtgcgtgactacgtgagtaacaattttgaatctcagaaaggaaataaaagtataatactgctacctactttgaggattcagcttgttacttaaaaccgtctttaaggtcaaatgctcaagattcattcaacaattgaaacgtctcacatgattaaaccatgtataaggatgctaaggtcttgcttgacaatgtttttctaggaatttcatctaactttttgagtgaaactatcaaataataattttaaaacaattttataagagaagctccggagataaaagggcatctaatctatgttagaagagtgaagtttactccctctgtcccaaaaatagaattctaagtatgaaatgatttttttgttatacgaaaggagtatatatcacaagattgatgtcagttatgcttagggcacgtacacgacgctggtgctttaggtagacgttaatcgttgtttctgcattttattttattttgttgccacggtgtacatttgggtagacgtttgtcacaggcattgccactcaaacaagcagccggcgcttggagcttttatagtttgaaaagtgacggttttaatgatgggtaagctgattagtatatgtaagtttagctttttccattgtaggttaagccttaaggctcttacacaattgtttcattattctcattctttaagagcccatataagcgttcatgaattgtacatatccttagatgtttttttttttgggtaaagctcgagcttctctatctaaaagtagagaaatcagaaaaagattcatgttttggtagttttgatttcttgcctccataataattttggtttaccattttttgtttgattttagttttagaagcgtttatagcaggatttaaaatccaaaactaccattatcttcaagtgaccgtcagtgagccgtttaacggcgtcgacaagtccaacggacaccaaccagtgaaccaccagcgtcgagccaagcgatgcaaacggaacggccgagacgttgacacctttggcgcggcacggcatgtcggatctccctctctggccagagagttccagctccacctccacctccacctccaccggtggcggtttccaagtccgttccgttccgttccgttccgttccgttccgcctcctgcctgctcctctcagacggcacgaaaccgtgacggcaccggcagcacggggggattccttttccactgctccttcctcttcccttcctcgcccgccgctataaatagccagccccgtccccagattctttcccaa

SEQ ID NO: 36 - DNA, 86 bp, Bouteloua gracilis
cctcatctttgttcggagcacgcacacaacccgatccccaattccctcgtctctcctcgcgagcctcgtcgaccccccccttcaag

SEQ ID NO: 37 - DNA, 1054 bp, Bouteloua gracilis
gtacggcgatcatcctccctccctccctctctctaccttctcttctctagactagatcggcgacccggtccatggttagggcctgctagttctgttcctgttttttccatggctgcgaggtaaaatagatctgatggcgttatgatggttaactcgtcatactcttgcgatctatggtccctttaggacatcgatttaatttcggatggttcgagatcggtgatccatggttagtaccctaggcagtggggttagatccgtgctgttagggttcgtagatggattctgattgctcagtaactgggaaacctgggatggttctagctgggaatcctgggatggttctagctggttcgcagatgagatcgatttcatggtctgctatatcttgtttcgttgcctaggttccgtttaatctgtccgtggtatgatgttagcctttgataaggttcgatcgtgctagctacgtcctgcgcagcatttaattgtcaggtcataatttttagcattcctgtttttgtttggtttggttttgtctggttgggctgtagatagtttcaatctacctgtcggtttattttattaaatttggattggatctgtatgtgtcacatatatcttcatgattaagatggttggaattatctcttcatcttttagatatatatggataggtatatatgttgctgtgggttttactggtactttattagatatattcatgcttagatacatgaagcaacgtgctgttacagtttaataattcttgtttatctaataaacaaataaggataggtatatgttgctgatggttttactgatactttattagatagtactttgacatgaaggaacatcctgcgacagcttaataattattcttcatctaataaaaagcttgctttttaattattttaattattttgatatacttggatgatgtcatgcagcagctatgtgtgaattttcggccctgtcttcatatgatgtttatttgcttgggactgtttctttggctgataacttaccctgttgtttggtgatccttctgcag

SEQ ID NO: 38 - DNA, 3142 bp, Bouteloua gracilis
gaatcccggcatggcatgttagaccggagtgagccggcccttttactggtatgacactccctctgtcttgagtgtcgctgtgccagcttgtacctctgtctatgttcacagcccgtgctgtgtacctagaccctccgtttgtccacattcattttaatctctattgtatcttgtcaaaacctaaaagcctaaaacgactctgataaagggacagaaagattatacaagagcaagtgtataatgaaataatgtaagcgagctatatgaattgtcacgtgtcatatttatgttgagacgaagaagagaaaataaacaccatgcaaatttatggcgagtgatagatggccagatgggcacaaggcctcctatttcttaaatcggattttgtaagaacgaaaaaagggacttataagagaataggatagaccatatatcaatgatgtagtatgcatcaagatctaactattatatgagtgaattgataaatttattctaggtgacatggccttaacgatgaacagtacgtggttaaatcaatagaacaatagccaactctagcggctctaaaaaaagatatatattcgtcgaggcactattatgcaaccacatagtcaacttcaacgccgcttgagtgcgttctcatgttttttttttcttgcaaattacgcttttctaaaataaaataatttggatcgtgcaattatttcactttaggtgtgcgtgactacgtgagtaacaattttgaatctcagaaaggaaataaaagtataatactgctacctactttgaggattcagcttgttacttaaaaccgtctttaaggtcaaatgctcaagattcattcaacaattgaaacgtctcacatgattaaaccatgtataaggatgctaaggtcttgcttgacaatgtttttctaggaatttcatctaactttttgagtgaaactatcaaataataattttaaaacaattttataagagaagctccggagataaaagggcatctaatctatgttagaagagtgaagtttactccctctgtcccaaaaatagaattctaagtatgaaatgatttttttgttatacgaaaggagtatatatcacaagattgatgtcagttatgcttagggcacgtacacgacgctggtgctttaggtagacgttaatcgttgtttctgcattttattttattttgttgccacggtgtacatttgggtagacgtttgtcacaggcattgccactcaaacaagcagccggcgcttggagcttttatagtttgaaaagtgacggttttaatgatgggtaagctgattagtatatgtaagtttagctttttccattgtaggttaagccttaaggctcttacacaattgtttcattattctcattctttaagagcccatataagcgttcatgaattgtacatatccttagatgtttttttttttgggtaaagctcgagcttctctatctaaaagtagagaaatcagaaaaagattcatgttttggtagttttgatttcttgcctccataataattttggtttaccattttttgtttgattttagttttagaagcgtttatagcaggatttaaaatccaaaactaccattatcttcaagtgaccgtcagtgagccgtttaacggcgtcgacaagtccaacggacaccaaccagtgaaccaccagcgtcgagccaagcgatgcaaacggaacggccgagacgttgacacctttggcgcggcacggcatgtcggatctccctctctggccagagagttccagctccacctccacctccacctccaccggtggcggtttccaagtccgttccgttccgttccgttccgttccgttccgcctcctgcctgctcctctcagacggcacgaaaccgtgacggcaccggcagcacggggggattccttttccactgctccttcctcttcccttcctcgcccgccgctataaatagccagccccgtccccagattctttcccaacctcatctttgttcggagcacgcacacaacccgatccccaattccctcgtctctcctcgcgagcctcgtcgaccccccccttcaaggtacggcgatcatcctccctccctccctctctctaccttctcttctctagactagatcggcgacccggtccatggttagggcctgctagttctgttcctgttttttccatggctgcgaggtaaaatagatctgatggcgttatgatggttaactcgtcatactcttgcgatctatggtccctttaggacatcgatttaatttcggatggttcgagatcggtgatccatggttagtaccctaggcagtggggttagatccgtgctgttagggttcgtagatggattctgattgctcagtaactgggaaacctgggatggttctagctgggaatcctgggatggttctagctggttcgcagatgagatcgatttcatggtctgctatatcttgtttcgttgcctaggttccgtttaatctgtccgtggtatgatgttagcctttgataaggttcgatcgtgctagctacgtcctgcgcagcatttaattgtcaggtcataatttttagcattcctgtttttgtttggtttggttttgtctggttgggctgtagatagtttcaatctacctgtcggtttattttattaaatttggattggatctgtatgtgtcacatatatcttcatgattaagatggttggaattatctcttcatcttttagatatatatggataggtatatatgttgctgtgggttttactggtactttattagatatattcatgcttagatacatgaagcaacgtgctgttacagtttaataattcttgtttatctaataaacaaataaggataggtatatgttgctgatggttttactgatactttattagatagtactttgacatgaaggaacatcctgcgacagcttaataattattcttcatctaataaaaagcttgctttttaattattttaattattttgatatacttggatgatgtcatgcagcagctatgtgtgaattttcggccctgtcttcatatgatgtttatttgcttgggactgtttctttggctgataacttaccctgttgtttggtgatccttctgcaggtg

SEQ ID NO: 39 - DNA, 1999 bp, Bouteloua gracilis
gaatcccggcatggcatgttagaccggagtgagccggcccttttactggtatgacactccctctgtcttgagtgtcgctgtgccagcttgtacctctgtctatgttcacagcccgtgctgtgtacctagaccctccgtttgtccacattcattttaatctctattgtatcttgtcaaaacctaaaagcctaaaacgactctgataaagggacagaaagattatacaagagcaagtgtataatgaaataatgtaagcgagctatatgaattgtcacgtgtcatatttatgttgagacgaagaagagaaaataaacaccatgcaaatttatggcgagtgatagatggccagatgggcacaaggcctcctatttcttaaatcggattttgtaagaacgaaaaaagggacttataagagaataggatagaccatatatcaatgatgtagtatgcatcaagatctaactattatatgagtgaattgataaatttattctaggtgacatggccttaacgatgaacagtacgtggttaaatcaatagaacaatagccaactctagcggctctaaaaaaagatatatattcgtcgaggcactattatgcaaccacatagtcaacttcaacgccgcttgagtgcgttctcatgttttttttttcttgcaaattacgcttttctaaaataaaataatttggatcgtgcaattatttcactttaggtgtgcgtgactacgtgagtaacaattttgaatctcagaaaggaaataaaagtataatactgctacctactttgaggattcagcttgttacttaaaaccgtctttaaggtcaaatgctcaagattcattcaacaattgaaacgtctcacatgattaaaccatgtataaggatgctaaggtcttgcttgacaatgtttttctaggaatttcatctaactttttgagtgaaactatcaaataataattttaaaacaattttataagagaagctccggagataaaagggcatctaatctatgttagaagagtgaagtttactccctctgtcccaaaaatagaattctaagtatgaaatgatttttttgttatacgaaaggagtatatatcacaagattgatgtcagttatgcttagggcacgtacacgacgctggtgctttaggtagacgttaatcgttgtttctgcattttattttattttgttgccacggtgtacatttgggtagacgtttgtcacaggcattgccactcaaacaagcagccggcgcttggagcttttatagtttgaaaagtgacggttttaatgatgggtaagctgattagtatatgtaagtttagctttttccattgtaggttaagccttaaggctcttacacaattgtttcattattctcattctttaagagcccatataagcgttcatgaattgtacatatccttagatgtttttttttttgggtaaagctcgagcttctctatctaaaagtagagaaatcagaaaaagattcatgttttggtagttttgatttcttgcctccataataattttggtttaccattttttgtttgattttagttttagaagcgtttatagcaggatttaaaatccaaaactaccattatcttcaagtgaccgtcagtgagccgtttaacggcgtcgacaagtccaacggacaccaaccagtgaaccaccagcgtcgagccaagcgatgcaaacggaacggccgagacgttgacacctttggcgcggcacggcatgtcggatctccctctctggccagagagttccagctccacctccacctccacctccaccggtggcggtttccaagtccgttccgttccgttccgttccgttccgttccgcctcctgcctgctcctctcagacggcacgaaaccgtgacggcaccggcagcacggggggattccttttccactgctccttcctcttcccttcctcgcccgccgctataaatagccagccccgtccccagattctttcccaa

SEQ ID NO: 40 - DNA, 1057 bp, Bouteloua gracilis
gtacggcgatcatcctccctccctccctctctctaccttctcttctctagactagatcggcgacccggtccatggttagggcctgctagttctgttcctgttttttccatggctgcgaggtaaaatagatctgatggcgttatgatggttaactcgtcatactcttgcgatctatggtccctttaggacatcgatttaatttcggatggttcgagatcggtgatccatggttagtaccctaggcagtggggttagatccgtgctgttagggttcgtagatggattctgattgctcagtaactgggaaacctgggatggttctagctgggaatcctgggatggttctagctggttcgcagatgagatcgatttcatggtctgctatatcttgtttcgttgcctaggttccgtttaatctgtccgtggtatgatgttagcctttgataaggttcgatcgtgctagctacgtcctgcgcagcatttaattgtcaggtcataatttttagcattcctgtttttgtttggtttggttttgtctggttgggctgtagatagtttcaatctacctgtcggtttattttattaaatttggattggatctgtatgtgtcacatatatcttcatgattaagatggttggaattatctcttcatcttttagatatatatggataggtatatatgttgctgtgggttttactggtactttattagatatattcatgcttagatacatgaagcaacgtgctgttacagtttaataattcttgtttatctaataaacaaataaggataggtatatgttgctgatggttttactgatactttattagatagtactttgacatgaaggaacatcctgcgacagcttaataattattcttcatctaataaaaagcttgctttttaattattttaattattttgatatacttggatgatgtcatgcagcagctatgtgtgaattttcggccctgtcttcatatgatgtttatttgcttgggactgtttctttggctgataacttaccctgttgtttggtgatccttctgcaggtg

SEQ ID NO: 41 - DNA, 2165 bp, Bouteloua gracilis
gagaagctccggagataaaagggcatctaatctatgttagaagagtgaagtttactccctctgtcccaaaaatagaattctaagtatgaaatgatttttttgttatacgaaaggagtatatatcacaagattgatgtcagttatgcttagggcacgtacacgacgctggtgctttaggtagacgttaatcgttgtttctgcattttattttattttgttgccacggtgtacatttgggtagacgtttgtcacaggcattgccactcaaacaagcagccggcgcttggagcttttatagtttgaaaagtgacggttttaatgatgggtaagctgattagtatatgtaagtttagctttttccattgtaggttaagccttaaggctcttacacaattgtttcattattctcattctttaagagcccatataagcgttcatgaattgtacatatccttagatgtttttttttttgggtaaagctcgagcttctctatctaaaagtagagaaatcagaaaaagattcatgttttggtagttttgatttcttgcctccataataattttggtttaccattttttgtttgattttagttttagaagcgtttatagcaggatttaaaatccaaaactaccattatcttcaagtgaccgtcagtgagccgtttaacggcgtcgacaagtccaacggacaccaaccagtgaaccaccagcgtcgagccaagcgatgcaaacggaacggccgagacgttgacacctttggcgcggcacggcatgtcggatctccctctctggccagagagttccagctccacctccacctccacctccaccggtggcggtttccaagtccgttccgttccgttccgttccgttccgttccgcctcctgcctgctcctctcagacggcacgaaaccgtgacggcaccggcagcacggggggattccttttccactgctccttcctcttcccttcctcgcccgccgctataaatagccagccccgtccccagattctttcccaacctcatctttgttcggagcacgcacacaacccgatccccaattccctcgtctctcctcgcgagcctcgtcgaccccccccttcaaggtacggcgatcatcctccctccctccctctctctaccttctcttctctagactagatcggcgacccggtccatggttagggcctgctagttctgttcctgttttttccatggctgcgaggtaaaatagatctgatggcgttatgatggttaactcgtcatactcttgcgatctatggtccctttaggacatcgatttaatttcggatggttcgagatcggtgatccatggttagtaccctaggcagtggggttagatccgtgctgttagggttcgtagatggattctgattgctcagtaactgggaaacctgggatggttctagctgggaatcctgggatggttctagctggttcgcagatgagatcgatttcatggtctgctatatcttgtttcgttgcctaggttccgtttaatctgtccgtggtatgatgttagcctttgataaggttcgatcgtgctagctacgtcctgcgcagcatttaattgtcaggtcataatttttagcattcctgtttttgtttggtttggttttgtctggttgggctgtagatagtttcaatctacctgtcggtttattttattaaatttggattggatctgtatgtgtcacatatatcttcatgattaagatggttggaattatctcttcatcttttagatatatatggataggtatatatgttgctgtgggttttactggtactttattagatatattcatgcttagatacatgaagcaacgtgctgttacagtttaataattcttgtttatctaataaacaaataaggataggtatatgttgctgatggttttactgatactttattagatagtactttgacatgaaggaacatcctgcgacagcttaataattattcttcatctaataaaaagcttgctttttaattattttaattattttgatatacttggatgatgtcatgcagcagctatgtgtgaattttcggccctgtcttcatatgatgtttatttgcttgggactgtttctttggctgataacttaccctgttgtttggtgatccttctgcaggtg

SEQ ID NO: 42 - DNA, 1022 bp, Bouteloua gracilis
gagaagctccggagataaaagggcatctaatctatgttagaagagtgaagtttactccctctgtcccaaaaatagaattctaagtatgaaatgatttttttgttatacgaaaggagtatatatcacaagattgatgtcagttatgcttagggcacgtacacgacgctggtgctttaggtagacgttaatcgttgtttctgcattttattttattttgttgccacggtgtacatttgggtagacgtttgtcacaggcattgccactcaaacaagcagccggcgcttggagcttttatagtttgaaaagtgacggttttaatgatgggtaagctgattagtatatgtaagtttagctttttccattgtaggttaagccttaaggctcttacacaattgtttcattattctcattctttaagagcccatataagcgttcatgaattgtacatatccttagatgtttttttttttgggtaaagctcgagcttctctatctaaaagtagagaaatcagaaaaagattcatgttttggtagttttgatttcttgcctccataataattttggtttaccattttttgtttgattttagttttagaagcgtttatagcaggatttaaaatccaaaactaccattatcttcaagtgaccgtcagtgagccgtttaacggcgtcgacaagtccaacggacaccaaccagtgaaccaccagcgtcgagccaagcgatgcaaacggaacggccgagacgttgacacctttggcgcggcacggcatgtcggatctccctctctggccagagagttccagctccacctccacctccacctccaccggtggcggtttccaagtccgttccgttccgttccgttccgttccgttccgcctcctgcctgctcctctcagacggcacgaaaccgtgacggcaccggcagcacggggggattccttttccactgctccttcctcttcccttcctcgcccgccgctataaatagccagccccgtccccagattctttcccaa

SEQ ID NO: 43 - DNA, 1903 bp, Bouteloua gracilis
actcaaacaagcagccggcgcttggagcttttatagtttgaaaagtgacggttttaatgatgggtaagctgattagtatatgtaagtttagctttttccattgtaggttaagccttaaggctcttacacaattgtttcattattctcattctttaagagcccatataagcgttcatgaattgtacatatccttagatgtttttttttttgggtaaagctcgagcttctctatctaaaagtagagaaatcagaaaaagattcatgttttggtagttttgatttcttgcctccataataattttggtttaccattttttgtttgattttagttttagaagcgtttatagcaggatttaaaatccaaaactaccattatcttcaagtgaccgtcagtgagccgtttaacggcgtcgacaagtccaacggacaccaaccagtgaaccaccagcgtcgagccaagcgatgcaaacggaacggccgagacgttgacacctttggcgcggcacggcatgtcggatctccctctctggccagagagttccagctccacctccacctccacctccaccggtggcggtttccaagtccgttccgttccgttccgttccgttccgttccgcctcctgcctgctcctctcagacggcacgaaaccgtgacggcaccggcagcacggggggattccttttccactgctccttcctcttcccttcctcgcccgccgctataaatagccagccccgtccccagattctttcccaacctcatctttgttcggagcacgcacacaacccgatccccaattccctcgtctctcctcgcgagcctcgtcgaccccccccttcaaggtacggcgatcatcctccctccctccctctctctaccttctcttctctagactagatcggcgacccggtccatggttagggcctgctagttctgttcctgttttttccatggctgcgaggtaaaatagatctgatggcgttatgatggttaactcgtcatactcttgcgatctatggtccctttaggacatcgatttaatttcggatggttcgagatcggtgatccatggttagtaccctaggcagtggggttagatccgtgctgttagggttcgtagatggattctgattgctcagtaactgggaaacctgggatggttctagctgggaatcctgggatggttctagctggttcgcagatgagatcgatttcatggtctgctatatcttgtttcgttgcctaggttccgtttaatctgtccgtggtatgatgttagcctttgataaggttcgatcgtgctagctacgtcctgcgcagcatttaattgtcaggtcataatttttagcattcctgtttttgtttggtttggttttgtctggttgggctgtagatagtttcaatctacctgtcggtttattttattaaatttggattggatctgtatgtgtcacatatatcttcatgattaagatggttggaattatctcttcatcttttagatatatatggataggtatatatgttgctgtgggttttactggtactttattagatatattcatgcttagatacatgaagcaacgtgctgttacagtttaataattcttgtttatctaataaacaaataaggataggtatatgttgctgatggttttactgatactttattagatagtactttgacatgaaggaacatcctgcgacagcttaataattattcttcatctaataaaaagcttgctttttaattattttaattattttgatatacttggatgatgtcatgcagcagctatgtgtgaattttcggccctgtcttcatatgatgtttatttgcttgggactgtttctttggctgataacttaccctgttgtttggtgatccttctgcaggtg

SEQ ID NO: 44 - DNA, 760 bp, Bouteloua gracilis
actcaaacaagcagccggcgcttggagcttttatagtttgaaaagtgacggttttaatgatgggtaagctgattagtatatgtaagtttagctttttccattgtaggttaagccttaaggctcttacacaattgtttcattattctcattctttaagagcccatataagcgttcatgaattgtacatatccttagatgtttttttttttgggtaaagctcgagcttctctatctaaaagtagagaaatcagaaaaagattcatgttttggtagttttgatttcttgcctccataataattttggtttaccattttttgtttgattttagttttagaagcgtttatagcaggatttaaaatccaaaactaccattatcttcaagtgaccgtcagtgagccgtttaacggcgtcgacaagtccaacggacaccaaccagtgaaccaccagcgtcgagccaagcgatgcaaacggaacggccgagacgttgacacctttggcgcggcacggcatgtcggatctccctctctggccagagagttccagctccacctccacctccacctccaccggtggcggtttccaagtccgttccgttccgttccgttccgttccgttccgcctcctgcctgctcctctcagacggcacgaaaccgtgacggcaccggcagcacggggggattccttttccactgctccttcctcttcccttcctcgcccgccgctataaatagccagccccgtccccagattctttcccaa

SEQ ID NO: 45 - DNA, 3234 bp, Bouteloua gracilis
ggcctctttacgtttggcacaacttagttgaatccggcttccggcaaactatatggcaagttagacccaagtgtgagccggccaccgcaagttattgtgacattatacgtaggaagcaagtgtataataagaatatgagataatgtaagcagctatatgaattatcacgtcatatttatgttaagatgaagaggagagaataaacggtacgtaaatttatagcgagtgatagacgggcacgaggcctcctagctatttccataaatcggattttgtaagaacaaaaaagaggacttattataagagaatgtggtaagtaagcatactccctccgtttcaaattataagttgttttaactttttttttatatctattttactatacattagatataataatgtgtctagatacataataaaatggatgaacaaaaaagtcaaagtgacttacaatttggaacggagggagtaagttcaagccatcaaggcacttctatgcaaccacatagtcaacttgaatgccgcttgagtgccttctcaagttttttttttcttgcaaaaattgtttctttttttttaaaaaagtataatttggatcgtgcaaatttctctctaggtgtgtgtgtgactgtgtgagtaacaatttctctagttgtgcgtgactgctgcttactttggagattacaatatatttctaaaatgcttcgattacttatttataaaccgtctctaaggccaattgctcaagattcattcaacaattgaaacgtctcacatgattaaatcatataaagtttctaagtcttgtttgacaagatttttttagattttcatctaaattggatgaaactatcaaacactaattttaaaaaatataagagaagctccggagataaaaggtcgtctatgttattataagagtaaagtcgtctattctcttcgtcccaacatatataattctaagcatgaattgctttctttttggacaaaaggagtatgccacaacacaagaatgatgtcaccgtcatgcttagatccttttatggtaaagcttcaccttctataatctaacaatagagaaatcggggaaaaatcatgttttggttgtttttatttctaacctccacaataactttggtttaccattttttgtttgattttagttttagagaagcgtttataacaggacctaaaatctttttttgagtacacagtacaacgcagacgctcatacacgcacgcacaatgtcctctatgaacacacgtaaggaaaccctacaccttgagcaccttcgaaggactgagccggcaaatctagagattctcgaagtcactattggcacctcgttatcaacgagaacgtcgcttaccacttaaagcataacaccgagaaatcccgtaacaaatccagtaaaatacgagcacccgtaccaagttgaatatttgaacccgagtgggtagattccaccgcaaaggacctaaccagatcatttcgcaaacaggaactaaaatcggtagagagcccagacaaaaaccttttctaagagcaactccagtgaaagcccctactttaggtataaaatgcaacactagtggagcttctaaataaacttctatttttcatgccctcctaaaatttactcctaaaaccctagctataggagcctcctatccatcctctattttattccactagaattgattataaatttagcctcttaaattttataagttgggagtcgagggtaactagagttgctctaaacggaccttatcttcaagtgacctcagtgagcccgtttaacggcgtcgacaagtctaatctaacggacaccaaccagagaaccaccgccagcgccgagccaagcgacgttgacatcttggcgcggcacggcatctccctggcgtctggtcccctcccgagacttccgctccacctcccaccggtggcggtttccgagtccgttccgcctcctctcacacggcacgaaaccttgacggcaccggcagcacgggggattccgttcccacggctccttccctttcccttcctcgcccgctgctataaatagccagccccatccccagcttcttccccaacctcatcttctcgtgttgttcggcccaacccgatcgatccccaattccctcgtcgtctctcgtcgcgagcctcgtcgatccccgcttcaaggtacagcgatcgatcgatcatcctcgctctctctaccttctctctcttagggcgtgctggttctgttcctgtttttccatggctgcgaggtacaatagattggcgattcatggttagggcctgctagttctgttcctgttttttttttttccatggctgcgaggcacaatagatctgatggcgttatgatggttaacttgtcatactcttgcgatctatggtccctttaggagtttaggacatcgatttaatttcggatagttcgagatctgtgatccatggttagtaccctaggcagtggggttagatccgtgctgttatggttcgtagatggattctgattgctcagtaactgggaatcctgggatggttctagctggttcgcagataagatcgatttcatgatatgctatatcttgtttggttgccgtggttccgttaaatctgtctgttatgatcttagtctttgataaggttcggtcgtgctagctacgtcctgtgcagcacttaattgtcaggtcataatttttagcatgccttttttttattggtttggttttgtctgactgggctgtagatagtttcaatctttgtctgactgggctgtagatagtttcaatcttcctgtctgtttattttattaaatttggatctgtatgtgtgtcatatatcttcatcttttagatatatcgataggtatatatgttgctgtcgttttttactgttcctttatgagatatattcatgcttagatacatgaaacaacgtgctgttacagtttaatagttcttgtttatctaataaacaaataaggataggtgctgcagttagttttactggtactttttttgacatgaacctacggcttaataattagtcttcatcaaataaaaagcatattttttaattatttcgatatacttgaatgatgtcatatgcagcatctgtgtgaatttttggccctgtcttcatatgatgtttatttgcttgggactgtttctttggctgataactcaccctgttgtttggtgatccttctgcag

SEQ ID NO: 46 - DNA, 2100 bp, Bouteloua gracilis
ggcctctttacgtttggcacaacttagttgaatccggcttccggcaaactatatggcaagttagacccaagtgtgagccggccaccgcaagttattgtgacattatacgtaggaagcaagtgtataataagaatatgagataatgtaagcagctatatgaattatcacgtcatatttatgttaagatgaagaggagagaataaacggtacgtaaatttatagcgagtgatagacgggcacgaggcctcctagctatttccataaatcggattttgtaagaacaaaaaagaggacttattataagagaatgtggtaagtaagcatactccctccgtttcaaattataagttgttttaactttttttttatatctattttactatacattagatataataatgtgtctagatacataataaaatggatgaacaaaaaagtcaaagtgacttacaatttggaacggagggagtaagttcaagccatcaaggcacttctatgcaaccacatagtcaacttgaatgccgcttgagtgccttctcaagttttttttttcttgcaaaaattgtttctttttttttaaaaaagtataatttggatcgtgcaaatttctctctaggtgtgtgtgtgactgtgtgagtaacaatttctctagttgtgcgtgactgctgcttactttggagattacaatatatttctaaaatgcttcgattacttatttataaaccgtctctaaggccaattgctcaagattcattcaacaattgaaacgtctcacatgattaaatcatataaagtttctaagtcttgtttgacaagatttttttagattttcatctaaattggatgaaactatcaaacactaattttaaaaaatataagagaagctccggagataaaaggtcgtctatgttattataagagtaaagtcgtctattctcttcgtcccaacatatataattctaagcatgaattgctttctttttggacaaaaggagtatgccacaacacaagaatgatgtcaccgtcatgcttagatccttttatggtaaagcttcaccttctataatctaacaatagagaaatcggggaaaaatcatgttttggttgtttttatttctaacctccacaataactttggtttaccattttttgtttgattttagttttagagaagcgtttataacaggacctaaaatctttttttgagtacacagtacaacgcagacgctcatacacgcacgcacaatgtcctctatgaacacacgtaaggaaaccctacaccttgagcaccttcgaaggactgagccggcaaatctagagattctcgaagtcactattggcacctcgttatcaacgagaacgtcgcttaccacttaaagcataacaccgagaaatcccgtaacaaatccagtaaaatacgagcacccgtaccaagttgaatatttgaacccgagtgggtagattccaccgcaaaggacctaaccagatcatttcgcaaacaggaactaaaatcggtagagagcccagacaaaaaccttttctaagagcaactccagtgaaagcccctactttaggtataaaatgcaacactagtggagcttctaaataaacttctatttttcatgccctcctaaaatttactcctaaaaccctagctataggagcctcctatccatcctctattttattccactagaattgattataaatttagcctcttaaattttataagttgggagtcgagggtaactagagttgctctaaacggaccttatcttcaagtgacctcagtgagcccgtttaacggcgtcgacaagtctaatctaacggacaccaaccagagaaccaccgccagcgccgagccaagcgacgttgacatcttggcgcggcacggcatctccctggcgtctggtcccctcccgagacttccgctccacctcccaccggtggcggtttccgagtccgttccgcctcctctcacacggcacgaaaccttgacggcaccggcagcacgggggattccgttcccacggctccttccctttcccttcctcgcccgctgctataaatagccagccccatccccagcttcttccccaa

SEQ ID NO: 47 - DNA, 91 bp, Bouteloua gracilis
cctcatcttctcgtgttgttcggcccaacccgatcgatccccaattccctcgtcgtctctcgtcgcgagcctcgtcgatccccgcttcaag

SEQ ID NO: 48 - DNA, 1043 bp, Bouteloua gracilis
gtacagcgatcgatcgatcatcctcgctctctctaccttctctctcttagggcgtgctggttctgttcctgtttttccatggctgcgaggtacaatagattggcgattcatggttagggcctgctagttctgttcctgttttttttttttccatggctgcgaggcacaatagatctgatggcgttatgatggttaacttgtcatactcttgcgatctatggtccctttaggagtttaggacatcgatttaatttcggatagttcgagatctgtgatccatggttagtaccctaggcagtggggttagatccgtgctgttatggttcgtagatggattctgattgctcagtaactgggaatcctgggatggttctagctggttcgcagataagatcgatttcatgatatgctatatcttgtttggttgccgtggttccgttaaatctgtctgttatgatcttagtctttgataaggttcggtcgtgctagctacgtcctgtgcagcacttaattgtcaggtcataatttttagcatgccttttttttattggtttggttttgtctgactgggctgtagatagtttcaatctttgtctgactgggctgtagatagtttcaatcttcctgtctgtttattttattaaatttggatctgtatgtgtgtcatatatcttcatcttttagatatatcgataggtatatatgttgctgtcgttttttactgttcctttatgagatatattcatgcttagatacatgaaacaacgtgctgttacagtttaatagttcttgtttatctaataaacaaataaggataggtgctgcagttagttttactggtactttttttgacatgaacctacggcttaataattagtcttcatcaaataaaaagcatattttttaattatttcgatatacttgaatgatgtcatatgcagcatctgtgtgaatttttggccctgtcttcatatgatgtttatttgcttgggactgtttctttggctgataactcaccctgttgtttggtgatccttctgcag

SEQ ID NO: 49 - DNA, 3176 bp, Bouteloua gracilis
aagttagacccaagtgtgagccggccaccgcaagttattgtgacattatacgtaggaagcaagtgtataataagaatatgagataatgtaagcagctatatgaattatcacgtcatatttatgttaagatgaagaggagagaataaacggtacgtaaatttatagcgagtgatagacgggcacgaggcctcctagctatttccataaatcggattttgtaagaacaaaaaagaggacttattataagagaatgtggtaagtaagcatactccctccgtttcaaattataagttgttttaactttttttttatatctattttactatacattagatataataatgtgtctagatacataataaaatggatgaacaaaaaagtcaaagtgacttacaatttggaacggagggagtaagttcaagccatcaaggcacttctatgcaaccacatagtcaacttgaatgccgcttgagtgccttctcaagttttttttttcttgcaaaaattgtttctttttttttaaaaaagtataatttggatcgtgcaaatttctctctaggtgtgtgtgtgactgtgtgagtaacaatttctctagttgtgcgtgactgctgcttactttggagattacaatatatttctaaaatgcttcgattacttatttataaaccgtctctaaggccaattgctcaagattcattcaacaattgaaacgtctcacatgattaaatcatataaagtttctaagtcttgtttgacaagatttttttagattttcatctaaattggatgaaactatcaaacactaattttaaaaaatataagagaagctccggagataaaaggtcgtctatgttattataagagtaaagtcgtctattctcttcgtcccaacatatataattctaagcatgaattgctttctttttggacaaaaggagtatgccacaacacaagaatgatgtcaccgtcatgcttagatccttttatggtaaagcttcaccttctataatctaacaatagagaaatcggggaaaaatcatgttttggttgtttttatttctaacctccacaataactttggtttaccattttttgtttgattttagttttagagaagcgtttataacaggacctaaaatctttttttgagtacacagtacaacgcagacgctcatacacgcacgcacaatgtcctctatgaacacacgtaaggaaaccctacaccttgagcaccttcgaaggactgagccggcaaatctagagattctcgaagtcactattggcacctcgttatcaacgagaacgtcgcttaccacttaaagcataacaccgagaaatcccgtaacaaatccagtaaaatacgagcacccgtaccaagttgaatatttgaacccgagtgggtagattccaccgcaaaggacctaaccagatcatttcgcaaacaggaactaaaatcggtagagagcccagacaaaaaccttttctaagagcaactccagtgaaagcccctactttaggtataaaatgcaacactagtggagcttctaaataaacttctatttttcatgccctcctaaaatttactcctaaaaccctagctataggagcctcctatccatcctctattttattccactagaattgattataaatttagcctcttaaattttataagttgggagtcgagggtaactagagttgctctaaacggaccttatcttcaagtgacctcagtgagcccgtttaacggcgtcgacaagtctaatctaacggacaccaaccagagaaccaccgccagcgccgagccaagcgacgttgacatcttggcgcggcacggcatctccctggcgtctggtcccctcccgagacttccgctccacctcccaccggtggcggtttccgagtccgttccgcctcctctcacacggcacgaaaccttgacggcaccggcagcacgggggattccgttcccacggctccttccctttcccttcctcgcccgctgctataaatagccagccccatccccagcttcttccccaacctcatcttctcgtgttgttcggcccaacccgatcgatccccaattccctcgtcgtctctcgtcgcgagcctcgtcgatccccgcttcaaggtacagcgatcgatcgatcatcctcgctctctctaccttctctctcttagggcgtgctggttctgttcctgtttttccatggctgcgaggtacaatagattggcgattcatggttagggcctgctagttctgttcctgttttttttttttccatggctgcgaggcacaatagatctgatggcgttatgatggttaacttgtcatactcttgcgatctatggtccctttaggagtttaggacatcgatttaatttcggatagttcgagatctgtgatccatggttagtaccctaggcagtggggttagatccgtgctgttatggttcgtagatggattctgattgctcagtaactgggaatcctgggatggttctagctggttcgcagataagatcgatttcatgatatgctatatcttgtttggttgccgtggttccgttaaatctgtctgttatgatcttagtcttgataaggttcggtcgtgctagctacgtcctgtgcagcacttaattgtcaggtcataatttttagcatgccttttttttattggtttggttttgtctgactgggctgtagatagtttcaatctttgtctgactgggctgtagatagtttcaatcttcctgtctgtttattttattaaatttggatctgtatgtgtgtcatatatcttcatcttttagatatatcgataggtatatatgttgctgtcgttttttactgttcctttatgagatatattcatgcttagatacatgaaacaacgtgctgttacagtttaatagttcttgtttatctaataaacaaataaggataggtgctgcagttagttttactggtactttttttgacatgaacctacggcttaataattagtcttcatcaaataaaaagcatattttttaattatttcgatatacttgaatgatgtcatatgcagcatctgtgtgaatttttggccctgtcttcatatgatgtttatttgcttgggactgtttctttggctgataactcaccctgttgtttggtgatccttctgcag

SEQ ID NO: 50 - DNA, 2043 bp, Bouteloua gracilis
aagttagacccaagtgtgagccggccaccgcaagttattgtgacattatacgtaggaagcaagtgtataataagaatatgagataatgtaagcagctatatgaattatcacgtcatatttatgttaagatgaagaggagagaataaacggtacgtaaatttatagcgagtgatagacgggcacgaggcctcctagctatttccataaatcggattttgtaagaacaaaaaagaggacttattataagagaatgtggtaagtaagcatactccctccgtttcaaattataagttgttttaactttttttttatatctattttactatacattagatataataatgtgtctagatacataataaaatggatgaacaaaaaagtcaaagtgacttacaatttggaacggagggagtaagttcaagccatcaaggcacttctatgcaaccacatagtcaacttgaatgccgcttgagtgccttctcaagttttttttttcttgcaaaaattgtttctttttttttaaaaaagtataatttggatcgtgcaaatttctctctaggtgtgtgtgtgactgtgtgagtaacaatttctctagttgtgcgtgactgctgcttactttggagattacaatatatttctaaaatgcttcgattacttatttataaaccgtctctaaggccaattgctcaagattcattcaacaattgaaacgtctcacatgattaaatcatataaagtttctaagtcttgtttgacaagatttttttagattttcatctaaattggatgaaactatcaaacactaattttaaaaaatataagagaagctccggagataaaaggtcgtctatgttattataagagtaaagtcgtctattctcttcgtcccaacatatataattctaagcatgaattgctttctttttggacaaaaggagtatgccacaacacaagaatgatgtcaccgtcatgcttagatccttttatggtaaagcttcaccttctataatctaacaatagagaaatcggggaaaaatcatgttttggttgtttttatttctaacctccacaataactttggtttaccattttttgtttgattttagttttagagaagcgtttataacaggacctaaaatctttttttgagtacacagtacaacgcagacgctcatacacgcacgcacaatgtcctctatgaacacacgtaaggaaaccctacaccttgagcaccttcgaaggactgagccggcaaatctagagattctcgaagtcactattggcacctcgttatcaacgagaacgtcgcttaccacttaaagcataacaccgagaaatcccgtaacaaatccagtaaaatacgagcacccgtaccaagttgaatatttgaacccgagtgggtagattccaccgcaaaggacctaaccagatcatttcgcaaacaggaactaaaatcggtagagagcccagacaaaaaccttttctaagagcaactccagtgaaagcccctactttaggtataaaatgcaacactagtggagcttctaaataaacttctatttttcatgccctcctaaaatttactcctaaaaccctagctataggagcctcctatccatcctctattttattccactagaattgattataaatttagcctcttaaattttataagttgggagtcgagggtaactagagttgctctaaacggaccttatcttcaagtgacctcagtgagcccgtttaacggcgtcgacaagtctaatctaacggacaccaaccagagaaccaccgccagcgccgagccaagcgacgttgacatcttggcgcggcacggcatctccctggcgtctggtcccctcccgagacttccgctccacctcccaccggtggcggtttccgagtccgttccgcctcctctcacacggcacgaaaccttgacggcaccggcagcacgggggattccgttcccacggctccttccctttcccttcctcgcccgctgctataaatagccagccccatccccagcttcttccccaa

SEQ ID NO: 51 - DNA, 1042 bp, Bouteloua gracilis
gtacagcgatcgatcgatcatcctcgctctctctaccttctctctcttagggcgtgctggttctgttcctgtttttccatggctgcgaggtacaatagattggcgattcatggttagggcctgctagttctgttcctgttttttttttttccatggctgcgaggcacaatagatctgatggcgttatgatggttaacttgtcatactcttgcgatctatggtccctttaggagtttaggacatcgatttaatttcggatagttcgagatctgtgatccatggttagtaccctaggcagtggggttagatccgtgctgttatggttcgtagatggattctgattgctcagtaactgggaatcctgggatggttctagctggttcgcagataagatcgatttcatgatatgctatatcttgtttggttgccgtggttccgttaaatctgtctgttatgatcttagtcttgataaggttcggtcgtgctagctacgtcctgtgcagcacttaattgtcaggtcataatttttagcatgccttttttttattggtttggttttgtctgactgggctgtagatagtttcaatctttgtctgactgggctgtagatagtttcaatcttcctgtctgtttattttattaaatttggatctgtatgtgtgtcatatatcttcatcttttagatatatcgataggtatatatgttgctgtcgttttttactgttcctttatgagatatattcatgcttagatacatgaaacaacgtgctgttacagtttaatagttcttgtttatctaataaacaaataaggataggtgctgcagttagttttactggtactttttttgacatgaacctacggcttaataattagtcttcatcaaataaaaagcatattttttaattatttcgatatacttgaatgatgtcatatgcagcatctgtgtgaatttttggccctgtcttcatatgatgtttatttgcttgggactgtttctttggctgataactcaccctgttgtttggtgatccttctgcag

SEQ ID NO: 52 - DNA, 3139 bp, Bouteloua gracilis
gacattatacgtaggaagcaagtgtataataagaatatgagataatgtaagcagctatatgaattatcacgtcatatttatgttaagatgaagaggagagaataaacggtacgtaaatttatagcgagtgatagacgggcacgaggcctcctagctatttccataaatcggattttgtaagaacaaaaaagaggacttattataagagaatgtggtaagtaagcatactccctccgtttcaaattataagttgttttaactttttttttatatctattttactatacattagatataataatgtgtctagatacataataaaatggatgaacaaaaaagtcaaagtgacttacaatttggaacggagggagtaagttcaagccatcaaggcacttctatgcaaccacatagtcaacttgaatgccgcttgagtgccttctcaagttttttttttcttgcaaaaattgtttctttttttttaaaaaagtataatttggatcgtgcaaatttctctctaggtgtgtgtgtgactgtgtgagtaacaatttctctagttgtgcgtgactgctgcttactttggagattacaatatatttctaaaatgcttcgattacttatttataaaccgtctctaaggccaattgctcaagattcattcaacaattgaaacgtctcacatgattaaatcatataaagtttctaagtcttgtttgacaagatttttttagattttcatctaaattggatgaaactatcaaacactaattttaaaaaatataagagaagctccggagataaaaggtcgtctatgttattataagagtaaagtcgtctattctcttcgtcccaacatatataattctaagcatgaattgctttctttttggacaaaaggagtatgccacaacacaagaatgatgtcaccgtcatgcttagatccttttatggtaaagcttcaccttctataatctaacaatagagaaatcggggaaaaatcatgttttggttgtttttatttctaacctccacaataactttggtttaccattttttgtttgattttagttttagagaagcgtttataacaggacctaaaatctttttttgagtacacagtacaacgcagacgctcatacacgcacgcacaatgtcctctatgaacacacgtaaggaaaccctacaccttgagcaccttcgaaggactgagccggcaaatctagagattctcgaagtcactattggcacctcgttatcaacgagaacgtcgcttaccacttaaagcataacaccgagaaatcccgtaacaaatccagtaaaatacgagcacccgtaccaagttgaatatttgaacccgagtgggtagattccaccgcaaaggacctaaccagatcatttcgcaaacaggaactaaaatcggtagagagcccagacaaaaaccttttctaagagcaactccagtgaaagcccctactttaggtataaaatgcaacactagtggagcttctaaataaacttctatttttcatgccctcctaaaatttactcctaaaaccctagctataggagcctcctatccatcctctattttattccactagaattgattataaatttagcctcttaaattttataagttgggagtcgagggtaactagagttgctctaaacggaccttatcttcaagtgacctcagtgagcccgtttaacggcgtcgacaagtctaatctaacggacaccaaccagagaaccaccgccagcgccgagccaagcgacgttgacatcttggcgcggcacggcatctccctggcgtctggtcccctcccgagacttccgctccacctcccaccggtggcggtttccgagtccgttccgcctcctctcacacggcacgaaaccttgacggcaccggcagcacgggggattccgttcccacggctccttccctttcccttcctcgcccgctgctataaatagccagccccatccccagcttcttccccaacctcatcttctcgtgttgttcggcccaacccgatcgatccccaattccctcgtcgtctctcgtcgcgagcctcgtcgatccccgcttcaaggtacagcgatcgatcgatcatcctcgctctctctaccttctctctcttagggcgtgctggttctgttcctgtttttccatggctgcgaggtacaatagattggcgattcatggttagggcctgctagttctgttcctgttttttttttttccatggctgcgaggcacaatagatctgatggcgttatgatggttaacttgtcatactcttgcgatctatggtccctttaggagtttaggacatcgatttaatttcggatagttcgagatctgtgatccatggttagtaccctaggcagtggggttagatccgtgctgttatggttcgtagatggattctgattgctcagtaactgggaatcctgggatggttctagctggttcgcagataagatcgatttcatgatatgctatatcttgtttggttgccgtggttccgttaaatctgtctgttatgatcttagtctttgataaggttcggtcgtgctagctacgtcctgtgcagcacttaattgtcaggtcataatttttagcatgccttttttttattggtttggttttgtctgactgggctgtagatagtttcaatctttgtctgactgggctgtagatagtttcaatcttcctgtctgtttattttattaaatttggatctgtatgtgtgtcatatatcttcatcttttagatatatcgataggtatatatgttgctgtcgttttttactgttcctttatgagatatattcatgcttagatacatgaaacaacgtgctgttacagtttaatagttcttgtttatctaataaacaaataaggataggtgctgcagttagttttactggtactttttttgacatgaacctacggcttaataattagtcttcatcaaataaaaagcatattttttaattatttcgatatacttgaatgatgtcatatgcagcatctgtgtgaatttttggccctgtcttcatatgatgtttatttgcttgggactgtttctttggctgataactcaccctgttgtttggtgatccttctgcaggtg

SEQ ID NO: 53 - DNA, 2002 bp, Bouteloua gracilis
gacattatacgtaggaagcaagtgtataataagaatatgagataatgtaagcagctatatgaattatcacgtcatatttatgttaagatgaagaggagagaataaacggtacgtaaatttatagcgagtgatagacgggcacgaggcctcctagctatttccataaatcggattttgtaagaacaaaaaagaggacttattataagagaatgtggtaagtaagcatactccctccgtttcaaattataagttgttttaactttttttttatatctattttactatacattagatataataatgtgtctagatacataataaaatggatgaacaaaaaagtcaaagtgacttacaatttggaacggagggagtaagttcaagccatcaaggcacttctatgcaaccacatagtcaacttgaatgccgcttgagtgccttctcaagttttttttttcttgcaaaaattgtttctttttttttaaaaaagtataatttggatcgtgcaaatttctctctaggtgtgtgtgtgactgtgtgagtaacaatttctctagttgtgcgtgactgctgcttactttggagattacaatatatttctaaaatgcttcgattacttatttataaaccgtctctaaggccaattgctcaagattcattcaacaattgaaacgtctcacatgattaaatcatataaagtttctaagtcttgtttgacaagatttttttagattttcatctaaattggatgaaactatcaaacactaattttaaaaaatataagagaagctccggagataaaaggtcgtctatgttattataagagtaaagtcgtctattctcttcgtcccaacatatataattctaagcatgaattgctttctttttggacaaaaggagtatgccacaacacaagaatgatgtcaccgtcatgcttagatccttttatggtaaagcttcaccttctataatctaacaatagagaaatcggggaaaaatcatgttttggttgtttttatttctaacctccacaataactttggtttaccattttttgtttgattttagttttagagaagcgtttataacaggacctaaaatctttttttgagtacacagtacaacgcagacgctcatacacgcacgcacaatgtcctctatgaacacacgtaaggaaaccctacaccttgagcaccttcgaaggactgagccggcaaatctagagattctcgaagtcactattggcacctcgttatcaacgagaacgtcgcttaccacttaaagcataacaccgagaaatcccgtaacaaatccagtaaaatacgagcacccgtaccaagttgaatatttgaacccgagtgggtagattccaccgcaaaggacctaaccagatcatttcgcaaacaggaactaaaatcggtagagagcccagacaaaaaccttttctaagagcaactccagtgaaagcccctactttaggtataaaatgcaacactagtggagcttctaaataaacttctatttttcatgccctcctaaaatttactcctaaaaccctagctataggagcctcctatccatcctctattttattccactagaattgattataaatttagcctcttaaattttataagttgggagtcgagggtaactagagttgctctaaacggaccttatcttcaagtgacctcagtgagcccgtttaacggcgtcgacaagtctaatctaacggacaccaaccagagaaccaccgccagcgccgagccaagcgacgttgacatcttggcgcggcacggcatctccctggcgtctggtcccctcccgagacttccgctccacctcccaccggtggcggtttccgagtccgttccgcctcctctcacacggcacgaaaccttgacggcaccggcagcacgggggattccgttcccacggctccttccctttcccttcctcgcccgctgctataaatagccagccccatccccagcttcttccccaa

SEQ ID NO: 54 - DNA, 1046 bp, Bouteloua gracilis
gtacagcgatcgatcgatcatcctcgctctctctaccttctctctcttagggcgtgctggttctgttcctgtttttccatggctgcgaggtacaatagattggcgattcatggttagggcctgctagttctgttcctgttttttttttttccatggctgcgaggcacaatagatctgatggcgttatgatggttaacttgtcatactcttgcgatctatggtccctttaggagtttaggacatcgatttaatttcggatagttcgagatctgtgatccatggttagtaccctaggcagtggggttagatccgtgctgttatggttcgtagatggattctgattgctcagtaactgggaatcctgggatggttctagctggttcgcagataagatcgatttcatgatatgctatatcttgtttggttgccgtggttccgttaaatctgtctgttatgatcttagtctttgataaggttcggtcgtgctagctacgtcctgtgcagcacttaattgtcaggtcataatttttagcatgccttttttttattggtttggttttgtctgactgggctgtagatagtttcaatctttgtctgactgggctgtagatagtttcaatcttcctgtctgtttattttattaaatttggatctgtatgtgtgtcatatatcttcatcttttagatatatcgataggtatatatgttgctgtcgttttttactgttcctttatgagatatattcatgcttagatacatgaaacaacgtgctgttacagtttaatagttcttgtttatctaataaacaaataaggataggtgctgcagttagttttactggtactttttttgacatgaacctacggcttaataattagtcttcatcaaataaaaagcatattttttaattatttcgatatacttgaatgatgtcatatgcagcatctgtgtgaatttttggccctgtcttcatatgatgtttatttgcttgggactgtttctttggctgataactcaccctgttgtttggtgatccttctgcaggtg

SEQ ID NO: 55 - DNA, 2160 bp, Bouteloua gracilis
gagaaatcggggaaaaatcatgttttggttgtttttatttctaacctccacaataactttggtttaccattttttgtttgattttagttttagagaagcgtttataacaggacctaaaatctttttttgagtacacagtacaacgcagacgctcatacacgcacgcacaatgtcctctatgaacacacgtaaggaaaccctacaccttgagcaccttcgaaggactgagccggcaaatctagagattctcgaagtcactattggcacctcgttatcaacgagaacgtcgcttaccacttaaagcataacaccgagaaatcccgtaacaaatccagtaaaatacgagcacccgtaccaagttgaatatttgaacccgagtgggtagattccaccgcaaaggacctaaccagatcatttcgcaaacaggaactaaaatcggtagagagcccagacaaaaaccttttctaagagcaactccagtgaaagcccctactttaggtataaaatgcaacactagtggagcttctaaataaacttctatttttcatgccctcctaaaatttactcctaaaaccctagctataggagcctcctatccatcctctattttattccactagaattgattataaatttagcctcttaaattttataagttgggagtcgagggtaactagagttgctctaaacggaccttatcttcaagtgacctcagtgagcccgtttaacggcgtcgacaagtctaatctaacggacaccaaccagagaaccaccgccagcgccgagccaagcgacgttgacatcttggcgcggcacggcatctccctggcgtctggtcccctcccgagacttccgctccacctcccaccggtggcggtttccgagtccgttccgcctcctctcacacggcacgaaaccttgacggcaccggcagcacgggggattccgttcccacggctccttccctttcccttcctcgcccgctgctataaatagccagccccatccccagcttcttccccaacctcatcttctcgtgttgttcggcccaacccgatcgatccccaattccctcgtcgtctctcgtcgcgagcctcgtcgatccccgcttcaaggtacagcgatcgatcgatcatcctcgctctctctaccttctctctcttagggcgtgctggttctgttcctgtttttccatggctgcgaggtacaatagattggcgattcatggttagggcctgctagttctgttcctgtttttttttttccatggctgcgaggcacaatagatctgatggcgttatgatggttaacttgtcatactcttgcgatctatggtccctttaggagtttaggacatcgatttaatttcggatagttcgagatctgtgatccatggttagtaccctaggcagtggggttagatccgtgctgttatggttcgtagatggattctgattgctcagtaactgggaatcctgggatggttctagctggttcgcagataagatcgatttcatgatatgctatatcttgtttggttgccgtggttccgttaaatctgtctgttatgatcttagtctttgataaggttcggtcgtgctagctacgtcctgtgcagcacttaattgtcaggtcataatttttagcatgccttttttttattggtttggttttgtctgactgggctgtagatagtttcaatctttgtctgactgggctgtagatagtttcaatcttcctgtctgtttattttattaaatttggatctgtatgtgtgtcatatatcttcatcttttagatatatcgataggtatatatgttgctgtcgttttttactgttcctttatgagatatattcatgcttagatacatgaaacaacgtgctgttacagtttaatagttcttgtttatctaataaacaaataaggataggtgctgcagttagttttactggtactttttttgacatgaacctacggcttaataattagtcttcatcaaataaaaagcatattttttaattatttcgatatacttgaatgatgtcatatgcagcatctgtgtgaatttttggccctgtcttcatatgatgtttatttgcttgggactgtttctttggctgataactcaccctgttgtttggtgatccttctgcaggtg

SEQ ID NO: 56 - DNA, 1024 bp, Bouteloua gracilis
gagaaatcggggaaaaatcatgttttggttgtttttatttctaacctccacaataactttggtttaccattttttgtttgattttagttttagagaagcgtttataacaggacctaaaatctttttttgagtacacagtacaacgcagacgctcatacacgcacgcacaatgtcctctatgaacacacgtaaggaaaccctacaccttgagcaccttcgaaggactgagccggcaaatctagagattctcgaagtcactattggcacctcgttatcaacgagaacgtcgcttaccacttaaagcataacaccgagaaatcccgtaacaaatccagtaaaatacgagcacccgtaccaagttgaatatttgaacccgagtgggtagattccaccgcaaaggacctaaccagatcatttcgcaaacaggaactaaaatcggtagagagcccagacaaaaaccttttctaagagcaactccagtgaaagcccctactttaggtataaaatgcaacactagtggagcttctaaataaacttctatttttcatgccctcctaaaatttactcctaaaaccctagctataggagcctcctatccatcctctattttattccactagaattgattataaatttagcctcttaaattttataagttgggagtcgagggtaactagagttgctctaaacggaccttatcttcaagtgacctcagtgagcccgtttaacggcgtcgacaagtctaatctaacggacaccaaccagagaaccaccgccagcgccgagccaagcgacgttgacatcttggcgcggcacggcatctccctggcgtctggtcccctcccgagacttccgctccacctcccaccggtggcggtttccgagtccgttccgcctcctctcacacggcacgaaaccttgacggcaccggcagcacgggggattccgttcccacggctccttccctttcccttcctcgcccgctgctataaatagccagccccatccccagcttcttccccaa

SEQ ID NO: 57 - DNA, 1045 bp, Bouteloua gracilis
gtacagcgatcgatcgatcatcctcgctctctctaccttctctctcttagggcgtgctggttctgttcctgtttttccatggctgcgaggtacaatagattggcgattcatggttagggcctgctagttctgttcctgtttttttttttccatggctgcgaggcacaatagatctgatggcgttatgatggttaacttgtcatactcttgcgatctatggtccctttaggagtttaggacatcgatttaatttcggatagttcgagatctgtgatccatggttagtaccctaggcagtggggttagatccgtgctgttatggttcgtagatggattctgattgctcagtaactgggaatcctgggatggttctagctggttcgcagataagatcgatttcatgatatgctatatcttgtttggttgccgtggttccgttaaatctgtctgttatgatcttagtctttgataaggttcggtcgtgctagctacgtcctgtgcagcacttaattgtcaggtcataatttttagcatgccttttttttattggtttggttttgtctgactgggctgtagatagtttcaatctttgtctgactgggctgtagatagtttcaatcttcctgtctgtttattttattaaatttggatctgtatgtgtgtcatatatcttcatcttttagatatatcgataggtatatatgttgctgtcgttttttactgttcctttatgagatatattcatgcttagatacatgaaacaacgtgctgttacagtttaatagttcttgtttatctaataaacaaataaggataggtgctgcagttagttttactggtactttttttgacatgaacctacggcttaataattagtcttcatcaaataaaaagcatattttttaattatttcgatatacttgaatgatgtcatatgcagcatctgtgtgaatttttggccctgtcttcatatgatgtttatttgcttgggactgtttctttggctgataactcaccctgttgtttggtgatccttctgcaggtg

SEQ ID NO: 58 - DNA, 2160 bp, Bouteloua gracilis
gagaaatcggggaaaaatcatgttttggttgtttttatttctaacctccacaataactttggtttaccattttttgtttgattttagttttagagaagcgtttataacaggacctaaaatctttttttgagtacacagtacaacgcagacgctcatacacgcacgcacaatgtcctctatgaacacacgtaaggaaaccctacaccttgagcaccttcgaaggactgagccggcaaatctagagattctcgaagtcactattggcacctcgttatcaacgagaacgtcgcttaccacttaaagcataacaccgagaaatcccgtaacaaatccagtaaaatacgagcacccgtaccaagttgaatatttgaacccgagtgggtagattccaccgcaaaggacctaaccagatcatttcgcaaacaggaactaaaatcggtagagagcccagacaaaaaccttttctaagagcaactccagtgaaagcccctactttaggtataaaatgcaacactagtggagcttctaaataaacttctatttttcatgccctcctaaaatttactcctaaaaccctagctataggagcctcctatccatcctctattttattccactagaattgattataaatttagcctcttaaattttataagttgggagtcgagggtaactagagttgctctaaacggaccttatcttcaagtgacctcagtgagcccgtttaacggcgtcgacaagtctaatctaacggacaccaaccagagaaccaccgccagcgccgagccaagcgacgttgacatcttggcgcggcacggcatctccctggcgtctggtcccctcccgagacttccgctccacctcccaccggtggcggtttccgagtccgttccgcctcctctcacacggcacgaaaccttgacggcaccggcagcacgggggattccgttcccacggctccttccctttcccttcctcgcccgctgctataaatagccagccccatccccagcttcttccccaacctcatcttctcgtgttgttcggcccaacccgatcgatccccaattccctcgtcgtctctcgtcgcgagcctcgtcgatccccgcttcaaggtacagcgatcgatcgatcatcctcgctctctctaccttctctctcttagggcgtgctggttctgttcctgtttttccatggctgcgaggtacaatagattggcgattcatggttagggcctgctagttctgttcctgttttttttttttccatggctgcgaggcacaatagatctgatggcgttatgatggttaacttgtcatactcttgcgatctatggtccctttaggagtttaggacatcgatttaatttcggatagttcgagatctgtgatccatggttagtaccctaggcagtggggttagatccgtgctgttatggttcgtagatggattctgattgctcagtaactgggaatcctgggatggttctagctggttcgcagataagatcgatttcatgatatgctatatcttgtttggttgccgtggttccgttaaatctgtctgttatgatcttagtcttgataaggttcggtcgtgctagctacgtcctgtgcagcacttaattgtcaggtcataatttttagcatgccttttttttattggtttggttttgtctgactgggctgtagatagtttcaatctttgtctgactgggctgtagatagtttcaatcttcctgtctgtttattttattaaatttggatctgtatgtgtgtcatatatcttcatcttttagatatatcgataggtatatatgttgctgtcgttttttactgttcctttatgagatatattcatgcttagatacatgaaacaacgtgctgttacagtttaatagttcttgtttatctaataaacaaataaggataggtgctgcagttagttttactggtactttttttgacatgaacctacggcttaataattagtcttcatcaaataaaaagcatattttttaattatttcgatatacttgaatgatgtcatatgcagcatctgtgtgaatttttggccctgtcttcatatgatgtttatttgcttgggactgtttctttggctgataactcaccctgttgtttggtgatccttctgcaggtg

SEQ ID NO: 59 - DNA, 1045 bp, Bouteloua gracilis
gtacagcgatcgatcgatcatcctcgctctctctaccttctctctcttagggcgtgctggttctgttcctgtttttccatggctgcgaggtacaatagattggcgattcatggttagggcctgctagttctgttcctgttttttttttttccatggctgcgaggcacaatagatctgatggcgttatgatggttaacttgtcatactcttgcgatctatggtccctttaggagtttaggacatcgatttaatttcggatagttcgagatctgtgatccatggttagtaccctaggcagtggggttagatccgtgctgttatggttcgtagatggattctgattgctcagtaactgggaatcctgggatggttctagctggttcgcagataagatcgatttcatgatatgctatatcttgtttggttgccgtggttccgttaaatctgtctgttatgatcttagtcttgataaggttcggtcgtgctagctacgtcctgtgcagcacttaattgtcaggtcataatttttagcatgccttttttttattggtttggttttgtctgactgggctgtagatagtttcaatctttgtctgactgggctgtagatagtttcaatcttcctgtctgtttattttattaaatttggatctgtatgtgtgtcatatatcttcatcttttagatatatcgataggtatatatgttgctgtcgttttttactgttcctttatgagatatattcatgcttagatacatgaaacaacgtgctgttacagtttaatagttcttgtttatctaataaacaaataaggataggtgctgcagttagttttactggtactttttttgacatgaacctacggcttaataattagtcttcatcaaataaaaagcatattttttaattatttcgatatacttgaatgatgtcatatgcagcatctgtgtgaatttttggccctgtcttcatatgatgtttatttgcttgggactgtttctttggctgataactcaccctgttgtttggtgatccttctgcaggtg

SEQ ID NO: 60 - DNA, 1885 bp, Bouteloua gracilis
caacgagaacgtcgcttaccacttaaagcataacaccgagaaatcccgtaacaaatccagtaaaatacgagcacccgtaccaagttgaatatttgaacccgagtgggtagattccaccgcaaaggacctaaccagatcatttcgcaaacaggaactaaaatcggtagagagcccagacaaaaaccttttctaagagcaactccagtgaaagcccctactttaggtataaaatgcaacactagtggagcttctaaataaacttctatttttcatgccctcctaaaatttactcctaaaaccctagctataggagcctcctatccatcctctattttattccactagaattgattataaatttagcctcttaaattttataagttgggagtcgagggtaactagagttgctctaaacggaccttatcttcaagtgacctcagtgagcccgtttaacggcgtcgacaagtctaatctaacggacaccaaccagagaaccaccgccagcgccgagccaagcgacgttgacatcttggcgcggcacggcatctccctggcgtctggtcccctcccgagacttccgctccacctcccaccggtggcggtttccgagtccgttccgcctcctctcacacggcacgaaaccttgacggcaccggcagcacgggggattccgttcccacggctccttccctttcccttcctcgcccgctgctataaatagccagccccatccccagcttcttccccaacctcatcttctcgtgttgttcggcccaacccgatcgatccccaattccctcgtcgtctctcgtcgcgagcctcgtcgatccccgcttcaaggtacagcgatcgatcgatcatcctcgctctctctaccttctctctcttagggcgtgctggttctgttcctgtttttccatggctgcgaggtacaatagattggcgattcatggttagggcctgctagttctgttcctgttttttttttttccatggctgcgaggcacaatagatctgatggcgttatgatggttaacttgtcatactcttgcgatctatggtccctttaggagtttaggacatcgatttaatttcggatagttcgagatctgtgatccatggttagtaccctaggcagtggggttagatccgtgctgttatggttcgtagatggattctgattgctcagtaactgggaatcctgggatggttctagctggttcgcagataagatcgatttcatgatatgctatatcttgtttggttgccgtggttccgttaaatctgtctgttatgatcttagtcttgataaggttcggtcgtgctagctacgtcctgtgcagcacttaattgtcaggtcataatttttagcatgccttttttttattggtttggttttgtctgactgggctgtagatagtttcaatctttgtctgactgggctgtagatagtttcaatcttcctgtctgtttattttattaaatttggatctgtatgtgtgtcatatatcttcatcttttagatatatcgataggtatatatgttgctgtcgttttttactgttcctttatgagatatattcatgcttagatacatgaaacaacgtgctgttacagtttaatagttcttgtttatctaataaacaaataaggataggtgctgcagttagttttactggtactttttttgacatgaacctacggcttaataattagtcttcatcaaataaaaagcatattttttaattatttcgatatacttgaatgatgtcatatgcagcatctgtgtgaatttttggccctgtcttcatatgatgtttatttgcttgggactgtttctttggctgataactcaccctgttgtttggtgatccttctgcaggtg

SEQ ID NO: 61 - DNA, 749 bp, Bouteloua gracilis
caacgagaacgtcgcttaccacttaaagcataacaccgagaaatcccgtaacaaatccagtaaaatacgagcacccgtaccaagttgaatatttgaacccgagtgggtagattccaccgcaaaggacctaaccagatcatttcgcaaacaggaactaaaatcggtagagagcccagacaaaaaccttttctaagagcaactccagtgaaagcccctactttaggtataaaatgcaacactagtggagcttctaaataaacttctatttttcatgccctcctaaaatttactcctaaaaccctagctataggagcctcctatccatcctctattttattccactagaattgattataaatttagcctcttaaattttataagttgggagtcgagggtaactagagttgctctaaacggaccttatcttcaagtgacctcagtgagcccgtttaacggcgtcgacaagtctaatctaacggacaccaaccagagaaccaccgccagcgccgagccaagcgacgttgacatcttggcgcggcacggcatctccctggcgtctggtcccctcccgagacttccgctccacctcccaccggtggcggtttccgagtccgttccgcctcctctcacacggcacgaaaccttgacggcaccggcagcacgggggattccgttcccacggctccttccctttcccttcctcgcccgctgctataaatagccagccccatccccagcttcttccccaa

SEQ ID NO: 62 - DNA, 6813 bp, Miscanthus sinesis
agcagactcgcattatcgatgggggaaatgaaattcagcgtttgacgtggatgcaacaactgcactgcacaggatatcttagccgttgtgtcgaagtttgctttgctaacgttttgagaaaaccagctttgaccaacacgagacgagcgccttacgtttggcacaatgtaatgtagcccggcacggcaagttagactagtatattgtgttagccggcctctttacgtttggcacagtttaattgaatccggcatggcaagttagactggagtgtgagccggtcattgcaaagttattatgacatatatataagagcacaagtgtataataagataatgtaagcaaggcagcaagctatatgaattgtcacgttatatttatgttgagatgttgagatgaagaagagaaaataaacagcctataaattcatagcgagtgatagacgggcacaaggcctcctatttcttaaaccgaattttgtaagaacaaaaaaaaggacttataggagaatgggatagaccatatatcaacgggaaaggtacacgttgctcgagtgttttaggcgttctgctcactcgatcctgtagctgtccgatctgcggcgtcaacacggcgcgcaacaagcggtggcgggcccctcggtagccgcggtcggaccggacgatggcctatggcgacccgcggcctgggcgtggcctgtgcgtgcatgcgccataggtcccggtgcatggtgcaggcggcaggtgcatgtgcatggagtaggctttggtgctggtgcaggctttggtcaggtgcaggaggggtaggttgcgcaggtgagaggtgaggtgcatgctgacccgtcacatcaccttactcctagcccctaagtcttgcatgtatgcagatttattcttttagcagcgacagattcagcagcgagagaccggctaccgtagcattttcatttttatttgataattagtatttaattatggactaattaggttcaaaatattcgtctcgcgatttccaaccaaactgtgcaattagtttttttcgtctacatttaatgctctatacacgtatcacaagattcaacgtgatggctactgtagcactttttgaaaaaactttttgcaactaaacaaggcctgaggtatcgtttaaatttaggtacaaaaaatataagggtgtcacatcgaatgttacacgagatatcatatgtgagtgttcggatagtaataataaaataaattacacaagtccttagtaatccacgagacgaatttattgagtctaattaatcagtcattagcacatggtgcattcatgcatctgcatattattttgtgttgcttggttgaaagttggatttcaaattgagttgaatttgcattttgaaattgctttggaaaaattagaaaaaaagaaaaaaaatgaatttccctccctcctttctcatttccctgctttcggcccctctgtgtagaactattcgagttctcaggtcgagtgctcgaatcatctagcttctcttttttgaggagagccagagagccagattcagaatagccagcctcctttttaggagagagctcatccccttttatagttgaaggcagcgacgaagccagcggggggctacccgtgctccagcctccctacggccatgatttacatggaacccgggcttagctcgggctaccgccatgaggaggaagaagaagataaggaggggctagaggaagaagaagaggaagctagccctggcttcgtcgattcctggcttcgtcgctggttgaaggggatgggctcttacaagtcagagaaagagagagaatgtatacgtgtgctatctagtcttgttgcccacgctgtcaggtacgagacggttgtcggcgcccacaatactgtttatgtccagatgcatgtggcaggctctaccgtgttcgcctgttatggcaaatgtcggcgcatacaatactatttgggttctgacacgcctgaaaggttgcatagtgcctatctggcatggcctggtggcaccgtccggcatgtgcgcaggatatgccagggtacggtccttggtattacggtttgacttgagcgccttaccttatctgctccgcctgatccccgggctcttaccgagcgggcgtccccggtcggtcgttcccagtcggccccgactgtgtcggtcggggaagagctgcaagcagaggtccggcgtatccccgatcgaaaaaggaagtcggagtcagactatgtctccaccttagccaggccttccggtcggggatcggatcattctcccggcctgtcattaggtatctgggtcggcccgagaggtgtgcgttgtcgctacgctgtctgctgggccgagtttctgttgggaagcgggtccattggggaccccgggtttatgaacccgacacgtggtcactatgctgcatactccctatacagccgctgaccagtacgctggttcaccgcgtcgcccgcgcgggacggaatgggatgtcacgacccgctgaacgccggggcatggcatcagcggcgaacaggcacccggcgtggagctgtccgtgtcaccatctacagtgttgacgggacccgcataaaaggagaaaaaaggcccgacggtcctggaagccttcctctccttagctcttctccctctttctctctgtgtaacctgctcttccccttcgtctataaaaagggaagtaggacgtcccaggaagagaagggcggttcaccactctacatggctatagacataaaaacacacgccttgggagcacactcacatcagagacttgggacctatccctctctcgctcgtttgtaacccctactacaaacttttagtgctagtaacacgagcagcagcgacgaactagacgtaaggactttctgcccgaaccagtataaacatcgtgtcatctaagcacaccatacgagccagacgcgcaatactagaaatttactagtcggtaactcgaaacaccgacatctagctaatctttttgttttatttggtttccctttgaaatcttctaatttagctttcatagaaataatctaggtattttttattttatatgttctatctgtttgcattaattttgatcatttgatctgaatgctgtggtcacgagaatcgagtgtttcatggccttaaaacactcgattatgccatctgacccgttttcaaccattctagtgtttctgagctatatcaatggtgcagcatgttagtatacatatctaactattactccgtatatgagtgagttgttaaatttattccaggtgaaatggcattaacgatagccaataggcggctaaattaatagccatactctaacagctctaaaaaacatatattcatcgaggcacctttatgcaaccacatagtcaacttcaacgtcgcttgcgtgcgttctcaagttttctttcttgcaaattacattttttttaaaaaaaagtataatttgtatcgtgcgattttttctctctaggtgtgcgtgactgtgggagtaacaattttgaatctcaagaaggaaataaaagaataatactgctgcctactttgaggatttcagtatttttctctaaaatgttttggtgtgatatctaaaccgtctttaaagccaattgctcaagattcattcaacaattgaaacgtctcacatgactaaatgatataaggttgctaaggtctttcttgataagcttttttatgaatttcatctaaattttcgagtgaaactattaaatactaaggttgctaagtgtcattctcgctcgagaagtctaacgctttaaactttaaccaaatatatacaagaaaatattaatatttatagtacataattagtatcattagatagatcgttgaatctattttcataacaaacttatttgaagaaacaaatgttgttcatatatttctatatacgaataccatagcgacacttattttagaatgtagggagtactccctttgtgccgctttgagtgtcgctttggcagctagtacctatgtccaccttcacagcttgtgcctagtacctagactctttctctgtccacattcatttaatctctgttgtaccttgttcggagataaaacgactctgataaagggacgaggaagtagtatgttagaggagtgaagtctactccctttgccgcaaaaaggtaatcctaagtgtgaattgtattcttttttgaccaaaggaatatacaacaagaatgatgtcatcatcatgcttcgatccttttttttggtaaagcttgagcttctgtaaaaatagagaaatcatgggaaaaatcacgttttggtggttttgatttctagcctccacaataactttggttttactattttttgtttgattttagtttcagaagtccacttttgtacgtgctcgtagagcctaaacaaaaggctttccaaaacgaccttatcttcgagtgttgtaaaaaaaatgagcccgtttaacggcgtcgacaagtctaacggacaccaaccagcgaaccaccagcgccgagccaagcgaagcagactgcagacggcacggccgagacgttgacaccttggcgcggcaacggcatctctctggccccctctcgagagttccgctccacctccgcatccacctccacctccacctccaccggtggcggtttccaagtccgtcccgttccgccacctgctcctctcacacggcacgaaaccgtcacggcaccggcagcacagcacgggggattcctttcccaccgctccgtccctttctcttcctcgcccgcccgttataaatagccagccccatccctcgtctctcgtgttgttcggagcgcacacacaacccgatccccaatcaatcgatccccgcttcaaggtacggcgatcctcctccctctctctctaccttctcttctctacactagatcggcggtccatggttagggcctgctagttccgttcctgtttttccatggctgcgaggtacaatagatctgatggcgttatgatggttaacttgtcatgcttttgcgatttatagtccctttagatagttcgagatcggtgatccatggttagtaccctaggctgtggagtcgggttagatccgcgctgttagggttcgtatatggaggcgagctgttctgattgttaacttgctgggaatcctgggatggttctagctgttccgcagatgagatcgatttcatgatctgctgtatctatccgtggtatgatgttagcctttgatatggttcgatcgtgctagctacgtcctgtgcacttaattgtcaggtcataatttttactatactttttttttggtttggtttggtttcgtctgatttggctgtcgttctagatcagagtagaaactgtttcaaactacctgttggatttattaaggtagcgtttggttcctggtatcgaatcatacacgcaccagtgcatcttggatagccagctggggcccacctgtccaaccgtttggttgccggatcgaacgagtccattcaagaccgaaccatgcagagcaatcgaatattctcttgtgacgctgtatcatccagttcggcaaaaaacaccgaatgccgccatacaggacaccgtactgagcgtctgcaactctgcatcccgctcactgctcacatctccgcttgccgcctcacccatccgactcagaccagagccacacggattactgctgctggtgtgtgtattaacaaaagatccatttgaccggagcacatgcagcttggatggaaaaaatttattatattcgtcagtgctgcatatgtactcatacttgcatgatggttttatttattcgacctcatcagtcctggcactatggaaagtcattgtagtatagattttttaatataatataaatcattggtgacttatcttgcttaattttattttcttattatgaaatatcgttgcattcataatagcaaatttgtgcaaatatatagaatctacgtgaaattcttggttggaccaatacaacaaacccctcaaacattctcttgtactgaaccataccattccgtacaaccatccaaacaaaaatcatgtatcatcatgtacatgtaaccaaacaattaacacgcaccatcctattcagacttgtctcatccataatctatccatccaggatgatccatcccattcatctatatacacccaatcaaacgctacctaaaatttggatctgtatgtgtcacatatatcttaataagatggatggaaatatctctttatcttttagatatggataggtatatatgttgctgtgggtttgttagttatatatatacgtgcttacatacgtgaagaaacctgctgctacagtttaataattcttgttcatctcaacaaataacgataggcgtatatgttgctgtgttttttactggtactttgttagatatatacatgcttacatacatgaagaacacatgctacagttcaaaaattcttgttcatctcataaacaaaaaggaggtgtatatgttgctgtgggttttactggtactttattagatatatacatgcttacatagatgaagcaacatgctgctatggtgtttaataattattgtttatctaataaacaaacatgctttttaattatcttgatatgtttggatgatggcatatgcagcagctatgtgtggattttaaatacccagcatcatgagcatgcatgaccctgccttagtatgcagttatttgcttgagactgtttcttttgttgatactcatcctttagttcggtcactcttctgcag

SEQ ID NO: 63 - DNA, 5359 bp, Miscanthus sinesis
agcagactcgcattatcgatgggggaaatgaaattcagcgtttgacgtggatgcaacaactgcactgcacaggatatcttagccgttgtgtcgaagtttgctttgctaacgttttgagaaaaccagctttgaccaacacgagacgagcgccttacgtttggcacaatgtaatgtagcccggcacggcaagttagactagtatattgtgttagccggcctctttacgtttggcacagtttaattgaatccggcatggcaagttagactggagtgtgagccggtcattgcaaagttattatgacatatatataagagcacaagtgtataataagataatgtaagcaaggcagcaagctatatgaattgtcacgttatatttatgttgagatgttgagatgaagaagagaaaataaacagcctataaattcatagcgagtgatagacgggcacaaggcctcctatttcttaaaccgaattttgtaagaacaaaaaaaaggacttataggagaatgggatagaccatatatcaacgggaaaggtacacgttgctcgagtgttttaggcgttctgctcactcgatcctgtagctgtccgatctgcggcgtcaacacggcgcgcaacaagcggtggcgggcccctcggtagccgcggtcggaccggacgatggcctatggcgacccgcggcctgggcgtggcctgtgcgtgcatgcgccataggtcccggtgcatggtgcaggcggcaggtgcatgtgcatggagtaggctttggtgctggtgcaggctttggtcaggtgcaggaggggtaggttgcgcaggtgagaggtgaggtgcatgctgacccgtcacatcaccttactcctagcccctaagtcttgcatgtatgcagatttattcttttagcagcgacagattcagcagcgagagaccggctaccgtagcattttcatttttatttgataattagtatttaattatggactaattaggttcaaaatattcgtctcgcgatttccaaccaaactgtgcaattagtttttttcgtctacatttaatgctctatacacgtatcacaagattcaacgtgatggctactgtagcactttttgaaaaaactttttgcaactaaacaaggcctgaggtatcgtttaaatttaggtacaaaaaatataagggtgtcacatcgaatgttacacgagatatcatatgtgagtgttcggatagtaataataaaataaattacacaagtccttagtaatccacgagacgaatttattgagtctaattaatcagtcattagcacatggtgcattcatgcatctgcatattattttgtgttgcttggttgaaagttggatttcaaattgagttgaatttgcattttgaaattgctttggaaaaattagaaaaaaagaaaaaaaatgaatttccctccctcctttctcatttccctgctttcggcccctctgtgtagaactattcgagttctcaggtcgagtgctcgaatcatctagcttctcttttttgaggagagccagagagccagattcagaatagccagcctcctttttaggagagagctcatccccttttatagttgaaggcagcgacgaagccagcggggggctacccgtgctccagcctccctacggccatgatttacatggaacccgggcttagctcgggctaccgccatgaggaggaagaagaagataaggaggggctagaggaagaagaagaggaagctagccctggcttcgtcgattcctggcttcgtcgctggttgaaggggatgggctcttacaagtcagagaaagagagagaatgtatacgtgtgctatctagtcttgttgcccacgctgtcaggtacgagacggttgtcggcgcccacaatactgtttatgtccagatgcatgtggcaggctctaccgtgttcgcctgttatggcaaatgtcggcgcatacaatactatttgggttctgacacgcctgaaaggttgcatagtgcctatctggcatggcctggtggcaccgtccggcatgtgcgcaggatatgccagggtacggtccttggtattacggtttgacttgagcgccttaccttatctgctccgcctgatccccgggctcttaccgagcgggcgtccccggtcggtcgttcccagtcggccccgactgtgtcggtcggggaagagctgcaagcagaggtccggcgtatccccgatcgaaaaaggaagtcggagtcagactatgtctccaccttagccaggccttccggtcggggatcggatcattctcccggcctgtcattaggtatctgggtcggcccgagaggtgtgcgttgtcgctacgctgtctgctgggccgagtttctgttgggaagcgggtccattggggaccccgggtttatgaacccgacacgtggtcactatgctgcatactccctatacagccgctgaccagtacgctggttcaccgcgtcgcccgcgcgggacggaatgggatgtcacgacccgctgaacgccggggcatggcatcagcggcgaacaggcacccggcgtggagctgtccgtgtcaccatctacagtgttgacgggacccgcataaaaggagaaaaaaggcccgacggtcctggaagccttcctctccttagctcttctccctctttctctctgtgtaacctgctcttccccttcgtctataaaaagggaagtaggacgtcccaggaagagaagggcggttcaccactctacatggctatagacataaaaacacacgccttgggagcacactcacatcagagacttgggacctatccctctctcgctcgtttgtaacccctactacaaacttttagtgctagtaacacgagcagcagcgacgaactagacgtaaggactttctgcccgaaccagtataaacatcgtgtcatctaagcacaccatacgagccagacgcgcaatactagaaatttactagtcggtaactcgaaacaccgacatctagctaatctttttgttttatttggtttccctttgaaatcttctaatttagctttcatagaaataatctaggtattttttattttatatgttctatctgtttgcattaattttgatcatttgatctgaatgctgtggtcacgagaatcgagtgtttcatggccttaaaacactcgattatgccatctgacccgttttcaaccattctagtgtttctgagctatatcaatggtgcagcatgttagtatacatatctaactattactccgtatatgagtgagttgttaaatttattccaggtgaaatggcattaacgatagccaataggcggctaaattaatagccatactctaacagctctaaaaaacatatattcatcgaggcacctttatgcaaccacatagtcaacttcaacgtcgcttgcgtgcgttctcaagttttctttcttgcaaattacattttttttaaaaaaaagtataatttgtatcgtgcgattttttctctctaggtgtgcgtgactgtgggagtaacaattttgaatctcaagaaggaaataaaagaataatactgctgcctactttgaggatttcagtatttttctctaaaatgttttggtgtgatatctaaaccgtctttaaagccaattgctcaagattcattcaacaattgaaacgtctcacatgactaaatgatataaggttgctaaggtctttcttgataagcttttttatgaatttcatctaaattttcgagtgaaactattaaatactaaggttgctaagtgtcattctcgctcgagaagtctaacgctttaaactttaaccaaatatatacaagaaaatattaatatttatagtacataattagtatcattagatagatcgttgaatctattttcataacaaacttatttgaagaaacaaatgttgttcatatatttctatatacgaataccatagcgacacttattttagaatgtagggagtactccctttgtgccgctttgagtgtcgctttggcagctagtacctatgtccaccttcacagcttgtgcctagtacctagactctttctctgtccacattcatttaatctctgttgtaccttgttcggagataaaacgactctgataaagggacgaggaagtagtatgttagaggagtgaagtctactccctttgccgcaaaaaggtaatcctaagtgtgaattgtattcttttttgaccaaaggaatatacaacaagaatgatgtcatcatcatgcttcgatccttttttttggtaaagcttgagcttctgtaaaaatagagaaatcatgggaaaaatcacgttttggtggttttgatttctagcctccacaataactttggttttactattttttgtttgattttagtttcagaagtccacttttgtacgtgctcgtagagcctaaacaaaaggctttccaaaacgaccttatcttcgagtgttgtaaaaaaaatgagcccgtttaacggcgtcgacaagtctaacggacaccaaccagcgaaccaccagcgccgagccaagcgaagcagactgcagacggcacggccgagacgttgacaccttggcgcggcaacggcatctctctggccccctctcgagagttccgctccacctccgcatccacctccacctccacctccaccggtggcggtttccaagtccgtcccgttccgccacctgctcctctcacacggcacgaaaccgtcacggcaccggcagcacagcacgggggattcctttcccaccgctccgtccctttctcttcctcgcccgcccgttataaatagccagccccatccctcgtctctcgtgttgttcggagcgcacacacaacccgatccccaatcaatcgatccccgcttcaaggtacggcgatcctcctccctctctctctaccttctcttctctacactagatcggcggtccatggttagggcctgctagttccgttcctgtttttccatggctgcgaggtacaatagatctgatggcgttatgatggttaacttgtcatgcttttgcgatttatagtccctttagatagttcgagatcggtgatccatggttagtaccctaggctgtggagtcgggttagatccgcgctgttagggttcgtatatggaggcgagctgttctgattgttaacttgctgggaatcctgggatggttctagctgttccgcagatgagatcgatttcatgatctgctgtatctatccgtggtatgatgttagcctttgatatggttcgatcgtgctagctacgtcctgtgcacttaattgtcaggtcataatttttactatactttttttttggtttggtttggtttcgtct

SEQ ID NO: 64 - DNA, 63 bp, Miscanthus sinesis
gatttggctgtcgttctagatcagagtagaaactgtttcaaactacctgttggatttattaag

SEQ ID NO: 65 - DNA, 1391 bp, Miscanthus sinesis
gtagcgtttggttcctggtatcgaatcatacacgcaccagtgcatcttggatagccagctggggcccacctgtccaaccgtttggttgccggatcgaacgagtccattcaagaccgaaccatgcagagcaatcgaatattctcttgtgacgctgtatcatccagttcggcaaaaaacaccgaatgccgccatacaggacaccgtactgagcgtctgcaactctgcatcccgctcactgctcacatctccgcttgccgcctcacccatccgactcagaccagagccacacggattactgctgctggtgtgtgtattaacaaaagatccatttgaccggagcacatgcagcttggatggaaaaaatttattatattcgtcagtgctgcatatgtactcatacttgcatgatggttttatttattcgacctcatcagtcctggcactatggaaagtcattgtagtatagattttttaatataatataaatcattggtgacttatcttgcttaattttattttcttattatgaaatatcgttgcattcataatagcaaatttgtgcaaatatatagaatctacgtgaaattcttggttggaccaatacaacaaacccctcaaacattctcttgtactgaaccataccattccgtacaaccatccaaacaaaaatcatgtatcatcatgtacatgtaaccaaacaattaacacgcaccatcctattcagacttgtctcatccataatctatccatccaggatgatccatcccattcatctatatacacccaatcaaacgctacctaaaatttggatctgtatgtgtcacatatatcttaataagatggatggaaatatctctttatcttttagatatggataggtatatatgttgctgtgggtttgttagttatatatatacgtgcttacatacgtgaagaaacctgctgctacagtttaataattcttgttcatctcaacaaataacgataggcgtatatgttgctgtgttttttactggtactttgttagatatatacatgcttacatacatgaagaacacatgctacagttcaaaaattcttgttcatctcataaacaaaaaggaggtgtatatgttgctgtgggttttactggtactttattagatatatacatgcttacatagatgaagcaacatgctgctatggtgtttaataattattgtttatctaataaacaaacatgctttttaattatcttgatatgtttggatgatggcatatgcagcagctatgtgtggattttaaatacccagcatcatgagcatgcatgaccctgccttagtatgcagttatttgcttgagactgtttcttttgttgatactcatcctttagttcggtcactcttctgcag

SEQ ID NO: 66 - DNA, 4402 bp, Miscanthus sinesis
cacgtggtcactatgctgcatactccctatacagccgctgaccagtacgctggttcaccgcgtcgcccgcgcgggacggaatgggatgtcacgacccgctgaacgccggggcatggcatcagcggcgaacaggcacccggcgtggagctgtccgtgtcaccatctacagtgttgacgggacccgcataaaaggagaaaaaaggcccgacggtcctggaagccttcctctccttagctcttctccctctttctctctgtgtaacctgctcttccccttcgtctataaaaagggaagtaggacgtcccaggaagagaagggcggttcaccactctacatggctatagacataaaaacacacgccttgggagcacactcacatcagagacttgggacctatccctctctcgctcgtttgtaacccctactacaaacttttagtgctagtaacacgagcagcagcgacgaactagacgtaaggactttctgcccgaaccagtataaacatcgtgtcatctaagcacaccatacgagccagacgcgcaatactagaaatttactagtcggtaactcgaaacaccgacatctagctaatctttttgttttatttggtttccctttgaaatcttctaatttagctttcatagaaataatctaggtattttttattttatatgttctatctgtttgcattaattttgatcatttgatctgaatgctgtggtcacgagaatcgagtgtttcatggccttaaaacactcgattatgccatctgacccgttttcaaccattctagtgtttctgagctatatcaatggtgcagcatgttagtatacatatctaactattactccgtatatgagtgagttgttaaatttattccaggtgaaatggcattaacgatagccaataggcggctaaattaatagccatactctaacagctctaaaaaacatatattcatcgaggcacctttatgcaaccacatagtcaacttcaacgtcgcttgcgtgcgttctcaagttttctttcttgcaaattacattttttttaaaaaaaagtataatttgtatcgtgcgattttttctctctaggtgtgcgtgactgtgggagtaacaattttgaatctcaagaaggaaataaaagaataatactgctgcctactttgaggatttcagtatttttctctaaaatgttttggtgtgatatctaaaccgtctttaaagccaattgctcaagattcattcaacaattgaaacgtctcacatgactaaatgatataaggttgctaaggtctttcttgataagcttttttatgaatttcatctaaattttcgagtgaaactattaaatactaaggttgctaagtgtcattctcgctcgagaagtctaacgctttaaactttaaccaaatatatacaagaaaatattaatatttatagtacataattagtatcattagatagatcgttgaatctattttcataacaaacttatttgaagaaacaaatgttgttcatatatttctatatacgaataccatagcgacacttattttagaatgtagggagtactccctttgtgccgctttgagtgtcgctttggcagctagtacctatgtccaccttcacagcttgtgcctagtacctagactctttctctgtccacattcatttaatctctgttgtaccttgttcggagataaaacgactctgataaagggacgaggaagtagtatgttagaggagtgaagtctactccctttgccgcaaaaaggtaatcctaagtgtgaattgtattcttttttgaccaaaggaatatacaacaagaatgatgtcatcatcatgcttcgatccttttttttggtaaagcttgagcttctgtaaaaatagagaaatcatgggaaaaatcacgttttggtggttttgatttctagcctccacaataactttggttttactattttttgtttgattttagtttcagaagtccacttttgtacgtgctcgtagagcctaaacaaaaggctttccaaaacgaccttatcttcgagtgttgtaaaaaaaatgagcccgtttaacggcgtcgacaagtctaacggacaccaaccagcgaaccaccagcgccgagccaagcgaagcagactgcagacggcacggccgagacgttgacaccttggcgcggcaacggcatctctctggccccctctcgagagttccgctccacctccgcatccacctccacctccacctccaccggtggcggtttccaagtccgtcccgttccgccacctgctcctctcacacggcacgaaaccgtcacggcaccggcagcacagcacgggggattcctttcccaccgctccgtccctttctcttcctcgcccgcccgttataaatagccagccccatccctcgtctctcgtgttgttcggagcgcacacacaacccgatccccaatcaatcgatccccgcttcaaggtacggcgatcctcctccctctctctctaccttctcttctctacactagatcggcggtccatggttagggcctgctagttccgttcctgtttttccatggctgcgaggtacaatagatctgatggcgttatgatggttaacttgtcatgcttttgcgatttatagtccctttagatagttcgagatcggtgatccatggttagtaccctaggctgtggagtcgggttagatccgcgctgttagggttcgtatatggaggcgagctgttctgattgttaacttgctgggaatcctgggatggttctagctgttccgcagatgagatcgatttcatgatctgctgtatctatccgtggtatgatgttagcctttgatatggttcgatcgtgctagctacgtcctgtgcacttaattgtcaggtcataatttttactatactttttttttggtttggtttggtttcgtctgatttggctgtcgttctagatcagagtagaaactgtttcaaactacctgttggatttattaaggtagcgtttggttcctggtatcgaatcatacacgcaccagtgcatcttggatagccagctggggcccacctgtccaaccgtttggttgccggatcgaacgagtccattcaagaccgaaccatgcagagcaatcgaatattctcttgtgacgctgtatcatccagttcggcaaaaaacaccgaatgccgccatacaggacaccgtactgagcgtctgcaactctgcatcccgctcactgctcacatctccgcttgccgcctcacccatccgactcagaccagagccacacggattactgctgctggtgtgtgtattaacaaaagatccatttgaccggagcacatgcagcttggatggaaaaaatttattatattcgtcagtgctgcatatgtactcatacttgcatgatggttttatttattcgacctcatcagtcctggcactatggaaagtcattgtagtatagattttttaatataatataaatcattggtgacttatcttgcttaattttattttcttattatgaaatatcgttgcattcataatagcaaatttgtgcaaatatatagaatctacgtgaaattcttggttggaccaatacaacaaacccctcaaacattctcttgtactgaaccataccattccgtacaaccatccaaacaaaaatcatgtatcatcatgtacatgtaaccaaacaattaacacgcaccatcctattcagacttgtctcatccataatctatccatccaggatgatccatcccattcatctatatacacccaatcaaacgctacctaaaatttggatctgtatgtgtcacatatatcttaataagatggatggaaatatctctttatcttttagatatggataggtatatatgttgctgtgggtttgttagttatatatatacgtgcttacatacgtgaagaaacctgctgctacagtttaataattcttgttcatctcaacaaataacgataggcgtatatgttgctgtgttttttactggtactttgttagatatatacatgcttacatacatgaagaacacatgctacagttcaaaaattcttgttcatctcataaacaaaaaggaggtgtatatgttgctgtgggttttactggtactttattagatatatacatgcttacatagatgaagcaacatgctgctatggtgtttaataattattgtttatctaataaacaaacatgctttttaattatcttgatatgtttggatgatggcatatgcagcagctatgtgtggattttaaatacccagcatcatgagcatgcatgaccctgccttagtatgcagttatttgcttgagactgtttcttttgttgatactcatcctttagttcggtcactcttctgcaggtg

SEQ ID NO: 67 - DNA, 2423 bp, Miscanthus sinesis
cacgtggtcactatgctgcatactccctatacagccgctgaccagtacgctggttcaccgcgtcgcccgcgcgggacggaatgggatgtcacgacccgctgaacgccggggcatggcatcagcggcgaacaggcacccggcgtggagctgtccgtgtcaccatctacagtgttgacgggacccgcataaaaggagaaaaaaggcccgacggtcctggaagccttcctctccttagctcttctccctctttctctctgtgtaacctgctcttccccttcgtctataaaaagggaagtaggacgtcccaggaagagaagggcggttcaccactctacatggctatagacataaaaacacacgccttgggagcacactcacatcagagacttgggacctatccctctctcgctcgtttgtaacccctactacaaacttttagtgctagtaacacgagcagcagcgacgaactagacgtaaggactttctgcccgaaccagtataaacatcgtgtcatctaagcacaccatacgagccagacgcgcaatactagaaatttactagtcggtaactcgaaacaccgacatctagctaatctttttgttttatttggtttccctttgaaatcttctaatttagctttcatagaaataatctaggtattttttattttatatgttctatctgtttgcattaattttgatcatttgatctgaatgctgtggtcacgagaatcgagtgtttcatggccttaaaacactcgattatgccatctgacccgttttcaaccattctagtgtttctgagctatatcaatggtgcagcatgttagtatacatatctaactattactccgtatatgagtgagttgttaaatttattccaggtgaaatggcattaacgatagccaataggcggctaaattaatagccatactctaacagctctaaaaaacatatattcatcgaggcacctttatgcaaccacatagtcaacttcaacgtcgcttgcgtgcgttctcaagttttctttcttgcaaattacattttttttaaaaaaaagtataatttgtatcgtgcgattttttctctctaggtgtgcgtgactgtgggagtaacaattttgaatctcaagaaggaaataaaagaataatactgctgcctactttgaggatttcagtatttttctctaaaatgttttggtgtgatatctaaaccgtctttaaagccaattgctcaagattcattcaacaattgaaacgtctcacatgactaaatgatataaggttgctaaggtctttcttgataagcttttttatgaatttcatctaaattttcgagtgaaactattaaatactaaggttgctaagtgtcattctcgctcgagaagtctaacgctttaaactttaaccaaatatatacaagaaaatattaatatttatagtacataattagtatcattagatagatcgttgaatctattttcataacaaacttatttgaagaaacaaatgttgttcatatatttctatatacgaataccatagcgacacttattttagaatgtagggagtactccctttgtgccgctttgagtgtcgctttggcagctagtacctatgtccaccttcacagcttgtgcctagtacctagactctttctctgtccacattcatttaatctctgttgtaccttgttcggagataaaacgactctgataaagggacgaggaagtagtatgttagaggagtgaagtctactccctttgccgcaaaaaggtaatcctaagtgtgaattgtattcttttttgaccaaaggaatatacaacaagaatgatgtcatcatcatgcttcgatccttttttttggtaaagcttgagcttctgtaaaaatagagaaatcatgggaaaaatcacgttttggtggttttgatttctagcctccacaataactttggttttactattttttgtttgattttagtttcagaagtccacttttgtacgtgctcgtagagcctaaacaaaaggctttccaaaacgaccttatcttcgagtgttgtaaaaaaaatgagcccgtttaacggcgtcgacaagtctaacggacaccaaccagcgaaccaccagcgccgagccaagcgaagcagactgcagacggcacggccgagacgttgacaccttggcgcggcaacggcatctctctggccccctctcgagagttccgctccacctccgcatccacctccacctccacctccaccggtggcggtttccaagtccgtcccgttccgccacctgctcctctcacacggcacgaaaccgtcacggcaccggcagcacagcacgggggattcctttcccaccgctccgtccctttctcttcctcgcccgcccgttataaatagccagccccatccctcgtctctcgt

SEQ ID NO: 68 - DNA, 55 bp, Miscanthus sinesis
gttgttcggagcgcacacacaacccgatccccaatcaatcgatccccgcttcaag

SEQ ID NO: 69 - DNA, 1924 bp, Miscanthus sinesis
gtacggcgatcctcctccctctctctctaccttctcttctctacactagatcggcggtccatggttagggcctgctagttccgttcctgtttttccatggctgcgaggtacaatagatctgatggcgttatgatggttaacttgtcatgcttttgcgatttatagtccctttagatagttcgagatcggtgatccatggttagtaccctaggctgtggagtcgggttagatccgcgctgttagggttcgtatatggaggcgagctgttctgattgttaacttgctgggaatcctgggatggttctagctgttccgcagatgagatcgatttcatgatctgctgtatctatccgtggtatgatgttagcctttgatatggttcgatcgtgctagctacgtcctgtgcacttaattgtcaggtcataatttttactatactttttttttggtttggtttggtttcgtctgatttggctgtcgttctagatcagagtagaaactgtttcaaactacctgttggatttattaaggtagcgtttggttcctggtatcgaatcatacacgcaccagtgcatcttggatagccagctggggcccacctgtccaaccgtttggttgccggatcgaacgagtccattcaagaccgaaccatgcagagcaatcgaatattctcttgtgacgctgtatcatccagttcggcaaaaaacaccgaatgccgccatacaggacaccgtactgagcgtctgcaactctgcatcccgctcactgctcacatctccgcttgccgcctcacccatccgactcagaccagagccacacggattactgctgctggtgtgtgtattaacaaaagatccatttgaccggagcacatgcagcttggatggaaaaaatttattatattcgtcagtgctgcatatgtactcatacttgcatgatggttttatttattcgacctcatcagtcctggcactatggaaagtcattgtagtatagattttttaatataatataaatcattggtgacttatcttgcttaattttattttcttattatgaaatatcgttgcattcataatagcaaatttgtgcaaatatatagaatctacgtgaaattcttggttggaccaatacaacaaacccctcaaacattctcttgtactgaaccataccattccgtacaaccatccaaacaaaaatcatgtatcatcatgtacatgtaaccaaacaattaacacgcaccatcctattcagacttgtctcatccataatctatccatccaggatgatccatcccattcatctatatacacccaatcaaacgctacctaaaatttggatctgtatgtgtcacatatatcttaataagatggatggaaatatctctttatcttttagatatggataggtatatatgttgctgtgggtttgttagttatatatatacgtgcttacatacgtgaagaaacctgctgctacagtttaataattcttgttcatctcaacaaataacgataggcgtatatgttgctgtgttttttactggtactttgttagatatatacatgcttacatacatgaagaacacatgctacagttcaaaaattcttgttcatctcataaacaaaaaggaggtgtatatgttgctgtgggttttactggtactttattagatatatacatgcttacatagatgaagcaacatgctgctatggtgtttaataattattgtttatctaataaacaaacatgctttttaattatcttgatatgtttggatgatggcatatgcagcagctatgtgtggattttaaatacccagcatcatgagcatgcatgaccctgccttagtatgcagttatttgcttgagactgtttcttttgttgatactcatcctttagttcggtcactcttctgcaggtg

SEQ ID NO: 70 - DNA, 3426 bp, Miscanthus sinesis
gcaaccacatagtcaacttcaacgtcgcttgcgtgcgttctcaagttttctttcttgcaaattacattttttttaaaaaaaagtataatttgtatcgtgcgattttttctctctaggtgtgcgtgactgtgggagtaacaattttgaatctcaagaaggaaataaaagaataatactgctgcctactttgaggatttcagtatttttctctaaaatgttttggtgtgatatctaaaccgtctttaaagccaattgctcaagattcattcaacaattgaaacgtctcacatgactaaatgatataaggttgctaaggtctttcttgataagcttttttatgaatttcatctaaattttcgagtgaaactattaaatactaaggttgctaagtgtcattctcgctcgagaagtctaacgctttaaactttaaccaaatatatacaagaaaatattaatatttatagtacataattagtatcattagatagatcgttgaatctattttcataacaaacttatttgaagaaacaaatgttgttcatatatttctatatacgaataccatagcgacacttattttagaatgtagggagtactccctttgtgccgctttgagtgtcgctttggcagctagtacctatgtccaccttcacagcttgtgcctagtacctagactctttctctgtccacattcatttaatctctgttgtaccttgttcggagataaaacgactctgataaagggacgaggaagtagtatgttagaggagtgaagtctactccctttgccgcaaaaaggtaatcctaagtgtgaattgtattcttttttgaccaaaggaatatacaacaagaatgatgtcatcatcatgcttcgatccttttttttggtaaagcttgagcttctgtaaaaatagagaaatcatgggaaaaatcacgttttggtggttttgatttctagcctccacaataactttggttttactattttttgtttgattttagtttcagaagtccacttttgtacgtgctcgtagagcctaaacaaaaggctttccaaaacgaccttatcttcgagtgttgtaaaaaaaatgagcccgtttaacggcgtcgacaagtctaacggacaccaaccagcgaaccaccagcgccgagccaagcgaagcagactgcagacggcacggccgagacgttgacaccttggcgcggcaacggcatctctctggccccctctcgagagttccgctccacctccgcatccacctccacctccacctccaccggtggcggtttccaagtccgtcccgttccgccacctgctcctctcacacggcacgaaaccgtcacggcaccggcagcacagcacgggggattcctttcccaccgctccgtccctttctcttcctcgcccgcccgttataaatagccagccccatccctcgtctctcgtgttgttcggagcgcacacacaacccgatccccaatcaatcgatccccgcttcaaggtacggcgatcctcctccctctctctctaccttctcttctctacactagatcggcggtccatggttagggcctgctagttccgttcctgtttttccatggctgcgaggtacaatagatctgatggcgttatgatggttaacttgtcatgcttttgcgatttatagtccctttagatagttcgagatcggtgatccatggttagtaccctaggctgtggagtcgggttagatccgcgctgttagggttcgtatatggaggcgagctgttctgattgttaacttgctgggaatcctgggatggttctagctgttccgcagatgagatcgatttcatgatctgctgtatctatccgtggtatgatgttagcctttgatatggttcgatcgtgctagctacgtcctgtgcacttaattgtcaggtcataatttttactatactttttttttggtttggtttggtttcgtctgatttggctgtcgttctagatcagagtagaaactgtttcaaactacctgttggatttattaaggtagcgtttggttcctggtatcgaatcatacacgcaccagtgcatcttggatagccagctggggcccacctgtccaaccgtttggttgccggatcgaacgagtccattcaagaccgaaccatgcagagcaatcgaatattctcttgtgacgctgtatcatccagttcggcaaaaaacaccgaatgccgccatacaggacaccgtactgagcgtctgcaactctgcatcccgctcactgctcacatctccgcttgccgcctcacccatccgactcagaccagagccacacggattactgctgctggtgtgtgtattaacaaaagatccatttgaccggagcacatgcagcttggatggaaaaaatttattatattcgtcagtgctgcatatgtactcatacttgcatgatggttttatttattcgacctcatcagtcctggcactatggaaagtcattgtagtatagattttttaatataatataaatcattggtgacttatcttgcttaattttattttcttattatgaaatatcgttgcattcataatagcaaatttgtgcaaatatatagaatctacgtgaaattcttggttggaccaatacaacaaacccctcaaacattctcttgtactgaaccataccattccgtacaaccatccaaacaaaaatcatgtatcatcatgtacatgtaaccaaacaattaacacgcaccatcctattcagacttgtctcatccataatctatccatccaggatgatccatcccattcatctatatacacccaatcaaacgctacctaaaatttggatctgtatgtgtcacatatatcttaataagatggatggaaatatctctttatcttttagatatggataggtatatatgttgctgtgggtttgttagttatatatatacgtgcttacatacgtgaagaaacctgctgctacagtttaataattcttgttcatctcaacaaataacgataggcgtatatgttgctgtgttttttactggtactttgttagatatatacatgcttacatacatgaagaacacatgctacagttcaaaaattcttgttcatctcataaacaaaaaggaggtgtatatgttgctgtgggttttactggtactttattagatatatacatgcttacatagatgaagcaacatgctgctatggtgtttaataattattgtttatctaataaacaaacatgctttttaattatcttgatatgtttggatgatggcatatgcagcagctatgtgtggattttaaatacccagcatcatgagcatgcatgaccctgccttagtatgcagttatttgcttgagactgtttcttttgttgatactcatcctttagttcggtcactcttctgcaggtg

SEQ ID NO: 71 - DNA, 1447 bp, Miscanthus sinesis
gcaaccacatagtcaacttcaacgtcgcttgcgtgcgttctcaagttttctttcttgcaaattacattttttttaaaaaaaagtataatttgtatcgtgcgattttttctctctaggtgtgcgtgactgtgggagtaacaattttgaatctcaagaaggaaataaaagaataatactgctgcctactttgaggatttcagtatttttctctaaaatgttttggtgtgatatctaaaccgtctttaaagccaattgctcaagattcattcaacaattgaaacgtctcacatgactaaatgatataaggttgctaaggtctttcttgataagcttttttatgaatttcatctaaattttcgagtgaaactattaaatactaaggttgctaagtgtcattctcgctcgagaagtctaacgctttaaactttaaccaaatatatacaagaaaatattaatatttatagtacataattagtatcattagatagatcgttgaatctattttcataacaaacttatttgaagaaacaaatgttgttcatatatttctatatacgaataccatagcgacacttattttagaatgtagggagtactccctttgtgccgctttgagtgtcgctttggcagctagtacctatgtccaccttcacagcttgtgcctagtacctagactctttctctgtccacattcatttaatctctgttgtaccttgttcggagataaaacgactctgataaagggacgaggaagtagtatgttagaggagtgaagtctactccctttgccgcaaaaaggtaatcctaagtgtgaattgtattcttttttgaccaaaggaatatacaacaagaatgatgtcatcatcatgcttcgatccttttttttggtaaagcttgagcttctgtaaaaatagagaaatcatgggaaaaatcacgttttggtggttttgatttctagcctccacaataactttggttttactattttttgtttgattttagtttcagaagtccacttttgtacgtgctcgtagagcctaaacaaaaggctttccaaaacgaccttatcttcgagtgttgtaaaaaaaatgagcccgtttaacggcgtcgacaagtctaacggacaccaaccagcgaaccaccagcgccgagccaagcgaagcagactgcagacggcacggccgagacgttgacaccttggcgcggcaacggcatctctctggccccctctcgagagttccgctccacctccgcatccacctccacctccacctccaccggtggcggtttccaagtccgtcccgttccgccacctgctcctctcacacggcacgaaaccgtcacggcaccggcagcacagcacgggggattcctttcccaccgctccgtccctttctcttcctcgcccgcccgttataaatagccagccccatccctcgtctctcgt

SEQ ID NO: 72 - DNA, 2878 bp, Miscanthus sinesis
ctatatacgaataccatagcgacacttattttagaatgtagggagtactccctttgtgccgctttgagtgtcgctttggcagctagtacctatgtccaccttcacagcttgtgcctagtacctagactctttctctgtccacattcatttaatctctgttgtaccttgttcggagataaaacgactctgataaagggacgaggaagtagtatgttagaggagtgaagtctactccctttgccgcaaaaaggtaatcctaagtgtgaattgtattcttttttgaccaaaggaatatacaacaagaatgatgtcatcatcatgcttcgatccttttttttggtaaagcttgagcttctgtaaaaatagagaaatcatgggaaaaatcacgttttggtggttttgatttctagcctccacaataactttggttttactattttttgtttgattttagtttcagaagtccacttttgtacgtgctcgtagagcctaaacaaaaggctttccaaaacgaccttatcttcgagtgttgtaaaaaaaatgagcccgtttaacggcgtcgacaagtctaacggacaccaaccagcgaaccaccagcgccgagccaagcgaagcagactgcagacggcacggccgagacgttgacaccttggcgcggcaacggcatctctctggccccctctcgagagttccgctccacctccgcatccacctccacctccacctccaccggtggcggtttccaagtccgtcccgttccgccacctgctcctctcacacggcacgaaaccgtcacggcaccggcagcacagcacgggggattcctttcccaccgctccgtccctttctcttcctcgcccgcccgttataaatagccagccccatccctcgtctctcgtgttgttcggagcgcacacacaacccgatccccaatcaatcgatccccgcttcaaggtacggcgatcctcctccctctctctctaccttctcttctctacactagatcggcggtccatggttagggcctgctagttccgttcctgtttttccatggctgcgaggtacaatagatctgatggcgttatgatggttaacttgtcatgcttttgcgatttatagtccctttagatagttcgagatcggtgatccatggttagtaccctaggctgtggagtcgggttagatccgcgctgttagggttcgtatatggaggcgagctgttctgattgttaacttgctgggaatcctgggatggttctagctgttccgcagatgagatcgatttcatgatctgctgtatctatccgtggtatgatgttagcctttgatatggttcgatcgtgctagctacgtcctgtgcacttaattgtcaggtcataatttttactatactttttttttggtttggtttggtttcgtctgatttggctgtcgttctagatcagagtagaaactgtttcaaactacctgttggatttattaaggtagcgtttggttcctggtatcgaatcatacacgcaccagtgcatcttggatagccagctggggcccacctgtccaaccgtttggttgccggatcgaacgagtccattcaagaccgaaccatgcagagcaatcgaatattctcttgtgacgctgtatcatccagttcggcaaaaaacaccgaatgccgccatacaggacaccgtactgagcgtctgcaactctgcatcccgctcactgctcacatctccgcttgccgcctcacccatccgactcagaccagagccacacggattactgctgctggtgtgtgtattaacaaaagatccatttgaccggagcacatgcagcttggatggaaaaaatttattatattcgtcagtgctgcatatgtactcatacttgcatgatggttttatttattcgacctcatcagtcctggcactatggaaagtcattgtagtatagattttttaatataatataaatcattggtgacttatcttgcttaattttattttcttattatgaaatatcgttgcattcataatagcaaatttgtgcaaatatatagaatctacgtgaaattcttggttggaccaatacaacaaacccctcaaacattctcttgtactgaaccataccattccgtacaaccatccaaacaaaaatcatgtatcatcatgtacatgtaaccaaacaattaacacgcaccatcctattcagacttgtctcatccataatctatccatccaggatgatccatcccattcatctatatacacccaatcaaacgctacctaaaatttggatctgtatgtgtcacatatatcttaataagatggatggaaatatctctttatcttttagatatggataggtatatatgttgctgtgggtttgttagttatatatatacgtgcttacatacgtgaagaaacctgctgctacagtttaataattcttgttcatctcaacaaataacgataggcgtatatgttgctgtgttttttactggtactttgttagatatatacatgcttacatacatgaagaacacatgctacagttcaaaaattcttgttcatctcataaacaaaaaggaggtgtatatgttgctgtgggttttactggtactttattagatatatacatgcttacatagatgaagcaacatgctgctatggtgtttaataattattgtttatctaataaacaaacatgctttttaattatcttgatatgtttggatgatggcatatgcagcagctatgtgtggattttaaatacccagcatcatgagcatgcatgaccctgccttagtatgcagttatttgcttgagactgtttcttttgttgatactcatcctttagttcggtcactcttctgcaggtg

SEQ ID NO: 73 - DNA, 899 bp, Miscanthus sinesis
ctatatacgaataccatagcgacacttattttagaatgtagggagtactccctttgtgccgctttgagtgtcgctttggcagctagtacctatgtccaccttcacagcttgtgcctagtacctagactctttctctgtccacattcatttaatctctgttgtaccttgttcggagataaaacgactctgataaagggacgaggaagtagtatgttagaggagtgaagtctactccctttgccgcaaaaaggtaatcctaagtgtgaattgtattcttttttgaccaaaggaatatacaacaagaatgatgtcatcatcatgcttcgatccttttttttggtaaagcttgagcttctgtaaaaatagagaaatcatgggaaaaatcacgttttggtggttttgatttctagcctccacaataactttggttttactattttttgtttgattttagtttcagaagtccacttttgtacgtgctcgtagagcctaaacaaaaggctttccaaaacgaccttatcttcgagtgttgtaaaaaaaatgagcccgtttaacggcgtcgacaagtctaacggacaccaaccagcgaaccaccagcgccgagccaagcgaagcagactgcagacggcacggccgagacgttgacaccttggcgcggcaacggcatctctctggccccctctcgagagttccgctccacctccgcatccacctccacctccacctccaccggtggcggtttccaagtccgtcccgttccgccacctgctcctctcacacggcacgaaaccgtcacggcaccggcagcacagcacgggggattcctttcccaccgctccgtccctttctcttcctcgcccgcccgttataaatagccagccccatccctcgtctctcgt

SEQ ID NO: 74 - DNA, 2670 bp, Miscanthus sinesis
gtatgttagaggagtgaagtctactccctttgccgcaaaaaggtaatcctaagtgtgaattgtattcttttttgaccaaaggaatatacaacaagaatgatgtcatcatcatgcttcgatccttttttttggtaaagcttgagcttctgtaaaaatagagaaatcatgggaaaaatcacgttttggtggttttgatttctagcctccacaataactttggttttactattttttgtttgattttagtttcagaagtccacttttgtacgtgctcgtagagcctaaacaaaaggctttccaaaacgaccttatcttcgagtgttgtaaaaaaaatgagcccgtttaacggcgtcgacaagtctaacggacaccaaccagcgaaccaccagcgccgagccaagcgaagcagactgcagacggcacggccgagacgttgacaccttggcgcggcaacggcatctctctggccccctctcgagagttccgctccacctccgcatccacctccacctccacctccaccggtggcggtttccaagtccgtcccgttccgccacctgctcctctcacacggcacgaaaccgtcacggcaccggcagcacagcacgggggattcctttcccaccgctccgtccctttctcttcctcgcccgcccgttataaatagccagccccatccctcgtctctcgtgttgttcggagcgcacacacaacccgatccccaatcaatcgatccccgcttcaaggtacggcgatcctcctccctctctctctaccttctcttctctacactagatcggcggtccatggttagggcctgctagttccgttcctgtttttccatggctgcgaggtacaatagatctgatggcgttatgatggttaacttgtcatgcttttgcgatttatagtccctttagatagttcgagatcggtgatccatggttagtaccctaggctgtggagtcgggttagatccgcgctgttagggttcgtatatggaggcgagctgttctgattgttaacttgctgggaatcctgggatggttctagctgttccgcagatgagatcgatttcatgatctgctgtatctatccgtggtatgatgttagcctttgatatggttcgatcgtgctagctacgtcctgtgcacttaattgtcaggtcataatttttactatactttttttttggtttggtttggtttcgtctgatttggctgtcgttctagatcagagtagaaactgtttcaaactacctgttggatttattaaggtagcgtttggttcctggtatcgaatcatacacgcaccagtgcatcttggatagccagctggggcccacctgtccaaccgtttggttgccggatcgaacgagtccattcaagaccgaaccatgcagagcaatcgaatattctcttgtgacgctgtatcatccagttcggcaaaaaacaccgaatgccgccatacaggacaccgtactgagcgtctgcaactctgcatcccgctcactgctcacatctccgcttgccgcctcacccatccgactcagaccagagccacacggattactgctgctggtgtgtgtattaacaaaagatccatttgaccggagcacatgcagcttggatggaaaaaatttattatattcgtcagtgctgcatatgtactcatacttgcatgatggttttatttattcgacctcatcagtcctggcactatggaaagtcattgtagtatagattttttaatataatataaatcattggtgacttatcttgcttaattttattttcttattatgaaatatcgttgcattcataatagcaaatttgtgcaaatatatagaatctacgtgaaattcttggttggaccaatacaacaaacccctcaaacattctcttgtactgaaccataccattccgtacaaccatccaaacaaaaatcatgtatcatcatgtacatgtaaccaaacaattaacacgcaccatcctattcagacttgtctcatccataatctatccatccaggatgatccatcccattcatctatatacacccaatcaaacgctacctaaaatttggatctgtatgtgtcacatatatcttaataagatggatggaaatatctctttatcttttagatatggataggtatatatgttgctgtgggtttgttagttatatatatacgtgcttacatacgtgaagaaacctgctgctacagtttaataattcttgttcatctcaacaaataacgataggcgtatatgttgctgtgttttttactggtactttgttagatatatacatgcttacatacatgaagaacacatgctacagttcaaaaattcttgttcatctcataaacaaaaaggaggtgtatatgttgctgtgggttttactggtactttattagatatatacatgcttacatagatgaagcaacatgctgctatggtgtttaataattattgtttatctaataaacaaacatgctttttaattatcttgatatgtttggatgatggcatatgcagcagctatgtgtggattttaaatacccagcatcatgagcatgcatgaccctgccttagtatgcagttatttgcttgagactgtttcttttgttgatactcatcctttagttcggtcactcttctgcaggtg

SEQ ID NO: 75 - DNA, 691 bp, Miscanthus sinesis
gtatgttagaggagtgaagtctactccctttgccgcaaaaaggtaatcctaagtgtgaattgtattcttttttgaccaaaggaatatacaacaagaatgatgtcatcatcatgcttcgatccttttttttggtaaagcttgagcttctgtaaaaatagagaaatcatgggaaaaatcacgttttggtggttttgatttctagcctccacaataactttggttttactattttttgtttgattttagtttcagaagtccacttttgtacgtgctcgtagagcctaaacaaaaggctttccaaaacgaccttatcttcgagtgttgtaaaaaaaatgagcccgtttaacggcgtcgacaagtctaacggacaccaaccagcgaaccaccagcgccgagccaagcgaagcagactgcagacggcacggccgagacgttgacaccttggcgcggcaacggcatctctctggccccctctcgagagttccgctccacctccgcatccacctccacctccacctccaccggtggcggtttccaagtccgtcccgttccgccacctgctcctctcacacggcacgaaaccgtcacggcaccggcagcacagcacgggggattcctttcccaccgctccgtccctttctcttcctcgcccgcccgttataaatagccagccccatccctcgtctctcgt

SEQ ID NO: 76 - DNA, 2485 bp, Miscanthus sinesis
gtggttttgatttctagcctccacaataactttggttttactattttttgtttgattttagtttcagaagtccacttttgtacgtgctcgtagagcctaaacaaaaggctttccaaaacgaccttatcttcgagtgttgtaaaaaaaatgagcccgtttaacggcgtcgacaagtctaacggacaccaaccagcgaaccaccagcgccgagccaagcgaagcagactgcagacggcacggccgagacgttgacaccttggcgcggcaacggcatctctctggccccctctcgagagttccgctccacctccgcatccacctccacctccacctccaccggtggcggtttccaagtccgtcccgttccgccacctgctcctctcacacggcacgaaaccgtcacggcaccggcagcacagcacgggggattcctttcccaccgctccgtccctttctcttcctcgcccgcccgttataaatagccagccccatccctcgtctctcgtgttgttcggagcgcacacacaacccgatccccaatcaatcgatccccgcttcaaggtacggcgatcctcctccctctctctctaccttctcttctctacactagatcggcggtccatggttagggcctgctagttccgttcctgtttttccatggctgcgaggtacaatagatctgatggcgttatgatggttaacttgtcatgcttttgcgatttatagtccctttagatagttcgagatcggtgatccatggttagtaccctaggctgtggagtcgggttagatccgcgctgttagggttcgtatatggaggcgagctgttctgattgttaacttgctgggaatcctgggatggttctagctgttccgcagatgagatcgatttcatgatctgctgtatctatccgtggtatgatgttagcctttgatatggttcgatcgtgctagctacgtcctgtgcacttaattgtcaggtcataatttttactatactttttttttggtttggtttggtttcgtctgatttggctgtcgttctagatcagagtagaaactgtttcaaactacctgttggatttattaaggtagcgtttggttcctggtatcgaatcatacacgcaccagtgcatcttggatagccagctggggcccacctgtccaaccgtttggttgccggatcgaacgagtccattcaagaccgaaccatgcagagcaatcgaatattctcttgtgacgctgtatcatccagttcggcaaaaaacaccgaatgccgccatacaggacaccgtactgagcgtctgcaactctgcatcccgctcactgctcacatctccgcttgccgcctcacccatccgactcagaccagagccacacggattactgctgctggtgtgtgtattaacaaaagatccatttgaccggagcacatgcagcttggatggaaaaaatttattatattcgtcagtgctgcatatgtactcatacttgcatgatggttttatttattcgacctcatcagtcctggcactatggaaagtcattgtagtatagattttttaatataatataaatcattggtgacttatcttgcttaattttattttcttattatgaaatatcgttgcattcataatagcaaatttgtgcaaatatatagaatctacgtgaaattcttggttggaccaatacaacaaacccctcaaacattctcttgtactgaaccataccattccgtacaaccatccaaacaaaaatcatgtatcatcatgtacatgtaaccaaacaattaacacgcaccatcctattcagacttgtctcatccataatctatccatccaggatgatccatcccattcatctatatacacccaatcaaacgctacctaaaatttggatctgtatgtgtcacatatatcttaataagatggatggaaatatctctttatcttttagatatggataggtatatatgttgctgtgggtttgttagttatatatatacgtgcttacatacgtgaagaaacctgctgctacagtttaataattcttgttcatctcaacaaataacgataggcgtatatgttgctgtgttttttactggtactttgttagatatatacatgcttacatacatgaagaacacatgctacagttcaaaaattcttgttcatctcataaacaaaaaggaggtgtatatgttgctgtgggttttactggtactttattagatatatacatgcttacatagatgaagcaacatgctgctatggtgtttaataattattgtttatctaataaacaaacatgctttttaattatcttgatatgtttggatgatggcatatgcagcagctatgtgtggattttaaatacccagcatcatgagcatgcatgaccctgccttagtatgcagttatttgcttgagactgtttcttttgttgatactcatcctttagttcggtcactcttctgcaggtg

SEQ ID NO: 77 - DNA, 506 bp, Miscanthus sinesis
gtggttttgatttctagcctccacaataactttggttttactattttttgtttgattttagtttcagaagtccacttttgtacgtgctcgtagagcctaaacaaaaggctttccaaaacgaccttatcttcgagtgttgtaaaaaaaatgagcccgtttaacggcgtcgacaagtctaacggacaccaaccagcgaaccaccagcgccgagccaagcgaagcagactgcagacggcacggccgagacgttgacaccttggcgcggcaacggcatctctctggccccctctcgagagttccgctccacctccgcatccacctccacctccacctccaccggtggcggtttccaagtccgtcccgttccgccacctgctcctctcacacggcacgaaaccgtcacggcaccggcagcacagcacgggggattcctttcccaccgctccgtccctttctcttcctcgcccgcccgttataaatagccagccccatccctcgtctctcgt

SEQ ID NO: 78 - DNA, 4079 bp, Schizachyium scoparium
ctctatgcctgtgtcattgtgccagcccctacctctgtcaatgttcaagatccaaataagagaatgggatagaccatatattaatggtgtagtatgcatcaagatctgaatattatatgagtgaattgataaatttattctaggtgacatggccttaacgatggccagtacgtggttaaatcaatgaatcaatagccatactctaatagctctaaaaaaggatatatatttgtcgaggcactattatgcaaccacatagtcaacttcaaagccgcttgagtgcgttctaaaaaaaaaatttcttgtaaattacgcttttctcaaaaaaattggatcatgcatttatttcactctaggtgtgcgtgactacgtgaataacaattttgaatctcagcaaggaaataaaagtataataccgctgtctactttgaagatcacaatatctttctcttagaatgtttctgtttgttatttaaaaccatcgttattaaggtcaaatgatcaagattcattcaacaattgaaacttctcacatgattacatcatatataaggttgctaaggtcttgcttgacaaggtatctctagtaacatctagtttttttgagtgaaataataaaattttaaagcaatgttacaagagaagctctggagataaaagttagaagggtgaagtttactccctctatcccaaagatgtaattctaagaatgacttaaattttttatacaaaaggagtatatatcacaagattgatgtcatcgttatgcttaggccacgtacacgacgctggcgcttatgtggacgttaatcggtaattcttcattttattttattttgttgtcaccgcgtacatttgggttaggcgtttgttaaaggcattgccactcaaacaagcagccgcgtttggagcttttatagtttgaaaagtgacggttgtaaagatgagtaagctgattattagtagagtaaattataattatcatacaacaactctcaaagtgggtgcacgttagtccaacatcttataatttatccaactcaatacaacaactatataggtgggtgcatgttggtccaacatcttctaatttgtttaatttgatacgagaacttgtcttattggtacatatatgatccaaagcattgtaacaacgtgtttatgtatactcttaatcatggtcatcagaagctaacacacacgctcatgccatccatatcattcaacttttgaatcgtttactatacaatattatttctaaatttggctgtaaagatggcattgatttcataaatatgaaaaataccaaattgcacattttctttctatattataatattgttttcatctattttcaccccgtaacctttaatttggtcatttagggctcactaaaactgatatgtgggttgtgcatcgcataagaatcaagaacccagaagtaattttcaatactaagaaacaacaaaatttggtttttttttgtttggtttcgattatagccgaactaaccaaatttaagaaagctttttatatttggccacataagaaatgatatcatttaatattgtaactgattcaagctgagtaatagatgagatgagtgtgttaggatgtgtagcttccgatgatagagaattagagtgtacaaagacgcatcgttacaatatttggaccttatatgcaccaatgtgtcaagtctcgcttcaaattaactatattaaaagatgttggatcaacatgcactcacttagatatcagtcgtattaaattgaacaaattacaagatattggactatgcacccactcaaatagttgttatatagtgaatacagtttactcttagtagtatatgtaagttcagccttttctattgtaggttaagccttaattaaggctcttacacaattgtttcattattcgcgttcgaagcagcttcttcgtagattttgcgagggaaggctgcctcggttttgccttccctagcactcatgtgagagcctctggcaataggtcttctcatttttattcacattctttaagagcccatataagcgttcatgacttgtatatactcttagatctttttttgtgggtaaagctcaagctaatctaaaaatagagaaatcaggaacaaagaatcatgttttggtggttttgatttctagcctccacaataattttagtttacctttttttgtttgattttaattttagaagggtttatagcaggacttaaaatccaaaatgaccattatcttcgagtaataacccgtttaacggcgtcgacaagtctaacggacaccaacccatgaaccaccagcgccgagccaagaactgaaggtcgagacgttgacacctttggcgcgacacggcatgttggcatctccctctctggccccctctcgagaattccgctccaccgcctcaaccggagacggtttccaaagttgtgcttagatgctcaaaagttggtgaaatcatttttatttggcaatttgtgtccaactatagactaattaggctcaaaagatttgtctcgtaaagtacattcaaactgtgtaattagttattttatttatctacatttaatactctatgaatgcgtcaagagatttgatgtgactttaatgtgacggacaatctgaaacttttacgcaacttgcatataaacagagcccaagtccgttccgttccgttccgcttcctcctcccagacggcacgaaaccgtgacggcaccggcagcacggggattcctttcccaccgctccttccttttcccttcatcgcccgcagctataaatagccacccccgtccgcaacttctttccccaacctcatcttttgttcggagcacgcacacaatccgatcgatccccaatcccctcgtctctcctcgcgagcctcgtcgatccgccattcaaggtacggcgatcatcctccctccctctctacctgctcttctgtagatcggcgaccccatccatggttagggcctgctagttctgttcctgttttttttccatggctgcgaggtagaatagatctgatggcgttatgatggttaatttgtcatactcttgcggtctatgggtccctttaggtcatcaatttaattttgggtggttgagatcggtgatccatggttagtaccctagtcagtggggttggatccgtgctattagggttcgtagatggattctgatggctcagtaactgggaatcctaggatggttccatctggtttgcagatgagaacgatttcatcatctgctatatcttgtttcgttgcgtaggttctgtttaaactaatccgtggtatgatgttagcctttgataaggttgatttcatcatctgctatatcttgtttcgttgcgtaggttctgtttaaactaatccgtggtatgatgttagcctttgataaggtttgattgtgctagctacgtcctgtgcagcagttaattgtcaggtcatacgtcataatttttagcatgtctgtttttgtttgatttcgttgtctgattaggctgtagatagtttcgatctacctgtcggtttattttattaaaatttggatccgtatgtgtgtcacatatatcttcatgattaagatggagttatatgggtaggttatacatgtggctgtggatcatgattaagatggattgaagtatctctttatcttttagttaggatagattattatatatgttgctgttgattttattggttctttattatatatattcatgcttatatacataaaagcaatgtgctattacagtttaatagttcttgattatctaataaacaaataaggataggtatatttgttgctgttggttttactggtactctattagatagtactttgacatgaagcaacatcctgctatggattaataattattcttcgtctaataaaaagcatggtttttaattattttgatttgatatacttggatgatgtcatatgcagcagctatttgtgaatttttcggccgtatcttcatattgcttgggactgtttctttggttgataactcaccctgttgtttggtgatccttctgcaggtg

SEQ ID NO: 79 - DNA, 2831 bp, Schizachyium scoparium
ctctatgcctgtgtcattgtgccagcccctacctctgtcaatgttcaagatccaaataagagaatgggatagaccatatattaatggtgtagtatgcatcaagatctgaatattatatgagtgaattgataaatttattctaggtgacatggccttaacgatggccagtacgtggttaaatcaatgaatcaatagccatactctaatagctctaaaaaaggatatatatttgtcgaggcactattatgcaaccacatagtcaacttcaaagccgcttgagtgcgttctaaaaaaaaaatttcttgtaaattacgcttttctcaaaaaaattggatcatgcatttatttcactctaggtgtgcgtgactacgtgaataacaattttgaatctcagcaaggaaataaaagtataataccgctgtctactttgaagatcacaatatctttctcttagaatgtttctgtttgttatttaaaaccatcgttattaaggtcaaatgatcaagattcattcaacaattgaaacttctcacatgattacatcatatataaggttgctaaggtcttgcttgacaaggtatctctagtaacatctagtttttttgagtgaaataataaaattttaaagcaatgttacaagagaagctctggagataaaagttagaagggtgaagtttactccctctatcccaaagatgtaattctaagaatgacttaaattttttatacaaaaggagtatatatcacaagattgatgtcatcgttatgcttaggccacgtacacgacgctggcgcttatgtggacgttaatcggtaattcttcattttattttattttgttgtcaccgcgtacatttgggttaggcgtttgttaaaggcattgccactcaaacaagcagccgcgtttggagcttttatagtttgaaaagtgacggttgtaaagatgagtaagctgattattagtagagtaaattataattatcatacaacaactctcaaagtgggtgcacgttagtccaacatcttataatttatccaactcaatacaacaactatataggtgggtgcatgttggtccaacatcttctaatttgtttaatttgatacgagaacttgtcttattggtacatatatgatccaaagcattgtaacaacgtgtttatgtatactcttaatcatggtcatcagaagctaacacacacgctcatgccatccatatcattcaacttttgaatcgtttactatacaatattatttctaaatttggctgtaaagatggcattgatttcataaatatgaaaaataccaaattgcacattttctttctatattataatattgttttcatctattttcaccccgtaacctttaatttggtcatttagggctcactaaaactgatatgtgggttgtgcatcgcataagaatcaagaacccagaagtaattttcaatactaagaaacaacaaaatttggtttttttttgtttggtttcgattatagccgaactaaccaaatttaagaaagctttttatatttggccacataagaaatgatatcatttaatattgtaactgattcaagctgagtaatagatgagatgagtgtgttaggatgtgtagcttccgatgatagagaattagagtgtacaaagacgcatcgttacaatatttggaccttatatgcaccaatgtgtcaagtctcgcttcaaattaactatattaaaagatgttggatcaacatgcactcacttagatatcagtcgtattaaattgaacaaattacaagatattggactatgcacccactcaaatagttgttatatagtgaatacagtttactcttagtagtatatgtaagttcagccttttctattgtaggttaagccttaattaaggctcttacacaattgtttcattattcgcgttcgaagcagcttcttcgtagattttgcgagggaaggctgcctcggttttgccttccctagcactcatgtgagagcctctggcaataggtcttctcatttttattcacattctttaagagcccatataagcgttcatgacttgtatatactcttagatctttttttgtgggtaaagctcaagctaatctaaaaatagagaaatcaggaacaaagaatcatgttttggtggttttgatttctagcctccacaataattttagtttacctttttttgtttgattttaattttagaagggtttatagcaggacttaaaatccaaaatgaccattatcttcgagtaataacccgtttaacggcgtcgacaagtctaacggacaccaacccatgaaccaccagcgccgagccaagaactgaaggtcgagacgttgacacctttggcgcgacacggcatgttggcatctccctctctggccccctctcgagaattccgctccaccgcctcaaccggagacggtttccaaagttgtgcttagatgctcaaaagttggtgaaatcatttttatttggcaatttgtgtccaactatagactaattaggctcaaaagatttgtctcgtaaagtacattcaaactgtgtaattagttattttatttatctacatttaatactctatgaatgcgtcaagagatttgatgtgactttaatgtgacggacaatctgaaacttttacgcaacttgcatataaacagagcccaagtccgttccgttccgttccgcttcctcctcccagacggcacgaaaccgtgacggcaccggcagcacggggattcctttcccaccgctccttccttttcccttcatcgcccgcagctataaatagccacccccgtccgcaacttctttc

SEQ ID NO: 80 - DNA, 95 bp, Schizachyium scoparium
cccaacctcatcttttgttcggagcacgcacacaatccgatcgatccccaatcccctcgtctctcctcgcgagcctcgtcgatccgccattcaag

SEQ ID NO: 81 - DNA, 1153 bp, Schizachyium scoparium
gtacggcgatcatcctccctccctctctacctgctcttctgtagatcggcgaccccatccatggttagggcctgctagttctgttcctgttttttttccatggctgcgaggtagaatagatctgatggcgttatgatggttaatttgtcatactcttgcggtctatgggtccctttaggtcatcaatttaattttgggtggttgagatcggtgatccatggttagtaccctagtcagtggggttggatccgtgctattagggttcgtagatggattctgatggctcagtaactgggaatcctaggatggttccatctggtttgcagatgagaacgatttcatcatctgctatatcttgtttcgttgcgtaggttctgtttaaactaatccgtggtatgatgttagcctttgataaggttgatttcatcatctgctatatcttgtttcgttgcgtaggttctgtttaaactaatccgtggtatgatgttagcctttgataaggtttgattgtgctagctacgtcctgtgcagcagttaattgtcaggtcatacgtcataatttttagcatgtctgtttttgtttgatttcgttgtctgattaggctgtagatagtttcgatctacctgtcggtttattttattaaaatttggatccgtatgtgtgtcacatatatcttcatgattaagatggagttatatgggtaggttatacatgtggctgtggatcatgattaagatggattgaagtatctctttatcttttagttaggatagattattatatatgttgctgttgattttattggttctttattatatatattcatgcttatatacataaaagcaatgtgctattacagtttaatagttcttgattatctaataaacaaataaggataggtatatttgttgctgttggttttactggtactctattagatagtactttgacatgaagcaacatcctgctatggattaataattattcttcgtctaataaaaagcatggtttttaattattttgatttgatatacttggatgatgtcatatgcagcagctatttgtgaatttttcggccgtatcttcatattgcttgggactgtttctttggttgataactcaccctgttgtttggtgatccttctgcaggtg

SEQ ID NO: 82 - DNA, 3281 bp, Schizachyium scoparium
gtggacgttaatcggtaattcttcattttattttattttgttgtcaccgcgtacatttgggttaggcgtttgttaaaggcattgccactcaaacaagcagccgcgtttggagcttttatagtttgaaaagtgacggttgtaaagatgagtaagctgattattagtagagtaaattataattatcatacaacaactctcaaagtgggtgcacgttagtccaacatcttataatttatccaactcaatacaacaactatataggtgggtgcatgttggtccaacatcttctaatttgtttaatttgatacgagaacttgtcttattggtacatatatgatccaaagcattgtaacaacgtgtttatgtatactcttaatcatggtcatcagaagctaacacacacgctcatgccatccatatcattcaacttttgaatcgtttactatacaatattatttctaaatttggctgtaaagatggcattgatttcataaatatgaaaaataccaaattgcacattttctttctatattataatattgttttcatctattttcaccccgtaacctttaatttggtcatttagggctcactaaaactgatatgtgggttgtgcatcgcataagaatcaagaacccagaagtaattttcaatactaagaaacaacaaaatttggtttttttttgtttggtttcgattatagccgaactaaccaaatttaagaaagctttttatatttggccacataagaaatgatatcatttaatattgtaactgattcaagctgagtaatagatgagatgagtgtgttaggatgtgtagcttccgatgatagagaattagagtgtacaaagacgcatcgttacaatatttggaccttatatgcaccaatgtgtcaagtctcgcttcaaattaactatattaaaagatgttggatcaacatgcactcacttagatatcagtcgtattaaattgaacaaattacaagatattggactatgcacccactcaaatagttgttatatagtgaatacagtttactcttagtagtatatgtaagttcagccttttctattgtaggttaagccttaattaaggctcttacacaattgtttcattattcgcgttcgaagcagcttcttcgtagattttgcgagggaaggctgcctcggttttgccttccctagcactcatgtgagagcctctggcaataggtcttctcatttttattcacattctttaagagcccatataagcgttcatgacttgtatatactcttagatcttttttttgtgggtaaagctcaagctaatctaaaaatagagaaatcaggaacaaagaatcatgttttggtggttttgatttctagcctccacaataattttagtttacctttttttgtttgattttaattttagaagggtttatagcaggacttaaaatccaaaatgaccattatcttcgagtaataacccgtttaacggcgtcgacaagtctaacggacaccaacccatgaaccaccagcgccgagccaagaactgaaggtcgagacgttgacacctttggcgcgacacggcatgttggcatctccctctctggccccctctcgagaattccgctccaccgcctcaaccggagacggtttccaaagttgtgcttagatgctcaaaagttggtgaaatcatttttatttggcaatttgtgtccaactatagactaattaggctcaaaagatttgtctcgtaaagtacattcaaactgtgtaattagttattttatttatctacatttaatactctatgaatgcgtcaagagatttgatgtgactttaatgtgacggacaatctgaaacttttacgcaacttgcatataaacagagcccaagtccgttccgttccgttccgcttcctcctcccagacggcacgaaaccgtgacggcaccggcagcacggggattcctttcccaccgctccttccttttcccttcatcgcccgcagctataaatagccacccccgtccgcaacttctttccccaacctcatcttttgttcggagcacgcacacaatccgatcgatccccaatcccctcgtctctcctcgcgagcctcgtcgatccgccattcaaggtacggcgatcatcctccctccctctctacctgctcttctgtagatcggcgaccccatccatggttagggcctgctagttctgttcctgttttttttccatggctgcgaggtagaatagatctgatggcgttatgatggttaatttgtcatactcttgcggtctatgggtccctttaggtcatcaatttaattttgggtggttgagatcggtgatccatggttagtaccctagtcagtggggttggatccgtgctattagggttcgtagatggattctgatggctcagtaactgggaatcctaggatggttccatctggtttgcagatgagaacgatttcatcatctgctatatcttgtttcgttgcgtaggttctgtttaaactaatccgtggtatgatgttagcctttgataaggttgatttcatcatctgctatatcttgtttcgttgcgtaggttctgtttaaactaatccgtggtatgatgttagcctttgataaggtttgattgtgctagctacgtcctgtgcagcagttaattgtcaggtcatacgtcataatttttagcatgtctgtttttgtttgatttcgttgtctgattaggctgtagatagtttcgatctacctgtcggtttattttattaaaatttggatccgtatgtgtgtcacatatatcttcatgattaagatggagttatatgggtaggttatacatgtggctgtggatcatgattaagatggattgaagtatctctttatcttttagttaggatagattattatatatgttgctgttgattttattggttctttattatatatattcatgcttatatacataaaagcaatgtgctattacagtttaatagttcttgattatctaataaacaaataaggataggtatatttgttgctgttggttttactggtactctattagatagtactttgacatgaagcaacatcctgctatggattaataattattcttcgtctaataaaaagcatggtttttaattattttgatttgatatacttggatgatgtcatatgcagcagctatttgtgaatttttcggccgtatcttcatattgcttgggactgtttctttggttgataactcaccctgttgtttggtgatccttctgcaggtg

SEQ ID NO: 83 - DNA, 2033 bp, Schizachyium scoparium
gtggacgttaatcggtaattcttcattttattttattttgttgtcaccgcgtacatttgggttaggcgtttgttaaaggcattgccactcaaacaagcagccgcgtttggagcttttatagtttgaaaagtgacggttgtaaagatgagtaagctgattattagtagagtaaattataattatcatacaacaactctcaaagtgggtgcacgttagtccaacatcttataatttatccaactcaatacaacaactatataggtgggtgcatgttggtccaacatcttctaatttgtttaatttgatacgagaacttgtcttattggtacatatatgatccaaagcattgtaacaacgtgtttatgtatactcttaatcatggtcatcagaagctaacacacacgctcatgccatccatatcattcaacttttgaatcgtttactatacaatattatttctaaatttggctgtaaagatggcattgatttcataaatatgaaaaataccaaattgcacattttctttctatattataatattgttttcatctattttcaccccgtaacctttaatttggtcatttagggctcactaaaactgatatgtgggttgtgcatcgcataagaatcaagaacccagaagtaattttcaatactaagaaacaacaaaatttggtttttttttgtttggtttcgattatagccgaactaaccaaatttaagaaagctttttatatttggccacataagaaatgatatcatttaatattgtaactgattcaagctgagtaatagatgagatgagtgtgttaggatgtgtagcttccgatgatagagaattagagtgtacaaagacgcatcgttacaatatttggaccttatatgcaccaatgtgtcaagtctcgcttcaaattaactatattaaaagatgttggatcaacatgcactcacttagatatcagtcgtattaaattgaacaaattacaagatattggactatgcacccactcaaatagttgttatatagtgaatacagtttactcttagtagtatatgtaagttcagccttttctattgtaggttaagccttaattaaggctcttacacaattgtttcattattcgcgttcgaagcagcttcttcgtagattttgcgagggaaggctgcctcggttttgccttccctagcactcatgtgagagcctctggcaataggtcttctcatttttattcacattctttaagagcccatataagcgttcatgacttgtatatactcttagatcttttttttgtgggtaaagctcaagctaatctaaaaatagagaaatcaggaacaaagaatcatgttttggtggttttgatttctagcctccacaataattttagtttacctttttttgtttgattttaattttagaagggtttatagcaggacttaaaatccaaaatgaccattatcttcgagtaataacccgtttaacggcgtcgacaagtctaacggacaccaacccatgaaccaccagcgccgagccaagaactgaaggtcgagacgttgacacctttggcgcgacacggcatgttggcatctccctctctggccccctctcgagaattccgctccaccgcctcaaccggagacggtttccaaagttgtgcttagatgctcaaaagttggtgaaatcatttttatttggcaatttgtgtccaactatagactaattaggctcaaaagatttgtctcgtaaagtacattcaaactgtgtaattagttattttatttatctacatttaatactctatgaatgcgtcaagagatttgatgtgactttaatgtgacggacaatctgaaacttttacgcaacttgcatataaacagagcccaagtccgttccgttccgttccgcttcctcctcccagacggcacgaaaccgtgacggcaccggcagcacggggattcctttcccaccgctccttccttttcccttcatcgcccgcagctataaatagccacccccgtccgcaacttctttc

SEQ ID NO: 84 - DNA, 2294 bp, Schizachyium scoparium
gatattggactatgcacccactcaaatagttgttatatagtgaatacagtttactcttagtagtatatgtaagttcagccttttctattgtaggttaagccttaattaaggctcttacacaattgtttcattattcgcgttcgaagcagcttcttcgtagattttgcgagggaaggctgcctcggttttgccttccctagcactcatgtgagagcctctggcaataggtcttctcatttttattcacattctttaagagcccatataagcgttcatgacttgtatatactcttagatcttttttttgtgggtaaagctcaagctaatctaaaaatagagaaatcaggaacaaagaatcatgttttggtggttttgatttctagcctccacaataattttagtttacctttttttgtttgattttaattttagaagggtttatagcaggacttaaaatccaaaatgaccattatcttcgagtaataacccgtttaacggcgtcgacaagtctaacggacaccaacccatgaaccaccagcgccgagccaagaactgaaggtcgagacgttgacacctttggcgcgacacggcatgttggcatctccctctctggccccctctcgagaattccgctccaccgcctcaaccggagacggtttccaaagttgtgcttagatgctcaaaagttggtgaaatcatttttatttggcaatttgtgtccaactatagactaattaggctcaaaagatttgtctcgtaaagtacattcaaactgtgtaattagttattttatttatctacatttaatactctatgaatgcgtcaagagatttgatgtgactttaatgtgacggacaatctgaaacttttacgcaacttgcatataaacagagcccaagtccgttccgttccgttccgcttcctcctcccagacggcacgaaaccgtgacggcaccggcagcacggggattcctttcccaccgctccttccttttcccttcatcgcccgcagctataaatagccacccccgtccgcaacttctttccccaacctcatcttttgttcggagcacgcacacaatccgatcgatccccaatcccctcgtctctcctcgcgagcctcgtcgatccgccattcaaggtacggcgatcatcctccctccctctctacctgctcttctgtagatcggcgaccccatccatggttagggcctgctagttctgttcctgttttttttccatggctgcgaggtagaatagatctgatggcgttatgatggttaatttgtcatactcttgcggtctatgggtccctttaggtcatcaatttaattttgggtggttgagatcggtgatccatggttagtaccctagtcagtggggttggatccgtgctattagggttcgtagatggattctgatggctcagtaactgggaatcctaggatggttccatctggtttgcagatgagaacgatttcatcatctgctatatcttgtttcgttgcgtaggttctgtttaaactaatccgtggtatgatgttagcctttgataaggttgatttcatcatctgctatatcttgtttcgttgcgtaggttctgtttaaactaatccgtggtatgatgttagcctttgataaggtttgattgtgctagctacgtcctgtgcagcagttaattgtcaggtcatacgtcataatttttagcatgtctgtttttgtttgatttcgttgtctgattaggctgtagatagtttcgatctacctgtcggtttattttattaaaatttggatccgtatgtgtgtcacatatatcttcatgattaagatggagttatatgggtaggttatacatgtggctgtggatcatgattaagatggattgaagtatctctttatcttttagttaggatagattattatatatgttgctgttgattttattggttctttattatatatattcatgcttatatacataaaagcaatgtgctattacagtttaatagttcttgattatctaataaacaaataaggataggtatatttgttgctgttggttttactggtactctattagatagtactttgacatgaagcaacatcctgctatggattaataattattcttcgtctaataaaaagcatggtttttaattattttgatttgatatacttggatgatgtcatatgcagcagctatttgtgaatttttcggccgtatcttcatattgcttgggactgtttctttggttgataactcaccctgttgtttggtgatccttctgcaggtg

SEQ ID NO: 85 - DNA, 1046 bp, Schizachyium scoparium
gatattggactatgcacccactcaaatagttgttatatagtgaatacagtttactcttagtagtatatgtaagttcagccttttctattgtaggttaagccttaattaaggctcttacacaattgtttcattattcgcgttcgaagcagcttcttcgtagattttgcgagggaaggctgcctcggttttgccttccctagcactcatgtgagagcctctggcaataggtcttctcatttttattcacattctttaagagcccatataagcgttcatgacttgtatatactcttagatcttttttttgtgggtaaagctcaagctaatctaaaaatagagaaatcaggaacaaagaatcatgttttggtggttttgatttctagcctccacaataattttagtttacctttttttgtttgattttaattttagaagggtttatagcaggacttaaaatccaaaatgaccattatcttcgagtaataacccgtttaacggcgtcgacaagtctaacggacaccaacccatgaaccaccagcgccgagccaagaactgaaggtcgagacgttgacacctttggcgcgacacggcatgttggcatctccctctctggccccctctcgagaattccgctccaccgcctcaaccggagacggtttccaaagttgtgcttagatgctcaaaagttggtgaaatcatttttatttggcaatttgtgtccaactatagactaattaggctcaaaagatttgtctcgtaaagtacattcaaactgtgtaattagttattttatttatctacatttaatactctatgaatgcgtcaagagatttgatgtgactttaatgtgacggacaatctgaaacttttacgcaacttgcatataaacagagcccaagtccgttccgttccgttccgcttcctcctcccagacggcacgaaaccgtgacggcaccggcagcacggggattcctttcccaccgctccttccttttcccttcatcgcccgcagctataaatagccacccccgtccgcaacttctttc

SEQ ID NO: 86 - DNA, 1795 bp, Schizachyium scoparium
gtcgacaagtctaacggacaccaacccatgaaccaccagcgccgagccaagaactgaaggtcgagacgttgacacctttggcgcgacacggcatgttggcatctccctctctggccccctctcgagaattccgctccaccgcctcaaccggagacggtttccaaagttgtgcttagatgctcaaaagttggtgaaatcatttttatttggcaatttgtgtccaactatagactaattaggctcaaaagatttgtctcgtaaagtacattcaaactgtgtaattagttattttatttatctacatttaatactctatgaatgcgtcaagagatttgatgtgactttaatgtgacggacaatctgaaacttttacgcaacttgcatataaacagagcccaagtccgttccgttccgttccgcttcctcctcccagacggcacgaaaccgtgacggcaccggcagcacggggattcctttcccaccgctccttccttttcccttcatcgcccgcagctataaatagccacccccgtccgcaacttctttccccaacctcatcttttgttcggagcacgcacacaatccgatcgatccccaatcccctcgtctctcctcgcgagcctcgtcgatccgccattcaaggtacggcgatcatcctccctccctctctacctgctcttctgtagatcggcgaccccatccatggttagggcctgctagttctgttcctgttttttttccatggctgcgaggtagaatagatctgatggcgttatgatggttaatttgtcatactcttgcggtctatgggtccctttaggtcatcaatttaattttgggtggttgagatcggtgatccatggttagtaccctagtcagtggggttggatccgtgctattagggttcgtagatggattctgatggctcagtaactgggaatcctaggatggttccatctggtttgcagatgagaacgatttcatcatctgctatatcttgtttcgttgcgtaggttctgtttaaactaatccgtggtatgatgttagcctttgataaggttgatttcatcatctgctatatcttgtttcgttgcgtaggttctgtttaaactaatccgtggtatgatgttagcctttgataaggtttgattgtgctagctacgtcctgtgcagcagttaattgtcaggtcatacgtcataatttttagcatgtctgtttttgtttgatttcgttgtctgattaggctgtagatagtttcgatctacctgtcggtttattttattaaaatttggatccgtatgtgtgtcacatatatcttcatgattaagatggagttatatgggtaggttatacatgtggctgtggatcatgattaagatggattgaagtatctctttatcttttagttaggatagattattatatatgttgctgttgattttattggttctttattatatatattcatgcttatatacataaaagcaatgtgctattacagtttaatagttcttgattatctaataaacaaataaggataggtatatttgttgctgttggttttactggtactctattagatagtactttgacatgaagcaacatcctgctatggattaataattattcttcgtctaataaaaagcatggtttttaattattttgatttgatatacttggatgatgtcatatgcagcagctatttgtgaatttttcggccgtatcttcatattgcttgggactgtttctttggttgataactcaccctgttgtttggtgatccttctgcaggtg

SEQ ID NO: 87 - DNA, 547 bp, Schizachyium scoparium
gtcgacaagtctaacggacaccaacccatgaaccaccagcgccgagccaagaactgaaggtcgagacgttgacacctttggcgcgacacggcatgttggcatctccctctctggccccctctcgagaattccgctccaccgcctcaaccggagacggtttccaaagttgtgcttagatgctcaaaagttggtgaaatcatttttatttggcaatttgtgtccaactatagactaattaggctcaaaagatttgtctcgtaaagtacattcaaactgtgtaattagttattttatttatctacatttaatactctatgaatgcgtcaagagatttgatgtgactttaatgtgacggacaatctgaaacttttacgcaacttgcatataaacagagcccaagtccgttccgttccgttccgcttcctcctcccagacggcacgaaaccgtgacggcaccggcagcacggggattcctttcccaccgctccttccttttcccttcatcgcccgcagctataaatagccacccccgtccgcaacttctttc

SEQ ID NO: 88 - DNA, 3357 bp, Sorghastrum nutans
gtggccagcttttgttctagttcaacggtccgggccttccgggaacctaatgcactaattgattattattaatctactattgcagctaacctcaaaagaaatgctctgcagttagttgtccgtcccaatcaatccaccagcagactcacattattgatggaggaaattaaattcagcctttgacgtggatgcaacaactgcacaagataccatctactttgcttaatttgctgatgttttgagaaaattaaaccagctttgaccaacacatgagatgggcgccttacgtttggcacaatgtaatgtagtccggcacggcaagttagactctgtgtgtagtgttatattagccggcctctttaggtttggcacaatttaattgaatccggcatggcaagttagactgcagtgtgagccggtcaccgcaagttaggatataatatacaagagcaagtatacaataaagtgacattagcgtaaagttatatgacatatggaatataagagaaaatacggagtatataataaggtgaactgtatagcgatcaaatttatgctaagcgaagaaaagagaagataaataggttgaaaacttatagtgagctttggctcataatctaaataattatgagagagtgggatcgaccacatattcattttgtagtacgtactctctccgttttttataagttgctttgatttttttttatatcaattttgctatacatctaaacataataggaatatcaagttcatgaaggtcgtgatttgcactaaatatgttcccttattagatagacgagttgtttagttttattgtagatgatatagcgcttgcatatagcatgtgaaccggctaaattattagccatacacgactataaaaaatgacattcctttgaggaacttttatgcaaccaaatagtcaacttcaatgttgctagagcgggctttaagccaaaagcagctgctgctttgtttccgagagaagggacattctagttgatagcaaaacaaatacgtagcagttgtagcgagtgtgtgagtaataatttttctctagtgtgtacgagtatgcgagtaataattttaaatctctagaaggaagaaaaataatattgctacctactttgaggatatcaatacctttctctaaaatgttttggtgaagccatctttaaagctaattgttcaagattcaaccattgggacgtctcaaatgattagatcctataatactcctacgtactaaattataagtcgttttgattttattggtacatacattttgctatgtgtttagatataataatatgtctagatacattggatgaaccgaaaaaatcgaaacgacttataatttggatcgaaaggagtatttgctaaagtccttttcgaagttccggctctaaatttttggataaaattttatgaaatactatcttaagaagtaatttgactagagaagcttgaagagtataatctcttaattttgtgctacaggagtgaagccaacgtcgtatttagatctagatgctgtcaggtagtgaggacggagggagtattggataaagtcattccaagatcttagaaaattaaagtatattaagtttgattaaatttatatgacaagtaataacattcatgatgccaattaagtatcattagattcttcatcaactatattttcatagtatacttatttaatgttataaatttttataattttttttataattttagctaaactcgagatcgattcttataattaaaaataaactgaaaaaaaatcacatgttcaagtgacaggaggagccagtttaacggcgtcgacaagtctaacggacaccaaccagcgaaccaccagcgccgagccaatcccaagcgaagccgactgcagacggccgagacgttgacacctttggcgcggcatccatctctccggccccctcttgagagttccgccccaccggcggcggtttccaagtccgttccgcccgccttcgcggttggacttgttccggtggcgcctggcggatcgcgtggcggagcggagacgacgaggtgagccgtgggcgttcctcctcctgctcctctcacacggcacggaacggaaccgtgacggcaccgggcagcacgggcgggattccttccccacctctccttcggtcctccctccatcataaatagccacccccctcccaccttctttccccacctcgtctcccctcgtgttattcggagcacagacacaccccgatccccaatcctctcctcgcgagcctcgtcgatccccgcttcaaggtacggcgatcatcctccctccctaactccaatccgtggttagggcctgctagatcgtcctccctccctacctgcgatccgtggttcgcgcctgctagttctgtttcctgtttgtcgatggctgcgaggtataatagatctgatggcgtgcggtgtgacggttaaattcacatgctcttgcgatttatacgcgaatcgatctgggattgctcgagatcggtgatccatggttagaaccctaggcggtggagtcgggttaaatccgtgctgttagggttcgtaggtggatgcgacctgttctggttgtttacttgtcagtatttaggaatcctactaggatggttctagctggttcgcagatgagatcgatttcatgatctgctatatctttcgttgcctaagtttcgtttaatctgtccgtggtatgatgttagcctttgatatgcttcgatcgtgctagctacctcctgtgcactaaattatcagctcgtaatttttagcatgcccttttttttttgggtattgttcgattgaggtgtcgttctagatcagagtaggaagactgtttcaaactacctgctggatttattaaatttggatctgtatgagtatcacatatatctccataatttagatggatggaaatatccctttttcttttagatactgtttggtatagattttgctgtgggttttactggtacttagatactcttcgtttagatatggatatgtttacatgcagatacatgaagcaacatgctgctacagtttaatatggataggtgtatatgttgttgtgggtcctttacttacatgcttagatacatgaagcaacatgctgctacgtttaataattattgtttatctgatctgatttaaacaaacatgctttttaattgtcctgaaatgcttggatgatggcatatgcagcagctatgtgtggattttaaatacccagcatgagcatgcatgaccctaacttagtatgctgtttatttgcttgacttttcttttgttgatactcacccttttgtttgttgactcttgcag

SEQ ID NO: 89 - DNA, 2218 bp, Sorghastrum nutans
gtggccagcttttgttctagttcaacggtccgggccttccgggaacctaatgcactaattgattattattaatctactattgcagctaacctcaaaagaaatgctctgcagttagttgtccgtcccaatcaatccaccagcagactcacattattgatggaggaaattaaattcagcctttgacgtggatgcaacaactgcacaagataccatctactttgcttaatttgctgatgttttgagaaaattaaaccagctttgaccaacacatgagatgggcgccttacgtttggcacaatgtaatgtagtccggcacggcaagttagactctgtgtgtagtgttatattagccggcctctttaggtttggcacaatttaattgaatccggcatggcaagttagactgcagtgtgagccggtcaccgcaagttaggatataatatacaagagcaagtatacaataaagtgacattagcgtaaagttatatgacatatggaatataagagaaaatacggagtatataataaggtgaactgtatagcgatcaaatttatgctaagcgaagaaaagagaagataaataggttgaaaacttatagtgagctttggctcataatctaaataattatgagagagtgggatcgaccacatattcattttgtagtacgtactctctccgttttttataagttgctttgatttttttttatatcaattttgctatacatctaaacataataggaatatcaagttcatgaaggtcgtgatttgcactaaatatgttcccttattagatagacgagttgtttagttttattgtagatgatatagcgcttgcatatagcatgtgaaccggctaaattattagccatacacgactataaaaaatgacattcctttgaggaacttttatgcaaccaaatagtcaacttcaatgttgctagagcgggctttaagccaaaagcagctgctgctttgtttccgagagaagggacattctagttgatagcaaaacaaatacgtagcagttgtagcgagtgtgtgagtaataatttttctctagtgtgtacgagtatgcgagtaataattttaaatctctagaaggaagaaaaataatattgctacctactttgaggatatcaatacctttctctaaaatgttttggtgaagccatctttaaagctaattgttcaagattcaaccattgggacgtctcaaatgattagatcctataatactcctacgtactaaattataagtcgttttgattttattggtacatacattttgctatgtgtttagatataataatatgtctagatacattggatgaaccgaaaaaatcgaaacgacttataatttggatcgaaaggagtatttgctaaagtccttttcgaagttccggctctaaatttttggataaaattttatgaaatactatcttaagaagtaatttgactagagaagcttgaagagtataatctcttaattttgtgctacaggagtgaagccaacgtcgtatttagatctagatgctgtcaggtagtgaggacggagggagtattggataaagtcattccaagatcttagaaaattaaagtatattaagtttgattaaatttatatgacaagtaataacattcatgatgccaattaagtatcattagattcttcatcaactatattttcatagtatacttatttaatgttataaatttttataattttttttataattttagctaaactcgagatcgattcttataattaaaaataaactgaaaaaaaatcacatgttcaagtgacaggaggagccagtttaacggcgtcgacaagtctaacggacaccaaccagcgaaccaccagcgccgagccaatcccaagcgaagccgactgcagacggccgagacgttgacacctttggcgcggcatccatctctccggccccctcttgagagttccgccccaccggcggcggtttccaagtccgttccgcccgccttcgcggttggacttgttccggtggcgcctggcggatcgcgtggcggagcggagacgacgaggtgagccgtgggcgttcctcctcctgctcctctcacacggcacggaacggaaccgtgacggcaccgggcagcacgggcgggattccttccccacctctccttcggtcctccctccatcataaatagccacccccctcccaccttctttccccac

SEQ ID NO: 90 - DNA, 86 bp, Sorghastrum nutans
ctcgtctcccctcgtgttattcggagcacagacacaccccgatccccaatcctctcctcgcgagcctcgtcgatccccgcttcaag

SEQ ID NO: 91 - DNA, 1053 bp, Sorghastrum nutans
gtacggcgatcatcctccctccctaactccaatccgtggttagggcctgctagatcgtcctccctccctacctgcgatccgtggttcgcgcctgctagttctgtttcctgtttgtcgatggctgcgaggtataatagatctgatggcgtgcggtgtgacggttaaattcacatgctcttgcgatttatacgcgaatcgatctgggattgctcgagatcggtgatccatggttagaaccctaggcggtggagtcgggttaaatccgtgctgttagggttcgtaggtggatgcgacctgttctggttgtttacttgtcagtatttaggaatcctactaggatggttctagctggttcgcagatgagatcgatttcatgatctgctatatctttcgttgcctaagtttcgtttaatctgtccgtggtatgatgttagcctttgatatgcttcgatcgtgctagctacctcctgtgcactaaattatcagctcgtaatttttagcatgcccttttttttttgggtattgttcgattgaggtgtcgttctagatcagagtaggaagactgtttcaaactacctgctggatttattaaatttggatctgtatgagtatcacatatatctccataatttagatggatggaaatatccctttttcttttagatactgtttggtatagattttgctgtgggttttactggtacttagatactcttcgtttagatatggatatgtttacatgcagatacatgaagcaacatgctgctacagtttaatatggataggtgtatatgttgttgtgggtcctttacttacatgcttagatacatgaagcaacatgctgctacgtttaataattattgtttatctgatctgatttaaacaaacatgctttttaattgtcctgaaatgcttggatgatggcatatgcagcagctatgtgtggattttaaatacccagcatgagcatgcatgaccctaacttagtatgctgtttatttgcttgacttttcttttgttgatactcacccttttgtttgttgactcttgcag

SEQ ID NO: 92 - DNA, 3106 bp, Sorghastrum nutans
agctttgaccaacacatgagatgggcgccttacgtttggcacaatgtaatgtagtccggcacggcaagttagactctgtgtgtagtgttatattagccggcctctttaggtttggcacaatttaattgaatccggcatggcaagttagactgcagtgtgagccggtcaccgcaagttaggatataatatacaagagcaagtatacaataaagtgacattagcgtaaagttatatgacatatggaatataagagaaaatacggagtatataataaggtgaactgtatagcgatcaaatttatgctaagcgaagaaaagagaagataaataggttgaaaacttatagtgagctttggctcataatctaaataattatgagagagtgggatcgaccacatattcattttgtagtacgtactctctccgttttttataagttgctttgatttttttttatatcaattttgctatacatctaaacataataggaatatcaagttcatgaaggtcgtgatttgcactaaatatgttcccttattagatagacgagttgtttagttttattgtagatgatatagcgcttgcatatagcatgtgaaccggctaaattattagccatacacgactataaaaaatgacattcctttgaggaacttttatgcaaccaaatagtcaacttcaatgttgctagagcgggctttaagccaaaagcagctgctgctttgtttccgagagaagggacattctagttgatagcaaaacaaatacgtagcagttgtagcgagtgtgtgagtaataatttttctctagtgtgtacgagtatgcgagtaataattttaaatctctagaaggaagaaaaataatattgctacctactttgaggatatcaatacctttctctaaaatgttttggtgaagccatctttaaagctaattgttcaagattcaaccattgggacgtctcaaatgattagatcctataatactcctacgtactaaattataagtcgttttgattttattggtacatacattttgctatgtgtttagatataataatatgtctagatacattggatgaaccgaaaaaatcgaaacgacttataatttggatcgaaaggagtatttgctaaagtccttttcgaagttccggctctaaatttttggataaaattttatgaaatactatcttaagaagtaatttgactagagaagcttgaagagtataatctcttaattttgtgctacaggagtgaagccaacgtcgtatttagatctagatgctgtcaggtagtgaggacggagggagtattggataaagtcattccaagatcttagaaaattaaagtatattaagtttgattaaatttatatgacaagtaataacattcatgatgccaattaagtatcattagattcttcatcaactatattttcatagtatacttatttaatgttataaatttttataattttttttataattttagctaaactcgagatcgattcttataattaaaaataaactgaaaaaaaatcacatgttcaagtgacaggaggagccagtttaacggcgtcgacaagtctaacggacaccaaccagcgaaccaccagcgccgagccaatcccaagcgaagccgactgcagacggccgagacgttgacacctttggcgcggcatccatctctccggccccctcttgagagttccgccccaccggcggcggtttccaagtccgttccgcccgccttcgcggttggacttgttccggtggcgcctggcggatcgcgtggcggagcggagacgacgaggtgagccgtgggcgttcctcctcctgctcctctcacacggcacggaacggaaccgtgacggcaccgggcagcacgggcgggattccttccccacctctccttcggtcctccctccatcataaatagccacccccctcccaccttctttccccacctcgtctcccctcgtgttattcggagcacagacacaccccgatccccaatcctctcctcgcgagcctcgtcgatccccgcttcaaggtacggcgatcatcctccctccctaactccaatccgtggttagggcctgctagatcgtcctccctccctacctgcgatccgtggttcgcgcctgctagttctgtttcctgtttgtcgatggctgcgaggtataatagatctgatggcgtgcggtgtgacggttaaattcacatgctcttgcgatttatacgcgaatcgatctgggattgctcgagatcggtgatccatggttagaaccctaggcggtggagtcgggttaaatccgtgctgttagggttcgtaggtggatgcgacctgttctggttgtttacttgtcagtatttaggaatcctactaggatggttctagctggttcgcagatgagatcgatttcatgatctgctatatctttcgttgcctaagtttcgtttaatctgtccgtggtatgatgttagcctttgatatgcttcgatcgtgctagctacctcctgtgcactaaattatcagctcgtaatttttagcatgcccttttttttttgggtattgttcgattgaggtgtcgttctagatcagagtaggaagactgtttcaaactacctgctggatttattaaatttggatctgtatgagtatcacatatatctccataatttagatggatggaaatatccctttttcttttagatactgtttggtatagattttgctgtgggttttactggtacttagatactcttcgtttagatatggatatgtttacatgcagatacatgaagcaacatgctgctacagtttaatatggataggtgtatatgttgttgtgggtcctttacttacatgcttagatacatgaagcaacatgctgctacgtttaataattattgtttatctgatctgatttaaacaaacatgctttttaattgtcctgaaatgcttggatgatggcatatgcagcagctatgtgtggattttaaatacccagcatgagcatgcatgaccctaacttagtatgctgtttatttgcttgacttttcttttgttgatactcacccttttgtttgttgactcttgcaggtg

SEQ ID NO: 93 - DNA, 1964 bp, Sorghastrum nutans
agctttgaccaacacatgagatgggcgccttacgtttggcacaatgtaatgtagtccggcacggcaagttagactctgtgtgtagtgttatattagccggcctctttaggtttggcacaatttaattgaatccggcatggcaagttagactgcagtgtgagccggtcaccgcaagttaggatataatatacaagagcaagtatacaataaagtgacattagcgtaaagttatatgacatatggaatataagagaaaatacggagtatataataaggtgaactgtatagcgatcaaatttatgctaagcgaagaaaagagaagataaataggttgaaaacttatagtgagctttggctcataatctaaataattatgagagagtgggatcgaccacatattcattttgtagtacgtactctctccgttttttataagttgctttgatttttttttatatcaattttgctatacatctaaacataataggaatatcaagttcatgaaggtcgtgatttgcactaaatatgttcccttattagatagacgagttgtttagttttattgtagatgatatagcgcttgcatatagcatgtgaaccggctaaattattagccatacacgactataaaaaatgacattcctttgaggaacttttatgcaaccaaatagtcaacttcaatgttgctagagcgggctttaagccaaaagcagctgctgctttgtttccgagagaagggacattctagttgatagcaaaacaaatacgtagcagttgtagcgagtgtgtgagtaataatttttctctagtgtgtacgagtatgcgagtaataattttaaatctctagaaggaagaaaaataatattgctacctactttgaggatatcaatacctttctctaaaatgttttggtgaagccatctttaaagctaattgttcaagattcaaccattgggacgtctcaaatgattagatcctataatactcctacgtactaaattataagtcgttttgattttattggtacatacattttgctatgtgtttagatataataatatgtctagatacattggatgaaccgaaaaaatcgaaacgacttataatttggatcgaaaggagtatttgctaaagtccttttcgaagttccggctctaaatttttggataaaattttatgaaatactatcttaagaagtaatttgactagagaagcttgaagagtataatctcttaattttgtgctacaggagtgaagccaacgtcgtatttagatctagatgctgtcaggtagtgaggacggagggagtattggataaagtcattccaagatcttagaaaattaaagtatattaagtttgattaaatttatatgacaagtaataacattcatgatgccaattaagtatcattagattcttcatcaactatattttcatagtatacttatttaatgttataaatttttataattttttttataattttagctaaactcgagatcgattcttataattaaaaataaactgaaaaaaaatcacatgttcaagtgacaggaggagccagtttaacggcgtcgacaagtctaacggacaccaaccagcgaaccaccagcgccgagccaatcccaagcgaagccgactgcagacggccgagacgttgacacctttggcgcggcatccatctctccggccccctcttgagagttccgccccaccggcggcggtttccaagtccgttccgcccgccttcgcggttggacttgttccggtggcgcctggcggatcgcgtggcggagcggagacgacgaggtgagccgtgggcgttcctcctcctgctcctctcacacggcacggaacggaaccgtgacggcaccgggcagcacgggcgggattccttccccacctctccttcggtcctccctccatcataaatagccacccccctcccaccttctttccccac

SEQ ID NO: 94 - DNA, 1056 bp, Sorghastrum nutans
gtacggcgatcatcctccctccctaactccaatccgtggttagggcctgctagatcgtcctccctccctacctgcgatccgtggttcgcgcctgctagttctgtttcctgtttgtcgatggctgcgaggtataatagatctgatggcgtgcggtgtgacggttaaattcacatgctcttgcgatttatacgcgaatcgatctgggattgctcgagatcggtgatccatggttagaaccctaggcggtggagtcgggttaaatccgtgctgttagggttcgtaggtggatgcgacctgttctggttgtttacttgtcagtatttaggaatcctactaggatggttctagctggttcgcagatgagatcgatttcatgatctgctatatctttcgttgcctaagtttcgtttaatctgtccgtggtatgatgttagcctttgatatgcttcgatcgtgctagctacctcctgtgcactaaattatcagctcgtaatttttagcatgcccttttttttttgggtattgttcgattgaggtgtcgttctagatcagagtaggaagactgtttcaaactacctgctggatttattaaatttggatctgtatgagtatcacatatatctccataatttagatggatggaaatatccctttttcttttagatactgtttggtatagattttgctgtgggttttactggtacttagatactcttcgtttagatatggatatgtttacatgcagatacatgaagcaacatgctgctacagtttaatatggataggtgtatatgttgttgtgggtcctttacttacatgcttagatacatgaagcaacatgctgctacgtttaataattattgtttatctgatctgatttaaacaaacatgctttttaattgtcctgaaatgcttggatgatggcatatgcagcagctatgtgtggattttaaatacccagcatgagcatgcatgaccctaacttagtatgctgtttatttgcttgacttttcttttgttgatactcacccttttgtttgttgactcttgcaggtg

SEQ ID NO: 95 - DNA, 2165 bp, Sorghastrum nutans
gattcaaccattgggacgtctcaaatgattagatcctataatactcctacgtactaaattataagtcgttttgattttattggtacatacattttgctatgtgtttagatataataatatgtctagatacattggatgaaccgaaaaaatcgaaacgacttataatttggatcgaaaggagtatttgctaaagtccttttcgaagttccggctctaaatttttggataaaattttatgaaatactatcttaagaagtaatttgactagagaagcttgaagagtataatctcttaattttgtgctacaggagtgaagccaacgtcgtatttagatctagatgctgtcaggtagtgaggacggagggagtattggataaagtcattccaagatcttagaaaattaaagtatattaagtttgattaaatttatatgacaagtaataacattcatgatgccaattaagtatcattagattcttcatcaactatattttcatagtatacttatttaatgttataaatttttataattttttttataattttagctaaactcgagatcgattcttataattaaaaataaactgaaaaaaaatcacatgttcaagtgacaggaggagccagtttaacggcgtcgacaagtctaacggacaccaaccagcgaaccaccagcgccgagccaatcccaagcgaagccgactgcagacggccgagacgttgacacctttggcgcggcatccatctctccggccccctcttgagagttccgccccaccggcggcggtttccaagtccgttccgcccgccttcgcggttggacttgttccggtggcgcctggcggatcgcgtggcggagcggagacgacgaggtgagccgtgggcgttcctcctcctgctcctctcacacggcacggaacggaaccgtgacggcaccgggcagcacgggcgggattccttccccacctctccttcggtcctccctccatcataaatagccacccccctcccaccttctttccccacctcgtctcccctcgtgttattcggagcacagacacaccccgatccccaatcctctcctcgcgagcctcgtcgatccccgcttcaaggtacggcgatcatcctccctccctaactccaatccgtggttagggcctgctagatcgtcctccctccctacctgcgatccgtggttcgcgcctgctagttctgtttcctgtttgtcgatggctgcgaggtataatagatctgatggcgtgcggtgtgacggttaaattcacatgctcttgcgatttatacgcgaatcgatctgggattgctcgagatcggtgatccatggttagaaccctaggcggtggagtcgggttaaatccgtgctgttagggttcgtaggtggatgcgacctgttctggttgtttacttgtcagtatttaggaatcctactaggatggttctagctggttcgcagatgagatcgatttcatgatctgctatatctttcgttgcctaagtttcgtttaatctgtccgtggtatgatgttagcctttgatatgcttcgatcgtgctagctacctcctgtgcactaaattatcagctcgtaatttttagcatgcccttttttttttgggtattgttcgattgaggtgtcgttctagatcagagtaggaagactgtttcaaactacctgctggatttattaaatttggatctgtatgagtatcacatatatctccataatttagatggatggaaatatccctttttcttttagatactgtttggtatagattttgctgtgggttttactggtacttagatactcttcgtttagatatggatatgtttacatgcagatacatgaagcaacatgctgctacagtttaatatggataggtgtatatgttgttgtgggtcctttacttacatgcttagatacatgaagcaacatgctgctacgtttaataattattgtttatctgatctgatttaaacaaacatgctttttaattgtcctgaaatgcttggatgatggcatatgcagcagctatgtgtggattttaaatacccagcatgagcatgcatgaccctaacttagtatgctgtttatttgcttgacttttcttttgttgatactcacccttttgtttgttgactcttgcaggtg

SEQ ID NO: 96 - DNA, 1023 bp, Sorghastrum nutans
gattcaaccattgggacgtctcaaatgattagatcctataatactcctacgtactaaattataagtcgttttgattttattggtacatacattttgctatgtgtttagatataataatatgtctagatacattggatgaaccgaaaaaatcgaaacgacttataatttggatcgaaaggagtatttgctaaagtccttttcgaagttccggctctaaatttttggataaaattttatgaaatactatcttaagaagtaatttgactagagaagcttgaagagtataatctcttaattttgtgctacaggagtgaagccaacgtcgtatttagatctagatgctgtcaggtagtgaggacggagggagtattggataaagtcattccaagatcttagaaaattaaagtatattaagtttgattaaatttatatgacaagtaataacattcatgatgccaattaagtatcattagattcttcatcaactatattttcatagtatacttatttaatgttataaatttttataattttttttataattttagctaaactcgagatcgattcttataattaaaaataaactgaaaaaaaatcacatgttcaagtgacaggaggagccagtttaacggcgtcgacaagtctaacggacaccaaccagcgaaccaccagcgccgagccaatcccaagcgaagccgactgcagacggccgagacgttgacacctttggcgcggcatccatctctccggccccctcttgagagttccgccccaccggcggcggtttccaagtccgttccgcccgccttcgcggttggacttgttccggtggcgcctggcggatcgcgtggcggagcggagacgacgaggtgagccgtgggcgttcctcctcctgctcctctcacacggcacggaacggaaccgtgacggcaccgggcagcacgggcgggattccttccccacctctccttcggtcctccctccatcataaatagccacccccctcccaccttctttccccac

SEQ ID NO: 97 - DNA, 1866 bp, Sorghastrum nutans
gtgctacaggagtgaagccaacgtcgtatttagatctagatgctgtcaggtagtgaggacggagggagtattggataaagtcattccaagatcttagaaaattaaagtatattaagtttgattaaatttatatgacaagtaataacattcatgatgccaattaagtatcattagattcttcatcaactatattttcatagtatacttatttaatgttataaatttttataattttttttataattttagctaaactcgagatcgattcttataattaaaaataaactgaaaaaaaatcacatgttcaagtgacaggaggagccagtttaacggcgtcgacaagtctaacggacaccaaccagcgaaccaccagcgccgagccaatcccaagcgaagccgactgcagacggccgagacgttgacacctttggcgcggcatccatctctccggccccctcttgagagttccgccccaccggcggcggtttccaagtccgttccgcccgccttcgcggttggacttgttccggtggcgcctggcggatcgcgtggcggagcggagacgacgaggtgagccgtgggcgttcctcctcctgctcctctcacacggcacggaacggaaccgtgacggcaccgggcagcacgggcgggattccttccccacctctccttcggtcctccctccatcataaatagccacccccctcccaccttctttccccacctcgtctcccctcgtgttattcggagcacagacacaccccgatccccaatcctctcctcgcgagcctcgtcgatccccgcttcaaggtacggcgatcatcctccctccctaactccaatccgtggttagggcctgctagatcgtcctccctccctacctgcgatccgtggttcgcgcctgctagttctgtttcctgtttgtcgatggctgcgaggtataatagatctgatggcgtgcggtgtgacggttaaattcacatgctcttgcgatttatacgcgaatcgatctgggattgctcgagatcggtgatccatggttagaaccctaggcggtggagtcgggttaaatccgtgctgttagggttcgtaggtggatgcgacctgttctggttgtttacttgtcagtatttaggaatcctactaggatggttctagctggttcgcagatgagatcgatttcatgatctgctatatctttcgttgcctaagtttcgtttaatctgtccgtggtatgatgttagcctttgatatgcttcgatcgtgctagctacctcctgtgcactaaattatcagctcgtaatttttagcatgcccttttttttttgggtattgttcgattgaggtgtcgttctagatcagagtaggaagactgtttcaaactacctgctggatttattaaatttggatctgtatgagtatcacatatatctccataatttagatggatggaaatatccctttttcttttagatactgtttggtatagattttgctgtgggttttactggtacttagatactcttcgtttagatatggatatgtttacatgcagatacatgaagcaacatgctgctacagtttaatatggataggtgtatatgttgttgtgggtcctttacttacatgcttagatacatgaagcaacatgctgctacgtttaataattattgtttatctgatctgatttaaacaaacatgctttttaattgtcctgaaatgcttggatgatggcatatgcagcagctatgtgtggattttaaatacccagcatgagcatgcatgaccctaacttagtatgctgtttatttgcttgacttttcttttgttgatactcacccttttgtttgttgactcttgcaggtg

SEQ ID NO: 98 - DNA, 724 bp, Sorghastrum nutans
gtgctacaggagtgaagccaacgtcgtatttagatctagatgctgtcaggtagtgaggacggagggagtattggataaagtcattccaagatcttagaaaattaaagtatattaagtttgattaaatttatatgacaagtaataacattcatgatgccaattaagtatcattagattcttcatcaactatattttcatagtatacttatttaatgttataaatttttataattttttttataattttagctaaactcgagatcgattcttataattaaaaataaactgaaaaaaaatcacatgttcaagtgacaggaggagccagtttaacggcgtcgacaagtctaacggacaccaaccagcgaaccaccagcgccgagccaatcccaagcgaagccgactgcagacggccgagacgttgacacctttggcgcggcatccatctctccggccccctcttgagagttccgccccaccggcggcggtttccaagtccgttccgcccgccttcgcggttggacttgttccggtggcgcctggcggatcgcgtggcggagcggagacgacgaggtgagccgtgggcgttcctcctcctgctcctctcacacggcacggaacggaaccgtgacggcaccgggcagcacgggcgggattccttccccacctctccttcggtcctccctccatcataaatagccacccccctcccaccttctttccccac

SEQ ID NO: 99 - DNA, 2625 bp, Setaria italica
actgccgcgacacgcctcactggcgggagggctccgagcgctctctccccggcggccggcggagcagcgatctggattggagagaatagaggaaagagagggaaaaggagagagatagcgcaaagagctgaaaagataaggttgtgcgggctgtggtgattagaggaccactaatccctccatctcctaatgacgcggtgcccaagaccagtgccgcggcacaccagcgtctaagtgaacttccgctaaccttccggtcattgcgcctgaaagatgtcatgtggcgaggcccccctctcagtagattgccaactgcctaccgtgccactcttccatgcatgattgctcccgtctatcccgtttctcacaacagatagacaacagtaagcatcactaaagcaagcatgtgtagaaccttaaaaaaaggcttatactaccagtatactatcaaccagcatgccgtttttgaagtatccaggattagaagcttctactgcgcttttatattatagctgtggacccgtggtaacctttctcttttggcgcttgcttaatctcggccgtgctggtccatgcttaggcactaggcagagatagagccgggggtgaatggggctaaagctcagctgctcgaggggccgtgggctggtttccactagcctacagctgtgccacgtgcggccgcgcaagccgaagcaagcacgctgagccgttggacagcttgtcataatgccattacgtggattacacgtaactggccctgtaactactcgttcggccatcatcaaacgacgacgtccgctaggcgacgacacgggtaatgcacgcagccacccaggcgcgcgcgctagcggagcacggtcaggtgacacgggcgtcgtgacgcttccgagttgaaggggttaacgccagaaacagtgtttggccagggtatgaacataacaaaaaatattcacacgaaagaatggaagtatggagctgctactgtgtaaatgccaagcaggaaactcacgcccgctaacatccaacggccaacagctcgacgtgccggtcagcagagcatcggaacactggtgattggtggagccggcagtatgcgccccagcacggccgaggtggtggtggcccgtggccctgctgtctgcgcggctcgggacaacttgaaactgggccaccgcctcgtcgcaactcgcaacccgttggcggaagaaaggaatggctcgtaggggcccgggtagaatcgaagaatgttgcgctgggcttcgattcacataacatgggcctgaagctctaaaacgacggcccggtcgccgcgcgatggaaagagaccggatcctcctcgtgaattctggaaggccacacgagagcgacccaccaccgacgcggaggagtcgtgcgtggtccaacacggccggcgggctgggctgcgaccttaaccagcaaggcacgccacgacccgccccgccctcgaggcataaataccctcccatcccgttgccgcaagactcagatcagattccgatccccagttcttccccaatcaccttgtggtctctcgtgtcgcggttcccagggacgcctccggctcgtcgctcgacagcgatctccgccccagcaaggtatagattcagttccttgctccgatcccaatctggttgagatgttgctccgatgcgacttgattatgtcatatatctgcggtttgcaccgatctgaagcctagggtttctcgagcgacccagttatttgcaatttgcgatttgctcgtttgttgcgcagcgtagtttatgtttggagtaatcgaggatttgtatgcggcgtcggcgctacctgcttaatcacgccatgtgacgcggttacttgcagaggctgggttctgttatgtcgtgatctaagaatctagattaggctcagtcgttcttgctgtcgactagtttgttttgatatccatgtagtacaagttacttaaaatttaggtccaatatattttgcatgcttttggcctgttattcttgccaacaagttgtcctggtaaaaagtagatgtgaaagtcacgtattgggacaaattgatggtttagtgctatagttctatagttctgtgatacatctatctgattttttttggtctattggtgcctaacttatctgaaaatcatggaacatgaggctagtttgatcatggtttagttcattgtgattaataatgtatgatttagtagctattttggtgatcgtgtcattttatttgtgaatggaatcattgtatgtaaatgaagctagttcaggggttacgatgtagctggctttgtattctaaaggctgctattattcatccatcgatttcacctatatgtaatccagagcttttgatgtgaaatttgtctgatccttcactaggaaggacagaacattgttaatattttggcacatctgtcttattctcatcctttgtttgaacatgttagcctgttcaaacagatactgttgtaatgtcctagttatataggtacatatgtgttctctattgagtttatggacttttgtgtgtgaagttatatttcattttgctcaaaactcatgtttgcaagctttctgacattattctattgttctgaaacagggt

SEQ ID NO: 100 - DNA, 1492 bp, Setaria italica
actgccgcgacacgcctcactggcgggagggctccgagcgctctctccccggcggccggcggagcagcgatctggattggagagaatagaggaaagagagggaaaaggagagagatagcgcaaagagctgaaaagataaggttgtgcgggctgtggtgattagaggaccactaatccctccatctcctaatgacgcggtgcccaagaccagtgccgcggcacaccagcgtctaagtgaacttccgctaaccttccggtcattgcgcctgaaagatgtcatgtggcgaggcccccctctcagtagattgccaactgcctaccgtgccactcttccatgcatgattgctcccgtctatcccgtttctcacaacagatagacaacagtaagcatcactaaagcaagcatgtgtagaaccttaaaaaaaggcttatactaccagtatactatcaaccagcatgccgtttttgaagtatccaggattagaagcttctactgcgcttttatattatagctgtggacccgtggtaacctttctcttttggcgcttgcttaatctcggccgtgctggtccatgcttaggcactaggcagagatagagccgggggtgaatggggctaaagctcagctgctcgaggggccgtgggctggtttccactagcctacagctgtgccacgtgcggccgcgcaagccgaagcaagcacgctgagccgttggacagcttgtcataatgccattacgtggattacacgtaactggccctgtaactactcgttcggccatcatcaaacgacgacgtccgctaggcgacgacacgggtaatgcacgcagccacccaggcgcgcgcgctagcggagcacggtcaggtgacacgggcgtcgtgacgcttccgagttgaaggggttaacgccagaaacagtgtttggccagggtatgaacataacaaaaaatattcacacgaaagaatggaagtatggagctgctactgtgtaaatgccaagcaggaaactcacgcccgctaacatccaacggccaacagctcgacgtgccggtcagcagagcatcggaacactggtgattggtggagccggcagtatgcgccccagcacggccgaggtggtggtggcccgtggccctgctgtctgcgcggctcgggacaacttgaaactgggccaccgcctcgtcgcaactcgcaacccgttggcggaagaaaggaatggctcgtaggggcccgggtagaatcgaagaatgttgcgctgggcttcgattcacataacatgggcctgaagctctaaaacgacggcccggtcgccgcgcgatggaaagagaccggatcctcctcgtgaattctggaaggccacacgagagcgacccaccaccgacgcggaggagtcgtgcgtggtccaacacggccggcgggctgggctgcgaccttaaccagcaaggcacgccacgacccgccccgccctcgaggcataaataccctcccatcc

SEQ ID NO: 101 - DNA, 127 bp, Setaria italica
cgttgccgcaagactcagatcagattccgatccccagttcttccccaatcaccttgtggtctctcgtgtcgcggttcccagggacgcctccggctcgtcgctcgacagcgatctccgccccagcaag

SEQ ID NO: 102 - DNA, 1006 bp, Setaria italica
gtatagattcagttccttgctccgatcccaatctggttgagatgttgctccgatgcgacttgattatgtcatatatctgcggtttgcaccgatctgaagcctagggtttctcgagcgacccagttatttgcaatttgcgatttgctcgtttgttgcgcagcgtagtttatgtttggagtaatcgaggatttgtatgcggcgtcggcgctacctgcttaatcacgccatgtgacgcggttacttgcagaggctgggttctgttatgtcgtgatctaagaatctagattaggctcagtcgttcttgctgtcgactagtttgttttgatatccatgtagtacaagttacttaaaatttaggtccaatatattttgcatgcttttggcctgttattcttgccaacaagttgtcctggtaaaaagtagatgtgaaagtcacgtattgggacaaattgatggtttagtgctatagttctatagttctgtgatacatctatctgattttttttggtctattggtgcctaacttatctgaaaatcatggaacatgaggctagtttgatcatggtttagttcattgtgattaataatgtatgatttagtagctattttggtgatcgtgtcattttatttgtgaatggaatcattgtatgtaaatgaagctagttcaggggttacgatgtagctggctttgtattctaaaggctgctattattcatccatcgatttcacctatatgtaatccagagcttttgatgtgaaatttgtctgatccttcactaggaaggacagaacattgttaatattttggcacatctgtcttattctcatcctttgtttgaacatgttagcctgttcaaacagatactgttgtaatgtcctagttatataggtacatatgtgttctctattgagtttatggacttttgtgtgtgaagttatatttcattttgctcaaaactcatgtttgcaagctttctgacattattctattgttctgaaacagggt

SEQ ID NO: 103 - DNA, 2625 bp, Setaria italica
actgccgcgacacgcctcactggcgggagggctccgagcgctctctccccggcggccggcggagcagcgatctggattggagagaatagaggaaagagagggaaaaggagagagatagcgcaaagagctgaaaagataaggttgtgcgggctgtggtgattagaggaccactaatccctccatctcctaatgacgcggtgcccaagaccagtgccgcggcacaccagcgtctaagtgaacttccgctaaccttccggtcattgcgcctgaaagatgtcatgtggcgaggcccccctctcagtagattgccaactgcctaccgtgccactcttccatgcatgattgctcccgtctatcccgtttctcacaacagatagacaacagtaagcatcactaaagcaagcatgtgtagaaccttaaaaaaaggcttatactaccagtatactatcaaccagcatgccgtttttgaagtatccaggattagaagcttctactgcgcttttatattatagctgtggacctgtggtaacctttctcttttggcgcttgcttaatctcggccgtgctggtccatgcttaggcactaggcagagatagagccgggggtgaatggggctaaagctcagctgctcgaggggccgtgggctggtttccactagcctacagctgtgccacgtgcggccgcgcaagccgaagcaagcacgctgagccgttggacagcttgtcataatgccattacgtggattacacgtaactggccctgtaactactcgttcggccatcatcaaacgacgacgtccgctaggcgacgacacgggtaatgcacgcagccacccaggcgcgcgcgctagcggagcacggtcaggtgacacgggcgtcgtgacgcttccgagttgaaggggttaacgccagaaacagtgtttggccagggtatgaacataacaaaaaatattcacacgaaagaatggaagtatggagctgctactgtgtaaatgccaagcaggaaactcacgcccgctaacatccaacggccaacagctcgacgtgccggtcagcagagcatcggaacactggtgattggtggagccggcagtatgcgccccagcacggccgaggtggtggtggcccgtggccctgctgtctgcgcggctcgggacaacttgaaactgggccaccgcctcgtcgcaactcgcaacccgttggcggaagaaaggaatggctcgtaggggcccgggtagaatcgaagaatgttgcgctgggcttcgattcacataacatgggcctgaagctctaaaacgacggcccggtcgccgcgcgatggaaagagaccggatcctcctcgtgaattctggaaggccacacgagagcgacccaccaccgacgcggaggagtcgtgcgtggtccaacacggccggcgggctgggctgcgaccttaaccagcaaggcacgccacgacccgccccgccctcgaggcataaataccctcccatcccgttgccgcaagactcagatcagattccgatccccagttcttccccaatcaccttgtggtctctcgtgtcgcggttcccagggacgcctccggctcgtcgctcgacagcgatctccgccccagcaaggtatagattcagttccttgctccgatcccaatctggttgagatgttgctccgatgcgacttgattatgtcatatatctgcggtttgcaccgatctgaagcctagggtttctcgagcgacccagttatttgcaatttgcgatttgctcgtttgttgcgcagcgtagtttatgtttggagtaatcgaggatttgtatgcggcgtcggcgctacctgcttaatcacgccatgtgacgcggttacttgcagaggctgggttctgttatgtcgtgatctaagaatctagattaggctcagtcgttcttgctgtcgactagtttgttttgatatccatgtagtacaagttacttaaaatttaggtccaatatattttgcatgcttttggcctgttattcttgccaacaagttgtcctggtaaaaagtagatgtgaaagtcacgtattgggacaaattgatggtttagtgctatagttctatagttctgtgatacatctatctgattttttttggtctattggtgcctaacttatctgaaaatcatggaacatgaggctagtttgatcatggtttagttcattgtgattaataatgtatgatttagtagctattttggtgatcgtgtcattttatttgtgaatggaatcattgtatgtaaatgaagctagttcaggggttacgatgtagctggctttgtattctaaaggctgctattattcatccatcgatttcacctatatgtaatccagagcttttgatgtgaaatttgtctgatccttcactaggaaggacagaacattgttaatattttggcacatctgtcttattctcatcctttgtttgaacatgttagcctgttcaaacagatactgttgtaatgtcctagttatataggtacatatgtgttctctattgagtttatggacttttgtgtgtgaagttatatttcattttgctcaaaactcatgtttgcaagctttctgacattattctattgttctgaaacaggtg

SEQ ID NO: 104 - DNA, 1492 bp, Setaria italica
actgccgcgacacgcctcactggcgggagggctccgagcgctctctccccggcggccggcggagcagcgatctggattggagagaatagaggaaagagagggaaaaggagagagatagcgcaaagagctgaaaagataaggttgtgcgggctgtggtgattagaggaccactaatccctccatctcctaatgacgcggtgcccaagaccagtgccgcggcacaccagcgtctaagtgaacttccgctaaccttccggtcattgcgcctgaaagatgtcatgtggcgaggcccccctctcagtagattgccaactgcctaccgtgccactcttccatgcatgattgctcccgtctatcccgtttctcacaacagatagacaacagtaagcatcactaaagcaagcatgtgtagaaccttaaaaaaaggcttatactaccagtatactatcaaccagcatgccgtttttgaagtatccaggattagaagcttctactgcgcttttatattatagctgtggacctgtggtaacctttctcttttggcgcttgcttaatctcggccgtgctggtccatgcttaggcactaggcagagatagagccgggggtgaatggggctaaagctcagctgctcgaggggccgtgggctggtttccactagcctacagctgtgccacgtgcggccgcgcaagccgaagcaagcacgctgagccgttggacagcttgtcataatgccattacgtggattacacgtaactggccctgtaactactcgttcggccatcatcaaacgacgacgtccgctaggcgacgacacgggtaatgcacgcagccacccaggcgcgcgcgctagcggagcacggtcaggtgacacgggcgtcgtgacgcttccgagttgaaggggttaacgccagaaacagtgtttggccagggtatgaacataacaaaaaatattcacacgaaagaatggaagtatggagctgctactgtgtaaatgccaagcaggaaactcacgcccgctaacatccaacggccaacagctcgacgtgccggtcagcagagcatcggaacactggtgattggtggagccggcagtatgcgccccagcacggccgaggtggtggtggcccgtggccctgctgtctgcgcggctcgggacaacttgaaactgggccaccgcctcgtcgcaactcgcaacccgttggcggaagaaaggaatggctcgtaggggcccgggtagaatcgaagaatgttgcgctgggcttcgattcacataacatgggcctgaagctctaaaacgacggcccggtcgccgcgcgatggaaagagaccggatcctcctcgtgaattctggaaggccacacgagagcgacccaccaccgacgcggaggagtcgtgcgtggtccaacacggccggcgggctgggctgcgaccttaaccagcaaggcacgccacgacccgccccgccctcgaggcataaataccctcccatcc

SEQ ID NO: 105 - DNA, 1006 bp, Setaria italica
gtatagattcagttccttgctccgatcccaatctggttgagatgttgctccgatgcgacttgattatgtcatatatctgcggtttgcaccgatctgaagcctagggtttctcgagcgacccagttatttgcaatttgcgatttgctcgtttgttgcgcagcgtagtttatgtttggagtaatcgaggatttgtatgcggcgtcggcgctacctgcttaatcacgccatgtgacgcggttacttgcagaggctgggttctgttatgtcgtgatctaagaatctagattaggctcagtcgttcttgctgtcgactagtttgttttgatatccatgtagtacaagttacttaaaatttaggtccaatatattttgcatgcttttggcctgttattcttgccaacaagttgtcctggtaaaaagtagatgtgaaagtcacgtattgggacaaattgatggtttagtgctatagttctatagttctgtgatacatctatctgattttttttggtctattggtgcctaacttatctgaaaatcatggaacatgaggctagtttgatcatggtttagttcattgtgattaataatgtatgatttagtagctattttggtgatcgtgtcattttatttgtgaatggaatcattgtatgtaaatgaagctagttcaggggttacgatgtagctggctttgtattctaaaggctgctattattcatccatcgatttcacctatatgtaatccagagcttttgatgtgaaatttgtctgatccttcactaggaaggacagaacattgttaatattttggcacatctgtcttattctcatcctttgtttgaacatgttagcctgttcaaacagatactgttgtaatgtcctagttatataggtacatatgtgttctctattgagtttatggacttttgtgtgtgaagttatatttcattttgctcaaaactcatgtttgcaagctttctgacattattctattgttctgaaacaggtg

SEQ ID NO: 106 - DNA, 2167 bp, Setaria italica
gccgtttttgaagtatccaggattagaagcttctactgcgcttttatattatagctgtggacctgtggtaacctttctcttttggcgcttgcttaatctcggccgtgctggtccatgcttaggcactaggcagagatagagccgggggtgaatggggctaaagctcagctgctcgaggggccgtgggctggtttccactagcctacagctgtgccacgtgcggccgcgcaagccgaagcaagcacgctgagccgttggacagcttgtcataatgccattacgtggattacacgtaactggccctgtaactactcgttcggccatcatcaaacgacgacgtccgctaggcgacgacacgggtaatgcacgcagccacccaggcgcgcgcgctagcggagcacggtcaggtgacacgggcgtcgtgacgcttccgagttgaaggggttaacgccagaaacagtgtttggccagggtatgaacataacaaaaaatattcacacgaaagaatggaagtatggagctgctactgtgtaaatgccaagcaggaaactcacgcccgctaacatccaacggccaacagctcgacgtgccggtcagcagagcatcggaacactggtgattggtggagccggcagtatgcgccccagcacggccgaggtggtggtggcccgtggccctgctgtctgcgcggctcgggacaacttgaaactgggccaccgcctcgtcgcaactcgcaacccgttggcggaagaaaggaatggctcgtaggggcccgggtagaatcgaagaatgttgcgctgggcttcgattcacataacatgggcctgaagctctaaaacgacggcccggtcgccgcgcgatggaaagagaccggatcctcctcgtgaattctggaaggccacacgagagcgacccaccaccgacgcggaggagtcgtgcgtggtccaacacggccggcgggctgggctgcgaccttaaccagcaaggcacgccacgacccgccccgccctcgaggcataaataccctcccatcccgttgccgcaagactcagatcagattccgatccccagttcttccccaatcaccttgtggtctctcgtgtcgcggttcccagggacgcctccggctcgtcgctcgacagcgatctccgccccagcaaggtatagattcagttccttgctccgatcccaatctggttgagatgttgctccgatgcgacttgattatgtcatatatctgcggtttgcaccgatctgaagcctagggtttctcgagcgacccagttatttgcaatttgcgatttgctcgtttgttgcgcagcgtagtttatgtttggagtaatcgaggatttgtatgcggcgtcggcgctacctgcttaatcacgccatgtgacgcggttacttgcagaggctgggttctgttatgtcgtgatctaagaatctagattaggctcagtcgttcttgctgtcgactagtttgttttgatatccatgtagtacaagttacttaaaatttaggtccaatatattttgcatgcttttggcctgttattcttgccaacaagttgtcctggtaaaaagtagatgtgaaagtcacgtattgggacaaattgatggtttagtgctatagttctatagttctgtgatacatctatctgattttttttggtctattggtgcctaacttatctgaaaatcatggaacatgaggctagtttgatcatggtttagttcattgtgattaataatgtatgatttagtagctattttggtgatcgtgtcattttatttgtgaatggaatcattgtatgtaaatgaagctagttcaggggttacgatgtagctggctttgtattctaaaggctgctattattcatccatcgatttcacctatatgtaatccagagcttttgatgtgaaatttgtctgatccttcactaggaaggacagaacattgttaatattttggcacatctgtcttattctcatcctttgtttgaacatgttagcctgttcaaacagatactgttgtaatgtcctagttatataggtacatatgtgttctctattgagtttatggacttttgtgtgtgaagttatatttcattttgctcaaaactcatgtttgcaagctttctgacattattctattgttctgaaacaggtg

SEQ ID NO: 107 - DNA, 1034 bp, Setaria italica
gccgtttttgaagtatccaggattagaagcttctactgcgcttttatattatagctgtggacctgtggtaacctttctcttttggcgcttgcttaatctcggccgtgctggtccatgcttaggcactaggcagagatagagccgggggtgaatggggctaaagctcagctgctcgaggggccgtgggctggtttccactagcctacagctgtgccacgtgcggccgcgcaagccgaagcaagcacgctgagccgttggacagcttgtcataatgccattacgtggattacacgtaactggccctgtaactactcgttcggccatcatcaaacgacgacgtccgctaggcgacgacacgggtaatgcacgcagccacccaggcgcgcgcgctagcggagcacggtcaggtgacacgggcgtcgtgacgcttccgagttgaaggggttaacgccagaaacagtgtttggccagggtatgaacataacaaaaaatattcacacgaaagaatggaagtatggagctgctactgtgtaaatgccaagcaggaaactcacgcccgctaacatccaacggccaacagctcgacgtgccggtcagcagagcatcggaacactggtgattggtggagccggcagtatgcgccccagcacggccgaggtggtggtggcccgtggccctgctgtctgcgcggctcgggacaacttgaaactgggccaccgcctcgtcgcaactcgcaacccgttggcggaagaaaggaatggctcgtaggggcccgggtagaatcgaagaatgttgcgctgggcttcgattcacataacatgggcctgaagctctaaaacgacggcccggtcgccgcgcgatggaaagagaccggatcctcctcgtgaattctggaaggccacacgagagcgacccaccaccgacgcggaggagtcgtgcgtggtccaacacggccggcgggctgggctgcgaccttaaccagcaaggcacgccacgacccgccccgccctcgaggcataaataccctcccatcc

SEQ ID NO: 108 - DNA, 1813 bp, Setaria italica
cacgggtaatgcacgcagccacccaggcgcgcgcgctagcggagcacggtcaggtgacacgggcgtcgtgacgcttccgagttgaaggggttaacgccagaaacagtgtttggccagggtatgaacataacaaaaaatattcacacgaaagaatggaagtatggagctgctactgtgtaaatgccaagcaggaaactcacgcccgctaacatccaacggccaacagctcgacgtgccggtcagcagagcatcggaacactggtgattggtggagccggcagtatgcgccccagcacggccgaggtggtggtggcccgtggccctgctgtctgcgcggctcgggacaacttgaaactgggccaccgcctcgtcgcaactcgcaacccgttggcggaagaaaggaatggctcgtaggggcccgggtagaatcgaagaatgttgcgctgggcttcgattcacataacatgggcctgaagctctaaaacgacggcccggtcgccgcgcgatggaaagagaccggatcctcctcgtgaattctggaaggccacacgagagcgacccaccaccgacgcggaggagtcgtgcgtggtccaacacggccggcgggctgggctgcgaccttaaccagcaaggcacgccacgacccgccccgccctcgaggcataaataccctcccatcccgttgccgcaagactcagatcagattccgatccccagttcttccccaatcaccttgtggtctctcgtgtcgcggttcccagggacgcctccggctcgtcgctcgacagcgatctccgccccagcaaggtatagattcagttccttgctccgatcccaatctggttgagatgttgctccgatgcgacttgattatgtcatatatctgcggtttgcaccgatctgaagcctagggtttctcgagcgacccagttatttgcaatttgcgatttgctcgtttgttgcgcagcgtagtttatgtttggagtaatcgaggatttgtatgcggcgtcggcgctacctgcttaatcacgccatgtgacgcggttacttgcagaggctgggttctgttatgtcgtgatctaagaatctagattaggctcagtcgttcttgctgtcgactagtttgttttgatatccatgtagtacaagttacttaaaatttaggtccaatatattttgcatgcttttggcctgttattcttgccaacaagttgtcctggtaaaaagtagatgtgaaagtcacgtattgggacaaattgatggtttagtgctatagttctatagttctgtgatacatctatctgattttttttggtctattggtgcctaacttatctgaaaatcatggaacatgaggctagtttgatcatggtttagttcattgtgattaataatgtatgatttagtagctattttggtgatcgtgtcattttatttgtgaatggaatcattgtatgtaaatgaagctagttcaggggttacgatgtagctggctttgtattctaaaggctgctattattcatccatcgatttcacctatatgtaatccagagcttttgatgtgaaatttgtctgatccttcactaggaaggacagaacattgttaatattttggcacatctgtcttattctcatcctttgtttgaacatgttagcctgttcaaacagatactgttgtaatgtcctagttatataggtacatatgtgttctctattgagtttatggacttttgtgtgtgaagttatatttcattttgctcaaaactcatgtttgcaagctttctgacattattctattgttctgaaacaggtg

SEQ ID NO: 109 - DNA, 680 bp, Setaria italica
cacgggtaatgcacgcagccacccaggcgcgcgcgctagcggagcacggtcaggtgacacgggcgtcgtgacgcttccgagttgaaggggttaacgccagaaacagtgtttggccagggtatgaacataacaaaaaatattcacacgaaagaatggaagtatggagctgctactgtgtaaatgccaagcaggaaactcacgcccgctaacatccaacggccaacagctcgacgtgccggtcagcagagcatcggaacactggtgattggtggagccggcagtatgcgccccagcacggccgaggtggtggtggcccgtggccctgctgtctgcgcggctcgggacaacttgaaactgggccaccgcctcgtcgcaactcgcaacccgttggcggaagaaaggaatggctcgtaggggcccgggtagaatcgaagaatgttgcgctgggcttcgattcacataacatgggcctgaagctctaaaacgacggcccggtcgccgcgcgatggaaagagaccggatcctcctcgtgaattctggaaggccacacgagagcgacccaccaccgacgcggaggagtcgtgcgtggtccaacacggccggcgggctgggctgcgaccttaaccagcaaggcacgccacgacccgccccgccctcgaggcataaataccctcccatcc

SEQ ID NO: 110 - DNA, 2634 bp, Setaria viridis
actgccgcgacacgcctcactggcgggagggctccgagcgctctctccccggcggccggcggagcagcgatctggattggagagaatagaggaaagagagggaaaaggagagagatagcgcaaagagctgaaaagataaggttgtgcgggctgtggtgattagaggaccactaatccctccatctcctaatgacgcggtgcccaagaccagtgccgcggcacaccagcgtctaagtgaacttccgctaaccttccggtcattgcgcctgaaagatgtcatgtggcgaggcccccctctcagtagattgccaactgcctaccgtgccactcttccatgcatgattgctcccgtctatcccgtttctcacaacagatagacaacagtaagcatcactaaagcaagcatgtgtagaaccttaaaaaaaggcttatactaccagtatactatcaaccagcatgccgtttttgaagtatccaggattagaagcttctactgcgcttttatattatagctgtggacctgtggtaacctttctcttttggcgcttgcttaatctcggccgtgctggtccatgcttaggcactaggcagagatagagccgggggtgaatggggctaaagctcagctgctcgaggggccgtgggctggtttccactagcctacagctgtgccacgtgcggccgcgcaagccgaagcaagcacgctgagccgttggacagcttgtcataatgccattacgtggattacaggtaactggccctgtaactactcgttcggccatcatcaaacgacgacgtccgctaggcgacgacacgggtaatgcacgcagccacccaggcgcgcgcgctagcggagcacggtcaggtgacacgggcgtcgtgacgcttccgagttgaaggggttaacgccagaaacagtgtttggccagggtatgaacataacaaaaaatattcacacgaaagaatggaagtatggagctgctactgtgtaaatgccaagcaggaaactcacgcccgctaacatccaacggccaacagctcgacgtgccggtcagcagagacatcggaacactggtgattggtggagccggcagtatgcgccccagcacggccgaggtggtggtggcccgtggccctgctgtctgcgcggctcgggacaacttgaaactgggccaccgcctcgtcgcaactcgcaacccgttggcggaagaaaggaatggctcgtaggggcccgggtagaatccaagaatgttgcgctgggcttcgattcacataacatgggcctgaagctctaaaacgacggcccggtcaccgggcgatggaaagagaccggatcctcctcgtgaattctggaaggccacacgagagcgacccaccaccgacgcggaggagtcgtgcgtggtccaacacggccggcgggctgggctgcgaccttaaccagcaaggcacgccacgacccgcctcgccctcgaggcataaataccctcccatcccgttgccgcaagactcagatcagattccgatccccagttcttccccaatcaccttgtggtctctcgtgtcgcggttcccagggacgcctccggctcgtcgctcgacagcgatctccgccccagcaaggtatagattcagttccttgctccgatcccaatctggttgagatgttgctccgatgcgacttgattatgtcatatatctgcggtttgcaccgatctgaagcctagggtttctcgagcgacccagttgtttgcaatttgcgatttgctcgtttgttgcgcatcgtagtttatgtttggagtaatcgaggatttgtatgcggcgtcggcgctacctgcttaatcacgccatgtgacgcggttacttgcagaggctgggttagtgggttctgttatgtcgtgatctaagaatctagattaggctcagtcgttcttgctgtcgactagtttgttttgatatccatgtagtacaagttacttaaaatttaggtccaatatattttgcatgcttttggcctgttattcttgccaacaagttgtcctggtaaaaagtagatgtgaaagtcacgtattgggacaaattgatggttaagtgctatagttctatagttctgtgatacatctatctgattttttttggtctattggtgcctaacttatctgaaaatcatggaacatgaggctagtttgatcatggtttagttcattgtgattaataatgtatgatttagtagctattttggtgatcgtgtcattttatttgtgaatggaatcattgtatgtaaatgaagctagttcaggggttatgatgtagctggctttgtattctaaaggctgctattattcatccatcgatttcacctatatgtaatccagagctttcgatgtgaaatttgtctgatccttcactaggaaggacagaacattgttaatattttggcacatctgtcttattctcatcctttgtttgaacatgttagcctgttcaaacagatactgttgtaatgtcctagttatataggtacatatgtgttctctattgagtttatggacttttgtgtgtgaagttatatttcattttgctcaaaactcatgtttgcaagctttctgacattattctattgttctgaaacaggtg

SEQ ID NO: 111 - DNA, 1493 bp, Setaria viridis
actgccgcgacacgcctcactggcgggagggctccgagcgctctctccccggcggccggcggagcagcgatctggattggagagaatagaggaaagagagggaaaaggagagagatagcgcaaagagctgaaaagataaggttgtgcgggctgtggtgattagaggaccactaatccctccatctcctaatgacgcggtgcccaagaccagtgccgcggcacaccagcgtctaagtgaacttccgctaaccttccggtcattgcgcctgaaagatgtcatgtggcgaggcccccctctcagtagattgccaactgcctaccgtgccactcttccatgcatgattgctcccgtctatcccgtttctcacaacagatagacaacagtaagcatcactaaagcaagcatgtgtagaaccttaaaaaaaggcttatactaccagtatactatcaaccagcatgccgtttttgaagtatccaggattagaagcttctactgcgcttttatattatagctgtggacctgtggtaacctttctcttttggcgcttgcttaatctcggccgtgctggtccatgcttaggcactaggcagagatagagccgggggtgaatggggctaaagctcagctgctcgaggggccgtgggctggtttccactagcctacagctgtgccacgtgcggccgcgcaagccgaagcaagcacgctgagccgttggacagcttgtcataatgccattacgtggattacaggtaactggccctgtaactactcgttcggccatcatcaaacgacgacgtccgctaggcgacgacacgggtaatgcacgcagccacccaggcgcgcgcgctagcggagcacggtcaggtgacacgggcgtcgtgacgcttccgagttgaaggggttaacgccagaaacagtgtttggccagggtatgaacataacaaaaaatattcacacgaaagaatggaagtatggagctgctactgtgtaaatgccaagcaggaaactcacgcccgctaacatccaacggccaacagctcgacgtgccggtcagcagagacatcggaacactggtgattggtggagccggcagtatgcgccccagcacggccgaggtggtggtggcccgtggccctgctgtctgcgcggctcgggacaacttgaaactgggccaccgcctcgtcgcaactcgcaacccgttggcggaagaaaggaatggctcgtaggggcccgggtagaatccaagaatgttgcgctgggcttcgattcacataacatgggcctgaagctctaaaacgacggcccggtcaccgggcgatggaaagagaccggatcctcctcgtgaattctggaaggccacacgagagcgacccaccaccgacgcggaggagtcgtgcgtggtccaacacggccggcgggctgggctgcgaccttaaccagcaaggcacgccacgacccgcctcgccctcgaggcataaataccctcccatcc

SEQ ID NO: 112 - DNA, 127 bp, Setaria viridis; identical to SEQ ID NO: 101

SEQ ID NO: 113 - DNA, 1014 bp, Setaria viridis
gtatagattcagttccttgctccgatcccaatctggttgagatgttgctccgatgcgacttgattatgtcatatatctgcggtttgcaccgatctgaagcctagggtttctcgagcgacccagttgtttgcaatttgcgatttgctcgtttgttgcgcatcgtagtttatgtttggagtaatcgaggatttgtatgcggcgtcggcgctacctgcttaatcacgccatgtgacgcggttacttgcagaggctgggttagtgggttctgttatgtcgtgatctaagaatctagattaggctcagtcgttcttgctgtcgactagtttgttttgatatccatgtagtacaagttacttaaaatttaggtccaatatattttgcatgcttttggcctgttattcttgccaacaagttgtcctggtaaaaagtagatgtgaaagtcacgtattgggacaaattgatggttaagtgctatagttctatagttctgtgatacatctatctgattttttttggtctattggtgcctaacttatctgaaaatcatggaacatgaggctagtttgatcatggtttagttcattgtgattaataatgtatgatttagtagctattttggtgatcgtgtcattttatttgtgaatggaatcattgtatgtaaatgaagctagttcaggggttatgatgtagctggctttgtattctaaaggctgctattattcatccatcgatttcacctatatgtaatccagagctttcgatgtgaaatttgtctgatccttcactaggaaggacagaacattgttaatattttggcacatctgtcttattctcatcctttgtttgaacatgttagcctgttcaaacagatactgttgtaatgtcctagttatataggtacatatgtgttctctattgagtttatggacttttgtgtgtgaagttatatttcattttgctcaaaactcatgtttgcaagctttctgacattattctattgttctgaaacaggtg

SEQ ID NO: 114 - DNA, 2634 bp, Setaria viridis
actgccgcgacacgcctcactggcgggagggctccgagcgctctctccccggcggccggcggagcagcgatctggattggagagaatagaggaaagagagggaaaaggagagagatagcgcaaagagctgaaaagataaggttgtgcgggctgtggtgattagaggaccactaatccctccatctcctaatgacgcggtgcccaagaccagtgccgcggcacaccagcgtctaagtgaacttccgctaaccttccggtcattgcgcctgaaagatgtcatgtggcgaggcccccctctcagtagattgccaactgcctaccgtgccactcttccatgcatgattgctcccgtctatcccgtttctcacaacagatagacaacagtaagcatcactaaagcaagcatgtgtagaaccttaaaaaaaggcttatactaccagtatactatcaaccagcatgccgtttttgaagtatccaggattagaagcttctactgcgcttttatattatagctgtggacctgtggtaacctttctcttttggcgcttgcttaatctcggccgtgctggtccatgcttaggcactaggcagagatagagccgggggtgaatggggctaaagctcagctgctcgaggggccgtgggctggtttccactagcctacagctgtgccacgtgcggccgcgcaagccgaagcaagcacgctgagccgttggacagcttgtcataatgccattacgtggattacaggtaactggccctgtaactactcgttcggccatcatcaaacgacgacgtccgctaggcgacgacacgggtaatgcacgcagccacccaggcgcgcgcgctagcggagcacggtcaggtgacacgggcgtcgtgacgcttccgagttgaaggggttaacgccagaaacagtgtttggccagggtatgaacataacaaaaaatattcacacgaaagaatggaagtatggagctgctactgtgtaaatgccaagcaggaaactcacgcccgctaacatccaacggccaacagctcgacgtgccggtcagcagagacatcggaacactggtgattggtggagccggcagtatgcgccccagcacggccgaggtggtggtggcccgtggccctgctgtctgcgcggctcgggacaacttgaaactgggccaccgcctcgtcgcaactcgcaacccgttggcggaagaaaggaatggctcgtaggggcccgggtagaatccaagaatgttgcgctgggcttcgattcacataacatgggcctgaagctctaaaacgacggcccggtcaccgggcgatggaaagagaccggatcctcctcgtgaattctggaaggccacacgagagcgacccaccaccgacgcggaggagtcgtgcgtggtccaacacggccggcgggctgggctgcgaccttaaccagcaaggcacgccacgacccgcctcgccctcgaggcataaataccctcccatcccgttgccgcaagactcagatcagattccgatccccagttcttccccaatcaccttgtggtctctcgtgtcgcggttcccagggacgcctccggctcgtcgctcgacagcgatctccgccccagcaaggtatagattcagttccttgctccgatcccaatctggttgagatgttgctccgatgcgacttgattatgtcatatatctgcggtttgcaccgatctgaagcctagggtttctcgagcgacccagttgtttgcaatttgcgatttgctcgtttgttgcgcatcgtagtttatgtttggagtaatcgaggatttgtatgcggcgtcggcgctacctgcttaatcacgccatgtgacgcggttacttgcagaggctgggttagtgggttctgttatgtcgtgatctaagaatctagattaggctcagtcgttcttgctgtcgactagtttgttttgatatccatgtagtacaagttacttaaaatttaggtccaatatattttgcatgcttttggcctgttattcttgccaacaagttgtcctggtaaaaagtagatgtgaaagtcacgtattgggacaaattgatggttaagtgctatagttctatagttctgtgatacatctatctgattttttttggtctattggtgcctaacttatctgaaaatcatggaacatgaggctagtttgatcatggtttagttcattgtgattaataatgtatgatttagtagctattttggtgatcgtgtcattttatttgtgaatggaatcattgtatgtaaatgaagctagttcaggggttatgatgtagctggctttgtattctaaaggctgctattattcatccatcgatttcacctatatgtaatccagagctttcgatgtgaaatttgtctgatccttcactaggaaggacagaacattgttaatattttggcacatctgtcttattctcatcctttgtttgaacatgttagcctgttcaaacagatactgttgtaatgtcctagttatataggtacatatgtgttctctattgagtttatggacttttgtgtgtgaagttatatttcattttgctcaaaactcatgtttgcaagctttctgacattattctattgttctgaaacagggt

SEQ ID NO: 115 - DNA, 1014 bp, Setaria viridis
gtatagattcagttccttgctccgatcccaatctggttgagatgttgctccgatgcgacttgattatgtcatatatctgcggtttgcaccgatctgaagcctagggtttctcgagcgacccagttgtttgcaatttgcgatttgctcgtttgttgcgcatcgtagtttatgtttggagtaatcgaggatttgtatgcggcgtcggcgctacctgcttaatcacgccatgtgacgcggttacttgcagaggctgggttagtgggttctgttatgtcgtgatctaagaatctagattaggctcagtcgttcttgctgtcgactagtttgttttgatatccatgtagtacaagttacttaaaatttaggtccaatatattttgcatgcttttggcctgttattcttgccaacaagttgtcctggtaaaaagtagatgtgaaagtcacgtattgggacaaattgatggttaagtgctatagttctatagttctgtgatacatctatctgattttttttggtctattggtgcctaacttatctgaaaatcatggaacatgaggctagtttgatcatggtttagttcattgtgattaataatgtatgatttagtagctattttggtgatcgtgtcattttatttgtgaatggaatcattgtatgtaaatgaagctagttcaggggttatgatgtagctggctttgtattctaaaggctgctattattcatccatcgatttcacctatatgtaatccagagctttcgatgtgaaatttgtctgatccttcactaggaaggacagaacattgttaatattttggcacatctgtcttattctcatcctttgtttgaacatgttagcctgttcaaacagatactgttgtaatgtcctagttatataggtacatatgtgttctctattgagtttatggacttttgtgtgtgaagttatatttcattttgctcaaaactcatgtttgcaagctttctgacattattctattgttctgaaacagggt

SEQ ID NO: 116 - DNA, 2176 bp, Setaria viridis
gccgtttttgaagtatccaggattagaagcttctactgcgcttttatattatagctgtggacctgtggtaacctttctcttttggcgcttgcttaatctcggccgtgctggtccatgcttaggcactaggcagagatagagccgggggtgaatggggctaaagctcagctgctcgaggggccgtgggctggtttccactagcctacagctgtgccacgtgcggccgcgcaagccgaagcaagcacgctgagccgttggacagcttgtcataatgccattacgtggattacaggtaactggccctgtaactactcgttcggccatcatcaaacgacgacgtccgctaggcgacgacacgggtaatgcacgcagccacccaggcgcgcgcgctagcggagcacggtcaggtgacacgggcgtcgtgacgcttccgagttgaaggggttaacgccagaaacagtgtttggccagggtatgaacataacaaaaaatattcacacgaaagaatggaagtatggagctgctactgtgtaaatgccaagcaggaaactcacgcccgctaacatccaacggccaacagctcgacgtgccggtcagcagagacatcggaacactggtgattggtggagccggcagtatgcgccccagcacggccgaggtggtggtggcccgtggccctgctgtctgcgcggctcgggacaacttgaaactgggccaccgcctcgtcgcaactcgcaacccgttggcggaagaaaggaatggctcgtaggggcccgggtagaatccaagaatgttgcgctgggcttcgattcacataacatgggcctgaagctctaaaacgacggcccggtcaccgggcgatggaaagagaccggatcctcctcgtgaattctggaaggccacacgagagcgacccaccaccgacgcggaggagtcgtgcgtggtccaacacggccggcgggctgggctgcgaccttaaccagcaaggcacgccacgacccgcctcgccctcgaggcataaataccctcccatcccgttgccgcaagactcagatcagattccgatccccagttcttccccaatcaccttgtggtctctcgtgtcgcggttcccagggacgcctccggctcgtcgctcgacagcgatctccgccccagcaaggtatagattcagttccttgctccgatcccaatctggttgagatgttgctccgatgcgacttgattatgtcatatatctgcggtttgcaccgatctgaagcctagggtttctcgagcgacccagttgtttgcaatttgcgatttgctcgtttgttgcgcatcgtagtttatgtttggagtaatcgaggatttgtatgcggcgtcggcgctacctgcttaatcacgccatgtgacgcggttacttgcagaggctgggttagtgggttctgttatgtcgtgatctaagaatctagattaggctcagtcgttcttgctgtcgactagtttgttttgatatccatgtagtacaagttacttaaaatttaggtccaatatattttgcatgcttttggcctgttattcttgccaacaagttgtcctggtaaaaagtagatgtgaaagtcacgtattgggacaaattgatggttaagtgctatagttctatagttctgtgatacatctatctgattttttttggtctattggtgcctaacttatctgaaaatcatggaacatgaggctagtttgatcatggtttagttcattgtgattaataatgtatgatttagtagctattttggtgatcgtgtcattttatttgtgaatggaatcattgtatgtaaatgaagctagttcaggggttatgatgtagctggctttgtattctaaaggctgctattattcatccatcgatttcacctatatgtaatccagagctttcgatgtgaaatttgtctgatccttcactaggaaggacagaacattgttaatattttggcacatctgtcttattctcatcctttgtttgaacatgttagcctgttcaaacagatactgttgtaatgtcctagttatataggtacatatgtgttctctattgagtttatggacttttgtgtgtgaagttatatttcattttgctcaaaactcatgtttgcaagctttctgacattattctattgttctgaaacaggtg

SEQ ID NO: 117 - DNA, 1035 bp, Setaria viridis
gccgtttttgaagtatccaggattagaagcttctactgcgcttttatattatagctgtggacctgtggtaacctttctcttttggcgcttgcttaatctcggccgtgctggtccatgcttaggcactaggcagagatagagccgggggtgaatggggctaaagctcagctgctcgaggggccgtgggctggtttccactagcctacagctgtgccacgtgcggccgcgcaagccgaagcaagcacgctgagccgttggacagcttgtcataatgccattacgtggattacaggtaactggccctgtaactactcgttcggccatcatcaaacgacgacgtccgctaggcgacgacacgggtaatgcacgcagccacccaggcgcgcgcgctagcggagcacggtcaggtgacacgggcgtcgtgacgcttccgagttgaaggggttaacgccagaaacagtgtttggccagggtatgaacataacaaaaaatattcacacgaaagaatggaagtatggagctgctactgtgtaaatgccaagcaggaaactcacgcccgctaacatccaacggccaacagctcgacgtgccggtcagcagagacatcggaacactggtgattggtggagccggcagtatgcgccccagcacggccgaggtggtggtggcccgtggccctgctgtctgcgcggctcgggacaacttgaaactgggccaccgcctcgtcgcaactcgcaacccgttggcggaagaaaggaatggctcgtaggggcccgggtagaatccaagaatgttgcgctgggcttcgattcacataacatgggcctgaagctctaaaacgacggcccggtcaccgggcgatggaaagagaccggatcctcctcgtgaattctggaaggccacacgagagcgacccaccaccgacgcggaggagtcgtgcgtggtccaacacggccggcgggctgggctgcgaccttaaccagcaaggcacgccacgacccgcctcgccctcgaggcataaataccctcccatcc

SEQ ID NO: 118 - DNA, 1822 bp, Setaria viridis
cacgggtaatgcacgcagccacccaggcgcgcgcgctagcggagcacggtcaggtgacacgggcgtcgtgacgcttccgagttgaaggggttaacgccagaaacagtgtttggccagggtatgaacataacaaaaaatattcacacgaaagaatggaagtatggagctgctactgtgtaaatgccaagcaggaaactcacgcccgctaacatccaacggccaacagctcgacgtgccggtcagcagagacatcggaacactggtgattggtggagccggcagtatgcgccccagcacggccgaggtggtggtggcccgtggccctgctgtctgcgcggctcgggacaacttgaaactgggccaccgcctcgtcgcaactcgcaacccgttggcggaagaaaggaatggctcgtaggggcccgggtagaatccaagaatgttgcgctgggcttcgattcacataacatgggcctgaagctctaaaacgacggcccggtcaccgggcgatggaaagagaccggatcctcctcgtgaattctggaaggccacacgagagcgacccaccaccgacgcggaggagtcgtgcgtggtccaacacggccggcgggctgggctgcgaccttaaccagcaaggcacgccacgacccgcctcgccctcgaggcataaataccctcccatcccgttgccgcaagactcagatcagattccgatccccagttcttccccaatcaccttgtggtctctcgtgtcgcggttcccagggacgcctccggctcgtcgctcgacagcgatctccgccccagcaaggtatagattcagttccttgctccgatcccaatctggttgagatgttgctccgatgcgacttgattatgtcatatatctgcggtttgcaccgatctgaagcctagggtttctcgagcgacccagttgtttgcaatttgcgatttgctcgtttgttgcgcatcgtagtttatgtttggagtaatcgaggatttgtatgcggcgtcggcgctacctgcttaatcacgccatgtgacgcggttacttgcagaggctgggttagtgggttctgttatgtcgtgatctaagaatctagattaggctcagtcgttcttgctgtcgactagtttgttttgatatccatgtagtacaagttacttaaaatttaggtccaatatattttgcatgcttttggcctgttattcttgccaacaagttgtcctggtaaaaagtagatgtgaaagtcacgtattgggacaaattgatggttaagtgctatagttctatagttctgtgatacatctatctgattttttttggtctattggtgcctaacttatctgaaaatcatggaacatgaggctagtttgatcatggtttagttcattgtgattaataatgtatgatttagtagctattttggtgatcgtgtcattttatttgtgaatggaatcattgtatgtaaatgaagctagttcaggggttatgatgtagctggctttgtattctaaaggctgctattattcatccatcgatttcacctatatgtaatccagagctttcgatgtgaaatttgtctgatccttcactaggaaggacagaacattgttaatattttggcacatctgtcttattctcatcctttgtttgaacatgttagcctgttcaaacagatactgttgtaatgtcctagttatataggtacatatgtgttctctattgagtttatggacttttgtgtgtgaagttatatttcattttgctcaaaactcatgtttgcaagctttctgacattattctattgttctgaaacaggtg

SEQ ID NO: 119 - DNA, 681 bp, Setaria viridis
cacgggtaatgcacgcagccacccaggcgcgcgcgctagcggagcacggtcaggtgacacgggcgtcgtgacgcttccgagttgaaggggttaacgccagaaacagtgtttggccagggtatgaacataacaaaaaatattcacacgaaagaatggaagtatggagctgctactgtgtaaatgccaagcaggaaactcacgcccgctaacatccaacggccaacagctcgacgtgccggtcagcagagacatcggaacactggtgattggtggagccggcagtatgcgccccagcacggccgaggtggtggtggcccgtggccctgctgtctgcgcggctcgggacaacttgaaactgggccaccgcctcgtcgcaactcgcaacccgttggcggaagaaaggaatggctcgtaggggcccgggtagaatccaagaatgttgcgctgggcttcgattcacataacatgggcctgaagctctaaaacgacggcccggtcaccgggcgatggaaagagaccggatcctcctcgtgaattctggaaggccacacgagagcgacccaccaccgacgcggaggagtcgtgcgtggtccaacacggccggcgggctgggctgcgaccttaaccagcaaggcacgccacgacccgcctcgccctcgaggcataaataccctcccatcc

SEQ ID NO: 120 - DNA, 1822 bp, Setaria viridis
cacgggtaatgcacgcagccacccaggcgcgcgcgctagcggagcacggtcaggtgacacgggcgtcgtgacgcttccgagttgaaggggttaacgccagaaacagtgtttggccagggtatgaacataacaaaaaatattcacacgaaagaatggaagtatggagctgctactgtgtaaatgccaagcaggaaactcacgcccgctaacatccaacggccaacagctcgacgtgccggtcagcagagacatcggaacactggtgattggtggagccggcagtatgcgccccagcacggccgaggtggtggtggcccgtggccctgctgtctgcgcggctcgggacaacttgaaactgggccaccgcctcgtcgcaactcgcaacccgttggcggaagaaaggaatggctcgtaggggcccgggtagaatccaagaatgttgcgctgggcttcgattcacataacatgggcctgaagctctaaaacgacggcccggtcaccgggcgatggaaagagaccggatcctccttgtgaattctggaaggccacacgagagcgacccaccaccgacgcggaggagtcgtgcgtggtccaacacggccggcgggctgggctgcgaccttaaccagcaaggcacgccacgacccgcctcgccctcgaggcataaataccctcccatcccgttgccgcaagactcagatcagattccgatccccagttcttccccaatcaccttgtggtctctcgtgtcgcggttcccagggacgcctccggctcgtcgctcgacagcgatctccgccccagcaaggtatagattcagttccttgctccgatcccaatctggttgagatgttgctccgatgcgacttgattatgtcatatatctgcggtttgcaccgatctgaagcctagggtttctcgagcgacccagttgtttgcaatttgcgatttgctcgtttgttgcgcatcgtagtttatgtttggagtaatcgaggatttgtatgcggcgtcggcgctacctgcttaatcacgccatgtgacgcggttacttgcagaggctgggttagtgggttctgttatgtcgtgatctaagaatctagattaggctcagtcgttcttgctgtcgactagtttgttttgatatccatgtagtacaagttacttaaaatttaggtccaatatattttgcatgcttttggcctgttattcttgccaacaagttgtcctggtaaaaagtagatgtgaaagtcacgtattgggacaaattgatggttaagtgctatagttctatagttctgtgatacatctatctgattttttttggtctattggtgcctaacttatctgaaaatcatggaacatgaggctagtttgatcatggtttagttcattgtgattaataatgtatgatttagtagctattttggtgatcgtgtcattttatttgtgaatggaatcattgtatgtaaatgaagctagttcaggggttatgatgtagctggctttgtattctaaaggctgctattattcatccatcgatttcacctatatgtaatccagagctttcgatgtgaaatttgtctgatccttcactaggaaggacagaacattgttaatattttggcacatctgtcttattctcatcctttgtttgaacatgttagcctgttcaaacagatactgttgtaatgtcctagttatataggtacatatgtgttctctattgagtttatggacttttgtgtgtgaagttatatttcattttgctcaaaactcatgtttgcaagctttctgacattattctattgttctgaaacagggt

SEQ ID NO: 121 - DNA, 681 bp, Setaria viridis
cacgggtaatgcacgcagccacccaggcgcgcgcgctagcggagcacggtcaggtgacacgggcgtcgtgacgcttccgagttgaaggggttaacgccagaaacagtgtttggccagggtatgaacataacaaaaaatattcacacgaaagaatggaagtatggagctgctactgtgtaaatgccaagcaggaaactcacgcccgctaacatccaacggccaacagctcgacgtgccggtcagcagagacatcggaacactggtgattggtggagccggcagtatgcgccccagcacggccgaggtggtggtggcccgtggccctgctgtctgcgcggctcgggacaacttgaaactgggccaccgcctcgtcgcaactcgcaacccgttggcggaagaaaggaatggctcgtaggggcccgggtagaatccaagaatgttgcgctgggcttcgattcacataacatgggcctgaagctctaaaacgacggcccggtcaccgggcgatggaaagagaccggatcctccttgtgaattctggaaggccacacgagagcgacccaccaccgacgcggaggagtcgtgcgtggtccaacacggccggcgggctgggctgcgaccttaaccagcaaggcacgccacgacccgcctcgccctcgaggcataaataccctcccatcc

SEQ ID NO: 122 - DNA, 1925 bp, Zea mays subsp. Mexicana
gtcgtgcccctctctagagataatgagcattgcatgtctaagttataaaaaattaccacatatttttttttgtcacacttgtgtttgaagtgcagtttatctatctctatacatatatttaaacttcactatatgaataatatagtctatagtattaaaataatatcaatgttttagatgattatataactgaactgctagacatggtctaaaggacaaccgagtattttgacaacatgactctacagttttatctttttagtgtgcatgtgttctttttacttttgcaaatagcttcacctatataatacttcatccattttattagtacatccatttactaaatttttagtacatctattttattctattttagcctctaaattaagaaaacttaaactctattttagttttttatttaataatttagatataaaatagaataaaataaagtgactaaaaaataactaaataccttttaagaaataaaaaaactaaggaaccatttttcttgttccgagtagataatgacagcctgttcaacgccgtcgacgagtctaacggacaccaaccagcgaaccagcagcgtcgcgtcgggccaagcgaagcagacggcacggcatctctgtagctgcctctggacccctctcgagagttccgctccaccgttggacttgctccgctgtcggcatccagaaattgcgtggcggagcggcagacgtgagccggcacggcaggcggcctcctctcacggcaccggcagctacgggggattcctttcccaccgctccttcgctttcccttcctcgcccgccgtaataaatagaccccctccacaccctctttccccaacctcgtgttcgttcggagcgcgcacacacacaaccagatctcccccaaatccacccgtcggcacctccgcttcaaggtacgccgctcatcctcctcccccccctctctctaccttctctagatcggcgtttcggtccatggttagggcccggtagttctacttctgttcatgtttgtgttagatccgtgtttgtgttagatccgtgctgctagatttcgtacacggatgcgacctgtacatcagacatgttctgattgctaacttgccagtgtttctctttggggaatcctgggatggctctagccgttccgcagacgggatcgatttcatgaattttttttgtttcgttgcatagggtttggtttgcccttttcctttatttcaatatatgccgtgcacttgtttgtcgggtcatcttttcatgttttttttggcttggttgtgatgatgtggtctggttgggcggtcgttctagatcggagtagaatactgtttcaaactacctggtggatttattaaaggatctgtatgtatgtgccatacatcttcatagttacgagtttaagatgatggatggaaatatcgatctaggataggtatacatgttgatgcgggttttactgatgcatatacagagatgcttttttttcgcttggttgtgatgatgtggtctggtcgggcggtcgttctagatcggagtagaatactgtttcaaactacctggtggatttattaattttggatctgtatgtgtgtcatacatcttcatagttacgagtttaagatcgatggaaatatcgatctaggataggtatacatgttgatgtgggttttactgatgcatatacatggcatatgcagcatctattcatatgctctaaccttgagtacctatctattataataaacaagtatgttttataattattttgatcttgatatacttggatgatggcatatgcagcagctatatgtggatttttttagccctgccttcatacgctatttatttgcttggtactgtttcttttgtcgatgctcaccctgttgtttggtgatacttctgcaggtc

SEQ ID NO: 123 - DNA, 850 bp, Zea mays subsp. Mexicana
gtcgtgcccctctctagagataatgagcattgcatgtctaagttataaaaaattaccacatatttttttttgtcacacttgtgtttgaagtgcagtttatctatctctatacatatatttaaacttcactatatgaataatatagtctatagtattaaaataatatcaatgttttagatgattatataactgaactgctagacatggtctaaaggacaaccgagtattttgacaacatgactctacagttttatctttttagtgtgcatgtgttctttttacttttgcaaatagcttcacctatataatacttcatccattttattagtacatccatttactaaatttttagtacatctattttattctattttagcctctaaattaagaaaacttaaactctattttagttttttatttaataatttagatataaaatagaataaaataaagtgactaaaaaataactaaataccttttaagaaataaaaaaactaaggaaccatttttcttgttccgagtagataatgacagcctgttcaacgccgtcgacgagtctaacggacaccaaccagcgaaccagcagcgtcgcgtcgggccaagcgaagcagacggcacggcatctctgtagctgcctctggacccctctcgagagttccgctccaccgttggacttgctccgctgtcggcatccagaaattgcgtggcggagcggcagacgtgagccggcacggcaggcggcctcctctcacggcaccggcagctacgggggattcctttcccaccgctccttcgctttcccttcctcgcccgccgtaataaatagaccccctccacaccctctttcccc

SEQ ID NO: 124 - DNA, 78 bp, Zea mays subsp. Mexicana
aacctcgtgttcgttcggagcgcgcacacacacaaccagatctcccccaaatccacccgtcggcacctccgcttcaag

SEQ ID NO: 125 - DNA, 997 bp, Zea mays subsp. Mexicana
gtacgccgctcatcctcctcccccccctctctctaccttctctagatcggcgtttcggtccatggttagggcccggtagttctacttctgttcatgtttgtgttagatccgtgtttgtgttagatccgtgctgctagatttcgtacacggatgcgacctgtacatcagacatgttctgattgctaacttgccagtgtttctctttggggaatcctgggatggctctagccgttccgcagacgggatcgatttcatgaattttttttgtttcgttgcatagggtttggtttgcccttttcctttatttcaatatatgccgtgcacttgtttgtcgggtcatcttttcatgttttttttggcttggttgtgatgatgtggtctggttgggcggtcgttctagatcggagtagaatactgtttcaaactacctggtggatttattaaaggatctgtatgtatgtgccatacatcttcatagttacgagtttaagatgatggatggaaatatcgatctaggataggtatacatgttgatgcgggttttactgatgcatatacagagatgcttttttttcgcttggttgtgatgatgtggtctggtcgggcggtcgttctagatcggagtagaatactgtttcaaactacctggtggatttattaattttggatctgtatgtgtgtcatacatcttcatagttacgagtttaagatcgatggaaatatcgatctaggataggtatacatgttgatgtgggttttactgatgcatatacatggcatatgcagcatctattcatatgctctaaccttgagtacctatctattataataaacaagtatgttttataattattttgatcttgatatacttggatgatggcatatgcagcagctatatgtggatttttttagccctgccttcatacgctatttatttgcttggtactgtttcttttgtcgatgctcaccctgttgtttggtgatacttctgcaggtc

SEQ ID NO: 126 - DNA, 1925 bp, Zea mays subsp. Mexicana
gtcgtgcccctctctagagataatgagcattgcatgtctaagttataaaaaattaccacatatttttttttgtcacacttgtgtttgaagtgcagtttatctatctctatacatatatttaaacttcactatatgaataatatagtctatagtattaaaataatatcaatgttttagatgattatataactgaactgctagacatggtctaaaggacaaccgagtattttgacaacatgactctacagttttatctttttagtgtgcatgtgttctttttacttttgcaaatagcttcacctatataatacttcatccattttattagtacatccatttactaaatttttagtacatctattttattctattttagcctctaaattaagaaaacttaaactctattttagttttttatttaataatttagatataaaatagaataaaataaagtgactaaaaaataactaaataccttttaagaaataaaaaaactaaggaaccatttttcttgttccgagtagataatgacagcctgttcaacgccgtcgacgagtctaacggacaccaaccagcgaaccagcagcgtcgcgtcgggccaagcgaagcagacggcacggcatctctgtagctgcctctggacccctctcgagagttccgctccaccgttggacttgctccgctgtcggcatccagaaattgcgtggcggagcggcagacgtgagccggcacggcaggcggcctcctctcacggcaccggcagctacgggggattcctttcccaccgctccttcgctttcccttcctcgcccgccgtaataaatagaccccctccacaccctctttccccaacctcgtgttcgttcggagcgcgcacacacacaaccagatctcccccaaatccacccgtcggcacctccgcttcaaggtacgccgctcatcctcctcccccccctctctctaccttctctagatcggcgtttcggtccatggttagggcccggtagttctacttctgttcatgtttgtgttagatccgtgtttgtgttagatccgtgctgctagatttcgtacacggatgcgacctgtacatcagacatgttctgattgctaacttgccagtgtttctctttggggaatcctgggatggctctagccgttccgcagacgggatcgatttcatgaattttttttgtttcgttgcatagggtttggtttgcccttttcctttatttcaatatatgccgtgcacttgtttgtcgggtcatcttttcatgttttttttggcttggttgtgatgatgtggtctggttgggcggtcgttctagatcggagtagaatactgtttcaaactacctggtggatttattaaaggatctgtatgtatgtgccatacatcttcatagttacgagtttaagatgatggatggaaatatcgatctaggataggtatacatgttgatgcgggttttactgatgcatatacagagatgcttttttttcgcttggttgtgatgatgtggtctggtcgggcggtcgttctagatcggagtagaatactgtttcaaactacctggtggatttattaattttggatctgtatgtgtgtcatacatcttcatagttacgagtttaagatcgatggaaatatcgatctaggataggtatacatgttgatgtgggttttactgatgcatatacatggcatatgcagcatctattcatatgctctaaccttgagtacctatctattataataaacaagtatgttttataattattttgatcttgatatacttggatgatggcatatgcagcagctatatgtggatttttttagccctgccttcatacgctatttatttgcttggtactgtttcttttgtcgatgctcaccctgttgtttggtgatacttctgcagggt

SEQ ID NO: 127 - DNA, 997 bp, Zea mays subsp. Mexicana
gtacgccgctcatcctcctcccccccctctctctaccttctctagatcggcgtttcggtccatggttagggcccggtagttctacttctgttcatgtttgtgttagatccgtgtttgtgttagatccgtgctgctagatttcgtacacggatgcgacctgtacatcagacatgttctgattgctaacttgccagtgtttctctttggggaatcctgggatggctctagccgttccgcagacgggatcgatttcatgaattttttttgtttcgttgcatagggtttggtttgcccttttcctttatttcaatatatgccgtgcacttgtttgtcgggtcatcttttcatgttttttttggcttggttgtgatgatgtggtctggttgggcggtcgttctagatcggagtagaatactgtttcaaactacctggtggatttattaaaggatctgtatgtatgtgccatacatcttcatagttacgagtttaagatgatggatggaaatatcgatctaggataggtatacatgttgatgcgggttttactgatgcatatacagagatgcttttttttcgcttggttgtgatgatgtggtctggtcgggcggtcgttctagatcggagtagaatactgtttcaaactacctggtggatttattaattttggatctgtatgtgtgtcatacatcttcatagttacgagtttaagatcgatggaaatatcgatctaggataggtatacatgttgatgtgggttttactgatgcatatacatggcatatgcagcatctattcatatgctctaaccttgagtacctatctattataataaacaagtatgttttataattattttgatcttgatatacttggatgatggcatatgcagcagctatatgtggatttttttagccctgccttcatacgctatttatttgcttggtactgtttcttttgtcgatgctcaccctgttgtttggtgatacttctgcagggt

SEQ ID NO: 128 - DNA, 1974 bp, Zea mays subsp. Mexicana
gtcgtgcccctctctagagataaagagcattgcatgtctaagttataaaaaattaccacatattttttttgtcacacttgtttgaagtgcagtttatctatctttatacatatatttaaactttactctacgaataatataatctatagtactacaataatatcagtgttttagagaatcatataaatgaacagttagacatggtctaaaggacaattgagtattttgacaacaggactctacagttttatctttttagtgtgcatgtgttctccttttttttttgcaaatagcttcacctatataatacttcatccattttattagtacatccatttagggtttagggttaatggtttttatagactaatttttttagtacatctattttattctattttagcctctaaattaagaaaactaaaactctattttagtttttttatttaataatttagatataaaatagaataaaataaagtgactaaaaattaaacaaataccctttaagaaattaaaaaaactaaggaaacatttttcttgtttcgagtagataatgccagcctgttaaacgccgtcgacgagtctaacggacaccaaccagcgaaccagcagcgtcgcgtcgggccaagcgaagcagacggcacggcatctctgtcgctgcctctggacccctctcgagagttccgctccaccgttggacttgctccgctgtcggcatccagaaattgcgtggcggagcggcagacgtgagccggcacggcaggcggcctcctcctcctctcacggcaccggcagctacgggggattcctttcccaccgctccttcgctttcccttcctcgcccgccgtaataaatagacaccccctccacaccttctttccccaacctcgtgttgttcggagcgcacacacacacaaccagatctcccccaaatccacccgtcggcacctccgcttcaaggtacgccgctcatcctcccccccccctctctaccttctctagatcggcgttccggtccatggttagggcccggtagttctacttctgttcatgtttgtgttagatccgtgtttgtgttagatccgtgctgctagcgttcgtacacggatgcgacctgtacgtcagacacgttctgattgctaacttgccagtgtttctctttggggaatcctgggatggctctagccgttccgcagacgggatcgatttcatgattttttttgtttcgttgcatagggtttggtttgcccttttcctttatttcaatatatgccgtgcacttgtttgtcgggtcatcttttcatgcttttttttgtcttggttgtgatgatgtggtctggttgggcggtcgttctagatcggagaagaattctgtttcaaactacctggtggatttattaattttggatctgtatgtgtgtgccatacatattcatagttacgaattgaagatgatggatggaaatatcgatctaggataggtatacatgttgatgcgggttttactgatgcatatacagagatgctttttgttcgcttggttgtgatgatgtggtctggttgggcggtcgttcattcgttctagatcggagtagaatactgtttcaaactacctggtgtatttattaattttggaactgtatgtgtgtgtcatacatcttcatagttacgagtttaagatggatggaaatatcgatctaggataggtatacatgttgatgtgggttttactgatgcatatacatgatggcatatgcagcatctattcatatgctctaaccttgagtacctatctattataataaacaagtatgttttataattattttgatcttgatatacttggatgatggcatatgcagcagctatatgtggatttttttagccctgccttcatacgctatttatttgcttggtactgtttcttttgtcgatgctcaccctgttgtttggtgatacttctgcaggtc

SEQ ID NO: 129 - DNA, 887 bp, Zea mays subsp. Mexicana
gtcgtgcccctctctagagataaagagcattgcatgtctaagttataaaaaattaccacatattttttttgtcacacttgtttgaagtgcagtttatctatctttatacatatatttaaactttactctacgaataatataatctatagtactacaataatatcagtgttttagagaatcatataaatgaacagttagacatggtctaaaggacaattgagtattttgacaacaggactctacagttttatctttttagtgtgcatgtgttctccttttttttttgcaaatagcttcacctatataatacttcatccattttattagtacatccatttagggtttagggttaatggtttttatagactaatttttttagtacatctattttattctattttagcctctaaattaagaaaactaaaactctattttagtttttttatttaataatttagatataaaatagaataaaataaagtgactaaaaattaaacaaataccctttaagaaattaaaaaaactaaggaaacatttttcttgtttcgagtagataatgccagcctgttaaacgccgtcgacgagtctaacggacaccaaccagcgaaccagcagcgtcgcgtcgggccaagcgaagcagacggcacggcatctctgtcgctgcctctggacccctctcgagagttccgctccaccgttggacttgctccgctgtcggcatccagaaattgcgtggcggagcggcagacgtgagccggcacggcaggcggcctcctcctcctctcacggcaccggcagctacgggggattcctttcccaccgctccttcgctttcccttcctcgcccgccgtaataaatagacaccccctccacaccttctttcccc

SEQ ID NO: 130 - DNA, 77 bp, Zea mays subsp. Mexicana
aacctcgtgttgttcggagcgcacacacacacaaccagatctcccccaaatccacccgtcggcacctccgcttcaag

SEQ ID NO: 131 - DNA, 1010 bp, Zea mays subsp. Mexicana
gtacgccgctcatcctcccccccccctctctaccttctctagatcggcgttccggtccatggttagggcccggtagttctacttctgttcatgtttgtgttagatccgtgtttgtgttagatccgtgctgctagcgttcgtacacggatgcgacctgtacgtcagacacgttctgattgctaacttgccagtgtttctctttggggaatcctgggatggctctagccgttccgcagacgggatcgatttcatgattttttttgtttcgttgcatagggtttggtttgcccttttcctttatttcaatatatgccgtgcacttgtttgtcgggtcatcttttcatgcttttttttgtcttggttgtgatgatgtggtctggttgggcggtcgttctagatcggagaagaattctgtttcaaactacctggtggatttattaattttggatctgtatgtgtgtgccatacatattcatagttacgaattgaagatgatggatggaaatatcgatctaggataggtatacatgttgatgcgggttttactgatgcatatacagagatgctttttgttcgcttggttgtgatgatgtggtctggttgggcggtcgttcattcgttctagatcggagtagaatactgtttcaaactacctggtgtatttattaattttggaactgtatgtgtgtgtcatacatcttcatagttacgagtttaagatggatggaaatatcgatctaggataggtatacatgttgatgtgggttttactgatgcatatacatgatggcatatgcagcatctattcatatgctctaaccttgagtacctatctattataataaacaagtatgttttataattattttgatcttgatatacttggatgatggcatatgcagcagctatatgtggatttttttagccctgccttcatacgctatttatttgcttggtactgtttcttttgtcgatgctcaccctgttgtttggtgatacttctgcaggtc

SEQ ID NO: 132 - DNA, 1974 bp, Zea mays subsp. Mexicana
gtcgtgcccctctctagagataaagagcattgcatgtctaagttataaaaaattaccacatattttttttgtcacacttgtttgaagtgcagtttatctatctttatacatatatttaaactttactctacgaataatataatctatagtactacaataatatcagtgttttagagaatcatataaatgaacagttagacatggtctaaaggacaattgagtattttgacaacaggactctacagttttatctttttagtgtgcatgtgttctccttttttttttgcaaatagcttcacctatataatacttcatccattttattagtacatccatttagggtttagggttaatggtttttatagactaatttttttagtacatctattttattctattttagcctctaaattaagaaaactaaaactctattttagtttttttatttaataatttagatataaaatagaataaaataaagtgactaaaaattaaacaaataccctttaagaaattaaaaaaactaaggaaacatttttcttgtttcgagtagataatgccagcctgttaaacgccgtcgacgagtctaacggacaccaaccagcgaaccagcagcgtcgcgtcgggccaagcgaagcagacggcacggcatctctgtcgctgcctctggacccctctcgagagttccgctccaccgttggacttgctccgctgtcggcatccagaaattgcgtggcggagcggcagacgtgagccggcacggcaggcggcctcctcctcctctcacggcaccggcagctacgggggattcctttcccaccgctccttcgctttcccttcctcgcccgccgtaataaatagacaccccctccacaccttctttccccaacctcgtgttgttcggagcgcacacacacacaaccagatctcccccaaatccacccgtcggcacctccgcttcaaggtacgccgctcatcctcccccccccctctctaccttctctagatcggcgttccggtccatggttagggcccggtagttctacttctgttcatgtttgtgttagatccgtgtttgtgttagatccgtgctgctagcgttcgtacacggatgcgacctgtacgtcagacacgttctgattgctaacttgccagtgtttctctttggggaatcctgggatggctctagccgttccgcagacgggatcgatttcatgattttttttgtttcgttgcatagggtttggtttgcccttttcctttatttcaatatatgccgtgcacttgtttgtcgggtcatcttttcatgcttttttttgtcttggttgtgatgatgtggtctggttgggcggtcgttctagatcggagaagaattctgtttcaaactacctggtggatttattaattttggatctgtatgtgtgtgccatacatattcatagttacgaattgaagatgatggatggaaatatcgatctaggataggtatacatgttgatgcgggttttactgatgcatatacagagatgctttttgttcgcttggttgtgatgatgtggtctggttgggcggtcgttcattcgttctagatcggagtagaatactgtttcaaactacctggtgtatttattaattttggaactgtatgtgtgtgtcatacatcttcatagttacgagtttaagatggatggaaatatcgatctaggataggtatacatgttgatgtgggttttactgatgcatatacatgatggcatatgcagcatctattcatatgctctaaccttgagtacctatctattataataaacaagtatgttttataattattttgatcttgatatacttggatgatggcatatgcagcagctatatgtggatttttttagccctgccttcatacgctatttatttgcttggtactgtttcttttgtcgatgctcaccctgttgtttggtgatacttctgcagggt

SEQ ID NO: 133 - DNA, 1010 bp, Zea mays subsp. Mexicana
gtacgccgctcatcctcccccccccctctctaccttctctagatcggcgttccggtccatggttagggcccggtagttctacttctgttcatgtttgtgttagatccgtgtttgtgttagatccgtgctgctagcgttcgtacacggatgcgacctgtacgtcagacacgttctgattgctaacttgccagtgtttctctttggggaatcctgggatggctctagccgttccgcagacgggatcgatttcatgattttttttgtttcgttgcatagggtttggtttgcccttttcctttatttcaatatatgccgtgcacttgtttgtcgggtcatcttttcatgcttttttttgtcttggttgtgatgatgtggtctggttgggcggtcgttctagatcggagaagaattctgtttcaaactacctggtggatttattaattttggatctgtatgtgtgtgccatacatattcatagttacgaattgaagatgatggatggaaatatcgatctaggataggtatacatgttgatgcgggttttactgatgcatatacagagatgctttttgttcgcttggttgtgatgatgtggtctggttgggcggtcgttcattcgttctagatcggagtagaatactgtttcaaactacctggtgtatttattaattttggaactgtatgtgtgtgtcatacatcttcatagttacgagtttaagatggatggaaatatcgatctaggataggtatacatgttgatgtgggttttactgatgcatatacatgatggcatatgcagcatctattcatatgctctaaccttgagtacctatctattataataaacaagtatgttttataattattttgatcttgatatacttggatgatggcatatgcagcagctatatgtggatttttttagccctgccttcatacgctatttatttgcttggtactgtttcttttgtcgatgctcaccctgttgtttggtgatacttctgcagggt

SEQ ID NO: 134 - DNA, 2008 bp, Zea mays subsp. Mexicana
gtcgtgcccctctctagagataaagagcattgcatgtctaaagtataaaaaattaccacatatttttttgtcacacttatttgaagtgtagtttatctatctctatacatatatttaaacttcactctacaaataatatagtctataatactaaaataatattagtgttttagaggatcatataaataaactgctagacatggtctaaaggataattgaatattttgacaatctacagttttatctttttagtgtgcatgtgatctctctgttttttttgcaaatagcttgacctatataatacttcatccattttattagtacatccatttaggatttagggttgatggtttctatagactaatttttagtacatccattttattctttttagtctctaaattttttaaaactaaaactctattttagttttttatttaataatttagatataaaatgaaataaaataaattgactacaaataaaacaaataccctttaagaaataaaaaaactaagcaaacatttttcttgtttcgagtagataatgacaggctgttcaacgccgtcgacgagtctaacggacaccaaccagcgaaccagcagcgtcgcgtcgggccaagcgaagcagacggcacggcatctctgtagctgcctctggacccctctcgagagttccgctccaccgttggacttgctccgctgtcggcatccagaaattgcgtggcggagcggcagacgtgaggcggcacggcaggcggcctcttcctcctctcacggcaccggcagctacgggggattcctttcccaccgctccttcgctttcccttcctcgcccgccgtaataaatagacaccccctccacaccctctttccccaacctcgtgttcgttcggagcgcacacacacgcaaccagatctcccccaaatccagccgtcggcacctccgcttcaaggtacgccgctcatcctccccccccccctctctctaccttctctagatcggcgatccggtccatggttagggcccggtagttctacttctgttcatgtttgtgttagagcaaacatgttcatgttcatgtttgtgatgatgtggtctggttgggcggtcgttctagatcggagtaggatactgtttcaagctacctggtggatttattaattttgtatctgtatgtgtgtgccatacatcttcatagttacgagtttaagatgatggatggaaatatcgatctaggataggtatacatgttgatgcgggttttactgatgcatatacagagatgctttttttctcgcttggttgtgatgatatggtctggttgggcggtcgttctagatcggagtagaatactgtttcaaactacctggtggatttattaaaggataaagggtcgttctagatcggagtagaatactgtttcaaactacctggtggatttattaaaggatctgtatgtatgtgcctacatcttcatagttacgagtttaagatgatggatggaaatatcgatctaggataggtatacatgttgatgcgggttttactgatgcatatacagagatgctttttttcgcttggttgtgatgatgtggtctggttgggcggtcgttctagatcggagtagaatactgtttcaaactacctggtggatttattaattttgtatctttatgtgtgtgccatacatcttcatagttacgagtttaagatgatggatggaaatattgatctaggataggtatacatgttgatgtgggttttactgatgcatatacatgatggcatatgcggcatctattcatatgctctaaccttgagtacctatctattataataaacaagtatgttttataattattttgatcttgatatacttggatgatggcatatgcagcagctatatgtggattttttagccctgccttcatacgctatttatttgcttggtactgtttcttttgtccgatgctcaccctgttgttgggtgatacttctgcaggtc

SEQ ID NO: 135 - DNA, 877 bp, Zea mays subsp. Mexicana
gtcgtgcccctctctagagataaagagcattgcatgtctaaagtataaaaaattaccacatatttttttgtcacacttatttgaagtgtagtttatctatctctatacatatatttaaacttcactctacaaataatatagtctataatactaaaataatattagtgttttagaggatcatataaataaactgctagacatggtctaaaggataattgaatattttgacaatctacagttttatctttttagtgtgcatgtgatctctctgttttttttgcaaatagcttgacctatataatacttcatccattttattagtacatccatttaggatttagggttgatggtttctatagactaatttttagtacatccattttattctttttagtctctaaattttttaaaactaaaactctattttagttttttatttaataatttagatataaaatgaaataaaataaattgactacaaataaaacaaataccctttaagaaataaaaaaactaagcaaacatttttcttgtttcgagtagataatgacaggctgttcaacgccgtcgacgagtctaacggacaccaaccagcgaaccagcagcgtcgcgtcgggccaagcgaagcagacggcacggcatctctgtagctgcctctggacccctctcgagagttccgctccaccgttggacttgctccgctgtcggcatccagaaattgcgtggcggagcggcagacgtgaggcggcacggcaggcggcctcttcctcctctcacggcaccggcagctacgggggattcctttcccaccgctccttcgctttcccttcctcgcccgccgtaataaatagacaccccctccacaccctctttcccc

SEQ ID NO: 136 - DNA, 78 bp, Zea mays subsp. Mexicana
aacctcgtgttcgttcggagcgcacacacacgcaaccagatctcccccaaatccagccgtcggcacctccgcttcaag

SEQ ID NO: 137 - DNA, 1053 bp, Zea mays subsp. Mexicana
gtacgccgctcatcctccccccccccctctctctaccttctctagatcggcgatccggtccatggttagggcccggtagttctacttctgttcatgtttgtgttagagcaaacatgttcatgttcatgtttgtgatgatgtggtctggttgggcggtcgttctagatcggagtaggatactgtttcaagctacctggtggatttattaattttgtatctgtatgtgtgtgccatacatcttcatagttacgagtttaagatgatggatggaaatatcgatctaggataggtatacatgttgatgcgggttttactgatgcatatacagagatgctttttttctcgcttggttgtgatgatatggtctggttgggcggtcgttctagatcggagtagaatactgtttcaaactacctggtggatttattaaaggataaagggtcgttctagatcggagtagaatactgtttcaaactacctggtggatttattaaaggatctgtatgtatgtgcctacatcttcatagttacgagtttaagatgatggatggaaatatcgatctaggataggtatacatgttgatgcgggttttactgatgcatatacagagatgctttttttcgcttggttgtgatgatgtggtctggttgggcggtcgttctagatcggagtagaatactgtttcaaactacctggtggatttattaattttgtatctttatgtgtgtgccatacatcttcatagttacgagtttaagatgatggatggaaatattgatctaggataggtatacatgttgatgtgggttttactgatgcatatacatgatggcatatgcggcatctattcatatgctctaaccttgagtacctatctattataataaacaagtatgttttataattattttgatcttgatatacttggatgatggcatatgcagcagctatatgtggattttttagccctgccttcatacgctatttatttgcttggtactgtttcttttgtccgatgctcaccctgttgttgggtgatacttctgcaggtc

SEQ ID NO: 138 - DNA, 2008 bp, Zea mays subsp. Mexicana
gtcgtgcccctctctagagataaagagcattgcatgtctaaagtataaaaaattaccacatatttttttgtcacacttatttgaagtgtagtttatctatctctatacatatatttaaacttcactctacaaataatatagtctataatactaaaataatattagtgttttagaggatcatataaataaactgctagacatggtctaaaggataattgaatattttgacaatctacagttttatctttttagtgtgcatgtgatctctctgttttttttgcaaatagcttgacctatataatacttcatccattttattagtacatccatttaggatttagggttgatggtttctatagactaatttttagtacatccattttattctttttagtctctaaattttttaaaactaaaactctattttagttttttatttaataatttagatataaaatgaaataaaataaattgactacaaataaaacaaataccctttaagaaataaaaaaactaagcaaacatttttcttgtttcgagtagataatgacaggctgttcaacgccgtcgacgagtctaacggacaccaaccagcgaaccagcagcgtcgcgtcgggccaagcgaagcagacggcacggcatctctgtagctgcctctggacccctctcgagagttccgctccaccgttggacttgctccgctgtcggcatccagaaattgcgtggcggagcggcagacgtgaggcggcacggcaggcggcctcttcctcctctcacggcaccggcagctacgggggattcctttcccaccgctccttcgctttcccttcctcgcccgccgtaataaatagacaccccctccacaccctctttccccaacctcgtgttcgttcggagcgcacacacacgcaaccagatctcccccaaatccagccgtcggcacctccgcttcaaggtacgccgctcatcctccccccccccctctctctaccttctctagatcggcgatccggtccatggttagggcccggtagttctacttctgttcatgtttgtgttagagcaaacatgttcatgttcatgtttgtgatgatgtggtctggttgggcggtcgttctagatcggagtaggatactgtttcaagctacctggtggatttattaattttgtatctgtatgtgtgtgccatacatcttcatagttacgagtttaagatgatggatggaaatatcgatctaggataggtatacatgttgatgcgggttttactgatgcatatacagagatgctttttttctcgcttggttgtgatgatatggtctggttgggcggtcgttctagatcggagtagaatactgtttcaaactacctggtggatttattaaaggataaagggtcgttctagatcggagtagaatactgtttcaaactacctggtggatttattaaaggatctgtatgtatgtgcctacatcttcatagttacgagtttaagatgatggatggaaatatcgatctaggataggtatacatgttgatgcgggttttactgatgcatatacagagatgctttttttcgcttggttgtgatgatgtggtctggttgggcggtcgttctagatcggagtagaatactgtttcaaactacctggtggatttattaattttgtatctttatgtgtgtgccatacatcttcatagttacgagtttaagatgatggatggaaatattgatctaggataggtatacatgttgatgtgggttttactgatgcatatacatgatggcatatgcggcatctattcatatgctctaaccttgagtacctatctattataataaacaagtatgttttataattattttgatcttgatatacttggatgatggcatatgcagcagctatatgtggattttttagccctgccttcatacgctatttatttgcttggtactgtttcttttgtccgatgctcaccctgttgttgggtgatacttctgcagggt

SEQ ID NO: 139 - DNA, 1053 bp, Zea mays subsp. Mexicana
gtacgccgctcatcctccccccccccctctctctaccttctctagatcggcgatccggtccatggttagggcccggtagttctacttctgttcatgtttgtgttagagcaaacatgttcatgttcatgtttgtgatgatgtggtctggttgggcggtcgttctagatcggagtaggatactgtttcaagctacctggtggatttattaattttgtatctgtatgtgtgtgccatacatcttcatagttacgagtttaagatgatggatggaaatatcgatctaggataggtatacatgttgatgcgggttttactgatgcatatacagagatgctttttttctcgcttggttgtgatgatatggtctggttgggcggtcgttctagatcggagtagaatactgtttcaaactacctggtggatttattaaaggataaagggtcgttctagatcggagtagaatactgtttcaaactacctggtggatttattaaaggatctgtatgtatgtgcctacatcttcatagttacgagtttaagatgatggatggaaatatcgatctaggataggtatacatgttgatgcgggttttactgatgcatatacagagatgctttttttcgcttggttgtgatgatgtggtctggttgggcggtcgttctagatcggagtagaatactgtttcaaactacctggtggatttattaattttgtatctttatgtgtgtgccatacatcttcatagttacgagtttaagatgatggatggaaatattgatctaggataggtatacatgttgatgtgggttttactgatgcatatacatgatggcatatgcggcatctattcatatgctctaaccttgagtacctatctattataataaacaagtatgttttataattattttgatcttgatatacttggatgatggcatatgcagcagctatatgtggattttttagccctgccttcatacgctatttatttgcttggtactgtttcttttgtccgatgctcaccctgttgttgggtgatacttctgcagggt

SEQ ID NO: 140 - DNA, 1635 bp, Sorghum bicolor
ccaagtccaaatgtcaattcccttgaagatgatctatttttatcttttgcattttgttatggaagtttgcaaatagcaacaaatgctaagtcaatttgccaaagtctttggagatgctcttagtctataattgaacaatatttgtaaaatacaaaaaaaaatagtactatttttattttaaaaaatttttggaagtaaacaaggccgaggatggggaaacggaagtccaacacgtcgttttctaagttgggctcaaaagcccatcacggaactgacctgctatgggtcggaggagagcgcgtccagatggttccagaggctggtggtggtgggccaaacgcggaactccgccaccgccacggcctcgtgcgcaagcgcagcgcgttgccgtgagccgtgacgtaaccctccgttgcccacgataaaagctccacccccgaccccggccccccgatttcccctacggaccagtctccccccgatcgcaatcgcgaattcgtcgcaccatcggcacgcagacgaacgaagcaaggctctccccatcggctcgtcaaggtatgcgttccctagatttgttcccttcctctctcggtttgtctatatatatgcatgtatggtcgattcccgatctcgtcgattctcggtttcgccttccgtacgaagattcgtttagattgttcatatgttctgttgtgttaccagattgatcggatcaacttgatccagttatcttcgctcctccgattagatccgtttctatttcagtatatatatactagtatagtatctagggttcacactgttgaccgactggttacttggaattgatccgtgctgagttcagttgttgccgtccataaaggcccgtgctattgtctgttctgaaacgaaatcctgtagatttcttagggttagtgttcaattcatcaaaaggttgattagtgaattatcaaatttgagagggttaaatcattctcatcatgttgtctcgaatgtaatcccaaagatattatagactgtgtttcgatttgatggattgatttgtgtatcatctaaatcaacaaggctaagtcatcagttcatagaatcatgtttaggtttccgttcaatagactagttttatcaatatataaaattataagaagggtagggtaaatcacgttgcctcaaatgccatcctgtatggtttggtttcaattcaattagtttggttgattagggtatgctctggattaagatggttaaatcttccctagcatcttccctgcctatccttacttgatccgtttcggatatgttggaagtacagcgagcttatttcatgttgatagtgacccctttcagattatactattgaatattgtatgtttgccacttctgtatgttgaattatcctgctaaattagcaatggaattagcatattggcaattggtatgcatggacctaatcaggacggatgtggttatgttagtttcaattcattgtcaattcattgttcacctgcgttagatatatatgatgatttttacgtgtagttcatagttcttgagttttggatctttcttatctgatatatgctttcctgtgcctgtgctttattgtgtcttaccatgcgatttttgtctatgcaggtc

SEQ ID NO: 141 - DNA, 401 bp, Sorghum bicolor
ccaagtccaaatgtcaattcccttgaagatgatctatttttatcttttgcattttgttatggaagtttgcaaatagcaacaaatgctaagtcaatttgccaaagtctttggagatgctcttagtctataattgaacaatatttgtaaaatacaaaaaaaaatagtactatttttattttaaaaaatttttggaagtaaacaaggccgaggatggggaaacggaagtccaacacgtcgttttctaagttgggctcaaaagcccatcacggaactgacctgctatgggtcggaggagagcgcgtccagatggttccagaggctggtggtggtgggccaaacgcggaactccgccaccgccacggcctcgtgcgcaagcgcagcgcgttgccgtgagccgtgac

SEQ ID NO: 142 - DNA, 154 bp, Sorghum bicolor
gtaaccctccgttgcccacgataaaagctccacccccgaccccggccccccgatttcccctacggaccagtctccccccgatcgcaatcgcgaattcgtcgcaccatcggcacgcagacgaacgaagcaaggctctccccatcggctcgtcaag

SEQ ID NO: 143 - DNA, 1080 bp, Sorghum bicolor
gtatgcgttccctagatttgttcccttcctctctcggtttgtctatatatatgcatgtatggtcgattcccgatctcgtcgattctcggtttcgccttccgtacgaagattcgtttagattgttcatatgttctgttgtgttaccagattgatcggatcaacttgatccagttatcttcgctcctccgattagatccgtttctatttcagtatatatatactagtatagtatctagggttcacactgttgaccgactggttacttggaattgatccgtgctgagttcagttgttgccgtccataaaggcccgtgctattgtctgttctgaaacgaaatcctgtagatttcttagggttagtgttcaattcatcaaaaggttgattagtgaattatcaaatttgagagggttaaatcattctcatcatgttgtctcgaatgtaatcccaaagatattatagactgtgtttcgatttgatggattgatttgtgtatcatctaaatcaacaaggctaagtcatcagttcatagaatcatgtttaggtttccgttcaatagactagttttatcaatatataaaattataagaagggtagggtaaatcacgttgcctcaaatgccatcctgtatggtttggtttcaattcaattagtttggttgattagggtatgctctggattaagatggttaaatcttccctagcatcttccctgcctatccttacttgatccgtttcggatatgttggaagtacagcgagcttatttcatgttgatagtgacccctttcagattatactattgaatattgtatgtttgccacttctgtatgttgaattatcctgctaaattagcaatggaattagcatattggcaattggtatgcatggacctaatcaggacggatgtggttatgttagtttcaattcattgtcaattcattgttcacctgcgttagatatatatgatgatttttacgtgtagttcatagttcttgagttttggatctttcttatctgatatatgctttcctgtgcctgtgctttattgtgtcttaccatgcgatttttgtctatgcaggtc

SEQ ID NO: 144 - DNA, 2067 bp, Sorghum bicolor
cattaaaagtcattatgtgcatgcgtcgtaactaacatggatatgttgctgcactatctcctcgcactagctgcgcatgataaagccacaagccaaaattaattattatgggtgagaataaatacgtaccagcaccggccatagaaaaagtacattattaaaggtctaatttggaaacagtctgaaaacgacgtgcgctgcagaggtaaatgtaattttcggcactaaaaccattatcaactaattcattcaataacagttatttagaaaatgtatagctcgctctaaaaaaacagtttagaaaaacagtcaaaataattcgaccaacaaacagttaataaggttcattaaatatataatgcacggtgctatttgatcttttaaaggaaaaagaggaatagtcgtgggcgccaggcgggaattggggcgcgggagtctgccggacgacgcgttccgtccgaacggccggacccgacgaggcccccccgccgccccacgtcgcagaaccgtccgtgggtggtaatctggccgggtacaccagccgtccccttgggcggcctcacagcactgggctcacacgtgagttttgttctgggcttcggatcgcaccatatgggcctcggcatcagaaagacggggcccgtctgggatagaagagacaggaacctcctcgtggattccagaagccagccacgagcgaccaccgacgcggaggatactcgtcgtccaagtccaacacggcgggcgggcgggcggacgcgtgggctgggctaactgcctaaccttaacctccaaggcacgccaaggcccgcttctcccacccgacataaatatccccccatccaggcaaggcgcagagcctcagaccagattccgatcaatcacccataagctccccccaaatctgttcctcgtctcccgtctcgcggtttcctacttccctcggacgcctccggcaagtcgctcgaccgcgcgattccgcccgctcaaggtatcaactcggttcaccactccaatctacgtctgatttagatgttacttccatctatgtctaatttagatgttactccgatgcgattggattatgtttatgcggtttgcactgctctggaaactggaatctagggtttcgagtgatttgatcgatcgcgatctgtgatttcgttgcgccttgtgtatgcttggagtgatctaggcttgtatatgcggcatcgcgatctgacgcggttgctttgtagaggctgggggtctaggctgtgattttagaatcaaataaagctgttccttaccgtagatgtttcctacatgttctgtccagtactccagtgctatattcacattgtttgaggcttgagttttgtcgatcagtggtcatgagaaaaatatatctcatgattttagaggcacctattgggaaaggtagatggttccgttttacatgttttatagaccttgtggcatggctcctttgttctatgggtgctttattttcctgaataacagtaatgcgagactggtctatgggtgctttgaccagtaatgcgagactagttatttgatcatggtgcagttcctagtgattacgaacaacaatttggtagctcagttcattcagcattggtttctacgatccttatcattttacttctgaatgaatttatttatttaagatattacagtgcaataaactgctgtataatatcagtaacaaactgctattactagtaaatgcctagattcataataattcattattctacttgaaaatgatcttaggcctttttatgcggtcctacgcatccttccacaggacttgctgtttgtttgttttttgtaatccctcgctgggacgcagaatggttcatctgtgctaataatttttttgcatatataagtttatagttctcattattcatgtggctatggtagcctgtaaaatctattgtaataacatattagtcagccatacatctgttccaacttgctcaattgcaaatcatatctccacttaaagcacatgtttgcaagctttctgacaagtttctttgtgtttgattgaaacaggtg

SEQ ID NO: 145 - DNA, 855 bp, Sorghum bicolor
cattaaaagtcattatgtgcatgcgtcgtaactaacatggatatgttgctgcactatctcctcgcactagctgcgcatgataaagccacaagccaaaattaattattatgggtgagaataaatacgtaccagcaccggccatagaaaaagtacattattaaaggtctaatttggaaacagtctgaaaacgacgtgcgctgcagaggtaaatgtaattttcggcactaaaaccattatcaactaattcattcaataacagttatttagaaaatgtatagctcgctctaaaaaaacagtttagaaaaacagtcaaaataattcgaccaacaaacagttaataaggttcattaaatatataatgcacggtgctatttgatcttttaaaggaaaaagaggaatagtcgtgggcgccaggcgggaattggggcgcgggagtctgccggacgacgcgttccgtccgaacggccggacccgacgaggcccccccgccgccccacgtcgcagaaccgtccgtgggtggtaatctggccgggtacaccagccgtccccttgggcggcctcacagcactgggctcacacgtgagttttgttctgggcttcggatcgcaccatatgggcctcggcatcagaaagacggggcccgtctgggatagaagagacaggaacctcctcgtggattccagaagccagccacgagcgaccaccgacgcggaggatactcgtcgtccaagtccaacacggcgggcgggcgggcggacgcgtgggctgggctaactgcctaaccttaacctccaaggcacgccaaggcccgcttctcccacccgacataaatatccccccatccaggcaaggcgc

SEQ ID NO: 146 - DNA, 136 bp, Sorghum bicolor
agagcctcagaccagattccgatcaatcacccataagctccccccaaatctgttcctcgtctcccgtctcgcggtttcctacttccctcggacgcctccggcaagtcgctcgaccgcgcgattccgcccgctcaag

SEQ ID NO: 147 - DNA, 1076 bp, Sorghum bicolor
gtatcaactcggttcaccactccaatctacgtctgatttagatgttacttccatctatgtctaatttagatgttactccgatgcgattggattatgtttatgcggtttgcactgctctggaaactggaatctagggtttcgagtgatttgatcgatcgcgatctgtgatttcgttgcgccttgtgtatgcttggagtgatctaggcttgtatatgcggcatcgcgatctgacgcggttgctttgtagaggctgggggtctaggctgtgattttagaatcaaataaagctgttccttaccgtagatgtttcctacatgttctgtccagtactccagtgctatattcacattgtttgaggcttgagttttgtcgatcagtggtcatgagaaaaatatatctcatgattttagaggcacctattgggaaaggtagatggttccgttttacatgttttatagaccttgtggcatggctcctttgttctatgggtgctttattttcctgaataacagtaatgcgagactggtctatgggtgctttgaccagtaatgcgagactagttatttgatcatggtgcagttcctagtgattacgaacaacaatttggtagctcagttcattcagcattggtttctacgatccttatcattttacttctgaatgaatttatttatttaagatattacagtgcaataaactgctgtataatatcagtaacaaactgctattactagtaaatgcctagattcataataattcattattctacttgaaaatgatcttaggcctttttatgcggtcctacgcatccttccacaggacttgctgtttgtttgttttttgtaatccctcgctgggacgcagaatggttcatctgtgctaataatttttttgcatatataagtttatagttctcattattcatgtggctatggtagcctgtaaaatctattgtaataacatattagtcagccatacatctgttccaacttgctcaattgcaaatcatatctccacttaaagcacatgtttgcaagctttctgacaagtttctttgtgtttgattgaaacaggtg

SEQ ID NO: 148 - DNA, 2067 bp, Sorghum bicolor
cattaaaagtcattatgtgcatgcgtcgtaactaacatggatatgttgctgcactatctcctcgcactagctgcgcatgataaagccacaagccaaaattaattattatgggtgagaataaatacgtaccagcaccggccatagaaaaagtacattattaaaggtctaatttggaaacagtctgaaaacgacgtgcgctgcagaggtaaatgtaattttcggcactaaaaccattatcaactaattcattcaataacagttatttagaaaatgtatagctcgctctaaaaaaacagtttagaaaaacagtcaaaataattcgaccaacaaacagttaataaggttcattaaatatataatgcacggtgctatttgatcttttaaaggaaaaagaggaatagtcgtgggcgccaggcgggaattggggcgcgggagtctgccggacgacgcgttccgtccgaacggccggacccgacgaggcccccccgccgccccacgtcgcagaaccgtccgtgggtggtaatctggccgggtacaccagccgtccccttgggcggcctcacagcactgggctcacacgtgagttttgttctgggcttcggatcgcaccatatgggcctcggcatcagaaagacggggcccgtctgggatagaagagacaggaacctcctcgtggattccagaagccagccacgagcgaccaccgacgcggaggatactcgtcgtccaagtccaacacggcgggcgggcgggcggacgcgtgggctgggctaactgcctaaccttaacctccaaggcacgccaaggcccgcttctcccacccgacataaatatccccccatccaggcaaggcgcagagcctcagaccagattccgatcaatcacccataagctccccccaaatctgttcctcgtctcccgtctcgcggtttcctacttccctcggacgcctccggcaagtcgctcgaccgcgcgattccgcccgctcaaggtatcaactcggttcaccactccaatctacgtctgatttagatgttacttccatctatgtctaatttagatgttactccgatgcgattggattatgtttatgcggtttgcactgctctggaaactggaatctagggtttcgagtgatttgatcgatcgcgatctgtgatttcgttgcgccttgtgtatgcttggagtgatctaggcttgtatatgcggcatcgcgatctgacgcggttgctttgtagaggctgggggtctaggctgtgattttagaatcaaataaagctgttccttaccgtagatgtttcctacatgttctgtccagtactccagtgctatattcacattgtttgaggcttgagttttgtcgatcagtggtcatgagaaaaatatatctcatgattttagaggcacctattgggaaaggtagatggttccgttttacatgttttatagaccttgtggcatggctcctttgttctatgggtgctttattttcctgaataacagtaatgcgagactggtctatgggtgctttgaccagtaatgcgagactagttatttgatcatggtgcagttcctagtgattacgaacaacaatttggtagctcagttcattcagcattggtttctacgatccttatcattttacttctgaatgaatttatttatttaagatattacagtgcaataaactgctgtataatatcagtaacaaactgctattactagtaaatgcctagattcataataattcattattctacttgaaaatgatcttaggcctttttatgcggtcctacgcatccttccacaggacttgctgtttgtttgttttttgtaatccctcgctgggacgcagaatggttcatctgtgctaataatttttttgcatatataagtttatagttctcattattcatgtggctatggtagcctgtaaaatctattgtaataacatattagtcagccatacatctgttccaacttgctcaattgcaaatcatatctccacttaaagcacatgtttgcaagctttctgacaagtttctttgtgtttgattgaaacagggt

SEQ ID NO: 149 - DNA, 1076 bp, Sorghum bicolor
gtatcaactcggttcaccactccaatctacgtctgatttagatgttacttccatctatgtctaatttagatgttactccgatgcgattggattatgtttatgcggtttgcactgctctggaaactggaatctagggtttcgagtgatttgatcgatcgcgatctgtgatttcgttgcgccttgtgtatgcttggagtgatctaggcttgtatatgcggcatcgcgatctgacgcggttgctttgtagaggctgggggtctaggctgtgattttagaatcaaataaagctgttccttaccgtagatgtttcctacatgttctgtccagtactccagtgctatattcacattgtttgaggcttgagttttgtcgatcagtggtcatgagaaaaatatatctcatgattttagaggcacctattgggaaaggtagatggttccgttttacatgttttatagaccttgtggcatggctcctttgttctatgggtgctttattttcctgaataacagtaatgcgagactggtctatgggtgctttgaccagtaatgcgagactagttatttgatcatggtgcagttcctagtgattacgaacaacaatttggtagctcagttcattcagcattggtttctacgatccttatcattttacttctgaatgaatttatttatttaagatattacagtgcaataaactgctgtataatatcagtaacaaactgctattactagtaaatgcctagattcataataattcattattctacttgaaaatgatcttaggcctttttatgcggtcctacgcatccttccacaggacttgctgtttgtttgttttttgtaatccctcgctgggacgcagaatggttcatctgtgctaataatttttttgcatatataagtttatagttctcattattcatgtggctatggtagcctgtaaaatctattgtaataacatattagtcagccatacatctgttccaacttgctcaattgcaaatcatatctccacttaaagcacatgtttgcaagctttctgacaagtttctttgtgtttgattgaaacagggt

SEQ ID NO: 150 - DNA, 2003 bp, Sorghum bicolor
agaagtaaaaaaaaagttcgtttcagaatcataaaggtaagttaaaaaaagaccatacaaaaaagaggtatttaatgataaactataatccagaatttgttaggatagtatataagaataagaccttgtttagtttcaaaaaaatttgcaaaattttccagattcctcgtcacatcaaatctttagaggtatgcatggagtattaaatatagacaagacctaaataagaaaacatgaaatgttcacgaaaaaaatcaagccaatgcatgatcgaagcaaacggtatagtaacggtgttaacctgatccattgatctttgtaatctttaacggccacctaccgcgggcagcaaacggcgtccccctcctcgatatctccgcggcggcctctggctttttccgcggaattgcgcggtggggacggattccacgagaccgcaacgcaaccgcctctcgccgctgggccccacaccgctcggtgccgtagcccgtagcctcacgggattctttctccctcctcccccgtgtataaattggcttcatcccctccctgcctcatccatccaaatcccactccccaatcccatcccgtcggagaaattcatcgaagcgaagcgaagcgaatcctcccgatcctctcaaggtacgcgagttttcgaatcccctccagacccctcgtatgctttccctgttcgttttcgtcgtagcgtttgattaggtatgctttccctgttcgtgttcgtcgtagggttcgattaggtcgtgtgaggccatggcctgctgtgataaatttatttgttgttatatcggatctgtagtcgatttgggggtcgtggtgtagatccgcgggctgtgatgaagttatttggtgtgattgtgctcgcgtgattctgcgcgttgagctcgagtagatctgatggttggacgaccgattggttcgttggctggctgcgctaaggttgggctgggctcatgttgcgttcgctgttgcgcgtgattccgcggatggacttgcgcttgattgccgccagatcacgttacgattatgtgatttcgtttggaactttttagatttgtagcttctgcttattatatgacagatgcgcctactgctcatatgcctgtggtaaataatggatggctgtgggtcaaactagttgattgtcgagtcatgtatcatatacaggtgtatagacttgcgtctaattgtttgcatgttgcagttatatgatttgttttagattgtttgttccactcatctaggctgtaaaagggacactacttattagcttgttgtttaatctttttattagtagattatattggtaatgttttactaattattattatgttatatgtgacttctgctcatgcctgattataatcatagatcactgtagttgattgttgaatcatgtgtcaaatacccgtatacataacactacacatttgcttagttgtttccttaactcatgcaaattgaacaccatgtatgatttgcatggtgctgtaatgttaaatactacagtcctgttggtacttgtttagtaagaatctgcttcatacaactatatgctatgcctgatgataatcatatatctttgtgtaattaataattagttgactgttgaataatgtatcgagtacataccatggcacaattgcttagtcacttccttaaccatgcatattgaactgaccccttcatgttctgctgaattgttctattctgattagaccatacatcatgtattgcaatctttatttgcaattgtaatgtaatggttcggttctcaaatgttaaatgctatagttgtgctactttctaatgttaaatgctatagctgtgctacttgtaagatctgcttcatagtttagttaaattaggatgatgagctttgatgctgtaactttgtttgattatgttcatagttgatcagtttttgttagactcacagtaacttatggtctcactcttcttctggtctttgatgtttgcagcgg

SEQ ID NO: 151 - DNA, 565 bp, Sorghum bicolor
agaagtaaaaaaaaagttcgtttcagaatcataaaggtaagttaaaaaaagaccatacaaaaaagaggtatttaatgataaactataatccagaatttgttaggatagtatataagaataagaccttgtttagtttcaaaaaaatttgcaaaattttccagattcctcgtcacatcaaatctttagaggtatgcatggagtattaaatatagacaagacctaaataagaaaacatgaaatgttcacgaaaaaaatcaagccaatgcatgatcgaagcaaacggtatagtaacggtgttaacctgatccattgatctttgtaatctttaacggccacctaccgcgggcagcaaacggcgtccccctcctcgatatctccgcggcggcctctggctttttccgcggaattgcgcggtggggacggattccacgagaccgcaacgcaaccgcctctcgccgctgggccccacaccgctcggtgccgtagcccgtagcctcacgggattctttctccctcctcccccgtgtataaattggcttcatcccctccctgcctcatccatcca

SEQ ID NO: 152 - DNA, 77 bp, Sorghum bicolor
aatcccactccccaatcccatcccgtcggagaaattcatcgaagcgaagcgaagcgaatcctcccgatcctctcaag

SEQ ID NO: 153 - DNA, 1361 bp, Sorghum bicolor
gtacgcgagttttcgaatcccctccagacccctcgtatgctttccctgttcgttttcgtcgtagcgtttgattaggtatgctttccctgttcgtgttcgtcgtagggttcgattaggtcgtgtgaggccatggcctgctgtgataaatttatttgttgttatatcggatctgtagtcgatttgggggtcgtggtgtagatccgcgggctgtgatgaagttatttggtgtgattgtgctcgcgtgattctgcgcgttgagctcgagtagatctgatggttggacgaccgattggttcgttggctggctgcgctaaggttgggctgggctcatgttgcgttcgctgttgcgcgtgattccgcggatggacttgcgcttgattgccgccagatcacgttacgattatgtgatttcgtttggaactttttagatttgtagcttctgcttattatatgacagatgcgcctactgctcatatgcctgtggtaaataatggatggctgtgggtcaaactagttgattgtcgagtcatgtatcatatacaggtgtatagacttgcgtctaattgtttgcatgttgcagttatatgatttgttttagattgtttgttccactcatctaggctgtaaaagggacactacttattagcttgttgtttaatctttttattagtagattatattggtaatgttttactaattattattatgttatatgtgacttctgctcatgcctgattataatcatagatcactgtagttgattgttgaatcatgtgtcaaatacccgtatacataacactacacatttgcttagttgtttccttaactcatgcaaattgaacaccatgtatgatttgcatggtgctgtaatgttaaatactacagtcctgttggtacttgtttagtaagaatctgcttcatacaactatatgctatgcctgatgataatcatatatctttgtgtaattaataattagttgactgttgaataatgtatcgagtacataccatggcacaattgcttagtcacttccttaaccatgcatattgaactgaccccttcatgttctgctgaattgttctattctgattagaccatacatcatgtattgcaatctttatttgcaattgtaatgtaatggttcggttctcaaatgttaaatgctatagttgtgctactttctaatgttaaatgctatagctgtgctacttgtaagatctgcttcatagtttagttaaattaggatgatgagctttgatgctgtaactttgtttgattatgttcatagttgatcagtttttgttagactcacagtaacttatggtctcactcttcttctggtctttgatgtttgcagcgg

SEQ ID NO: 154 - DNA, 1812 bp, Artificial sequence
  misc_feature (1)..(1812): Codon optimized coding sequence.
atggtccgtcctgtagaaaccccaacccgtgaaatcaaaaaactcgacggcctgtgggcattcagtctggatcgcgaaaactgtggaattgatcagcgttggtgggaaagcgcgttacaagaaagccgggcaattgctgtgccaggcagttttaacgatcagttcgccgatgcagatattcgtaattatgcgggcaacgtctggtatcagcgcgaagtctttataccgaaaggttgggcaggccagcgtatcgtgctgcgtttcgatgcggtcactcattacggcaaagtgtgggtcaataatcaggaagtgatggagcatcagggcggctatacgccatttgaagccgatgtcacgccgtatgttattgccgggaaaagtgtacgtatcaccgtttgtgtgaacaacgaactgaactggcagactatcccgccgggaatggtgattaccgacgaaaacggcaagaaaaagcagtcttacttccatgatttctttaactatgccggaatccatcgcagcgtaatgctctacaccacgccgaacacctgggtggacgatatcaccgtggtgacgcatgtcgcgcaagactgtaaccacgcgtctgttgactggcaggtggtggccaatggtgatgtcagcgttgaactgcgtgatgcggatcaacaggtggttgcaactggacaaggcactagcgggactttgcaagtggtgaatccgcacctctggcaaccgggtgaaggttatctctatgaactgtgcgtcacagccaaaagccagacagagtgtgatatctacccgcttcgcgtcggcatccggtcagtggcagtgaagggcgaacagttcctgattaaccacaaaccgttctactttactggctttggtcgtcatgaagatgcggacttgcgtggcaaaggattcgataacgtgctgatggtgcacgaccacgcattaatggactggattggggccaactcctaccgtacctcgcattacccttacgctgaagagatgctcgactgggcagatgaacatggcatcgtggtgattgatgaaactgctgctgtcggctttaacctctctttaggcattggtttcgaagcgggcaacaagccgaaagaactgtacagcgaagaggcagtcaacggggaaactcagcaagcgcacttacaggcgattaaagagctgatagcgcgtgacaaaaaccacccaagcgtggtgatgtggagtattgccaacgaaccggatacccgtccgcaaggtgcacgggaatatttcgcgccactggcggaagcaacgcgtaaactcgacccgacgcgtccgatcacctgcgtcaatgtaatgttctgcgacgctcacaccgataccatcagcgatctctttgatgtgctgtgcctgaaccgttattacggatggtatgtccaaagcggcgatttggaaacggcagagaaggtactggaaaaagaacttctggcctggcaggagaaactgcatcagccgattatcatcaccgaatacggcgtggatacgttagccgggctgcactcaatgtacaccgacatgtggagtgaagagtatcagtgtgcatggctggatatgtatcaccgcgtctttgatcgcgtcagcgccgtcgtcggtgaacaggtatggaatttcgccgattttgcgacctcgcaaggcatattgcgcgttggcggtaacaagaaagggatcttcactcgcgaccgcaaaccgaagtcggcggcttttctgctgcaaaaacgctggactggcatgaacttcggtgaaaaaccgcagcagggaggcaaacaatga

SEQ ID NO: 155 - DNA, 2001 bp, Artificial sequence
  misc_feature (1)..(2001): Chimeric coding sequence with processable intron.
atggtccgtcctgtagaaaccccaacccgtgaaatcaaaaaactcgacggcctgtgggcattcagtctggatcgcgaaaactgtggaattgatcagcgttggtgggaaagcgcgttacaagaaagccgggcaattgctgtgccaggcagttttaacgatcagttcgccgatgcagatattcgtaattatgcgggcaacgtctggtatcagcgcgaagtctttataccgaaaggttgggcaggccagcgtatcgtgctgcgtttcgatgcggtcactcattacggcaaagtgtgggtcaataatcaggaagtgatggagcatcagggcggctatacgccatttgaagccgatgtcacgccgtatgttattgccgggaaaagtgtacgtaagtttctgcttctacctttgatatatatataataattatcattaattagtagtaatataatatttcaaatatttttttcaaaataaaagaatgtagtatatagcaattgcttttctgtagtttataagtgtgtatattttaatttataacttttctaatatatgaccaaaatttgttgatgtgcaggtatcaccgtttgtgtgaacaacgaactgaactggcagactatcccgccgggaatggtgattaccgacgaaaacggcaagaaaaagcagtcttacttccatgatttctttaactatgccggaatccatcgcagcgtaatgctctacaccacgccgaacacctgggtggacgatatcaccgtggtgacgcatgtcgcgcaagactgtaaccacgcgtctgttgactggcaggtggtggccaatggtgatgtcagcgttgaactgcgtgatgcggatcaacaggtggttgcaactggacaaggcactagcgggactttgcaagtggtgaatccgcacctctggcaaccgggtgaaggttatctctatgaactgtgcgtcacagccaaaagccagacagagtgtgatatctacccgcttcgcgtcggcatccggtcagtggcagtgaagggcgaacagttcctgattaaccacaaaccgttctactttactggctttggtcgtcatgaagatgcggacttgcgtggcaaaggattcgataacgtgctgatggtgcacgaccacgcattaatggactggattggggccaactcctaccgtacctcgcattacccttacgctgaagagatgctcgactgggcagatgaacatggcatcgtggtgattgatgaaactgctgctgtcggctttaacctctctttaggcattggtttcgaagcgggcaacaagccgaaagaactgtacagcgaagaggcagtcaacggggaaactcagcaagcgcacttacaggcgattaaagagctgatagcgcgtgacaaaaaccacccaagcgtggtgatgtggagtattgccaacgaaccggatacccgtccgcaaggtgcacgggaatatttcgcgccactggcggaagcaacgcgtaaactcgacccgacgcgtccgatcacctgcgtcaatgtaatgttctgcgacgctcacaccgataccatcagcgatctctttgatgtgctgtgcctgaaccgttattacggatggtatgtccaaagcggcgatttggaaacggcagagaaggtactggaaaaagaacttctggcctggcaggagaaactgcatcagccgattatcatcaccgaatacggcgtggatacgttagccgggctgcactcaatgtacaccgacatgtggagtgaagagtatcagtgtgcatggctggatatgtatcaccgcgtctttgatcgcgtcagcgccgtcgtcggtgaacaggtatggaatttcgccgattttgcgacctcgcaaggcatattgcgcgttggcggtaacaagaaagggatcttcactcgcgaccgcaaaccgaagtcggcggcttttctgctgcaaaaacgctggactggcatgaacttcggtgaaaaaccgcagcagggaggcaaacaatga

SEQ ID NO: 156 - DNA, 1653 bp, Artificial sequence
  misc_feature (1)..(1653): Codon optimized coding sequence.
atggaagacgccaaaaacataaagaaaggcccggcgccattctatcctctagaggatggaaccgctggagagcaactgcataaggctatgaagagatacgccctggttcctggaacaattgcttttacagatgcacatatcgaggtgaacatcacgtacgcggaatacttcgaaatgtccgttcggttggcagaagctatgaaacgatatgggctgaatacaaatcacagaatcgtcgtatgcagtgaaaactctcttcaattctttatgccggtgttgggcgcgttatttatcggagttgcagttgcgcccgcgaacgacatttataatgaacgtgaattgctcaacagtatgaacatttcgcagcctaccgtagtgtttgtttccaaaaaggggttgcaaaaaattttgaacgtgcaaaaaaaattaccaataatccagaaaattattatcatggattctaaaacggattaccagggatttcagtcgatgtacacgttcgtcacatctcatctacctcccggttttaatgaatacgattttgtaccagagtcctttgatcgtgacaaaacaattgcactgataatgaattcctctggatctactgggttacctaagggtgtggcccttccgcatagaactgcctgcgtcagattctcgcatgccagagatcctatttttggcaatcaaatcattccggatactgcgattttaagtgttgttccattccatcacggttttggaatgtttactacactcggatatttgatatgtggatttcgagtcgtcttaatgtatagatttgaagaagagctgtttttacgatcccttcaggattacaaaattcaaagtgcgttgctagtaccaaccctattttcattcttcgccaaaagcactctgattgacaaatacgatttatctaatttacacgaaattgcttctgggggcgcacctctttcgaaagaagtcggggaagcggttgcaaaacgcttccatcttccagggatacgacaaggatatgggctcactgagactacatcagctattctgattacacccgagggggatgataaaccgggcgcggtcggtaaagttgttccattttttgaagcgaaggttgtggatctggataccgggaaaacgctgggcgttaatcagagaggcgaattatgtgtcagaggacctatgattatgtccggttatgtaaacaatccggaagcgaccaacgccttgattgacaaggatggatggctacattctggagacatagcttactgggacgaagacgaacacttcttcatagttgaccgcttgaagtctttaattaaatacaaaggatatcaggtggcccccgctgaattggaatcgatattgttacaacaccccaacatcttcgacgcgggcgtggcaggtcttcccgacgatgacgccggtgaacttcccgccgccgttgttgttttggagcacggaaagacgatgacggaaaaagagatcgtggattacgtcgccagtcaagtaacaaccgcgaaaaagttgcgcggaggagttgtgtttgtggacgaagtaccgaaaggtcttaccggaaaactcgacgcaagaaaaatcagagagatcctcataaaggccaagaagggcggaaagtccaaattgtaa

SEQ ID NO: 157 - DNA, 936 bp, Artificial sequence
  misc_feature (1)..(936): Codon optimized coding sequence.
atggcttccaaggtgtacgaccccgagcaacgcaaacgcatgatcactgggcctcagtggtgggctcgctgcaagcaaatgaacgtgctggactccttcatcaactactatgattccgagaagcacgccgagaacgccgtgatttttctgcatggtaacgctgcctccagctacctgtggaggcacgtcgtgcctcacatcgagcccgtggctagatgcatcatccctgatctgatcggaatgggtaagtccggcaagagcgggaatggctcatatcgcctcctggatcactacaagtacctcaccgcttggttcgagctgctgaaccttccaaagaaaatcatctttgtgggccacgactggggggcttgtctggcctttcactactcctacgagcaccaagacaagatcaaggccatcgtccatgctgagagtgtcgtggacgtgatcgagtcctgggacgagtggcctgacatcgaggaggatatcgccctgatcaagagcgaagagggcgagaaaatggtgcttgagaataacttcttcgtcgagaccatgctcccaagcaagatcatgcggaaactggagcctgaggagttcgctgcctacctggagccattcaaggagaagggcgaggttagacggcctaccctctcctggcctcgcgagatccctctcgttaagggaggcaagcccgacgtcgtccagattgtccgcaactacaacgcctaccttcgggccagcgacgatctgcctaagatgttcatcgagtccgaccctgggttcttttccaacgctattgtcgagggagctaagaagttccctaacaccgagttcgtgaaggtgaagggcctccacttcagccaggaggacgctccagatgaaatgggtaagtacatcaagagcttcgtggagcgcgtgctgaagaacgagcagtaa

SEQ ID NO: 158 - DNA, 253 bp, Agrobacterium tumefaciens
gatcgttcaaacatttggcaataaagtttcttaagattgaatcctgttgccggtcttgcgatgattatcatataatttctgttgaattacgttaagcatgtaataattaacatgtaatgcatgacgttatttatgagatgggtttttatgattagagtcccgcaattatacatttaatacgcgatagaaaacaaaatatagcgcgcaaactaggataaattatcgcgcgcggtgtcatctatgttactagatc

SEQ ID NO: 159 - DNA, 210 bp, Triticum aestivum
ctgcatgcgtttggacgtatgctcattcaggttggagccaatttggttgatgtgtgtgcgagttcttgcgagtctgatgagacatctctgtattgtgtttctttccccagtgttttctgtacttgtgtaatcggctaatcgccaacagattcggcgatgaataaatgagaaataaattgttctgattttgagtgcaaaaaaaaaggaatt

SEQ ID NO: 160 - DNA, 300 bp, Oryza sativa
attaatcgatcctccgatcccttaattaccataccattacaccatgcatcaatatccatatatatataaaccctttcgcacgtacttatactatgttttgtcatacatatatatgtgtcgaacgatcgatctatcactgatatgatatgattgatccatcagcctgatctctgtatcttgttatttgtataccgtcaaataaaagtttcttccacttgtgttaataattagctactctcatctcatgaaccctatatataactagtttaatttgctgtcaattgaacatgatgatcgatg

SEQ ID NO: 161 - DNA, 1204 bp, Artificial sequence
  misc_feature (1)..(1204): Chimeric transcriptional regulatory expression element group.
ggtccgattgagacttttcaacaaagggtaatatccggaaacctcctcggattccattgcccagctatctgtcactttattgtgaagatagtggaaaaggaaggtggctcctacaaatgccatcattgcgataaaggaaaggccatcgttgaagatgcctctgccgacagtggtcccaaagatggacccccacccacgaggagcatcgtggaaaaagaagacgttccaaccacgtcttcaaagcaagtggattgatgtgatggtccgattgagacttttcaacaaagggtaatatccggaaacctcctcggattccattgcccagctatctgtcactttattgtgaagatagtggaaaaggaaggtggctcctacaaatgccatcattgcgataaaggaaaggccatcgttgaagatgcctctgccgacagtggtcccaaagatggacccccacccacgaggagcatcgtggaaaaagaagacgttccaaccacgtcttcaaagcaagtggattgatgtgatatctccactgacgtaagggatgacgcacaatcccactatccttcgcaagacccttcctctatataaggaagttcatttcatttggagaggacacgctgacaagctgactctagcagatcctctagaaccatcttccacacactcaagccacactattggagaacacacagggacaacacaccataagatccaagggaggcctccgccgccgccggtaaccaccccgcccctctcctctttctttctccgtttttttttccgtctcggtctcgatctttggccttggtagtttgggtgggcgagaggcggcttcgtgcgcgcccagatcggtgcgcgggaggggcgggatctcgcggctggggctctcgccggcgtggatccggcccggatctcgcggggaatggggctctcggatgtagatctgcgatccgccgttgttgggggagatgatggggggtttaaaatttccgccgtgctaaacaagatcaggaagaggggaaaagggcactatggtttatatttttatatatttctgctgcttcgtcaggcttagatgtgctagatctttctttcttctttttgtgggtagaatttgaatccctcagcattgttcatcggtagtttttcttttcatgatttgtgacaaatgcagcctcgtgcggagcttttttgtaggtagaag

SEQ ID NO: 162 - DNA, 1396 bp, Oryza sativa
tcgaggtcattcatatgcttgagaagagagtcgggatagtccaaaataaaacaaaggtaagattacctggtcaaaagtgaaaacatcagttaaaaggtggtataaagtaaaatatcggtaataaaaggtggcccaaagtgaaatttactcttttctactattataaaaattgaggatgtttttgtcggtactttgatacgtcatttttgtatgaattggtttttaagtttattcgcttttggaaatgcatatctgtatttgagtcgggttttaagttcgtttgcttttgtaaatacagagggatttgtataagaaatatctttagaaaaacccatatgctaatttgacataatttttgagaaaaatatatattcaggcgaattctcacaatgaacaataataagattaaaatagctttcccccgttgcagcgcatgggtattttttctagtaaaaataaaagataaacttagactcaaaacatttacaaaaacaacccctaaagttcctaaagcccaaagtgctatccacgatccatagcaagcccagcccaacccaacccaacccagcccaccccagtccagccaactggacaatagtctccacacccccccactatcaccgtgagttgtccgcacgcaccgcacgtctcgcagccaaaaaaaaaaagaaagaaaaaaaagaaaaagaaaaaacagcaggtgggtccgggtcgtgggggccggaaacgcgaggaggatcgcgagccagcgacgaggccggccctccctccgcttccaaagaaacgccccccatcgccactatatacatacccccccctctcctcccatccccccaaccctaccaccaccaccaccaccacctccacctcctcccccctcgctgccggacgacgagctcctcccccctccccctccgccgccgccgcgccggtaaccaccccgcccctctcctctttctttctccgtttttttttccgtctcggtctcgatctttggccttggtagtttgggtgggcgagaggcggcttcgtgccgcccagatcggtgcgcgggaggggcgggatctcgcggctggctctcgcccccgtggatccggcccggatctcgcggggaatggggctctcggatgtagatctgcgatccgccgttgttggggccgatgatggggcccttaaaatttccgccgtgctaaacaagatcaggaagaggggaaaagggcactatggtttatatttttatatatttctgctgcttcgtcaggcttagatgtgctagatctttctttcttctttttgtgggtagaatttaatccctcagcattgttcatcggtagtttttcttttcatgattcgtgacaaatgcagcctcgtgcggacgtttttttgtaggtagaag

SEQ ID NO: 163 - DNA, 1446 bp, Artificial sequence
  misc_feature (1)..(1446): Chimeric transcriptional regulatory expression element group.
ggtccgattgagacttttcaacaaagggtaatatccggaaacctcctcggattccattgcccagctatctgtcactttattgtgaagatagtggaaaaggaaggtggctcctacaaatgccatcattgcgataaaggaaaggccatcgttgaagatgcctctgccgacagtggtcccaaagatggacccccacccacgaggagcatcgtggaaaaagaagacgttccaaccacgtcttcaaagcaagtggattgatgtgatggtccgattgagacttttcaacaaagggtaatatccggaaacctcctcggattccattgcccagctatctgtcactttattgtgaagatagtggaaaaggaaggtggctcctacaaatgccatcattgcgataaaggaaaggccatcgttgaagatgcctctgccgacagtggtcccaaagatggacccccacccacgaggagcatcgtggaaaaagaagacgttccaaccacgtcttcaaagcaagtggattgatgtgatatctccactgacgtaagggatgacgcacaatcccactatccttcgcaagacccttcctctatataaggaagttcatttcatttggagaggacacgctgacaagctgactctagcagatctaccgtcttcggtacgcgctcactccgccctctgcctttgttactgccacgtttctctgaatgctctcttgtgtggtgattgctgagagtggtttagctggatctagaattacactctgaaatcgtgttctgcctgtgctgattacttgccgtcctttgtagcagcaaaatatagggacatggtagtacgaaacgaagatagaacctacacagcaatacgagaaatgtgtaatttggtgcttagcggtatttatttaagcacatgttggtgttatagggcacttggattcagaagtttgctgttaatttaggcacaggcttcatactacatgggtcaatagtatagggattcatattataggcgatactataataatttgttcgtctgcagagcttattatttgccaaaattagatattcctattctgtttttgtttgtgtgctgttaaattgttaacgcctgaaggaataaatataaatgacgaaattttgatgtttatctctgctcctttattgtgaccataagtcaagatcagatgcacttgttttaaatattgttgtctgaagaaataagtactgacagtattttgatgcattgatctgcttgtttgttgtaacaaaatttaaaaataaagagtttcctttttgttgctctccttacctcctgatggtatctagtatctaccaactgacactatattgcttctctttacatacgtatcttgctcgatgccttctccctagtgttgaccagtgttactcacatagtctttgctcatttcattgtaatgcagataccaagcgg

SEQ ID NO: 164 - DNA, 675 bp, Artificial sequence
  misc_feature (1)..(675): Chimeric transcriptional regulatory expression element group.
ggtccgatgtgagacttttcaacaaagggtaatatccggaaacctcctcggattccattgcccagctatctgtcactttattgtgaagatagtggaaaaggaaggtggctcctacaaatgccatcattgcgataaaggaaaggccatcgttgaagatgcctctgccgacagtggtcccaaagatggacccccacccacgaggagcatcgtggaaaaagaagacgttccaaccacgtcttcaaagcaagtggattgatgtgatggtccgatgtgagacttttcaacaaagggtaatatccggaaacctcctcggattccattgcccagctatctgtcactttattgtgaagatagtggaaaaggaaggtggctcctacaaatgccatcattgcgataaaggaaaggccatcgttgaagatgcctctgccgacagtggtcccaaagatggacccccacccacgaggagcatcgtggaaaaagaagacgttccaaccacgtcttcaaagcaagtggattgatgtgatatctccactgacgtaagggatgacgcacaatcccactatccttcgcaagacccttcctctatataaggaagttcatttcatttggagaggaaccatcttccacacactcaagccacactattggagaacacacagggacaacacaccataa

SEQ ID NO: 165 - DNA, 804 bp, Zea mays
accgtcttcggtacgcgctcactccgccctctgcctttgttactgccacgtttctctgaatgctctcttgtgtggtgattgctgagagtggtttagctggatctagaattacactctgaaatcgtgttctgcctgtgctgattacttgccgtcctttgtagcagcaaaatatagggacatggtagtacgaaacgaagatagaacctacacagcaatacgagaaatgtgtaatttggtgcttagcggtatttatttaagcacatgttggtgttatagggcacttggattcagaagtttgctgttaatttaggcacaggcttcatactacatgggtcaatagtatagggattcatattataggcgatactataataatttgttcgtctgcagagcttattatttgccaaaattagatattcctattctgtttttgtttgtgtgctgttaaattgttaacgcctgaaggaataaatataaatgacgaaattttgatgtttatctctgctcctttattgtgaccataagtcaagatcagatgcacttgttttaaatattgttgtctgaagaaataagtactgacagtattttgatgcattgatctgcttgtttgttgtaacaaaatttaaaaataaagagtttcctttttgttgctctccttacctcctgatggtatctagtatctaccaactgacactatattgcttctctttacatacgtatcttgctcgatgccttctccctagtgttgaccagtgttactcacatagtctttgctcatttcattgtaatgcagataccaagcgg

SEQ ID NO: 166 - DNA, 623 bp, Cauliflower mosaic virus
ggtccgatgtgagacttttcaacaaagggtaatatccggaaacctcctcggattccattgcccagctatctgtcactttattgtgaagatagtggaaaaggaaggtggctcctacaaatgccatcattgcgataaaggaaaggccatcgttgaagatgcctctgccgacagtggtcccaaagatggacccccacccacgaggagcatcgtggaaaaagaagacgttccaaccacgtcttcaaagcaagtggattgatgtgatggtccgatgtgagacttttcaacaaagggtaatatccggaaacctcctcggattccattgcccagctatctgtcactttattgtgaagatagtggaaaaggaaggtggctcctacaaatgccatcattgcgataaaggaaaggccatcgttgaagatgcctctgccgacagtggtcccaaagatggacccccacccacgaggagcatcgtggaaaaagaagacgttccaaccacgtcttcaaagcaagtggattgatgtgatatctccactgacgtaagggatgacgcacaatcccactatccttcgcaagacccttcctctatataaggaagttcatttcatttggagaggacacgctga

SEQ ID NO: 167 - DNA, 8 bp, Cauliflower mosaic virus
acacgctg

SEQ ID NO: 168 - DNA, 1790 bp, Coix lacryma-jobi
gtgatgttcaagatattgtaatggtgtttattttctatcaaatagccataaaatgatatacaaaatgttattcatgattgatcctagttacattcaaagtattaaatagcttgcagatagtaaatagacagtcattgtataacctgtttttttgactgtctatgttcagttccaagaacttacagacaagaggttatgtgtagattgaacgtgcccttgacggcatccaactagcgaaccacgagggaagcagatggtggccgttgaggggctgttgacgcaaagcatctctctcggctgctctcgaaagctccattgcgggtggcggtctggtggcaccaggaaattgcgtgagccaaggcgggctcgtctcggtctcacaacacggcacgaaaccgtcacggcacacggcaccaggatttccttcccctcccctgccgttctcctcatcataaatagccaccccctcctcgcctcttttccccaactcatctgttcttcgtctcacacagccagatcccaatccctctcctcgcgaacttcgtcgatctcccttccctcgcctcgcttcaaggtacggcgatcatcctcccgctttccctcctcctcctctagatgtagtacggagtacttgccatcatgcatcatgctacatcacgctcgtgcgagctctgggtcctcgatctgggaacggaactgtgggatgctgctcgtgcgatttattattggggatctgggttctcgatctgggaacggaactgtgggatgctgctcgtgcgatttattattggggatctgggttctcgatctgggaacggaactgtgggatgcttgtaggcaggtcggagatgggtcggatcgttgcttagggttcgatctgctcgtggttttcttttaatccctgatgcatgatttatcggtcatcctattagatggaaccagtagggtgactctgatccgatatacttaacctcgatctggttcgatgttcctggctaggcttgtgcgtctgtttcgtcagaccagttttgctgtttttggtatggttgtgatgcccgtccaaatatgactaagcgagtgtagaatcattttatgaactaactgctggtcttattaaatctagatctgcatacgttgatgtactacgttcatagttgatacagtatgtatgaactagttgctggtcgtattaattttggatctgcatgtgtggtagcatataatgttcataatacaattgatacagtatgatgtatgaactatctgctggtttattaaatttggatctgcttgtggtaaaaaatatgttttttatatagttaccatgatggattaatctatacttctgatgtatatgctgcagttttctgctgaggctgtagttttttccagattaaaatacagcatgcatatttgctaagctctgggcgtgtgaacgcccaccatggcattgtccagtaatagtaatgaatttttttgtttgcctgatgtgggagaaaacacgcattgtccagttattttgttccatatgcattgtcctgttttgttggatatgcatgcttagaaaacatatgcagccactgtttgataatgctttagcatctgcctgttgaacatgcatgatctacctatctttattttgtatgtacttgggtagtggcatgttgctagttttccttgattctgtggcgtctacatgttgagcttgcatatatgtttgttgtccttcttttcctccttggtctactgctatatgcttacccttttgtttggctaattttcaggtgcag

SEQ ID NO: 169 - DNA, 481 bp, Coix lacryma-jobi
gtgatgttcaagatattgtaatggtgtttattttctatcaaatagccataaaatgatatacaaaatgttattcatgattgatcctagttacattcaaagtattaaatagcttgcagatagtaaatagacagtcattgtataacctgtttttttgactgtctatgttcagttccaagaacttacagacaagaggttatgtgtagattgaacgtgcccttgacggcatccaactagcgaaccacgagggaagcagatggtggccgttgaggggctgttgacgcaaagcatctctctcggctgctctcgaaagctccattgcgggtggcggtctggtggcaccaggaaattgcgtgagccaaggcgggctcgtctcggtctcacaacacggcacgaaaccgtcacggcacacggcaccaggatttccttcccctcccctgccgttctcctcatcataaatagccaccccctcctcgcctctttt

SEQ ID NO: 170 - DNA, 93 bp, Coix lacryma-jobi
ccccaactcatctgttcttcgtctcacacagccagatcccaatccctctcctcgcgaacttcgtcgatctcccttccctcgcctcgcttcaag

SEQ ID NO: 171 - DNA, 1216 bp, Coix lacryma-jobi
gtacggcgatcatcctcccgctttccctcctcctcctctagatgtagtacggagtacttgccatcatgcatcatgctacatcacgctcgtgcgagctctgggtcctcgatctgggaacggaactgtgggatgctgctcgtgcgatttattattggggatctgggttctcgatctgggaacggaactgtgggatgctgctcgtgcgatttattattggggatctgggttctcgatctgggaacggaactgtgggatgcttgtaggcaggtcggagatgggtcggatcgttgcttagggttcgatctgctcgtggttttcttttaatccctgatgcatgatttatcggtcatcctattagatggaaccagtagggtgactctgatccgatatacttaacctcgatctggttcgatgttcctggctaggcttgtgcgtctgtttcgtcagaccagttttgctgtttttggtatggttgtgatgcccgtccaaatatgactaagcgagtgtagaatcattttatgaactaactgctggtcttattaaatctagatctgcatacgttgatgtactacgttcatagttgatacagtatgtatgaactagttgctggtcgtattaattttggatctgcatgtgtggtagcatataatgttcataatacaattgatacagtatgatgtatgaactatctgctggtttattaaatttggatctgcttgtggtaaaaaatatgttttttatatagttaccatgatggattaatctatacttctgatgtatatgctgcagttttctgctgaggctgtagttttttccagattaaaatacagcatgcatatttgctaagctctgggcgtgtgaacgcccaccatggcattgtccagtaatagtaatgaatttttttgtttgcctgatgtgggagaaaacacgcattgtccagttattttgttccatatgcattgtcctgttttgttggatatgcatgcttagaaaacatatgcagccactgtttgataatgctttagcatctgcctgttgaacatgcatgatctacctatctttattttgtatgtacttgggtagtggcatgttgctagttttccttgattctgtggcgtctacatgttgagcttgcatatatgtttgttgtccttcttttcctccttggtctactgctatatgcttacccttttgtttggctaattttcaggtgcag